European Patent Specification EP 4 301 852 B1, published March 18, 2026. Title: NOVEL CRISPR-Cas NUCLEASES FROM METAGENOMES. Applicant: BRAIN Biotech AG. The sequence listing filed with the application follows.

SEQUENCE LISTING (65 sequences)

SEQ ID NO: 1 - protein, 1295 aa, Unknown bacterial species
  AA Sequence of BMC01
MIFNNFTQKFSLSKTLRFELRPVDAGGNVITDLTIFEETIKNDQKRYEAYLAIKPLVDETHKHFIQTVLSGLTDLIKSDEMKNYLEHKNLIRQKDVEEKVKTKSIDVINKIEKDWRKRVSDSFTKHPQYKKMFDKTLFADESPLYKLAENDFQRSQIKIFEKFTGYFNGFHENRKNLYVAEKQGTAIANRVINENLPKFIENANKLKRAFEKYPEFLSKISEDKSFQALLIKNQLSLEKLLQPLTFNLLISQTGIDSYNEVLGGYTPENSEPIKGLNQLINLYRQKINLARNDFPNLAPLYKQLLSDRETNSVVYKPLENVADVYSSVFELCQNLLSKQSDINKWIEDINISSGQIWIYKSHLSGLSVMLFGESGWGLIPRILNISEDDEEEIIKSKSKKSQQEYFSFAEIGNAINNYSFEDVNIKALAKQGLCLWQKQGNERLIKFGKLFSQMQNELQSPKEKWDSTEKEKIKELLDTGLEFVHWLKVISNQPEDKDEVFYAEWQALTDTWRGLPKLYDRVRNFATKKDYSQNKLKINFDKGTLLNGWDTNKETDNLGILLENKGQYYLGIMKDSSIFDYQWDIDNFQNPNSKQSVAKKNLHEAIVSDNTQDCWSKIVYKLLPGPNKMLPKVFFSDKRQKYFGADEKVIDINENGRHKKGDNFNISDCHYLIDFYKTAINKHPEWSQFNFKFSATKSYEDISQFYHEVQNQGYRIEFDHIRKDYIQKMVSEGKLFLFKIHSKDFSSYAKGRPNMHTIYWRAIFNPENLANVVVKLNGEAEFFYRKSSKDRIISHPQGLEVSNKNPSNPKKTSRFAYDLIKDKRFTQDKFFFHVPITLNFREGEGYRFNQSVIRELKKYYQTDKANLHIIGIDRGERHLLYYCVINVASGKIVEQGSFNQISTNYTPEQITDDGEIIKGETVNKTTDYHNLLNTKEGDRQKARKNWQTIENIKELKAGYLSNVIHKISQLMVKYNAFVVLEELKYGFKRGRFKVEKQVYQKFEKALIDKLNYLVFKDRAPAEVGGVLNALQLAPPVASYIDIGKQAGFLFYVPAHHTSKICPWTGFVDWLKPRYDGIDKAKAFFTCFESIHFNTQKNYFEFAFDYEKFRGNINHLPEGLKRTSWTLCSHNSLRDIATKDKNGNWPYKQINLTAELLEILKTLNPRNGENLVERIIEMNDKKFFESLMWALRVLLQLRYGYIKRNNEGIIIEEVDYILSPVANENGEFFDSRNFVNIEKADFPKDADANGAYNIARKGLLLIAQNINNAKINDKGEVKCDLQIDKTTWFNWVQSKS

SEQ ID NO: 2 - protein, 1107 aa, Unknown bacterial species
  AA Sequence of BMC02
MPKEDFDKACIYLSNFDKFSTYFVGFNQNRENLYTDEEQATAIPYRIINDNMVRHFDNCRKFEKIVKKYGDISNVLSTYKEFFAPDCFKNKLNQSQIDHYNNTIGHTADDIYGVGINQILSKYKQDNKLNSSDLPLISKLYKQILSDTESYAIENFADDKMMLNAVDKEYSRIKENDVFINIETCMNEYLTLENSHMIYLKNDSSLTDISNKLWEDWAFVKNAIQKYSKEILCLSDKKIEDMLKMSHYSISFVQNSVYYYVDNYMESCEDKRKSIIDYIKTFYSIKYNNVFSCYKEAEAVLRLDSIHKNRRSPVDKNGIGGEGFAQIEKIKNFLDSILEVKNFLNPLYLIKSGKMAEIEDKSEEFYNRFNELYNSLSDTTYLYNKVRNYLTKKPYKKEKFKMNFENSTLLSGWDVNKENCSNSIILIRNGKYYLGIIDKQCGNMFNFKIDAEDNEKKRKEKEDLAEDILSDGSDSYYEKMVYKLLPDPSKMLPKVFFSNKSIDFYAPSEDIKYIRENGLFKKDAKNKKALYIWIEFMQNSLKKHPEWSNYFNFNFKPSTEYADVSEFYKQVSDQGYSLSFDKIKDSYIESKIKSGELFLFEIYNKDFSPYSKGNPNLHTIYWKSIFDKENLSNVVIKLNGQAEIFFRPASLKRNEVVVHRAKENILNKNPLNPKKESMFEYDIVKDKRYTQDKFFFHCPITLNFKSGNVGKFNDKVNQFLKNNPDVNVIGFDRGERHLLYCNVLNQKGEIIEQKSFNVIENKNNGITQKVDYHNLLDRKEKERDASRKSWSTIENIKELKEGYLSNVVHEISELIIKYNAILVLEDLNFEFKKGRFKIEKQVYQKFEKALIDKLSYMVFKKEESNKPGHSLMAYQLASPFESFQKLGKQCGFIFYVNSNYTSKIDPVTGFVNLLKIKYESVDKSCKFINDKFDDIRYNADREYFEFTFDNGKWTACSHGKERYRYNRNDKKYNCFDVTEELKSLFNKYEIDFKAGTDIKKSICQVQDKNFHSELLFNLSLIVQLRHTYKNGDIEKDFILSPIMDKETGKFFDSREYENLENSLLPTNADSNGAYNIARKGLLTLRQIDKDGKPSNISNKEWFDFVQK

SEQ ID NO: 3 - protein, 1323 aa, Unknown bacterial species
  AA Sequence of BMC03
MEKNLNYLERFTKHYNTKKTLKNKLIPYGNTAENMIKNNIISNEKQIILSAKKQKQSIDFLQKEYIENKLSEITLPYLNDYYNEFIKNKKERDTDVIDNIEIAMRKHISKSLTENGNHKKYLNKEVFDIISEKKELYYDVTFKRNATYLSDYFQSRVNLYKDSNKSSTIASRCININLPIFAKNIVLFNFIKNKANIIFDDLKEITDDEYTLDSIFSIDFFNMVLSQKGIDYYNTILGGMTKEDGKKIKGINEYINLYNQNVKDEKNKLPYPKKLKKQLLSDINSYSARFEKFDTEQEMVKSIKSLVENDLFQGELFDKKVDILKETERLLERISEYDSNALFITEKNISYISIDIFNDKFFIKTAIEYFYENNICPDYRKIYDNASKNKRKQLGKEKNKVIKQKSFSISFLQDAITFYIKDSGINKISENCIINYFKKHTIKLTELFGKVYEDYNVIKPILEQHLVEYEGKSISKDSIKRSKIKLFSENLKNIFYFIRPLNIIEEALNYDTSFYTPFNILFEEIKKFNKLYDKIRNFITKKPFNDEEINLYFGIPNLGGGFIDSQTDKSNNGTQYCTYLFRKKNQLLNWEYFVGISKNKHLFREKENIELNSDETSFQRYSFYTPKDKSIYGSSYFSANEKNYKDDKQEFINIINNIVNNSGNELAIKELKKYINNSTENSETPNGCLSVLKNKCNEIYNLVINHDDFKEKNEDIINKLKNTLSKLSKVPQAKELINKKYNLFSEIISDISEICLTSTQRYYPIDDEELNSALNDENKPLYFFKISNKDLSADENILNGKRKSKGKDNIHTMILRAMMDDNVTNIIPTSCKISMREASIKKDDLVIHKANEPIKLKNSLANKKESTFSYDITKDRRYSRDEFFFSITASINSDCKENDYYFNQKVNEYLKNNSKINLLAVDLGETNIITISVIDQKGNIILQKDLDKFINKEKNIITDFNLLLSNRSKERDIAKRDWQEQQQIKNLKEGMISCIIHEICKLMIEHNAILIMEDLDANFKNRKKRIEKAIYQKFEIAILEKLNNLVFKDIPINEVGSVTKPLQLSDKFETYEKVGNQSGFVFKVSPFYTSIIDPTTGFINLFKKNFESVKYSIEFFSKFESIRYNTKEKYFEFAFDYKNFKEIKYTENIKTDWVACTTNIDRYEYDKKNKIYKKYDVTTDLKNLFENEEIYYQKGENILDVILKKNNREFFEKLTNLLKITMLFRYRNSHLKLDYISSPVKNSNGEFFSTENGLENYPIDSDTNGAYHIALKGKMILDRINSNSSEKLDTYISIEDWLKFIQKFSVNKITETKKNKKINIKYV

SEQ ID NO: 4 - protein, 1324 aa, Unknown bacterial species
  AA Sequence of BMC04
MKNLTEFTGLYPVSKTLRFELKPTDDFNWETFLESTIFKHDQERAEAYPIVKVIVDQFHKWFIEDALNKSTINWNSLYDAYFAPKNENSVENLRKEQDKIRKEIVDTYFKKHDWWKYVSKDHSKLFKIELPALLSDDAFIYEINDKYPNYTQEILIDALAKFQNFSVYFGGYFKNRDNMYKSDAQSTSIANRIVNENFTKFADNIKIYNRLKENCLSELQKVELDFTDELTGLTFDDIFSPSYFNKCLTQKGIEKLNLYIGGKTGKNKEDKVFGINRVGNEFLQFNKESKLKLKDLKMVKLYKQILSDREQPSFLPEQFRNEDELIKSIEDFHNLITEQKLFERLLKLMGRLKNGECEDLNKIHVVGSSLTQLSKVLYGNWEVLGTALRNKFQTNKTKKDKLESEKDIQEWMERKSFSLAQIIEVESSLQDDKSIKVIDLFTTFNAWQKVNEKPQLVDLIKLCKDDFQTRFRAVKDLIEKGEQIQGNESAKEEIKAVLDNYQNLLHVVKLLNLGKKESYLDKDETFYNEYKEILSSTESDNVCLEDIIPLYNKVRSFLTRKLGDEGKMLLKFDCSTLADGWDVGKESANNSTILIDNSKYYLIITNPENKPDLSTAITSNTDNVYKKIVYRQIADPTKDLPNLMVIDGKTQRKTGNKDDDGINRVLDQLKDKYLPQEVNRIRKLGSYLKTSEHFNKKDSQVYLAYYMQRLIEYKQGEMEFSFKNSEEYDSYSDFLDDITKQKYSLSFVNVSKEIITQWISEGKIFLFQIYNKDFEEKATGTPNLHTLYWKELFSEENLKDIVYKLNGEAELFYRKKMDGKPFTHNKGAVLVNKTFADGSPVEPEHYKEYVEYITGKVIEKQLSKEAKDKLHLVKTNKAKLDIIKDKRYFQHKLLFHVPITINFKSEGVPKFNDYTLNYLRENKKDINIIGIDRGERNLIYVSVINQKGENIIPPKHFNIVESDMFGMEDKRKFNYLEKLIQKEGNRDDARKNWSKIETIKDLKTGYLSLVVHEIAKLVVEHHAIVVLEDLNYGFKRGRFNVERQIYQNFEKMLIEKLNLLVFKNNSNSPDYGNILNGLQLTAPFGSFKELGKQSGWLFYVNASYTSKIDPQTGFANLFNMKDAKKDTKSFFEKITEIKYDDGMFKFTFDYRNGFSIVQTDYKNIWTVCTNDKRILVSKDNISGKFKHEYVDITESIKNLFINNNINDYHSISKETILSIKEKKFFDDLFFYFKLSLQMRNSIPNSDIDYLISPVQIKGKPFFDSRIPNNINIVDADANGAYHIALKGLYLVINDFPTEKKGKSEYLKKITNEDWFEFAQRRSLK

SEQ ID NO: 5 - protein, 1230 aa, Unknown bacterial species
  AA Sequence of BMC05
MRWDEKLQTFLNDQEIEDAYQVLKPVFDKLHENFIIGSLENTNNKKLFSFDKYLKLKNDLLHVNKKEQESDYKKKEKEFETEGKLLRNTFATVWINEGKNFKNTIVGGENDREILKEGGYKILTEAGILKYIKMNIDKFVELKLKTREDILWKKENRNLVEMADLEKSLGTIESWGVFEGFFTYFSGFNQNRENYYSTDEKATAVASRVIDENLPKFSDNVLEFNKKNDVYIGIFSFLKGKNIVLKGKSGNGEEQDLLPITEKIFEIEYFKNCLSEGEIERYNSDIGNANFLINLYNQQQDKKENKLRIFKTLYKQIGCGIKGDFIQLIKTDDELKKIFEDLKITGDNFFKNTQNLKEIILSLENFSGIYWSDKALNTVSGKYFANWASLKELLKNAKIFKKEKDEIKIPQTIELSDLFGVLDSNELIFKESFNENDELKQIILKSYEKNSIKLLKMIFVDVEENQKIFGNLKDGLPINDFKKDENTQIIKTWLDGLLNTNQILKYFKVRESKIKGAPLNPEVSERLNKILNVENPTVIYDVVRNYLTKKPTEGLNKLKLNFDNAVLAAGWDVNKESERGCLILKDGDNKKYLAILTNKTQKFFGEKVKYKEFVGDENWQKMDYKLLPGPNKMLPKVLLPKSDRYKFGATDEILKIYNEGGFKKNEPTFTKAKLAKIVDFFKDGLKNYPSAKSSWYNLFAFDFSDTEKYESIDRFYTEVEKQGYKLSWSAISKNFIFEKVDAGDMYLFEIRNKDNNLKNGKAKTGAKNLHTIYWGTIFGESENKPKLNGEAEIFYRPVVKDLIKDKDKNGDIIKASEKRFEQEKFVFHCPITLNFCLKSTRLNDVINQIMIENKKDVCFIGIDRGEKHLAYYSVVNQKGEILEQGSFNEINGQNYAKKLEEKAGHRDEARKNWKTIGTIKELKNGYISQVVRRIVDLAVKYNAYIVLEDLNSGFKRGRQKIEKSVYQKLELALAKKLNFLVDKSKKDGEIGSVQKALQLTPPATNFADIEKAKQFGIMLYVRANYTSQTDPVTGWRKTIYFKSTTQENLKKEICEKFSEIGFDGNDYYFEYKDENAEKKWTMYSGVSGKSLDRFRGKKDTHGIWKVEKQDIVELLKKIFGQQTSVVGDLKTKITNDNVNDLKYTIDLIQQIRNTGFNEIDNDFILSPVRDEKGNHFDSRKDGAILSNGDANGAYNIARKGVLAFERINAKPEKPELYIADVEWDKWLQSK

SEQ ID NO: 6 - protein, 1256 aa, Unknown bacterial species
  AA Sequence of BMC06
MDSFTQFTGLYSLSKTLRFELKPIGKTLAYIENKGLLVQDEHRADSYKIVKKIIDEYHKSFIEKSLNGLCLDGLEDYYFYYQIPKKDDNQKKIVEDILTKLRKQIAERFSKQDIYKNLFAKELIKDDLNSFVQEVEQKDLIKEFENFTTYFTGFHENRKNMYSAEDKSTAIAFRLIHQNLPKFLDNMRAFNKISVSPLAEKFKHILSDSELGPIVQVVAMEDVFNLAYFNETLTQSGIDIYNHLLGGYTPEEGKEKIKGLNEYINLYNQTVKKEERLPKLKPLFKQILSDRSTASFIPEQYKNDNEVLESIEKLYQEIKEHVFHSLKELFVHINEYDLHKIYLRNDVSMTDISQKMFGDWGVFTKAMNLYFDKQYKGKAKLGTEKYEDEQKKYFSNQESFSIGYINECLLLLGSNYHKKVEDYFKVAGKTEEQVQMLFEIIETKYQNIQDLLNSPYPTEKNLAQDQVQVDKIKGLLDSIKNLQWFIKPLLGKGNEAEKDERFYGEFTALWETLDQITPLYNKVRNYMTRKPYSTEKMKLNFDNSTLLDGWDINKEPDNTSVVLRKDGLFYLGIMDKKYNKTFKQEFIESNEPCFEKMEYKLLPGANKMLPKVFFSNSRIEEFNPTVDLLENYKNQTHKKGDKFNIAHCRNLIDFFKQSINKHDDWKQFGFAFSDTKNYDDLSGFYREVEQQGYKITFRNIPEKFINQMVEESKLYLFQIYNKDFSPYSKGTPNMHTLYWKMLFDTENLKDVVYKLNGQAEVFYRKASINDENIVVHKANEVIINKNTLNEKKQSRFDYDIIKDKRYTIDKFQFHVPITMNFKARGLNNINLEVNQYLQKENDIHIIGIDRGERHLLYLSLINSKGNIIEQYSLNEIINEYNGNHYHTNYHDLLDKREGNRTEERQNWKTIESIKELKEGYLSQVVHKISELMVEYNAIVVLEDLNMGFIRGRQKVEKSVYQQFEKMLIDKLNYLVDKKKKSFELGGTLHAYQLTNKFESFQKMGKQSGFLFYIPAWNTSKMDPVTGFVNLFDTRYENVVKAKAFFNKFESIRYNKDKDYFEFEVKKYSDFNAKAEDTRQEWIICTHGERIINYRNPEKNNEWDDKTVHPTTELKSLFTSKNIIFENGSCLKEQIALQKDTDKEFFEGLLKQFKNTLQMRNSKTKSEIDYLFSPVSNENGVFFDSRDYVDIDNRDRKFCVSTGKPTLPVNADANGAYNIARKGLWIVEQIKNPNTDLKKLKLAMTNKEWLQFVQNKG

SEQ ID NO: 7 - protein, 1274 aa, Unknown bacterial species
  AA Sequence of BMC07
MDNAFSDFTQKYTLSKTLRFELRPVGNTEKMLEDEKVFEKDKLIQEKYIKTKPYFDLLHREFVEEALKDVDISGLHNYFETYQKWAKDKKKYQKELQNKEQILRKEILVFLDSTAKYWAEKKYSELRIKKKDIEIFFEEDVFTILKKRYGEDSEAQIIDEVSGETVSIFDSWKGFTGYFKKFQETRKNLYRDDGTATAHATRIIDQNLKRFCDNLEIIKRIAGIIEFSEVEGNFKHSMGDVFSLSFYNKCLLQDGINFYNRILGGEVLQDGTKLKGINELINKYRQDNKGVKIPFLKLLDKQILSEKEEFLDGIEDDKELLAVLKKFYEVAEKKTSILKSLIQDFAQNNRQYNLEEVYISKEAFNTISRKWTHETSKFEEWLYNVMKPNKPTGLKYDKKEESYKFPDFIPLSYIQTALEQADIDGDFWKEHYSENSKANDGCLMGDESIWEQFIKIFEYEFQSLFEKEIIDRETGQPKKNGYNYVKDDFKGLLNGENFSVEIIKDFADTVLSIYQMAKYFAIEKKRKWLDEYDTGDFYENPEFGYKLFYDDAYKEIVQTYNNLRNYLTKKSYSEEKWKLNFENPTLADGWDKNKEPDNSAVILRKDGRYYLGLMKKGCNKIFDDRNKVEFSGGVDKDKYEKIVYKFFPDQAKMFPKVCFSAKGLDFFQPSEEILNIYKNSEFKKGDTFSVQSMQKLIDFYKDCLTKYEGWIAYEFKHLKSTDLYRNNISEFFSDVAEDGYKITFQDISDNYIDKKNQSEELYLFEIHNKDWNLKDEVKKTGSKNLHTLYFEALFSHENIQNNFPIKLNGQAEVFYRPKTDEEKLVKKKDKKGREVIDHKRYAENKIFFHVPLTLNRGKGDAYQFNAKINNFLANNSDINVIGVDRGEKHLAYYSVINQKGETLDSGSLNVVNKINYGEKLQEKASNRKQSIRDWKAVEGIKNLKKGYISQVVRKLADLAIEHNAIIIFEDLNMRFKQIRGGIEKSVYQQLEGALIEKLSFLVNKGEKDPKQAGNLLKAYQLAAPFTTFKDMGKQTGIIFYTQASYTSKIDPLTGWRPNLYLKYTNAEKTKEDIGNFSNIEFKNGIFEFTYDLRNFQKQKEYPKKTEWTLCSCVERFRWNRVLNQNKGGYDHYEDITHNFRDLFEKYDINFMSADIKGQIDTLDAKGNENFFKDFIFFFNLICQIRNTQQDKDGDENDFILSPIKPFFDSRDSKKFGENLPNNGDDNGAYNISRKGIIILNKISEFFDENGGCEKMKWGDLYISHKDWDDFARQI

SEQ ID NO: 8 - protein, 1335 aa, Unknown bacterial species
  AA Sequence of BMC08
MMQIMKNFDKFTNLYSVSKTLRFELRPEPKTLEYMRSNLRFDKNLQTFLADQEIEDAYQALKPIFDSLHERFITESLESGSAQKIDFSKYLEKYRNKRDLGIKALEGTEKLLRNNFAEIYKATAKSWKENAGKDGKGKEVFKKEGFNILTEKGILEYIEKNIDSFSAIKSPEEIRGALGAFDGFFTYFTGFNQNRENYYETKKEASTAVATRIVHENLPKFCDNILIFDERAEDYIGAYKALQKMGRALVNKEGGELPSISGDLFKITFFNKCFSQKQIEEYNTAIGNANSLVNLFNQAKRDEDGYKKLALFKTLYKQIGCDKKDSLFFAVTHDRRADAEKARENGQEAFSVEEVLVLAKHAGEKYFNKGNDDGEVNTTQEFISYIKDRSDYQGIYWSKAALNTISNKYFDNWYELIDQLKEAKVFTKTGSGSEDNVKIPDAIELEGFFQVLNKIQDWKTVFFKKSITADPQKLGIIESSETASAALLSLIFDDVAKHTKLFIDQSEDILKVENFVKPENKEDIKRWLDHSLAINQMLKYFLVKESRTKGAPIDPTLTKALDTLLRSQDAEWFKWYDVLRNYLTKKPQDGTKENKLKLSFENGTLANGWDVNKEPDNFCVILQNPEGKKFLAIIARQEGQKGFNQVFAKKHDNPLYKVDEGGVFWSKMEYKLLPGPNKMLPKCLMPKSNREKYGATEEVLKIYNQGSFKKTESNFSKKDLSRLINFYKSALQQYEDWRCFNFSFRATDSYEDIGQFYRDVESQGYKLDFQSINTDVLDELVEEGKIYLFEIKNQDSNQGKSSIHRDNLHTMYWNALFQEVLNRPKLNGGAELFYRKALSPEKIKELGSVDKNGKRIIRNYRFSKEKFIFHIPITLNFCLSDTRVNDTVNQELSRTSSSHFLGIDRGEKHLAYYFLVDQNGKIVLDEYGKAVQGTLNIPFLDNNGNVRKIKAKRRSLDENGKEKIEEVWCKDYNELLEARAGDRAYARKNWQTIGNIKELKEGYISQVVRKIVDLAIEYEAFIVLEDLNVGFKRGRQKIEKSVYQKLELALAKKLNFVVDKSAKIGGLKSVTNALQLAPPVSNFGDIEGRKQFGIMLYTRANYTSQTDPATGWRKSIYLKRGSEESIRKQIIDSFEEIGFDGEDYFFTYTDSVAGRTWILYSGKNGGSLDRFYGKRDNDKNQWVSMRQDVSKQLDGILANFEKDRSILAQIIDGEVDLIKVEQKYTAWESFRSTIDLIQQIRNTGTSERDGDFILSPVRDERGIHFDSRDTREGMPTSGDANGAYNIARKGTIMGEHIKREYSRMFISDEEWDAWLAGKQVWEKWLKDNEKILKKK

SEQ ID NO: 9 - protein, 1274 aa, Unknown bacterial species
  AA Sequence of BMC09
MKNSLEDFTNLYSLQKTLRFELKPIGNTQSMLEEDGVFDTDEKRKIAYSKTKPYIDRLHREFIEESLSDAQISKLDEYFKAYVDYKKDKKDTKRFNRIKQFKSVLRKEVVDHFNKQGKEWTTVKFAHLKIKKKDLEVLFEKQLPNILKEEYGTEKETQIIDEDSGEVTSIFDMWNGFMGYFTKFFETRKNFYKSDGTSTAIATRIIDQNLDRFIENILIYDSIKPKIDTSEVREFFNLESDTIFSMEFYNNCLLQAGIDQYNNFLGGKTLENGRKIRGINELINKYRQENPEDKIPFLKKLDKQIHSEKEKFIQQIETLEDLKEELQKFYNSSNEKIKILDNLLSRIEEFKPEGIFISKQAFNTISRRWTDQSEAFETSLFESLKEEKPITGTAKKKDDGYNFPEFISLQSIRNTLKKVQGEERFWKERYYRDNSESGILAGNEEIWTQFLMIFKSEFNSKFERNDPEDNGTIGYNLFKEDLEKLLKDLKITKDTKSIIKRFADEALHIYQVGKYFALEKDRVWISSYDDLLDTFYTDPNTGYLSFYEGAYEQIVQPYNMIRNYLTRKPYSDEKWKLNFENPTLANGWDKNKETDNSSIMLRKEGAYYLGIMKKGKNKLFEERNRQLFEPKNGEDTYEKLSYKLFPDPAKMIPKVCFSNKNIQMFSPSTEIMNIYNGETFKKNSDDFSVSSMQKLIAFYTKCLSQYEGWKYYDFKYIKSPDQYKDNIGEFYNDVAKSGYRVWFENISQSYVDSKNTMGELYLFKIHNKDWNQKDKKTKVGSKNLHTHYFEELFSQDNIENNFPLKLNGEAEVFYRPKTNPEKLGTKKDSKGREVIDRKRYASDKVLFHVPITLNRTPVTTTKLNKEINGFLANNPSINIIGVDRGEKHLVYYSVVNQRGKMLESGSFNTINGVDYHGKLEERADRREQARRDWQDVEGIKNLKKGYISLVVRELANLSIKYNAIIVMEDLNMRFKQIRGGIEKSAYQQLEKALIEKLNYLVNKTETDPQKTGHILKAYQLTSPIKSFKEMGKQTGIIFYTQASYTSVTDPITGWRPNLYLKYSSASKAKSDILKFSKISYNTNNNRFEFTYDLRNFVNMKAYPQKTAWTICSNVERFRWDRKGNKNNGEYIQYKDLTENFKTFFEEVSINYKGDILFQIKNLSEKGNEKFFRDLIFYISLISQIRNTQKDKKGDENDFILSPVEPFFDSRKSSTFGENLPLNGDANGAYNIARKGIIMLNKISKGSKNKVKEDIGWGDLYIPHTEWDDFATGSI

SEQ ID NO: 10 - protein, 1456 aa, Unknown bacterial species
  AA Sequence of BMC10
MSTKRSFSDFTNLYSVSKTLRFELKPIGKTLENMRERIYNDKKDYDSALQTFLHDQAIEDAYKTLKPILDSLHEEFINTSLNSSKAKNIDLSEYLNAYRERGNDTKTGEESKLSGIEKSLRKAIGETYLTWAKSFTEQAKNLIGIIEDIWDTEEEWDEEKKTKWLFKKKNFELLTESGILVFIEKKLDTMNISEQEKTDIKKALEEFKGFFTYFSGYNQNRKNYYETKAEKKTAIATRIVHENLPKFCDNVILFHGYQKILKDGSKREYKKKEEYLGMYAFLKLRNIETCIKDAESGEMIELYAITEDIFDISFFSSCLAQREIDEHNRIIGGIDKYNRIIGHYNALINLYNQARKKDEKFTKLSPFKELYKQIWCGNKKWSWIKAITHDTDEQILADTNHTGEAISVERILSLASKAGKKYFQPWKSTDDGIKTVPDFLDWLRGQTDWNGIYWSKAAINSISNVYFPNWGSIKETMKGDKTLVSYDKKREEQIKINEAVELSGLFDILDSTDGDWKQEWVLFKASLTKLLDASAENAEENSKRARRKDIIDRSSSPSQALLALITDFIEENMKHFLDQSHTILRLTEYSSPKSKEAIKSWMDLALSVSQTIRYFRVKESKTKGDTLNAELVGILTNLLDAEDATWFEWYDLLRNYLTKKPQDDAKENKLKLNFANSTLAAGWDVNKETDNTCVILQNPEWKTYLAVMNKNKKNVFQKEWNEWRWKKKTTKLNPLYEIDWGESWKKMEYDFWSDVSKMIPKCSTQLKKVIKHFKESDEDFIFPSGYKVTSGERFIEECRITKEQFELNNKVYKRDGDRIISAFRYELSETEEKTYIKSFQKGYLDMLLKSNNLPETEQEIYRKKYEDSLSKWINFCKYFIWKYPKTSLFEYQFDETDHYKSVDKFNLDVDIWSYKLKVDTKINKTILDTLVENGDIYLFEIKNQDSNIGKWENHKNNLHTTYWKSIFESVQNRPKLNGEAEIFYMKPLSPEKLQKKIDKKGKEIIDGYRFSRERFIFHCPITLNFCLGNEKINNIINFELSPKSDIYFLGLDRGEKHLVYYSIVDQNGKMIDQWSFNEIKWKDYHALLTKREWDRMESRKNWQTISNIAKLKEWYISLVIHEIIEKLKLNPWFIVLEDLNTGFKRGRQKIEKSIYQKFELALAKKLNFVVDKSAKLGEVGSVTNALQLTPPVSNYGDIENRKQVGIMLYTRANYTSQTDPATGWRKTIYLKTGSEENIKEQIVTQFSDIGFDGKDYYFEYTDKIGKTWILYSGKNGKSLTRFRGVRGKEKNEWNIKEINVRNMLDGIFANFDKDRSFLSQILDEWVEIKKIDEHTAWESLRFAIDLIQQIRNSGDKTQWEDDNFLFSPVRDAQGNHFDTREQKEGLPKDADANGAYNIARKWIIMNEHIRINEDTKDLDLFVSDEEWDMWLTDREKWKEMLPIFASRKAMEKRRGK

SEQ ID NO: 11 - protein, 1317 aa, Unknown bacterial species
  AA Sequence of BMC11
MSQNNTFEKFTNQYSLSKTLRFELRPVGNTEQMLEDENVFKKDEIIRKKYEQTKPFIDKLHKEVIKDSLHGKKIEGLDDYFKKFEIYSKNKKDSKIKKEFTDKESELRKQLNSHFKAESLFSEKVFSLLKEKYGTEDESFVKDENGNFVLDTVGEKISIFDEWKGFTGYFTKFQKTRENFYKDDGTSTAIVTRTIDENLYRFCENIKHFESIKNRVNFSEIEKNFNFKLENLFKADFYNSCLLQDGIDKYNDILGGKTLESGEKLKGLNEIINKYRQDNKVEKIGFFKMLDKQILGDKEKPSFIESIADDNELLLKLKEFYTNAEEKTEVLKKLFSDFSKNNDSYDLSKIYINKVGINTILLKWFDVAGRSDFEKNISTQTKKEKIVTFDKDSNSYKFPEFLAFSHIKEALSNGTYEVKEIWKERYYQSENKEKSEKAPLKKDSAISHWEEFLQIFSYEFDLLFVGAESQAGYNSNKNLFESLIKKNEKGFSISPEEKLVIKNFVDNTLWIYQMAKYFAIEKKRKWLESEYPTDSSFYDSEEFGFKNKFYDDAYDKIVKLRMLLQSHLTKKPFSTDKWKLNFENPTLAKGWDKNKESDNSAVLLRKEGRYYLAVMKKGNNKIFDDKNKSNFLENIEGGKYEKMVYKQMSDPSKDIQNLMVIDDKTVRKVGKKDPLDGVNRRLEELKKEYLPRDINTIREQKAYLKSSDNFNLGDANLFINYYKDRLVEYHKDIFVFSFRDRYSDFHDFSKHVAEQTYSLSFEDISEFYIQEKNNNGELFLFEIHNKDWNLEKKGGDRKSGAKNLHTVYFESLFSKENENNNFSIKLNGEAELFYRPKTDEQKLGNKNDLKGKIVLNKKRYAENKTFIHIPITLNRVASESKYFNQKLNDFLVGNPDINIIGIDRGEKHLIYYAGINQAGEFLKDEKGNLVLGSLNTINDVNYAQKLEERAKGRVKAKQDWQEIENIKDLKRGYISLVVRELADLIIKHNAIIVFEDLNMRFKQIRGGIEKSVYQQLEKALIDKLNFLVNKGEKDPTKAGHLLRAFQLTAPISAYKDMGKQTGVIFYTQASYTSKTCPECGFRPNVRWEPKSIKDKIKEGKLEITYKEDGFEISYKLSDFSKSQNQSKRRNILYTNVSKQDKFNLNTKDAVRCKWFRKTLSENELNKGEQKLNIQTETGVNIEYKISDCLIGLFEKYGLDYQNNLQEEIKNSGDSLPVKFYDKLSFYLHLLTNTRSSVSGTDIDHINCPNCGFCSKNGFKGGEFNGDANGAYNIARKGIIILDKLKNYKTENSNLEKMTWGDLFIDIDEWDKFTQNKT

SEQ ID NO: 12 - protein, 1385 aa, Unknown bacterial species
  AA Sequence of BMC12
METKNKSIWGDFTNKYSLSKTLRFELVPVGKTRENIQKHNPEFVQDQKIEEAYQILKSVFDKIHEDFITKSLESDEAKSINFSEYFDLYKKWNELKKKKTNEKNIEIKKEIQNEIEKIYKDNGGSKGEIQKIEDELRKRFEEIFKIQGKIFKEKACELNIKEGQEKDDDEEKDDNKKGFRKLLKAKFLYDYLCNLIESKNIIYKDFFENIKNKEGESISKEKTKDALIRFKGFTTYFGGFELNRLNYYTTKEEKSTAVATRIVNQNLPKFCDNVILFEIKKSEYLKIDEFLKNKNISLISKNQNGGEVELHKINKNFFEMMFFSKCLSQKEIQKYNLEIGNANNLINRYNQQQSDKSQKLKLFKTLHKQIGCGDRGGFIPSIKGEEDLRERLQEIKNNSIEYFENINDFIEYLKNHENYENVYWSDKAINTISSKYFSDWLNLKKEIWGKRDRKGNLKDEETKIPRAVQLKDLLENLDKITDWKLEGRLFKLSLFENGRKAKKLQQEDLNKFNKNKIENELEIEKLQIIEQNPSPFQALLNMIFADIKSKESAFLESRIFEISDFVHNEDKQIIKQWLDSILAINQIIKYWRVKDTFGTEGTLDEKLKNIIYSEKNPTRFYDIIRNYLTKKPQDELNKLKLNFENSTLAQGLDVNKEKDNFCIILRDDKQNQYLGILNSKNKNIFEIDQNEDIYQDDGLGWSKMMYKLIPGASKTLPKIFFSKRWTENNPTPDEISKIKKGETFKKGDNFIKRDLHELINFYKANLEKYPSVNESWAKLFIFNFSDTKTYESIDQFYNEVDKQGYKVSFISINKNTLDNFIDKEKLYLFQIKNKDNNLDKGEKKQSNKNLHSIYWEAIFGKALNKPKLNGGAEIFYRPALSEKKISELKIKDKNGKNIIIIKNYRYSKDKFIFHCPITLNFSAKSSKLNDEINDHIKNKKEFCFMGIDRGEKHLAYYSLVNQNGKILDKGQGTLNLPFVDKDGNKRCIKTEKYFEEDKKENEKWKPRIIDCPDYNCLLDARASNRDLARKNWQTIGTIKELKEGYISQVVRKIVDLAIENNAFIVLENLNIGFKRGRQKIEKQVYQKLELALARKLNFLVDKKAIIGEVGSVTKALQLTPPVNNFGDIGGKSQFGIMFYTKADYTSQTDPVTGWRKSIYLKRGPEDYIKDQILGNKNKNIEPAFEDICFDGQDYCFTYINKNTGKKWTLYSSKNGKSLDRYHRELVYENSDKKWLPKKQDVLEMLNNLFEGFDKKKSLLKQLETKNPNKTGEHPAWESLRFTIDLIQQIRNTGIKERDEDFILSPVRDKKGDHFDSREASPDLPNSGDANGAYNIARKGIIMAKHIEKGYFLYISDEEWDAWLAGEECWNRWAEKNTKSLLKNNY

SEQ ID NO: 13 - protein, 1385 aa, Unknown bacterial species
  AA Sequence of BMC13
MSTKTIFSDFTNLYELSKTLRFELKPVGETENLLNENQVFLTDKIRQKKYEEIKPFLDEFHLDFIHFCLSDLHLDYTEYKKSLDNYQKDKKNKDLEKKKENEEKKLREQIVGKFDSKVEDFLKTFGKVEKIKGKKDNEKFKVSLGKDWEIEFSKNNYEFLFEIGIFDLMKKKFEGNGDIYVADKETGEIYQDEKTGKDITIFDDWNGWLGYLTKFFETRKNLYKSDGTSTAIATRIINENLKKYCENLDIYNKLSQIENLKNKFQNLEADFGIKLEKFFSLENYNSCILQNGIENYNDIRGGKLEKNNNKIPGINEYINKYRQDSGEKLPFLQKLDKQILAGGKENFIEQIENEPSFEKCLKNFYNNSIKKVDILTQIFQDLSTYTNEDYKTIYFSKEAFNTLSHKFTDQVLNFEKLVFEELLLNKLVEKKDFDKKEEKYKFPDFIPLFYVKKGLENYHTKNLFYKSRYYENEIIEEDNDNIWQKFCTILNYEFQSLLSNTIINQNGEEIEVGFTISKNKLEKILDNFSLGENNNGIIKDFADISKTIYQMGKYFALEKKREWNNNFDLNDDFYKTEYSQENEKYGYLEFYNEAYEQIIVPYNLMRNFIAKKPWEDNKKWKLNFENSSLLKGWDKEFESYGSYIFEKAGLYYLGIINGTKLNKNEIEKLYNYNANNGAKRFVYDFQKPDNKNTPRLFIRSKGDNFAPSVKELNLPINNIIEIYDKELYKKDKEKPNKHKESLMKLIDYFKLGFRKHISYKHFNFVWKESNKYDNIADFYRDVEKSCYKPYWEEDINFDELKNLTKEKRMYLFQIYNKNFELDESISTDDYTFKGNGKDSVHTMYFKGLFSKDNLENKNGVNLKLSGGGELFFRPKSIEKKIDKNRKSKREIIENKRYSKDKILLHFPIQVNFKENKTSNFNNYINNFLANNPDINIIGIDRGEKHLAYYSVINQKQEIIESGSLNYIYQKDKDGKIIQKSEKKIQEVRNDEGKIIDYELVETGKLVDYEDYGILLDYKEKKRRLQRQSWKEVEQIKDLKKGYISAVVRKIADLIIEHNAIVIFEDLNMRFKQIRGGIEKSVYQQLEKALIDKLNFLVNKGEKDSEQAGNLLKAFQLTAPIGTFKDMGKQTGIIFYTQARYTSKIDPLTGWRPNLYIKKQSAELNKESILKFDSIIWNKEKEYFEITYDLEKFQSESTKNLKEKKEEKLERTKWTLSTRVERFKWNKNLNNNKGGYEHFENLNIHFKELFEKYGLDISGDILKQIHNLETKGNEAFFSHFLDLFKLVCQIRNTNQDKKGNENDFIYSPVFPFFDSRKQNTVGVKNGDDNGAFNIARKGIIILERIGKWKKENDMKIQKGEKEMYPDLFISNIGWDNFTQNHNIRDN

SEQ ID NO: 14 - protein, 1310 aa, Unknown bacterial species
  AA Sequence of BMC14
MSQNNIKEKSIFDEFTNKYSLQKTLRFELRPVLNTEQMLTDSGIIKLDEKRKLNYEKTKPFLNRLHQEFVTESLNGVRLKSLDGYAVLYANWKKSIDKKEKDAAYKVLEKKELEIRQEIVVLFDEKAVEWIGKLPADVKKPKKPNYEFLFEPAIFSILKKKYSDEVGTTIDEESIFDSWDKWTAYFGKFFETRKNFYKSDGKATAVATRIVNENLRRFCDDVSTFENIQSKIDLSPLEKEFDVSLKKVFDIQHYNQCLNQSGIDAFNTLLGGEVHENGEKIKGINEYINEHRQKTGEKLTRLKKLDKQIGSDKENFIDLIETDEQLKTTLVTFIANAKEKVDLLDKSVSYLTKDTDVKLSGIFFRKEAINTITRRWFVSHEKISDALVSAFSDKNVKFDQKREEYKFPDFISWHVIQNAVEKLASDGEEIWKKYYLEEEKLSLLDKTPWQQFLTVFECEYNNLKSKGHESEGRSFTELVQDIESLLKTDTLDRNDHVTEIIKSFSDRVLNIYRFAKYFALDKSCQWNPDGLDTDDFYVAYEQFYSDGYEKIVKVYDKVRNYMTKKPFNQDKWKLNFENPTLANGWDKNKETDNTAIILRRAGRYYLAVMERGHNTLFKKIPMSSSGYQKMTYKLFPDPSKMMPKVCFSKKGLEFFKPSAEIMRIYKNGEFKKGDTFSLSSMHVLIDFYKNALKTYDGWTMYDFSNLKKTSEYTENIGEFYRDVAESGYQINFDYIAEQYIEDANKEGKLYLFEIHNKDWNLKDGAIKTGSKNAHTLYFEQVFSDENAQNNFVVKLNGEAELFFRPATSTEKLGNHYDSKGNVVTKNKRYAHDKMFFHVPVTLNRTAPDARKFNQSVNVFLANNPDTNIIGIDRGEKHLAYLSVINQKGDILKIKSLNKIEVKDKDGNVIKEDDYAKLLEDRAKNRESARRDWKSVEQIKDLKKGYISNVVREIADLVIKYNAIVVFEDLNMRFKQVRGGIEKSVYQQLEKALIDKLNFLVDKNELDPQKAGHILHAYQLTAPFETFKDMGKQTGVLFYTQAEYTSQTDPVTGFRKNVYLSNSATVEKIKAFVEMFDVIGWDDKLKSYYFKYNPVNFVETKFKENTFSKDWVIYANVPRIKRERKNGYWEATVVNPNEEFLKLFKEWDFDNIYVEDIKEQIFQMFEEGRLDGTKEFDGKNRNFWHSFIFLFNLMLQVRNSTATQYKKDEDGNIIETVEGVDFIASPVFPFFTTDGGDFTEGCVNLAKLEDKFVGSNADKERFKKEFNGDANGAYNIARKGIIMLNNIKNNPEKPDLFVSKKDWDKFAQANQ

SEQ ID NO: 15 - protein, 1275 aa, Unknown bacterial species
  AA Sequence of BMC15
MNPTQTDKTPSKPFEKFTNLYCLSKTLRFELKPIGKTQKILEDNKVFENDKKRAKSYEEAKKYFNKLHREFIDESLKNITLSNNLIEKFEKKYLTWKNSKNKDNSTELKKSAKRLRIVILESFNKKANEWNSEYSNQVKNEKKKKKIQEITGIDLFFKVEVFDFLIHKYPEVQINGESIFSPFNKFSGYFKKFHETRKNFYKDDGTSTAIPTRIIDVNLEKFLENKDIYYTKYFQKYNSIFNKEETDIFKLESFKNCLTQSQIDKYNESIATLKSKINNLRQNNPEVNKHDLPFFKELFRQILGQPIKKETEQDNFIEILTNDEVFPVLQKNIDENELYIPKADTLFKEFLKSQIQETNEYNINEIYVASRFINSISNNWFAEWDTIINLLRTELKIKQNQKKLPDFISIASLKRVLQKSQDEIDAKDLFRNNYENLFESTTDFYKIFLKIWELEFNDNIKKYNLETENIRKIIIEDKKYLPNKKSILKNGETGIIHNEKILDYAQSALNIYQMMKYFSLEKGKEREWNPDGLNEDTTGGFYDDFNKYYQNVNTWKYFNEFRNYLTKKPYKTDKIKLYFGHKSLLGGFTESKTEKSNNGTQYGAYLLRKKHGLGGFDYYLGISTDPHLMSYFDPIDDSGDSEYERLNYYQVLTRTIYGPSYEGDYELDKKNLSEIEIIKKIKRSLSYYTSRVKKIQDIINNNYESVRDIHKDITDVLKEFGTIFDYKVITNSQIQKAFNCDKGFYLFEIYSKDFSKEKGDKSKNSKDNLHTTYFKSLMDRKQSTFDLGSGEIFFREKSVQSEIDSMRKTKNKITRFKRYTKNLIQFNLSITLNNNCTEVPQNKNARKAFINNFNIELSKKLLTNNSDINIIGIDRGEKHLAYYSVIDQQSNILETGSFNKIQERKDREPTDYQQKLDKIQKDRDWQRKSWQEISNIKDLKKGYISQVVYEISKLVKKYNAIIVFEDLNIGFKRGRFAIEKQVYQNLELSLAKKLNYLVFKDANEGESGHYLKAYQLTSPVNNFQDIGKQCGIIFYIPASYTSAICPSCGFHKNIPTSIKKLAKNKEFVEKFVITYELKKDRFYFGYKINDFYNSNLQDNVIFYSNVERLRYKRNKDNRSGEVQERLPNEELKKLFEQNHINYKDNPQISGQIKNQKLDNEKFYKPLIYEISLILQLRNSKTVKSEDGTINTNINRDFISCPACYFHSENNLMNLPNKYKGGKKFEFNGDANGAYNIARKGILLLNKLNNIKDIEKIEYNDLNISQEDWDNFVKNP

SEQ ID NO: 16 - DNA, 3888 bp, Unknown bacterial species
  NT Sequence of BMC01
atgatatttaataacttcacccagaaattttcactttccaaaactctccgctttgagcttcgtccggttgatgccggaggaaacgtaattacggatttaactatatttgaagaaaccattaaaaacgaccagaaacgatatgaggcctatcttgcgataaagcctttggttgatgaaacgcataagcattttattcaaacggttttatcgggtttaaccgatttaattaaatccgatgaaatgaagaattacttagagcataaaaatctaattcgccaaaaggatgttgaagaaaaagttaaaactaaatcaatagatgtgatcaataaaattgaaaaggattggcgaaagcgggtttctgatagtttcactaaacatccgcaatacaagaaaatgtttgataaaaccttatttgccgatgaaagcccgctttataaattagccgaaaatgattttcagagaagtcagattaaaatctttgaaaaattcaccggttattttaatggtttccatgaaaaccggaaaaacctatatgttgccgaaaaacaaggcacggcaatagccaatcgcgtaattaatgaaaatttgccgaagttcatagaaaacgccaataagctaaaacgggcatttgaaaagtatccggaatttttatccaaaatatctgaggataaatcttttcaggcattgctaattaaaaatcaattatcccttgaaaaacttcttcaaccactaacctttaatttattaatttctcagaccggtattgatagttataacgaggttttaggcggttatacaccggaaaattcagaaccaattaaaggtttaaatcagttaattaacttatatcgccagaaaattaatttagcccgcaatgactttcctaaccttgccccgttatacaaacagcttttatccgaccgcgaaaccaatagcgttgtctacaagccattggaaaatgttgcagatgtttatagcagtgtatttgagctttgccaaaatctactttcaaagcaaagcgatataaataagtggattgaggatattaatattagttccggacaaatctggatttataaaagccatctatcaggcttatcggttatgctctttggtgaaagcggctggggattaattcctcgcattctaaatatttctgaagatgacgaagaggaaattattaagtcaaaaagtaaaaaatcacagcaagaatatttttcatttgctgaaattggcaatgccattaataattattcttttgaggatgtaaacataaaagccttagcaaaacaaggcttatgcttatggcaaaagcagggaaatgaacgattgattaaatttggtaaattgtttagccaaatgcaaaatgaactgcaaagcccaaaagaaaaatgggatagcaccgaaaaggaaaaaataaaagaattattagatacaggattggagtttgtgcattggctgaaagtaattagcaatcagcccgaagacaaagatgaagttttttatgccgagtggcaggcacttactgatacttggcggggactgcccaaactatatgaccgcgtgagaaattttgcgactaaaaaagattacagccagaataagttaaaaattaattttgataaaggcactttgttaaacggctgggataccaacaaggaaaccgacaatttaggaatattattagaaaataaagggcagtattatttgggaataatgaaagattcctcaatatttgattaccaatgggatattgataattttcaaaatcccaattccaaacaatcggtggcgaagaaaaaccttcacgaggcaatagtatcggataacacacaagattgctggagcaagattgtctacaagcttttacccgggccaaataaaatgttaccgaaggtatttttttccgataaacggcaaaaatattttggtgccgatgaaaaagtaatagatattaatgaaaatggtcggcataaaaaaggcgataattttaatatttcggattgccattatcttattgacttttataaaaccgcgattaataagcatcctgaatggagtcaatttaattttaagttttctgctaccaaaagctacgaagatataagccagttttatcatgaagtgcagaatcaaggctatcggattgagtttgaccatatccgcaaagattacattcaaaagatggtaagtgagggcaaactatttttattcaaaattcacagtaaagatttttcgtcttatgccaaaggtcgcccgaatatgcataccatttattggcgggcaattttcaatccggaaaatttagcaaatgtggtcgtaaaattaaatggcgaagccgaatttttctatcggaaatcgtcgaaagatcggattatcagtcatccccagggtttagaggtttctaataaaaatcccagcaacccgaaaaagaccagtagatttgcttatgatttaattaaagacaaaagatttactcaggataaatttttctttcatgtgcccatcaccctgaatttccgcgaaggtgaaggctatcgttttaatcaatcggttattcgcgagcttaaaaagtattatcaaaccgacaaagccaacctgcatataatcggcattgaccgcggcgagcggcatttgctttattattgcgtaattaatgtggcgagcggaaaaatagttgagcagggaagttttaatcagatttccacaaactatacgcctgagcaaattaccgatgacggtgaaataattaaaggtgaaaccgtaaataaaactaccgactatcacaatctgctaaataccaaagaaggcgaccgccagaaagcccgcaaaaactggcagaccattgaaaatattaaagagttaaaagccggatatttatcgaatgtaattcacaaaatatcgcaattaatggtgaaatataatgccttcgtggttttggaagaattgaaatatggttttaagcgcgggcgttttaaggttgaaaaacaggtttatcaaaaatttgaaaaggcattaattgataaattaaattatctggtttttaaagaccgcgctccggcagaggtgggcggggtattaaatgctctgcaattagctccaccggtggcaagttatatagatattggtaaacaggcgggatttttattttatgtccccgcccatcacacctccaaaatctgcccgtggacgggttttgtcgattggttaaaaccgcgctacgatggcattgacaaggcgaaagcattttttacttgttttgagagcatccattttaatacgcagaaaaattattttgaatttgcctttgactatgaaaagttccgtgggaatattaatcatctgcctgaaggcctaaagcgaaccagctggacattatgctcacataacagccttcgcgacattgctaccaaagataaaaacggaaattggccatataagcaaattaatctcaccgccgaattgcttgaaatattaaaaaccctaaatccccgcaatggtgaaaaccttgtggagcggattattgaaatgaatgataaaaagttttttgaatcattaatgtgggctttgcgagtattgttgcaacttcgttatggatacattaaacgtaataatgaaggcataattattgaagaagttgattatattctttcgccggtggccaacgaaaatggtgagttttttgattcgcggaattttgtaaatattgaaaaggcagattttcccaaagatgccgatgccaatggcgcgtataacattgctcgcaaaggcttattattaatcgcccagaatattaataatgccaaaattaatgataagggcgaggttaaatgcgacctgcagattgataaaaccacttggtttaattgggtgcaaagtaaatcataa

SEQ ID NO: 17 - DNA, 3324 bp, Unknown bacterial species
  NT Sequence of BMC02
atgcccaaagaagattttgataaagcatgcatatatttgtctaactttgataagttttcaacttattttgttggttttaatcagaatcgagagaatctgtatacagatgaagaacaggctacggcaataccttatagaattattaatgataatatggtaagacattttgataactgccggaagtttgaaaagatagttaaaaaatatggagatatatctaatgtattatctacttataaagagtttttcgctcctgactgttttaaaaataaattaaatcagtctcaaattgatcattacaataatactataggacatactgcagatgatatatatggagtaggaattaatcagatactcagtaaatataagcaagataacaaacttaattccagcgatcttcctttaatatctaaactttataagcaaatacttagtgatactgagagctatgcaatagaaaattttgctgatgataaaatgatgttgaatgccgttgataaagaatactcaaggattaaagagaatgatgtttttatcaatatcgagacgtgtatgaatgaatatcttacattagaaaattctcatatgatttatctaaaaaatgattcctctcttactgatatctctaataaattatgggaagattgggcctttgttaaaaatgctatacagaaatattctaaagagatattatgccttagtgacaagaaaatagaagacatgctaaaaatgagtcattactctatttcttttgttcagaattctgtttattactatgtggataattatatggagtcatgtgaagataaaagaaaatcaattatagattatataaaaacattttattctataaaatataataatgtattttcttgttataaagaagcagaagctgttttaaggcttgactcgattcacaagaataggagatctcctgttgacaagaacggcataggaggagaaggttttgctcaaatagaaaaaataaaaaatttcttagatagtatattagaagtcaagaatttcttgaatcctctttatctgataaaatccggaaaaatggcagaaatagaagataagagtgaagagttctataaccgtttcaatgagttatataattctctttctgatacaacctatttatataataaagttaggaattatcttacaaaaaaaccttataaaaaagaaaaatttaaaatgaattttgaaaattccacgctattaagcggatgggatgttaataaggaaaattgcagtaactctattatactcatccgtaatgggaagtactatctgggtatcattgataagcaatgcggcaatatgtttaattttaaaattgatgcagaagataatgaaaaaaagagaaaagaaaaagaagatctggcagaggacatcctttcagatggttctgattcatattatgaaaaaatggtatataagcttctccctgatccttctaagatgttaccgaaagttttttttagcaataagagtatagacttttatgccccttcagaggatattaaatatattagagaaaatggacttttcaaaaaagatgctaaaaataaaaaagctctttatatatggatagagtttatgcagaattctcttaaaaaacatcctgaatggagtaattattttaattttaactttaaaccatcaacagaatatgctgatgtgtcagaattttataagcaagtttctgatcaagggtactctttgtcttttgataaaataaaagatagttatatagaaagtaaaataaaatcaggagaacttttcttatttgaaatttataataaagatttttctccatatagcaaaggtaatccaaatttacatactatctattggaaatcaatttttgataaagaaaatcttagcaatgttgttataaaattgaatggtcaggcagaaatattctttagaccagcttctttaaaaagaaatgaagtagttgttcacagagcgaaagagaatatattaaataagaatcctcttaaccctaaaaaagagagtatgtttgaatatgatattgtaaaagataaaagatatactcaagataaattcttctttcactgtcctataactttaaattttaagtcagggaatgtaggaaaattcaatgataaggttaatcaatttcttaaaaataatcctgatgtaaatgttataggattcgaccgaggagaaagacatttactctattgcaatgttcttaatcaaaaaggagagataatagagcaaaagagttttaatgtgatagaaaataaaaataatggaattacccaaaaagtagattatcacaacttgttggaccgcaaggaaaaagaaagagatgcttctcgcaaatcatggtcaaccattgaaaatatcaaagaattaaaggaaggatatctgtctaatgtggttcatgaaatttctgaactaataattaaatataatgctatcctagttctagaagatttaaatttcgaatttaaaaaaggtagatttaaaatagaaaaacaagtatatcaaaaatttgaaaaagcacttatagacaaactcagctacatggtttttaaaaaggaagaatctaataaaccggggcattctcttatggcatatcaattagcttctccttttgaaagtttccaaaaactagggaaacaatgtggatttattttttatgtaaatagtaattatacttctaaaatagatccagtaacaggattcgtaaatcttctaaaaatcaaatacgaatctgttgataaaagttgtaaatttattaatgataagtttgatgatatcagatacaatgccgatagggaatattttgaatttacttttgataatggcaaatggactgcttgttctcatggaaaagaaagatatcgttataatagaaatgataagaaatataattgttttgatgttactgaagaattaaaatcactgtttaataaatatgaaatagattttaaggcaggaacagatattaaaaaaagcatatgccaggtgcaagacaaaaactttcatagcgaattattgtttaatttatctctgatagttcagttaagacatacttataaaaatggagatatagaaaaagattttatcttatctcctattatggataaggaaactggaaaattctttgattctagagagtatgaaaatttagaaaattctttgttacctactaatgcggattctaatggagcatacaacatcgccagaaaaggattattaactttaaggcagatagacaaggacggaaaaccatcaaatatatccaacaaagaatggtttgatttcgtccaaaagtaa

SEQ ID NO: 18 - DNA, 3972 bp, Unknown bacterial species
  NT Sequence of BMC03
atggaaaaaaatttaaattatttagaaagatttactaagcattacaacactaaaaaaacattaaaaaataagttaataccttatggtaatactgctgagaacatgataaaaaataatatcatatcaaatgaaaaacaaataattttatcagcaaaaaaacaaaaacaaagtattgattttttacaaaaagaatatattgaaaataaattatcagaaattacattaccatatttaaatgattattataatgaatttattaaaaataaaaaagaacgtgatactgatgttatagacaatattgaaatagctatgagaaagcatatttcaaaatctttaacagaaaatggaaaccataaaaaatatttaaataaagaagtctttgatataatatcagaaaaaaaagaattatattatgatgtaacatttaaaagaaatgccacatatctatcagattattttcaaagcagagtaaatttatataaagattcaaataaatcatctacgattgcatcaagatgtattaatattaatttaccaatatttgcaaaaaatatagtattatttaattttattaaaaataaagcaaatattatttttgatgatttaaaagaaattacagatgatgaatacactttggattcaattttttcaatcgatttctttaatatggtattatctcaaaaaggtatagattattataatactattcttggtggcatgacaaaagaagatggaaaaaaaataaagggtataaatgaatatattaatttatataatcaaaatgtaaaagatgaaaaaaataaattaccttatccaaagaaattaaaaaaacaattattaagtgatattaattcttattcagcaagatttgaaaaatttgatacagaacaagaaatggttaaaagtattaaatctttagttgaaaatgacttatttcaaggagaattatttgataaaaaagttgatattctaaaggaaacagaaagacttttagaaagaatatctgaatatgattcaaatgctttatttattactgaaaaaaatatttcatatatttcaatagatatttttaatgataagttttttataaaaacagctattgaatatttttatgaaaataacatttgtccagattataggaaaatatatgataatgcttctaaaaataaacgtaagcaattaggaaaagaaaagaataaagttattaaacaaaaatctttttctatttcttttttacaagatgctataaccttttatattaaagatagtggtattaataaaatctctgagaattgtatcattaattattttaaaaagcatactatcaaactaacagaattatttggaaaagtatatgaagattataatgtaattaaacctattttagaacaacatttagtagaatatgaaggtaaatctatttcaaaagattctatcaaaagaagtaaaattaaattgttttcagaaaatttaaaaaatatattttattttattcgaccattaaatattatagaagaagcattaaattatgatacatctttttatacaccattcaatatattatttgaagaaataaaaaaattcaataaattatatgataaaataagaaattttattacaaaaaaaccattcaatgatgaagaaattaatttatatttcggtattccaaatttagggggtggttttatagatagccaaacagataaaagtaataatggtacacaatattgtacttatctttttaggaaaaaaaatcaattattaaattgggaatatttcgttggaattagtaaaaataaacatttatttagagaaaaagaaaatatagaattaaattctgatgaaacatcatttcaaagatattcattttacacccccaaagataaatctatttatggtagttcttatttttcagctaatgaaaaaaattataaagatgataaacaagaatttatcaatattatcaataatatagtaaataatagtggtaatgaattagctattaaagaacttaaaaaatatattaataattctactgaaaattctgaaacacctaatggttgtcttagtgttttaaaaaataaatgtaatgagatatataatcttgttattaaccatgatgattttaaagaaaaaaatgaagacattatcaataaacttaaaaacactcttagtaaattatctaaagtaccacaagctaaagaactaataaataaaaaatataatttgttttctgaaatcatatcagatattagtgaaatttgtctaacttcaacccaaagatattatcctattgatgatgaagaactaaattctgctttgaatgatgaaaataaaccattatatttctttaaaataagcaataaagatttaagtgctgatgaaaatattcttaatggtaaaagaaaaagtaaaggaaaagataatattcatactatgatattaagagccatgatggatgataatgtgacaaatattatacccacctcttgtaaaattagtatgagagaagcatctataaaaaaagatgatttagttattcataaagctaatgaaccaattaaacttaaaaattctctggctaataaaaaagaaagtactttttcatatgatataactaaagatagaagatatagtagggatgaatttttctttagtataacagcatctattaatagtgattgtaaggaaaatgattattactttaatcaaaaagttaatgaatatttaaaaaacaattccaaaattaatttattagctgttgatttaggagaaacaaatattattactataagtgttattgaccaaaaaggtaatataattttgcaaaaagatttagataaatttataaataaagaaaaaaatattattactgattttaatctacttctttctaatcgttctaaagaaagagatatagctaaaagagattggcaagaacaacaacaaattaaaaatcttaaagaaggtatgatttcatgcattatacatgagatatgtaaacttatgatagaacataatgctattcttattatggaagatttagatgctaattttaaaaataggaaaaaaagaatagaaaaagctatttaccaaaaatttgaaatagcaatacttgaaaaattaaacaatttagtttttaaagatataccaattaatgaagttggtagtgtaacgaaacctcttcaattaagcgataagtttgaaacatatgaaaaagttggtaatcaaagtggatttgtttttaaagtatcccctttttatacaagtataattgacccaacaacaggatttattaatttatttaagaaaaattttgaaagtgttaaatattctattgagttcttttcaaagtttgaaagtattagatataatacaaaagaaaaatactttgaatttgcttttgattataagaactttaaagaaattaaatatactgaaaatataaaaactgattgggtggcttgtacaacaaatatagatagatatgagtatgataaaaagaacaaaatctataaaaaatatgatgttactacggatttaaaaaatctttttgaaaatgaagaaatttattatcaaaagggtgaaaacattcttgatgtgattttaaaaaagaataatagagagttctttgaaaaactcacaaatctattaaagataactatgctatttagatatagaaattcacatttaaaattagactatatatcatcacctgtaaagaatagtaatggagaattttttagtactgaaaatggattagagaattatccgatagattctgatacaaatggtgcatatcatattgctcttaaaggaaaaatgattcttgaccgtattaatagtaattcatcagaaaaattagatacttatattagtattgaagattggcttaaatttattcaaaaatttagtgtgaataaaataactgaaaccaaaaagaataaaaaaataaatattaaatatgtttaa

SEQ ID NO: 19 - DNA, 3975 bp, Unknown bacterial species
  NT Sequence of BMC04
atgaagaatctaactgaatttacaggattgtatcctgtctccaaaactttgcgttttgaattaaaaccaactgatgatttcaattgggagacctttttggaatctaccatttttaaacatgaccaagaaagagctgaagcatatccaatcgtaaaggttatagtggatcaatttcataaatggtttattgaagatgctttaaataaatcgactatcaattggaattcactttatgatgcttatttcgcacctaaaaacgagaatagtgttgaaaacttgagaaaagaacaagataaaatccgcaaagaaatagtagatacatactttaaaaaacatgactggtggaagtacgtttcaaaagaccacagtaaattattcaaaatagaactaccagctttattatccgatgatgcttttatttatgaaattaacgataaatatccaaattatacgcaagaaatactgattgatgctttagcaaaatttcaaaatttctctgtttattttggaggttattttaagaacagggataatatgtataaatcggatgctcagagcacttcaattgctaatagaattgtaaatgagaattttacaaagttcgcagataacataaaaatttacaatagactaaaagaaaactgtttatctgaattacaaaaagtagagttagattttacagacgaattaactgggttgacctttgatgacattttttcaccttcttatttcaataaatgcctgactcaaaaaggaattgaaaaattgaatctttatattggaggaaaaacaggtaaaaataaggaagataaagtttttggaataaaccgagttggaaatgaatttttacaatttaataaagaatcgaagttaaaactcaaagaccttaaaatggtcaaactttacaagcaaatattaagcgatcgagaacaaccttcgtttttacctgagcaatttagaaatgaagatgaattaatcaaaagtattgaagatttccataatttgataacagagcaaaaactgtttgaaaggttattgaaattaatgggaagattaaaaaacggagaatgtgaagatttgaataaaatacatgttgttggcagttcattgacacaattgtcaaaagtattatatggaaattgggaagtacttggtactgctttacgcaacaaatttcaaacgaataaaacaaaaaaagacaaacttgaaagtgaaaaagatattcaggagtggatggaacgaaaatctttttcccttgctcaaatcatcgaagttgaatcatcattacaggatgataaaagtataaaagttatcgatttatttacgacattcaatgcgtggcaaaaggttaacgaaaaaccacagttagttgatttaatcaagttatgtaaagatgattttcaaacccgctttagagcagtgaaagatttgattgaaaaaggagaacaaatccaaggtaacgaatcggccaaagaagaaataaaagctgtactcgataactatcagaatttactccacgtagttaaattgttgaatctgggcaaaaaagaaagttatctggataaagatgaaactttttataatgaatataaggagattttatcatcaactgagtcggataatgtttgtcttgaagatattataccgttgtacaataaggtgagaagttttctgacacgaaaattaggggatgaggggaaaatgttgttgaaatttgattgtagtacattggctgatggttgggatgtgggaaaagaatctgccaacaactctacaattttaattgataatagtaagtattacctgataattacaaatcccgaaaataaaccagacttaagtactgcaattacctctaatacagataatgtttataaaaagattgtctatcgacaaattgctgatcccacaaaagacttacctaatttgatggttattgatggcaaaacacaacgaaaaacaggcaataaagatgatgacggaataaacagagtattggatcaacttaaagacaaatatttaccacaggaggttaatcgaattcgtaagttaggctcatatctaaaaacttcagaacacttcaataaaaaagattcacaagtatatttagcatattatatgcaaagacttattgaatacaaacagggagaaatggaattctcatttaagaattccgaagaatatgactcttattcggattttttagatgatattactaaacaaaaatactctctttcatttgtaaatgtctcgaaggaaattataacacaatggatttcagaaggaaaaatatttctctttcagatttacaataaagattttgaagaaaaggcaacaggtacacccaatttacatacactttattggaaagaattgtttagtgaagaaaatctaaaagatatagtttataaattaaatggtgaagcggagcttttttaccggaagaaaatggacggcaaaccatttacacacaacaaaggggctgttttagtgaataaaacctttgcggatggtagccctgtggaacctgaacattacaaagaatatgttgaatatattaccggaaaagtgattgaaaaacagctttcaaaagaggcaaaagataaactccatcttgtaaaaacaaacaaagcaaaactcgatataattaaggataaacgttattttcagcacaagttactattccatgttcccataacaattaatttcaagagtgaaggagtgccaaaatttaatgattatactttaaactatctgagagaaaataaaaaagatattaacataattggaattgaccgtggtgaacgaaatttaatttatgtttctgtaatcaatcagaaaggcgaaaatataataccgccaaaacatttcaatattgtagaatcggacatgtttgggatggaagataaacgaaagttcaactatcttgaaaaactaatacaaaaggagggaaaccgagatgatgcacgtaagaactggagtaaaattgaaactattaaagacttaaagacaggttatttatcattagtggttcatgaaatagctaaattagtggtagagcatcatgcaatcgttgtcttagaggatttgaactatggttttaaaagaggtagatttaatgttgaaagacagatttaccaaaattttgagaagatgctgattgaaaaactgaatcttcttgtttttaaaaataattctaattctccggattatggtaatattttaaatggtttacaacttactgcaccatttggcagtttcaaagaacttggcaaacagagtggatggctgttttatgtaaatgcatcttacacttcaaaaattgaccctcaaactggttttgcaaacctatttaatatgaaagatgcaaaaaaagatacgaagtcattctttgaaaagattacagaaattaaatatgatgatggaatgtttaaatttacatttgattatcgcaatggtttttctattgtacaaacagattataaaaatatatggactgtatgtaccaacgacaaacgtattttagttagtaaagataacatcagtggaaagttcaaacatgaatatgttgatattacagaaagcataaaaaatctttttataaacaacaatattaatgattaccactcgatttcaaaagaaactatcttatcaatcaaagaaaagaaattctttgatgatttgttcttttattttaagcttagtcttcaaatgcgaaattcaataccaaattcggacattgattatttgatttcaccagttcagataaaggggaagcctttctttgattctagaattccaaataatattaatattgttgatgccgatgcaaatggggcttaccatatagcattaaaaggattatatctggttataaatgattttccaactgagaaaaaaggaaaatctgaatacctaaagaaaataaccaacgaagattggtttgaatttgcacaaaggcgtagtttaaaataa

SEQ ID NO: 20 - DNA, 3693 bp, Unknown bacterial species
  NT Sequence of BMC05
atgagatgggatgaaaaactccagacttttttgaatgatcaggaaattgaggatgcttatcaggttttaaagcctgtatttgataaattacatgagaattttattattggcagtttagaaaatacaaataataaaaaactgttttcttttgataaatacttgaaactaaaaaatgatttgttgcacgttaataaaaaagaacaagagtcagattacaaaaagaaagaaaaggaatttgagacagagggaaagttattgcgtaatacttttgcaacggtttggataaatgaaggcaaaaattttaagaatacgattgttggaggtgaaaatgacagagaaattttaaaggaaggggggtataaaattttaacggaggcgggtattttgaagtatattaaaatgaatattgataagtttgtggaattaaaattaaagaccagagaggatattttatggaaaaaagagaatagaaacttggtagagatggctgatttggaaaagtctttgggaacaattgaatcatggggtgtttttgaaggattctttacttatttttcaggttttaatcaaaatcgagaaaattattattcaactgatgaaaaggcgacggctgtcgcaagtagagttattgatgagaacttaccaaaattttctgataatgttttggaatttaataaaaagaatgatgtttatatagggattttttcgttcttgaaaggaaaaaacattgtattgaagggcaagtcgggaaacggggaagaacaagatttattgccaatcaccgagaaaatttttgagattgaatattttaagaattgtttatcggaaggagaaatagaaaggtataattcggatattggaaatgcaaactttttaattaatttatacaatcagcaacaagataaaaaagaaaataaattgcgaattttcaagactttatataaacaaatcgggtgtggtattaaaggtgattttattcagttaattaaaacggatgatgaattaaaaaagatttttgaagacttaaaaattacgggcgataatttttttaagaacacgcaaaatttgaaagagataattttgagtttggaaaattttagcggaatttattggtcagacaaagcgttaaatacagtctctggtaaatactttgctaattgggcgagtctgaaggagcttttaaaaaacgctaaaattttcaaaaaggaaaaagatgaaattaaaatacctcaaactatagagttgtcggatttgtttggggtgttggattctaatgaactaatttttaaggaaagttttaatgaaaacgatgaattgaaacaaataattttaaagagctatgagaaaaattcaattaagcttttaaagatgatttttgtggatgttgaagaaaatcagaagatttttgggaatcttaaagatgggttgccgataaatgattttaagaaagatgagaacactcaaattattaagacctggttggatggtttgttgaatacaaatcaaattttgaaatattttaaagttcgtgaaagcaaaattaagggggcgccattgaatccggaggtttctgaaagacttaataaaattttgaatgttgaaaatccgactgttatttatgatgttgttcgtaattatttaacaaaaaaaccaacagaaggcttgaataagttgaaattaaattttgataatgcggttttggcggccggttgggatgttaacaaggagtctgagcgtggctgtttgattttgaaggatggtgataacaaaaaatatttggcaattttaacgaataaaacgcaaaagttttttggtgaaaaggtgaagtataaagaatttgttggtgatgaaaattggcaaaaaatggattacaaattgttaccaggacctaataagatgttacctaaggttttgttgcctaagagtgatagatataaatttggagcaactgatgaaatcttgaaaatttataatgagggtggttttaagaaaaatgaaccaacttttacgaaggcaaaactggccaaaatcgttgatttttttaaggatggtttgaaaaattatccgtctgcgaaaagtagttggtataatttgtttgcttttgatttttctgatacagaaaaatatgaaagtatagatcgattttatactgaggtggagaagcaggggtataaattatcttggagcgctattagcaaaaattttatttttgaaaaggtggatgcaggtgatatgtatttatttgaaattagaaataaagataataacttaaaaaatggcaaagcaaaaacaggagcaaaaaatttacatacaatttattgggggactatttttggggagtcagaaaataaaccaaagttaaatggtgaggcagaaattttctatcgtccagttgttaaggatttaattaaagataaggacaaaaacggagatataatcaaagcgagcgaaaaacgatttgaacaagaaaaatttgtttttcattgtccgataactttaaatttttgtttaaaatcaacaaggttgaatgatgtaataaatcaaataatgattgaaaacaagaaagatgtttgttttatcggcattgatcgtggcgaaaaacaccttgcttattattcggttgttaatcaaaagggtgaaattttggaacaggggagttttaacgaaattaacggacagaattatgcgaaaaagttggaagaaaaggctgggcatagagatgaagctagaaaaaactggaaaacaattggtacaattaaagaattaaaaaacggttatatttcgcaggttgtgcgaagaatcgttgatttagcagtaaaatataatgcttatattgttttggaggatttaaatagtggatttaagcgtggtcgtcaaaaaattgaaaaatcagtgtatcagaaattggaattggcattggctaaaaaattgaattttttggttgataagagtaagaaagatggtgaaattggtagcgttcagaaggctttgcagttgacgccccctgccactaattttgctgacattgaaaaagctaaacaatttggcattatgctttatgttcgtgctaattatacttctcaaacggatcctgtcactggttggcgaaagactatttactttaaatccactacccaagaaaatttaaaaaaggaaatttgtgaaaagtttagcgaaataggatttgatggaaatgactattattttgagtataaggatgagaatgcagaaaaaaaatggacaatgtattcaggtgttagtggtaaaagcttggatagatttcggggaaagaaagatacccatggtatttggaaagttgaaaaacaggatattgttgaattgttaaagaaaatttttggtcaacaaacaagcgttgtaggcgatttgaaaacaaaaattaccaacgacaatgtaaatgacttaaaatatacaattgatttaattcagcaaattagaaataccggatttaatgaaatagacaatgattttattttatcgccggtaagagatgaaaaggggaatcattttgatagtcggaaagatggtgcaattttgtctaatggtgatgcaaatggtgcatataatatagctcgtaaaggagtgttggcttttgagaggattaatgcgaaaccggaaaaaccggagctgtatattgcagatgtggaatgggataaatggttacaatctaaataa

SEQ ID NO: 21 - DNA, 3771 bp, Unknown bacterial species
  NT Sequence of BMC06
atggattcattcacacagtttacagggctttattctctatcgaaaacattgcggtttgagttgaaaccgataggaaaaaccttagcctatatcgaaaataaagggttattagtacaagacgaacaccgtgcagatagttacaaaatcgttaaaaaaattattgacgaataccataaatcatttattgaaaaatctttaaatgggttgtgtttggatggattggaggattattatttttattatcaaattccaaaaaaagatgataatcagaaaaaaatagttgaagatatactgacaaagctacgtaaacaaatagccgaacgattttcaaaacaggatatatataaaaatctttttgcaaaggaactgattaaagacgatttaaattcttttgtacaagaggtagaacaaaaggatttaattaaagaatttgaaaattttactacctattttacaggatttcacgagaaccgaaaaaatatgtattcggcagaagataaatcaacggcaatagctttccgtcttattcatcaaaacttacctaagtttcttgacaatatgcgagcatttaataaaataagtgtttcaccgcttgccgaaaaatttaagcatattctttccgacagcgaattaggtcctattgtacaggtagtagcgatggaagatgtatttaacttggcatattttaacgaaacactaacacaatcgggtattgatatatataaccatttacttggtggatatactcccgaagaagggaaagaaaaaattaaaggactaaacgaatatatcaatctatataatcaaaccgttaaaaaggaagaacgtttacctaaacttaaaccattgtttaaacagattttaagcgaccgttctacagcatcgtttattcccgaacaatataaaaacgataatgaggtattagaaagtattgaaaaattataccaagaaataaaggaacatgtttttcattcattgaaagagctatttgtacacataaatgagtatgatttgcataaaatctatttacggaatgatgtaagtatgaccgatatttcgcaaaaaatgtttggtgattggggggtgtttacaaaagccatgaatctatactttgataaacagtacaaggggaaagcaaagcttggtacggaaaaatacgaagatgaacaaaagaagtattttagcaatcaagagagtttttcaataggctatattaatgaatgcttgttgcttttaggtagtaattatcataaaaaagtggaagactattttaaagtggctggaaaaacggaagaacaagttcaaatgctttttgaaataattgaaacaaaatatcaaaacatacaagatttgcttaattcaccctatccgacagaaaaaaacttggcacaagaccaagttcaggttgataaaataaaaggactgttagacagcattaaaaacttgcaatggtttataaaaccattgcttggaaaagggaatgaagccgaaaaagacgaacgcttttacggtgaatttactgcactttgggaaacacttgaccaaattacacctctttataataaggtgcgtaactacatgactcgcaaaccatattctactgagaaaatgaagttaaatttcgacaattcaactttattagatggttgggatataaataaagagcctgataatacaagtgttgttttgcgaaaggatggtttattttatttgggtataatggataaaaaatataataaaacgtttaaacaggaatttattgaatcgaatgagccgtgtttcgagaaaatggaatacaaattattacccggagccaataaaatgttgcctaaggttttcttctcaaattccagaatagaggaatttaatcctactgtcgatttacttgaaaattataaaaaccaaacccataaaaaaggtgataaatttaatattgcccattgtcgaaatttgattgatttttttaaacaatccattaacaaacatgatgattggaaacaattcggctttgctttttcagatacaaaaaactatgacgatttaagcgggttttatcgagaggttgaacaacaaggttataaaattacctttagaaatatacctgaaaaatttataaatcaaatggtggaggaaagtaaactttaccttttccaaatttataacaaagatttttcaccctatagtaaaggtacaccaaacatgcatactttgtactggaaaatgttatttgataccgaaaatcttaaagatgtggtgtataagctaaacggacaggcggaagttttttaccgaaaagccagtattaatgacgaaaacatagtggttcataaagccaatgaagtcataatcaacaaaaatacacttaacgagaagaaacaaagtagatttgactatgacattataaaagacaaacgttacacgatagataaatttcagtttcatgtacctattaccatgaactttaaagctcgcgggttgaataacattaatttggaagttaatcaatacctgcaaaaagaaaatgatattcacattatcggtattgatcgtggcgaacgccatttattgtatctttcattaattaacagtaagggaaatatcattgaacaatattctttaaatgaaattattaatgaatataatggcaatcattaccacacaaattatcacgatttattggataagcgagaaggaaatcgcaccgaagaacggcaaaattggaaaacaattgaaagtattaaggaactaaaagaaggatatttgagtcaagttgtgcataaaatatccgaattaatggttgaatacaatgctattgttgtgcttgaggatttaaatatgggatttattcggggacgacaaaaagtagaaaaatcggtttatcaacaatttgaaaaaatgcttattgataaacttaattatttggtagataaaaagaaaaaatcgtttgaattaggaggaactttacatgcgtatcaattaaccaataagtttgaaagttttcaaaagatgggcaagcaaagcggttttctgttttatattccggcatggaataccagcaaaatggatcctgttaccggctttgtaaatctgtttgacacacgctatgaaaatgtagtgaaagcaaaagcattttttaataaatttgaatccattcgatacaacaaagacaaggactattttgaatttgaagtaaaaaaatattcagactttaatgccaaagccgaagacacacgtcaagagtggattatttgtactcacggcgaacgaattatcaattatcgtaatcctgaaaaaaacaatgaatgggacgacaaaacagtacatccgacaacggaattaaaatcactctttacatcaaaaaatattatttttgaaaacgggtcttgtttaaaagaacagattgccttgcaaaaagataccgataaagaattttttgaagggttactgaaacaatttaaaaatacgcttcaaatgcgaaacagtaaaacaaaatcagaaattgattatctattttctccggtatcaaatgaaaatggtgttttttttgattctcgtgattatgtggatattgataatagagatagaaaattttgcgtctctacgggaaaaccaacattgcctgtcaatgccgatgctaacggtgcctacaacattgctcgcaaagggttgtggattgttgaacaaataaaaaatccaaatacagacctgaaaaaactgaaattggcaatgaccaataaagaatggctacaattcgtacaaaacaaggggtaa

SEQ ID NO: 22 - DNA, 3825 bp, Unknown bacterial species
  NT Sequence of BMC07
atggataatgctttttctgattttacccagaagtatacgctttcaaaaacattgaggtttgagttgaggcctgtggggaataccgaaaagatgttggaagatgagaaagtatttgaaaaggacaagcttattcaagagaaatatataaaaacaaagccttattttgatctcttgcatagggagtttgttgaagaagcgctgaaggacgtagatatatcgggattacataattattttgaaacttaccaaaaatgggcgaaggacaagaaaaaataccaaaaggaactccaaaacaaagaacagatcctaagaaaggagatattagtttttttagacagtacggcgaaatattgggctgagaaaaaatactcggaacttagaataaagaaaaaagacatagagattttctttgaagaggatgtatttactatactaaagaagcgatatggagaagattctgaagctcaaataatagatgaagtatctggtgaaaccgtttctatttttgattcttggaaaggctttacgggctactttaaaaaatttcaggaaacacgaaagaatctatatagggatgatggcaccgctactgctcatgcaacacgaattattgatcagaacttaaagcgcttttgtgataatttggaaattataaaaagaatagcggggatcattgaattttcggaagtagaaggtaattttaaacactcgatgggtgacgtattttccttgagtttttataataagtgtctactgcaagatggtatcaatttctacaataggattttgggcggagaagttctgcaggatggtacaaaactaaaaggcatcaatgaacttatcaataaatatagacaggataataaaggagtaaaaattcccttcctgaaattactggataaacaaattcttagcgaaaaagaggagtttttagatggaattgaagatgataaagaacttttagccgtacttaaaaagttttacgaagtggctgagaagaagacatctatcctaaagtcgcttatccaagattttgctcaaaataataggcaatacaatcttgaggaggtttatatatcaaaagaggcattcaatactatttcgcgtaaatggacgcatgaaacctcaaaatttgaagaatggctttataatgtaatgaagccaaataagccgactggattaaaatatgacaaaaaagaagaaagttataaattcccggattttattcccctgtcttatatccaaaccgccttggagcaagccgatattgatggggatttttggaaggagcattattctgagaactcaaaagcaaatgatggttgcctaatgggagatgagtctatttgggaacagttcataaagattttcgaatatgaatttcaatctctttttgaaaaggaaattattgatagggaaaccggtcaacccaaaaaaaatggatataattatgttaaggatgattttaaaggattactcaatggagagaatttttctgtagaaataatcaaggattttgccgatactgtattgagtatttatcaaatggcaaagtactttgccattgagaaaaaaagaaaatggctagatgagtacgacacaggggatttttatgaaaaccctgaatttggctataagttattttatgatgatgcctataaagagatagttcaaacctacaataacctgagaaattatttaactaaaaagtcttatagcgaagaaaaatggaagttaaattttgaaaacccaacacttgccgatggatgggataagaataaggagcctgataattcagctgtgattttgaggaaagatggaaggtattatttagggttaatgaaaaaagggtgcaataaaatttttgatgacagaaataaggtggagttttctggaggagtagataaggataaatatgagaaaatagtttataaattttttccggatcaggcaaaaatgtttccaaaagtttgtttttctgctaagggattggatttttttcaaccttctgaagaaattttgaatatttataaaaattcagaatttaaaaagggcgatactttttcagttcaaagtatgcagaagcttatcgatttttataaagattgtcttacgaaatatgaaggatggatcgcatatgaatttaaacatttgaagtctacagatttgtaccgaaacaatattagtgaattttttagtgacgttgccgaagatggttataaaataacttttcaagatatttcggacaactatattgataaaaaaaatcagagtgaggaactctatctctttgaaattcacaacaaagactggaatctaaaagatgaggttaaaaaaacaggatcaaagaatctgcatactctttattttgaggcgctcttttcccatgaaaacattcagaataatttccctataaagcttaatggacaagctgaagttttttatagacctaaaactgatgaagaaaagcttgtgaagaagaaagataaaaagggtagagaagtcattgatcataagagatatgctgaaaataagatattttttcatgttcctttaaccttaaataggggcaagggggatgcctatcaatttaatgctaaaatcaataatttccttgccaataactccgatattaatgttattggagtagataggggagaaaagcatttagcttattattcggttattaatcaaaagggtgaaactttggatagtggatcgcttaatgtcgtgaataaaattaactatggcgaaaagcttcaagaaaaagcatccaatagaaaacaatctataagggattggaaggctgtagaaggtattaaaaatcttaaaaagggttatatttcacaagtggtgcgtaagttagcggatttggctattgaacataatgccatcatcatctttgaagatctaaatatgcgctttaaacaaattcgaggaggtattgaaaaaagcgtgtatcagcaactggaaggagccttgatagaaaaattgagttttcttgtaaataagggagaaaaagaccccaaacaggccggaaatttattgaaggcttatcagcttgccgctcctttcacaacctttaaggatatgggcaagcagaccggaatcattttctatacgcaagcttcttatacttcaaagattgatccattaacaggatggagacccaatctatatctgaaatatactaacgcagaaaaaacaaaagaggatattgggaatttctcaaatattgaatttaaaaatgggatatttgagtttacttatgatctaagaaacttccaaaagcagaaggagtatcctaagaaaactgaatggacgctctgctcatgcgttgaaagatttcgatggaatagagttctaaatcaaaacaaaggcggatatgaccattatgaagatataactcataattttcgagatctttttgaaaaatatgacataaactttatgagcgctgatatcaaaggtcaaatagatactcttgatgcaaaaggcaatgagaattttttcaaggattttatttttttctttaacttaatttgtcaaatcagaaatactcaacaagataaagatggtgatgaaaatgattttattctttctcccataaagccattttttgatagccgtgattctaaaaaatttggtgaaaatttaccgaataacggagatgataatggagcttataacatttcccgtaaaggaattattatcttaaataagatttcagaattctttgatgaaaatggtggatgtgagaaaatgaaatggggagatttatatatatctcataaggattgggatgactttgctcgtcaaatataa

SEQ ID NO: 23 - DNA, 4008 bp, Unknown bacterial species
  NT Sequence of BMC08
atgatgcaaattatgaaaaatttcgataaatttacgaatctatattctgtttctaagaccctacgatttgagttgaggccagaaccaaaaacattggagtatatgcgtagcaatctacgttttgataaaaatttacagacctttctggctgaccaagagatcgaggatgcatatcaagctttgaagccgatctttgattctttgcatgaaaggtttattacagaaagtcttgagtctggaagtgcgcagaagattgatttttcgaaatatttagaaaaatatcgaaacaaaagagatttaggaataaaagcccttgaaggtacagagaaacttttaaggaataattttgcagagatttataaagcaactgcaaagagctggaaagagaatgccggtaaggatggaaaaggtaaagaggtttttaaaaaggaagggtttaacattcttacagaaaaaggaattctcgaatatatcgaaaaaaatatagatagtttttcggctataaaatcacccgaagaaataagaggagccctaggggcatttgatggtttttttacatactttacgggttttaatcagaatcgtgagaattattatgaaacaaaaaaagaagcctctactgctgttgcgacccgtatcgttcatgaaaacttaccgaagttttgtgataatattttaattttcgacgagagagcggaagactatataggagcgtataaagcactccagaagatggggagagctttggtaaacaaagaaggaggggagttgccttctatttcaggcgatctttttaagattacgtttttcaataaatgtttttctcagaagcaaattgaagaatataacacagcaattggaaatgcgaattctctagttaacttattcaaccaggcaaaaagagatgaagatggatataagaagctcgcgctttttaaaactctctacaagcaaattggttgtgacaagaaagattcactcttttttgctgtcacacacgatagaagggcggacgcagaaaaggcaagggaaaatgggcaagaggcattttcggtggaagaggtgttggttttagcaaaacatgccggcgagaagtatttcaacaaggggaatgatgatggcgaggttaataccacccaagagtttatatcctatatcaaagatcgatcggattatcagggtatatattggtcaaaagcagcactcaatacaatttcaaataagtacttcgataattggtatgagttaatagatcaattaaaagaggcaaaggttttcacgaaaacaggtagtggcagtgaagataatgtaaaaatacccgatgctatagagctggaaggattttttcaggtactaaataaaatccaagactggaagacggtattttttaagaaatcaatcacagctgacccacaaaagctagggattattgaaagttccgaaactgcatcagcagcgcttctttcacttatttttgacgatgtcgctaaacatacaaaactttttattgatcaatccgaagatattttaaaggtagaaaattttgtaaaaccagaaaacaaggaagacattaagcgctggttagatcattcattggcaatcaatcagatgttgaaatattttcttgtaaaggaatctaggacaaaaggagcgcctatcgatcctactcttacaaaggctttggacaccttgttgcgctcgcaggatgcggagtggtttaaatggtatgacgtgcttcgaaactatcttactaaaaagccgcaggatggtacgaaagagaataaactcaagttaagttttgagaacggtaccctagctaatgggtgggatgttaataaggagccagataatttttgtgtcattctacaaaacccagagggtaaaaaatttcttgctattattgctcgccaagaaggacaaaaaggttttaatcaggtttttgcgaagaagcatgataacccactctacaaggttgatgaggggggagttttctggagcaagatggaatataaacttttgcctggaccaaataagatgctcccaaaatgtttgatgcccaagtcaaatagagagaagtatggagctacagaagaagttttgaaaatatataaccagggtagctttaagaaaacagaatcgaatttctcgaaaaaagatctatccaggttaattaatttttataaatctgctctccagcaatacgaagactggcggtgctttaatttttctttccgagcaacggattcttatgaggacataggtcaattctaccgagatgtcgaaagccaaggatataagttggatttccaaagcatcaacaccgacgttctagatgagttggttgaagaaggcaagatttatttgtttgaaataaaaaatcaagactcaaatcaaggcaaaagtagtattcatagagataatttacatacgatgtattggaatgctcttttccaagaagtattaaatcgtcctaaacttaacgggggcgcggaactgttttatagaaaggcgctctcaccagagaaaataaaagaactaggatcggtagataaaaatggcaagaggatcataagaaattatcgtttctcaaaagaaaagtttatttttcatattccaattacgttgaatttttgtttaagtgacacaagggtcaatgataccgtcaatcaagagttgtcaagaacttcgagtagtcactttcttggtattgaccggggagagaagcatcttgcgtactattttctggttgatcagaatgggaaaattgtgttggacgagtatggaaaagcagtgcaaggcactttgaatataccttttctcgacaacaacggtaatgtgcgaaagataaaagctaaaaggcgaagtctagatgagaatggaaaggaaaaaatagaggaggtttggtgcaaagactataacgagcttttagaggctcgagcgggtgatagagcctatgcacgcaaaaactggcaaacaataggaaatataaaggagttgaaggaggggtatatctcacaggtggtgcgaaaaatagttgatcttgctatagaatacgaagcgtttattgtcctcgaagatctcaatgttggctttaagcgtgggcggcaaaaaatcgaaaaatctgtatatcaaaaactggaacttgcgctggcgaaaaaacttaactttgttgtagataaatctgcaaaaataggaggattaaagtctgtcactaatgccttgcagcttgcgccccctgtatctaatttcggagatattgaaggtaggaagcagttcgggattatgctctacacgagagctaattacacttcacaaacagaccccgctacagggtggaggaaaagcatctatcttaagaggggatcggaagaaagcattaggaagcaaattatcgattcctttgaggagatcggctttgacggagaagattattttttcacttatacagattcggtagcgggtagaacctggattttatattcgggtaaaaatggaggctctttggaccgtttttatggcaagcgtgacaacgacaagaatcagtgggtaagtatgcggcaagatgtctctaagcaactagatgggattttagcaaatttcgaaaaggatcgctcaattcttgcacaaattattgatggggaggttgacctcattaaagtagagcaaaaatatactgcctgggaatcatttcgatctactatcgatttaattcagcaaattcggaatacaggtactagtgagagagatggagatttcattctttcgcctgttcgagacgagagaggtatccattttgactcacgggatactagggaagggatgcctacgtctggggatgcaaatggagcatacaatattgcaaggaaggggacgattatgggcgagcatataaaacgagagtatagtagaatgtttatttctgacgaagaatgggacgcgtggcttgctgggaagcaagtttgggaaaaatggttgaaggacaacgagaagatattaaagaaaaagtag

SEQ ID NO: 24 - DNA, 3825 bp, Unknown bacterial species
  NT Sequence of BMC09
atgaaaaattccttggaggactttacgaatctatacagtctccaaaagacacttagatttgagcttaaaccaataggcaatacacaatctatgttggaagaagatggtgtatttgataccgatgagaaaaggaaaatcgcatattctaaaacaaaaccgtatatagaccgtttacaccgtgaattcatcgaagagtccctcagtgatgcacaaataagtaaattggatgaatacttcaaagcatatgtcgactataaaaaggacaagaaggatactaaaagattcaataggataaaacaatttaaatcagtacttaggaaggaagttgttgatcacttcaataagcaagggaaggaatggactactgttaaatttgctcacctgaaaataaaaaagaaggatctagaagttttattcgaaaagcagttgccaaacattctaaaagaagaatatggtacagaaaaagaaactcaaataattgatgaggacagtggtgaagtaacatcgatattcgatatgtggaatgggtttatgggttactttacaaagttttttgagacaagaaaaaatttctacaaatcagacggtacctcaacagctatcgcaactaggattattgatcaaaacctcgaccgatttattgaaaatatactcatatatgactcaattaaacctaaaatcgataccagcgaggttagggaattcttcaatttagagtccgatactattttttccatggaattctataataattgcttacttcaagctggtatagaccaatacaacaactttttaggtggaaaaacccttgaaaatgggaggaagataagaggtataaatgaacttatcaataaatacagacaggagaacccagaagataagatcccttttctgaaaaagcttgacaagcaaatacacagtgagaaggagaagtttattcagcaaatagaaactcttgaggacctgaaagaagaattacaaaagttttataactcatctaatgagaaaatcaaaattctggataacctcctcagtagaattgaggagttcaagccagaaggtatttttatttcaaagcaagccttcaatacaatctctagaagatggacagaccaatcagaggcctttgaaaccagcctatttgagtcactaaaagaagagaaaccaataacagggacagcaaagaaaaaagacgatggttacaatttccctgaattcatatcattacaaagcattagaaatactcttaaaaaagttcaaggggaggaaaggttttggaaagaaaggtactaccgagacaacagtgaatccggtatcttggctggaaatgaagaaatctggacgcagtttttgatgatatttaaaagtgaattcaattcaaaattcgaaagaaatgatccggaagacaacggcaccattggatataatttatttaaagaagatctcgagaaactacttaaagaccttaaaataacaaaagacacaaaatctataattaagagatttgctgatgaagctctgcatatatatcaagttggcaagtatttcgcattagaaaaagacagggtatggatcagtagttatgatgacttactagacactttttatacagaccctaatactgggtatttgagtttctacgaaggggcgtatgaacagattgtacagccatacaatatgataagaaactatctaacaagaaagccatatagtgacgaaaagtggaagctgaattttgagaaccctactctagcgaatgggtgggataaaaataaagaaacagacaattcctcaataatgctccgaaaagaaggggcttactatcttggaattatgaaaaagggaaagaacaaattatttgaggaacgaaatagacaactgtttgagccaaagaatggtgaagatacttatgaaaaacttagttataaacttttcccagatcctgcaaaaatgattcctaaggtatgtttttcgaataaaaacatacagatgttttctccttctacagaaattatgaatatttataacggagaaacatttaagaaaaatagtgatgatttttcagtatctagtatgcaaaagctcattgctttctatactaaatgtttgagtcaatatgaaggttggaaatattatgacttcaaatatataaagtctcctgatcaatataaggataatataggagagttttataatgatgtcgcaaagtctgggtatagagtctggtttgaaaatatctctcagagttacgttgactcaaagaataccatgggagagttgtatttattcaaaatacacaacaaagactggaatcaaaaagacaaaaagaccaaagtgggaagtaaaaacctacacacacattattttgaagagcttttttcacaagacaatattgaaaataactttcctcttaaacttaatggggaagcagaggtcttttatagacctaaaacaaatccagagaagcttgggacaaaaaaagatagtaaagggagagaggtcattgatagaaagagatatgcatcagataaggtactattccatgtcccaataaccctaaacagaactcctgttacaactacaaagctcaataaagaaatcaacggtttcctagcaaataacccaagtatcaatataatcggagtagatagaggtgaaaaacatttagtctattactctgtagtaaatcaaagaggaaagatgctggaaagcggcagttttaatacaataaacggtgttgactatcacggtaagctcgaagaaagggcagaccggagagagcaggcacgcagagattggcaggatgttgaagggattaaaaaccttaaaaaaggttatatatctttggttgtaagagagttagcaaatctttctataaaatataacgctattatagtaatggaggatctcaacatgagatttaagcagataaggggaggaatagaaaaaagtgcataccaacagctagaaaaggcattaattgaaaaactaaactatcttgtaaataagacggaaacagatccacaaaagacaggtcatatactaaaagcataccagctaacatcccctattaaatcttttaaggaaatgggcaagcaaactgggatcattttttacactcaagcatcctatacttccgtaacagacccaataacagggtggagaccaaacctatatcttaaatatagtagtgcaagcaaagcgaagagtgacatactaaagttttcaaaaatctcatacaacacaaataacaatcgatttgagtttacatacgacctaagaaattttgtaaatatgaaggcttatcctcagaagactgcttggacaatctgttcaaatgtggagcgattcaggtgggataggaaaggaaataagaataatggagagtacatacaatacaaggatctaacagaaaactttaaaacattctttgaagaagttagtataaactacaaaggagatatactgtttcagattaaaaatctaagtgaaaaaggcaatgaaaaattctttagagaccttatcttctacattagtctaatttcccaaattagaaatacacaaaaagacaagaaaggagatgaaaatgatttcattctgtccccagtagaaccattctttgacagtagaaaatctagtacttttggagaaaacctaccactaaatggagatgcaaacggtgcctataatattgcaagaaaagggattattatgttaaataaaatctcaaaaggttcaaaaaataaagtcaaagaagatataggatggggagatctatacattccacatactgagtgggacgattttgccacagggagcatttag

SEQ ID NO: 25 - DNA, 4371 bp, Unknown bacterial species
  NT Sequence of BMC10
atgagtacaaaaaggagtttttcagattttacaaatttgtatagtgtaagtaagactcttagatttgagttgaaaccaatcggaaagacgctcgaaaatatgcgagagcgtatctataatgacaaaaaagattatgattctgccctacaaacatttctccatgatcaagcaatagaagatgcatataaaacactcaagcccattctagatagcttacacgaggaatttatcaataccagtctcaattcttccaaggcaaagaatatagatctttcagagtatctcaatgcatatagagaacgaggaaatgatacaaagactggtgaagaatcaaaattatcaggaattgaaaagagtcttcgaaaggcgataggagaaacatatcttacatgagcgaagagctttaccgaacaagcaaaaaatttgattggaataatagaggatatatgagatacggaagaagagtgagacgaggaaaagaaaacaaaatgactctttaagaaaaagaattttgaacttttgactgagtcggggattttggtatttatcgaaaaaaaactggataccatgaacattagtgagcaagaaaagacggatataaaaaaggctctcgaagagtttaaaggattttttacctatttttcaggttacaatcagaatagaaagaattactatgaaacaaaagcggaaaagaaaacagcaatcgcgacacgaatcgttcatgaaaatctcccaaaattttgtgacaatgtcatcttgtttcacggatatcaaaaaattctcaaggatggatcaaaacgagaatacaagaaaaaggaggagtatctcgggatgtatgcatttctcaaattaagaaacatagaaacatgcatcaaagatgctgagtcaggagagatgattgagctctatgctattactgaagatatttttgatatatctttcttctcatcgtgccttgctcaacgagaaattgatgagcataatcggatcattgggggaattgataaatacaatcgtattatcggacactacaatgctctcatcaatctctacaatcaggcacgcaagaaagacgaaaaattcacaaaactctcgccattcaaagagctctacaagcaaatctgatgcggtaataagaagtgaagttggatcaaagccattactcatgatactgacgagcagattcttgcagataccaatcatacaggagaggcaatttctgtagagcgtattctgagtcttgcgagcaaagcagggaagaaatattttcagccatgaaaaagcacggatgatgggataaaaacagttcctgattttctcgattggctcaggggacaaacagattggaatggcatatactggtcgaaagcagcgatcaacagtatctcaaatgtctattttccaaattggggaagcatcaaagaaaccatgaaaggcgacaaaacgctcgtttcttacgacaagaaacgagaggagcaaatcaaaatcaatgaagcagtggagctttctggactttttgatatattggatagcactgatggtgactggaagcaagaatgagtactcttcaaagcaagtcttacaaaattattggacgcatcagcagaaaatgccgaagaaaatagtaaacgagcgagaagaaaagatatcatcgatcgatcatcgtctccaagtcaagcacttcttgctctcattacagactttatagaagaaaatatgaagcattttctcgatcaatctcatacgattttgagactgaccgagtatagctctcccaaaagcaaagaagccataaaatcatggatggatctggcactctcagtgagtcaaacaattcgatattttcgagtcaaagaatccaagaccaaaggggatactctcaatgctgagttggtgggtattctcaccaatctgctggatgcagaagatgcaacttggtttgagtggtatgatctcctccgaaactatctcaccaaaaagccacaggatgatgcaaaagagaataagttgaagttgaattttgcaaacagtactctcgcagctggctgggatgtgaataaggaaacggataatacctgtgtcatcttgcaaaatcctgaatgaaaaacatatcttgcggtgatgaataaaaataaaaaaaacgtttttcagaaagaatggaatgaatgaagatgaaagaagaaaaccacaaaattgaatccattgtatgaaattgattgaggggaaagctggaaaaagatggagtatgatttttggtctgatgtctcaaaaatgataccaaaatgttcaactcaattaaaaaaggtcattaaacatttcaaagaatccgacgaagattttatttttccatccggatataaggttacttctggagaaagatttatcgaagaatgtagaattacaaaagaacaatttgagctcaacaataaagtttataagagggatggtgatagaattataagtgcatttagatatgagttgtctgagacggaagaaaaaacttatatcaaatcttttcagaaagggtatttggatatgttgttaaaaagcaataatctcccagaaactgaacaagaaatataccgaaaaaaatatgaagattcgctcagtaaatggattaacttctgtaagtatttcatttgaaaatatccaaaaacttcactttttgaatatcaatttgatgagactgatcattataagtctgtagataagttcaatcttgatgtagatatatgatcatataagcttaaggtagatacaaagataaacaaaaccattctcgatactctggtagaaaatggagatatttatctttttgagataaagaatcaagattctaatattggaaaatgagagaaccataaaaacaatcttcatacaacttattggaaatcaatttttgaatcagtccaaaatcgtccaaaactcaatggagaagcggagatattttatatgaagccactttctcctgaaaaattgcaaaagaaaatcgataaaaaaggaaaagaaataattgatggatatagattctctcgggaaagatttatatttcattgtcctattactctcaatttttgtcttggtaatgaaaagatcaacaatatcatcaattttgagctttcaccaaaatcagacatctattttctcggtcttgatcgaggagaaaaacatctcgtctactactctatagtggatcaaaacggaaaaatgatagatcagtgaagttttaatgaaatcaagtgaaaagattatcatgcacttctgacaaagcgagaatgagatcgtatggaatctcgcaagaattggcagacaataagcaatatcgccaaactcaaggagtgatatatttcacttgtcatccatgagatcatcgagaaactgaaattgaatccatgatttatcgtactggaagatcttaatactggattcaagcgaggacgccaaaagatcgagaaatccatctaccagaagtttgaacttgcccttgcgaaaaaactcaatttcgtcgtggacaaatcagcaaaactcggggaagtcggatcagttaccaatgctcttcagctgactccgccagtatcgaattatggcgatatcgagaatcggaagcaggttgggatcatgctctatacccgagcaaactatacgtctcagacagatcctgcgacaggatggagaaagacgatctatctcaaaacagggagcgaggaaaatatcaaagaacagattgtcactcaattttctgatattggttttgacggcaaagattattattttgaatacactgataaaatagggaagacttggattctatactctgggaaaaatgggaaaagtctcactcgatttcgcggagttcgcggaaaagaaaaaaatgaatggaacataaaagagataaatgtccgaaatatgcttgatggaatatttgcgaattttgataaggatcgctctttcctctctcaaatactcgatgaatgagtggaaatcaaaaaaatagatgaacatactgcttgggaatcacttcgatttgctattgatctgatccagcagattcgaaattcaggagacaaaactcaatgagaagatgataattttctcttttctcctgttcgagatgcacaggggaatcacttcgatacacgagaacaaaaagaggggttaccaaaagatgcagatgcaaacggtgcctacaatattgcccgcaagtgaatcatcatgaatgaacatattcgtatcaatgaagatacgaaagatcttgatctctttgtctctgatgaagagtgggatatgtggcttacagacagagaaaaatggaaagaaatgcttccgatatttgcatcgagaaaagctatggaaaaacggagagggaaatag

SEQ ID NO: 26 - DNA, 3954 bp, Unknown bacterial species
  NT Sequence of BMC11
atgtcgcagaacaacacttttgaaaagtttactaaccagtattcactaagcaagaccttgcggtttgaattgcgtcctgtaggaaatacagaacaaatgcttgaagatgaaaacgtcttcaaaaaagatgaaataattcgtaaaaaatacgaacagaccaaaccttttattgataaattacataaagaggttattaaagattctttacatggtaagaagattgaaggtttggatgattactttaaaaagttcgaaatttattcaaaaaataagaaagattctaaaataaagaaagaatttacagataaagaatcggaattaaggaaacaattaaatagtcactttaaggcagaaagtttattctctgagaaggtattttcgttgttgaaagaaaagtatggtacggaggatgagtcttttgttaaagatgaaaacggtaattttgttctagatactgttggtgaaaaaatttctatttttgatgagtggaaaggttttactggttactttacgaaatttcagaaaactagagagaacttttataaagatgatggaacttctacagcaattgtaactagaactatagatgagaacttatatagattttgtgaaaatatcaagcattttgaaagtataaaaaatagagtaaatttttcagaaattgagaagaattttaacttcaagttagaaaatttatttaaggcggatttttataattcttgcttactccaagacggaatagataaatacaatgatattttaggcggtaaaacattagaaagtggtgaaaaattaaaaggtttaaatgagattataaataaatatcgtcaagacaataaggttgaaaaaattggctttttcaaaatgcttgataagcaaattttgggtgataaggaaaaaccaagttttattgaatcaattgcagatgataatgaattactattaaaattaaaagaattctatacaaacgcagaagaaaaaactgaagtattaaaaaagttatttagtgatttttctaagaataatgatagctacgatttatcaaaaatctatataaataaagtcggaataaatactattctgttaaagtggtttgatgttgctggtagaagtgattttgagaaaaatatttctacacaaactaaaaaagaaaaaattgttacttttgacaaagatagtaatagttacaagtttccggaatttttagcttttagtcacataaaagaagctttaagtaacggaacttatgaagttaaagaaatttggaaagaaagatattatcagtcagaaaataaagaaaaatcagaaaaagcgccactgaaaaaagattcagctatttcacattgggaagaattcttacaaatttttagttatgaatttgatttgttgtttgtaggagctgaaagccaagcaggatacaattcaaataagaatctttttgaaagtttaataaaaaagaatgagaaaggtttttctatttctcctgaagaaaaattagtcattaaaaattttgtagataatactttgtggatttatcaaatggcaaaatactttgctattgaaaaaaagagaaagtggctagagtcagaatatccaactgatagtagtttttacgacagtgaagaatttggttttaaaaataaattttacgatgatgcgtatgacaaaattgtaaaattaagaatgcttttacaaagtcatctaactaaaaaaccttttagtactgataagtggaagttgaattttgaaaacccaactctagctaaaggttgggataaaaataaagaaagtgataattctgctgttcttctgagaaaagaaggcaggtattatttggcggtaatgaaaaaagggaataataagatttttgatgataaaaataaatcaaattttttagaaaatatagaaggtggaaaatatgaaaaaatggtttataagcagatgtctgatccgtcaaaagatatacagaatttgatggttattgacgacaagaccgttagaaaggttggaaaaaaagaccccctcgatggtgttaatagacgacttgaagaattaaagaaggaatatttacctagagacataaatactattcgagaacaaaaagcttatttaaaaagtagcgataacttcaacttaggggacgctaacttatttataaactactataaagataggctggtagaataccataaggacatttttgtctttagttttagagacaggtactctgattttcacgatttctctaaacatgtagcagaacaaacttacagcctaagctttgaagatatttctgagttttatattcaagaaaagaataataatggagaattatttttatttgaaatccataataaagattggaatttagaaaagaagggtggagatagaaagagtggtgctaaaaacttgcatacggtttattttgaaagcttattttcaaaagaaaacgaaaataataatttctcgattaaattaaatggtgaagccgaattgttttatagaccaaaaactgatgagcaaaaattaggaaataaaaatgatttgaaaggaaaaattgtcttgaacaaaaaaagatatgctgaaaataaaacttttattcatattcctattacattaaacagagttgcttctgagtctaaatacttcaatcaaaaattgaatgattttttggttgggaatcccgatataaatatcattggtattgatcgtggggaaaaacatttaatttactacgctggaatcaatcaagcaggggaatttttgaaagacgaaaaaggaaatctagttttaggaagcctaaacaccataaacgatgtaaactacgctcaaaaactagaagaacgtgccaaagggagggtaaaagctaagcaagactggcaagaaatagaaaatataaaagatttgaaaagaggatatatttctttggtggtaagggaattggctgatttgattattaaacataacgctatcattgtttttgaggatctcaatatgagatttaagcaaattcgtggcggtattgaaaagagtgtctatcagcaattagaaaaagctctaattgataagttaaactttttagttaataaaggtgaaaaagatccgacaaaggccggacatctcttacgagcctttcaattaactgctcctatttcggcttacaaagacatgggtaaacaaacaggggtgattttctatactcaagctagttatacttcaaaaacctgtcccgagtgcggttttcgaccaaacgtcaggtgggaaccaaaatcaattaaagataaaataaaagaaggtaagttagaaattacttataaagaagatggttttgaaatttcctataaattatctgattttagtaaatctcaaaatcaatcaaaaagaagaaatattctttatactaatgtttccaaacaagataagtttaatttaaacaccaaagatgctgttaggtgtaaatggtttagaaaaactttgtcagaaaatgaattaaataaaggagagcaaaaattaaacattcagactgagacaggggtaaatattgagtataaaatttctgattgtttgattggtttatttgagaaatatggactagattatcaaaataatctacaagaagaaattaaaaactcaggagactctttgccagttaagttttacgacaaattaagtttttatctgcatctcttaacaaataccagaagtagtgtttcgggaactgatattgatcacattaattgtccgaactgtggattctgtagcaagaatggatttaaaggaggggagtttaatggtgatgctaacggtgcttataatattgcacgaaaaggaattattattttggataagttaaaaaattataagacagaaaattctaacttggaaaaaatgacttggggcgatttattcattgatattgatgagtgggataaatttacccaaaacaaaacctaa

SEQ ID NO: 27 - DNA, 4158 bp, Unknown bacterial species
  NT Sequence of BMC12
atggaaacaaaaaataaaagtatttggggagattttactaataaatactctttaagtaagactttgcggtttgagttggtgccagtgggaaagactcgtgaaaatattcaaaaacacaaccctgagtttgttcaagaccaaaaaattgaagaagcttatcaaatattaaaatcggtttttgataaaattcatgaagattttattacaaaaagcttagagagtgatgaagctaaaagtataaatttttctgaatattttgatttatataaaaaatggaatgagttaaaaaagaagaaaaccaatgaaaaaaacatagagataaaaaaagagattcaaaatgaaatagaaaaaatttataaagataatggtggaagtaaaggtgaaattcaaaagatagaagacgaattaagaaaaaggtttgaagaaatatttaaaattcaaggaaaaatttttaaggaaaaagcgtgtgagttaaatattaaagaaggccaagaaaaagacgatgatgaagagaaagatgataataaaaaaggctttagaaaattattaaaagcaaaatttttatatgattatttgtgtaatttgattgaaagtaaaaatataatatataaagatttttttgaaaacataaagaataaagaaggagagagtatttcaaaagaaaagacaaaagacgctcttataagatttaaaggttttacaacttattttggcgggtttgagttaaatagattaaattattatacaacaaaggaagaaaaatctactgctgtagcaacaagaattgttaaccaaaatttaccaaagttttgtgacaatgttattctttttgaaattaaaaaatcagaatacctcaaaattgatgaatttttgaaaaataaaaatatttctttaatttctaaaaatcagaatggaggtgaggttgaattacataaaataaataaaaatttttttgaaatgatgttttttagcaaatgcttatctcaaaaagaaattcaaaaatataatttagaaattggaaatgcaaataacttaataaatagatacaaccagcaacaaagtgacaaatctcagaaattaaaattatttaaaactttacacaaacaaattggatgcggagatagaggtggatttattccatcaattaaaggtgaggaagacttaagggagagattgcaagaaattaagaataacagtattgagtattttgaaaatataaatgactttattgaatatttaaaaaatcatgaaaattatgagaatgtttactggtcagacaaggcaataaataccatttcttcaaaatatttttctgattggttaaatcttaaaaaagaaatttggggcaaaagagacagaaagggtaacttaaaagatgaagaaactaaaattccacgagccgttcaattaaaggatctgcttgaaaatctagacaaaatcacagactggaaattagaaggtagattatttaaactttctctatttgaaaatggtagaaaagctaaaaaattacagcaagaagatttaaataaatttaataaaaataaaatagagaatgaactagagattgaaaaattgcagattatagaacaaaacccaagtccttttcaggctttactaaatatgatttttgctgatatcaaaagcaaggaaagtgcctttttagagagtcggatatttgagatttctgattttgttcacaatgaagataaacaaattataaaacaatggcttgattctattttagctataaatcaaattataaaatattggagagtaaaagatacatttggaaccgaaggaactctcgatgaaaagttaaagaatattatttattcagaaaaaaatccaacaagattttatgatattattcgtaactatctgacaaaaaaaccacaagacgagttaaataaattgaagcttaattttgaaaattctactcttgctcaaggtttggacgtaaataaagaaaaagacaatttctgcataattttacgagacgacaaacaaaatcaatatctaggtattttgaatagtaaaaataaaaatatttttgagatagatcaaaatgaagatatatatcaggatgacggtctgggttggagtaaaatgatgtataaacttattcctggagcgagcaagacacttcctaaaatatttttctcaaagagatggacagaaaataacccaacaccagatgagattagtaaaataaaaaagggtgagacctttaaaaaaggggataattttattaagagagatcttcatgaattaattaatttttataaggctaacttagaaaagtatccatcggtaaatgagagttgggctaaactctttatttttaattttagtgatacaaaaacatatgaaagtatcgatcaattttacaatgaggttgataaacaaggatacaaggtttcttttatctcaataaataaaaacactctggataattttatagacaaagaaaaattatacctatttcagattaaaaataaagataataatctagataaaggcgagaaaaaacaaagcaataaaaatcttcatagtatttattgggaggctatttttggtaaagccttaaataaaccaaaattaaacggcggggccgaaattttttatcgtccagctttgtcagagaaaaaaataagtgaactaaaaattaaagataaaaatggaaaaaatataattataatcaaaaattatagatattcaaaagataaatttatttttcattgccctataactctaaattttagcgcaaagtcatctaaattaaatgatgaaataaatgatcacataaaaaacaaaaaagaattttgttttatgggaattgaccgtggcgaaaaacatcttgcttattattctttggtaaatcaaaatggaaaaattttagataaaggccaaggaactctaaatctcccatttgtagataaagacggaaataaaagatgcataaaaactgaaaaatattttgaggaggataaaaaagaaaacgagaaatggaagccaagaattattgattgtcctgattataattgtcttttggatgctcgtgcctctaatcgtgatttagctcgtaaaaactggcagacaattggaactataaaagaattgaaagaagggtatatttcccaggttgttagaaaaattgttgatctggcaatagagaataacgctttcatcgtattggaaaatctaaatattggttttaagaggggtcgtcaaaaaattgaaaagcaagtatatcaaaaattagaacttgctttggcaagaaaattaaatttcttagttgataaaaaagcaataatcggagaagttggttcagtcacaaaagcgttacaacttactccgccggtaaataacttcggtgacataggaggcaaaagtcaatttggtataatgttttatacaaaagctgattatacttcacaaactgaccctgtcacgggttggcggaaaagtatttacctaaaaagggggccggaagattatatcaaagaccaaatacttggcaataaaaacaaaaatattgaaccggcattcgaagacatttgttttgatggacaagattattgttttacttatataaataaaaatactggtaaaaaatggacactatactcaagtaaaaacggtaaaagtttagatagatatcatcgggaattagtatatgaaaatagcgacaaaaaatggttacccaaaaaacaagatgtcttagagatgctcaataatttatttgaagggtttgataagaaaaaatctttgcttaaacaattagaaactaaaaacccaaataaaacaggagaacaccccgcttgggagtctctaagatttacgattgatttaattcagcaaattagaaatacaggcataaaagaaagagatgaagactttattctttcgccggttagagataaaaaaggtgatcattttgactcacgcgaggcttccccagatttaccaaattcaggtgatgccaatggcgcctataatattgctcgcaaggggataattatggcgaaacacattgaaaaaggatactttctttatattagcgatgaagaatgggacgcctggcttgctggtgaagaatgctggaatcgttgggctgaaaaaaacactaaatctctactaaaaaacaattattga

SEQ ID NO: 28 - DNA, 4158 bp, Unknown bacterial species
  NT Sequence of BMC13
atgagtacaaaaacaattttttcagattttaccaatctctatgaattaagtaaaactttgaggtttgagttgaagcctgtttgagagactgaaaatttactaaatgaaaatcaagtatttttaactgacaaaatcagacaaaaaaagtatgaagaaataaaaccatttttagatgaatttcatttggattttatacatttttgtctttcagatttacatttagattatactgaatataaaaaatctttggataattatcaaaaagataaaaaaaataaagatttagaaaagaaaaaagaaaatgaagaaaaaaagctaagagaacaaattgtttgaaaatttgattcaaaagttgaagattttttaaaaactttttgaaaagttgaaaaaattaaatgaaaaaaagataatgaaaaatttaaagtaagtttatgaaaagattgggaaatagaattttctaaaaataactatgaatttctttttgaaatctgaatttttgatttgatgaaaaagaaatttgaatgaaactgagatatttatgtcgcagataaagaaacttgagagatttatcaggatgaaaaaacttgaaaagatatcactatttttgatgattggaattgatggcttggatatctaacaaagttttttgaaacaagaaaaaatttatataagtcagatggaacttctactgcaattgctacaagaattattaatgaaaatttaaaaaaatattgtgaaaatttagatatttataataaactttctcaaattgagaatttaaaaaataagtttcaaaacttagaagctgatttttgaattaaattagaaaagttttttagtttagagaattataactcttgtatattacaaaattgaatagaaaattataatgatatcaggtgatgaaaattagaaaaaaataacaataaaattccttgaataaatgaatatataaataaatataggcaagatagttgagaaaagcttccttttttacaaaaacttgataaacaaattttagcctgatgaaaagaaaattttatagaacaaatagaaaatgaaccatcttttgaaaaatgtttgaaaaatttttataataattcaataaaaaaagtagacattttaactcaaatttttcaagatttaagtacctacactaatgaagattataaaactatttatttttcaaaagaagctttcaataccctttctcataaatttacagaccaagttttaaactttgaaaaacttgtttttgaggaactcttactaaataaattagttgagaaaaaggattttgataaaaaagaagaaaaatataaatttcctgattttatacctttattttatgtgaagaaaggattagaaaattatcatacaaaaaatttattttataaatcaagatattatgaaaacgaaattatagaagaagataatgataatatatggcagaaattttgtactattctcaattatgaattccagtctttactttcaaatacgataataaaccaaaatggagaagaaatagaagttgggtttactatttcaaaaaataagttagagaaaattttagataacttctctctttgagaaaataataattgaattattaaagattttgcagatataagtaaaactatctatcaaatgtgaaaatattttgctttagagaaaaaaagagaatggaataataattttgatttaaatgatgatttttataaaacagaatattctcaagaaaatgaaaaatattgatatttagaattttataatgaagcttatgaacaaattatagttccatataatttgatgagaaattttatagcaaaaaaaccttgggaagataataaaaaatggaaattaaattttgaaaattctagtttattgaaatgatgggataaagaatttgaaagttatggatcttatatttttgaaaaagcttgattgtattatttatgaataataaattgaacaaaattaaataaaaatgaaattgagaaactctataattataatgcaaataattgagcaaaaagatttgtttatgattttcaaaaacctgataataaaaatacccctagattatttattagatcaaaatgagataattttgctccatcagttaaagaattaaatttaccaataaataacattattgaaatttatgataaagaattgtataaaaaagacaaagaaaaacctaacaaacataaagaaagtttaatgaaattgattgattattttaagctttgatttagaaaacatatatcttataagcattttaattttgtttggaaagagagtaataaatatgataatattgctgatttttatagagatgtagaaaaatcatgttataaaccatattgggaagaagatataaattttgatgaattaaaaaatcttacaaaagaaaaaagaatgtatttgtttcaaatttataataaaaattttgaattagatgaaagtatatctacagacgattatacttttaaatgaaattgaaaagatagtgttcatacaatgtattttaaatgattattttcaaaagataatttagaaaataaaaattgagtaaatctaaaattaagctgatgatgagaattgttttttagaccaaaatctatagaaaaaaagatagataaaaatagaaaaagtaaaagagaaattatagaaaataaaagatattctaaagataaaatactattacattttccaattcaagtaaattttaaagaaaataaaacttcaaattttaataattatataaacaattttctcgcaaataatccagatataaacattatttgaatagatagatgagaaaaacatttagcttactattcagtaataaaccaaaaacaagaaattattgaaagttgaagtctaaattatatttatcaaaaagataaagatggaaaaattattcaaaagtctgagaaaaaaatacaagaagtgagaaatgatgaatgaaaaatcattgattatgaattagtggaaacttgaaaattagtagattatgaagattattgaatattgcttgattataaagagaaaaaaagaagattgcaaagacaatcttggaaggaagtagaacaaataaaagatttaaagaaatgatatatctcagcagtggtaagaaaaattgcagatttaattattgagcataatgcaatagttatatttgaagatttaaatatgagattcaaacaaattagatgatgaatagaaaaaagtgtgtatcaacaattagaaaaagctctcatagataaactcaattttcttgtaaataaatgagaaaaagactcagaacaagcttgaaatttattaaaagcttttcagttaactgctccaatttgaacttttaaagatatgtgaaaacaaactggaatcattttttacactcaagcccgttatacttcaaaaattgatccactcacttgatggagaccaaatttatatattaaaaaacaaagtgctgaactcaataaagaaagtattttaaaatttgattctattatttggaataaagagaaagaatattttgaaataacttatgatttagagaaatttcaatcagaaagtacaaaaaatttaaaagagaaaaaagaagaaaaattagaaagaacaaaatggactctatcaacaagagttgagagattcaaatggaataaaaatctcaataataataaatgatgatatgaacactttgaaaatttaaatatacatttcaaagaactttttgaaaaatattgattagatatttcttgagatattttaaagcaaattcataatttagaaacaaagtgaaatgaagcattttttagtcattttttagatttatttaaacttgtatgtcagattcgaaacactaatcaagataaaaaatgaaacgaaaatgattttatttattctccagtttttcctttttttgatagtagaaaacaaaatacagtatgagttaaaaatggagatgataattgagcttttaatatagcaagaaaatgaattattatcttggagagaatttgaaaatggaaaaaagaaaatgatatgaaaatacaaaaatgagaaaaggaaatgtatccagatttatttatttcaaatataggttgggataattttactcagaatcataatattcgagataattaa

SEQ ID NO: 29 - DNA, 3933 bp, Unknown bacterial species
  NT Sequence of BMC14
atgtcgcagaacaatataaaagagaaaagtatttttgatgaatttaccaacaagtattcacttcaaaagacattgcggtttgaattacgtccggtactaaatacggagcagatgcttaccgacagtggaataatcaaactggatgaaaagcgaaagctgaactatgaaaaaacgaaaccgttcctcaatcgactacatcaagagtttgtcaccgagtctctaaatggtgtgcgtttaaaatcactcgacgggtacgcagttttatatgcaaattggaagaagagcatagataaaaaagaaaaagatgcagcttataaagttttagaaaaaaaggaactagaaatcagacaagagattgtagttttgtttgatgagaaagcggtagaatggattggtaagttacctgccgatgtaaaaaaaccgaaaaaaccaaactatgagtttttgtttgaaccagcgattttttcaatactcaagaaaaaatatagtgatgaggtaggaactactattgatgaggaatcaatttttgatagttgggataaatggacggcgtactttggaaagttttttgaaacacgcaaaaatttttataaaagtgacggtaaggctacagcagtagcgacaagaatagtgaatgaaaatttgagacgtttttgtgatgatgtctcaacttttgaaaatatacaatcaaaaatcgatttgtcaccactcgaaaaggagtttgacgttagccttaaaaaggtttttgatattcaacattacaatcaatgtttgaaccagtcaggtattgatgcgtttaacacattacttggaggagaggttcacgagaatggagaaaaaattaagggaattaacgaatatataaacgagcaccgacaaaaaactggcgaaaaattaacgcgcctaaaaaagttagataaacagattggcagtgataaggaaaattttattgatctcattgagacagatgaacaattgaagacaacgcttgtcacatttattgcaaacgctaaggaaaaagtagacttgttagataagagcgtctcgtatctcacgaaagatactgatgttaagttatctggtatttttttcagaaaggaagcgattaacacaatcaccaggcgatggtttgtgagtcatgaaaagatatcagatgcactcgtaagcgcctttagtgataagaatgtaaagttcgatcaaaagcgtgaagaatataagtttccagattttattagttggcacgtgatacaaaatgcggtcgaaaaacttgccagtgacggagaagagatttggaaaaagtattatcttgaggaagagaaattatcacttcttgataaaaccccatggcagcagtttttgacagtttttgaatgtgaatataacaacctaaaatcgaaaggtcatgaaagcgaaggaaggagctttactgaacttgtgcaagatattgaatctttgctgaagacagacaccctagatagaaacgaccatgtaacggagattataaaatccttttctgatcgggtgcttaatatctatcgatttgcgaaatattttgcactcgataaatcttgccaatggaatcctgatggtttggatactgacgatttttacgtggcctacgaacaattctatagtgatggatacgagaagatcgttaaggtgtacgacaaggttcgtaactatatgaccaagaagccgttcaatcaagacaaatggaaattgaactttgagaacccaactttggctaacggctgggacaagaacaaggagactgataacaccgcaataatcttgcgacgggcaggtcggtattatctagcggtgatggaaaggggtcataataccttgttcaagaaaatacctatgtcatcctctggctatcaaaagatgacatataaattgtttcctgatccatcaaagatgatgccgaaggtttgtttttcaaaaaaaggattggaattctttaaacctagtgctgaaataatgagaatatacaaaaacggcgagtttaaaaaaggtgacaccttctcactttcttcaatgcacgttctgattgatttctataaaaatgcactcaagacatacgacggctggactatgtatgacttcagtaatttaaagaaaacgagtgaatacacggagaacattggcgagttctatcgagatgtcgctgaaagtgggtatcaaatcaattttgactatattgcagagcaatatatagaagatgcaaataaagaaggaaaattgtatctcttcgaaatccataacaaggattggaatttgaaagatggggcaataaagaccggtagtaaaaatgcacacacgctttattttgagcaggttttttctgatgagaatgcccaaaataatttcgttgttaagctcaatggagaagcagaattatttttccgcccagcaaccagtactgaaaaacttggaaatcactacgatagtaaaggtaacgtagttacaaaaaacaaacgatatgcacacgataaaatgtttttccatgtgccagtgacgctcaaccgcactgctcctgacgctcgtaaatttaatcaatcagtcaatgtatttctagcaaataatcctgatacaaacatcatcggtattgatcggggagagaagcatttggcctacttgtccgtcattaaccagaaaggagatatattgaaaataaaatctttaaacaagattgaggttaaggataaggacggtaatgtgataaaggaagatgattatgcaaagctattggaagaccgtgctaagaatcgtgagagcgcacggcgcgactggaagagtgtagaacagattaaagaccttaagaaaggttatatctcaaatgttgtacgagagattgccgacctcgtcattaaatacaatgcgattgtagtatttgaagatttgaatatgcgcttcaagcaagtgcgcggtggcattgaaaagagcgtgtatcaacaacttgaaaaggccttgattgataaacttaacttcttggttgataaaaatgaacttgatccccagaaggcggggcacatattgcatgcgtaccaactcactgcaccatttgagacgtttaaagatatgggaaagcaaactggcgtactcttctacacccaagctgaatatacgtcgcaaaccgatccggtaacaggttttcgaaaaaatgtctatctgagcaattcggccaccgttgagaagataaaagcatttgtggaaatgtttgatgtaatcggctgggacgataaactaaaaagttactacttcaaatataacccggttaattttgttgaaactaagtttaaggaaaatacgttctcaaaagattgggtcatttatgccaatgtgccgcggattaagcgcgaacgcaaaaatgggtattgggaggcaaccgtggtcaatccaaacgaagaattcttgaaactttttaaggaatgggattttgataacatctatgttgaagacataaaagaacagatctttcagatgtttgaagagggaagattggacgggacaaaagaattcgatggcaaaaatcgtaatttttggcacagctttatcttcctattcaatcttatgttgcaagtaagaaattctaccgcaacccaatacaagaaggatgaagatggaaatatcattgagactgttgagggtgttgatttcattgcttcaccagtttttccattcttcaccaccgatggtggtgatttcaccgaaggatgcgtgaatctagcaaaacttgaagataaatttgtcggtagtaatgctgacaaagagcggttcaagaaagaatttaacggagacgcaaacggtgcatacaacattgctcgaaagggaattattatgttgaacaatattaaaaataatccggagaaaccagacctgttcgtgtctaaaaaagactgggacaaatttgctcaagcaaatcaataa

SEQ ID NO: 30 - DNA, 3828 bp, Unknown bacterial species
  NT Sequence of BMC15
atgaatccaacccaaacagacaaaaccccctcaaagccatttgaaaaatttaccaatttatactgcttgtcaaaaaccctgaggtttgagctgaaaccaatcggcaaaacgcaaaagatacttgaagataataaggttttcgaaaatgataaaaagagagctaaaagttatgaggaagcaaaaaaatattttaataaattacatagagaatttattgacgaatcactcaaaaatattacattatctaataatctaattgaaaaatttgaaaaaaaatatcttacctggaaaaatagtaaaaataaagataatagtactgaactaaaaaagtctgctaaaagattgagaatagtaattcttgagagtttcaataaaaaagctaatgaatggaactctgaatattcaaaccaagttaagaacgaaaagaaaaaaaagaaaatacaagaaataacaggaatagatttgtttttcaaagttgaagtttttgattttcttatacataaataccccgaggtgcagataaatggtgagagtatttttagtccattcaacaaatttagtggttactttaaaaaatttcacgaaacaagaaaaaacttttataaagacgatggaacctccacagcaattcccacaagaataattgatgttaatttagaaaaatttttagaaaataaggacatctactatacaaaatacttccaaaaatacaattctatttttaataaggaagaaacagatattttcaaactggaatcgtttaaaaattgtttaacacaatctcagattgataaatataatgaatcaatagccacattaaaatcaaaaatcaacaacttacgtcaaaataatcctgaggttaataaacatgatcttccattttttaaagaattattcaggcaaattctaggtcaaccaattaaaaaggagacagaacaggataacttcatagagatactaacaaatgacgaggtttttcctgttttacaaaaaaatattgatgaaaacgagttatatattcctaaagctgatactctctttaaagaatttttaaagagccaaattcaagagacaaatgaatataatattaacgaaatatatgttgcaagtcgttttataaactcaatatccaacaactggtttgctgaatgggataccattattaatttattacgtactgaactaaaaattaaacagaatcagaaaaaacttccagatttcatctcgattgcttcattaaaaagagtgttacaaaaatcccaagacgagatagatgctaaagatttatttagaaacaactatgagaatcttttcgaatctacaactgacttctataaaatatttcttaaaatttgggaattagaatttaatgataatattaaaaaatataatttggagacagagaatataagaaaaataataatagaagataaaaagtatcttccaaataaaaagagtatattaaagaatggtgagacaggtattattcataatgaaaaaatattagattatgcacaatctgcattaaatatttatcaaatgatgaaatatttttctttggaaaaaggaaaagaaagagagtggaatccggacggtctgaatgaagatacaacaggaggattttatgatgatttcaataaatactaccaaaatgtaaacacgtggaaatattttaatgaattcagaaattatttaacaaaaaaaccatataagacagataagattaaattatactttggtcacaagagtttattaggtggttttactgaaagcaaaacagagaaaagcaataacggcacacaatatggggcttatttattaagaaagaagcatggacttggaggctttgattattatcttggaattagtacagacccccatttaatgagttattttgatccaattgatgattcaggagatagcgaatatgaaaggttaaattattatcaagtattaacaagaacaatctacggtccttcttatgaaggcgattatgaattggacaaaaaaaatttatcagaaatagagataataaaaaaaataaaaagatcattatcttattacacttcaagggttaaaaaaatccaggacataatcaataataattatgagtctgttagagatattcataaagatataactgatgtactaaaagaatttggaacaatctttgattataaagtaataacaaacagtcaaatacaaaaggcatttaattgcgataaaggattttatctctttgagatatattcgaaggatttttcaaaagagaaaggtgataaaagtaagaatagcaaagataatttacatacaacgtattttaaatcattaatggatagaaagcagtctacatttgatttaggtagtggagaaatatttttcagagaaaaatctgttcagtctgaaattgattctatgagaaaaactaagaataaaataactaggttcaaacgatacacaaaaaatttaattcagttcaatttatcaattacccttaataataactgtacagaagttcctcagaataaaaatgcaagaaaagcatttattaataattttaatattgaactaagtaagaaactgttaacaaataattcagacataaatattattggtattgaccgtggagaaaaacatttggcctattactctgttatagaccagcaaagcaacattcttgaaacaggctcttttaataaaattcaagagagaaaagacagagaacctaccgattaccaacaaaaattagataaaattcaaaaggacagagactggcaaagaaaatcatggcaggaaatatcaaatatcaaagatttaaaaaaaggctatatttctcaagttgtctatgaaataagtaagttagttaaaaaatataatgcaatcatagtatttgaagacctgaatataggatttaagcgtggccgttttgcaatagaaaaacaagtataccaaaatttggagctttcattagcgaaaaaattaaattatttagtttttaaagatgcaaatgaaggagaatcaggacattatctaaaagcatatcaacttacatcccctgtcaacaattttcaagatattggtaaacaatgtggtataatattttatattcctgccagctacacatcagcaatttgtccttcatgtggattccataaaaacataccaacatcaattaaaaaacttgcaaagaataaagaatttgtagaaaaatttgttataacttatgaacttaaaaaagatcgtttttattttggttacaaaataaatgatttttacaattctaatttgcaagataatgtcattttctactcaaatgtagaaagattaagatataaaagaaataaggataaccgaagtggcgaagtacaagaacgattgcctaatgaagaattaaaaaaactctttgagcaaaatcacattaattataaagataatcctcaaatatctggtcaaattaaaaatcaaaaactagataatgaaaaattttataaacctcttatatatgaaatctctttaattttacaattaaggaatagtaaaacagtaaaaagtgaagatggaacaattaacacaaatataaatcgggatttcatttcttgtccagcttgttattttcattcagagaataatttaatgaatcttcctaataagtataaaggaggaaaaaaatttgaatttaacggagatgcaaatggagcatataatattgcacgaaaaggcattttgcttttaaacaaattaaataatatcaaagatatagaaaaaattgaatataatgacctcaatatatcacaagaagactgggataactttgtcaaaaacccctaa

SEQ ID NO: 31 - DNA, 19 bp, Artificial Sequence
  Stem-Loop Consensus Sequence
  variation 1,11: /replace="a,c,g,t"
natttctactnttgtagat

SEQ ID NO: 32 - DNA, 19 bp, Unknown bacterial species
  BMC01-15 Stem Loop Sequence
gatttctactattgtagat

SEQ ID NO: 33 - DNA, 3888 bp, Artificial Sequence
  Nucleotide sequence of BMC01 (E. coli codon otimized)
atgatcttcaacaacttcacccagaaattcagcctgagcaaaaccctgcgttttgaactgcgtccggttgatgccggtggtaatgttattaccgatctgaccattttcgaagaaaccatcaaaaacgatcagaaacgctatgaagcatacctggcaattaaaccgctggttgatgaaacccataaacactttattcagaccgttctgagtggtctgacagatctgattaaatccgatgagatgaagaactacctggaacacaaaaatctgatccgtcagaaagatgtggaagagaaagttaaaaccaaaagcatcgacgtgatcaacaaaatcgaaaaagattggcgtaaacgtgtgagcgatagctttaccaaacatccgcagtacaaaaagatgttcgataaaaccctgtttgccgatgaaagtccgctgtataaactggccgaaaatgattttcagcgtagccagattaaaatcttcgagaaatttaccggctacttcaacggctttcatgagaatcgtaaaaatctgtatgtggcggaaaaacagggcaccgcaattgcaaatcgtgtgattaatgaaaacctgccgaaatttatcgagaacgccaataaactgaaacgtgcctttgaaaaatatcccgaatttctgtccaaaatcagcgaggataaaagctttcaggcactgctgattaaaaaccagctgagcctggaaaaactgctgcagccgctgacctttaatctgctgatttctcagaccggtatcgatagctataatgaagtgttaggtggttacacaccggaaaatagcgaaccgattaaaggcctgaatcaactgattaatctgtaccgccagaaaattaacctggcacgtaacgattttccgaatctggcaccgctgtacaaacagctgctgagcgatcgtgaaaccaatagcgttgtgtataaacctctggaaaatgtggcagatgtttatagcagtgtgtttgaactgtgtcagaacctgctgagcaaacagagcgatattaataaatggatcgaggatatcaacatcagcagcggtcagatttggatctataaaagccatctgagcggtctgtcagttatgctgtttggtgaaagtggttggggtctgattccgcgtattctgaatattagcgaagatgatgaagaagagatcatcaaatccaaaagcaaaaagagccagcaagagtatttcagctttgcggaaattggtaacgccatcaacaactatagctttgaggatgtgaacattaaagcactggcaaaacagggtctgtgtctgtggcagaaacaaggtaatgaacgtctgatcaaattcggcaaactgtttagccagatgcagaatgaactgcagagcccgaaagaaaaatgggatagcaccgaaaaagagaaaatcaaagaactgctggatacaggcctggaatttgttcattggctgaaagttattagcaaccagccggaagataaagatgaagtcttttatgccgaatggcaggcactgaccgatacctggcgtggtctgccgaaactgtatgatcgtgttcgtaattttgccaccaaaaaagattacagccagaacaagctgaagatcaactttgataaaggcaccctgctgaatggttgggataccaataaagaaaccgataatctgggtatcctgctggaaaataaaggccagtattatctgggcatcatgaaagatagcagcatctttgattatcagtgggacattgacaattttcagaacccgaatagcaaacagtcagtggccaaaaaaaacctgcatgaagcaattgttagcgataacacccaggattgttggagcaaaattgtgtacaaactgttaccgggtccgaataaaatgctgccgaaagtgttttttagtgacaagcgccagaaatactttggtgcggatgaaaaagtgatcgacattaacgaaaatggccgtcataaaaaaggcgacaactttaacattagcgattgccactatctgatcgacttctataaaaccgccatcaataaacatccggaatggtcccagttcaacttcaaatttagcgcgaccaaaagctacgaagatatcagccagttttatcacgaagttcagaatcagggttatcgcatcgagtttgatcatatccgcaaagactatatccagaaaatggtgagcgaaggtaaactgttcctgtttaaaatccacagcaaagattttagcagctatgcaaaaggtcgtccgaatatgcataccatctattggcgtgccatttttaacccggaaaatctggccaatgttgtggttaaactgaatggtgaagccgaattcttttatcgcaaaagcagtaaagatcgcattatcagccatccgcaaggtctggaagttagcaataaaaacccgagcaatccgaaaaaaaccagtcgttttgcatacgacctgatcaaagataaacgtttcacgcaggacaagttttttttccatgttccgattacgctgaattttcgtgaaggtgaaggttatcgctttaaccagagcgttattcgtgagctgaaaaaatactatcagaccgataaagccaacctgcatatcattggtattgatcgtggtgaacgtcatctgctgtattattgcgttattaatgttgccagcggcaaaatcgttgaacagggtagcttcaatcagatcagcaccaattatacaccggaacaaattaccgatgatggcgaaatcattaaaggcgaaaccgtgaataaaaccaccgattatcataacctgcttaacaccaaagaaggtgatcgccagaaagcacgtaaaaattggcagaccattgaaaacatcaaagagctgaaagccggttatctgagcaatgtgattcataaaatcagccagctgatggtgaaatataacgcctttgttgttctggaagaactgaaatatggttttaaacgcggtcgcttcaaggttgagaaacaggtttatcagaaatttgagaaagccctgatcgacaagcttaactatctggtgtttaaagatcgtgcccctgccgaagttggtggtgttctgaatgcactgcagctggcacctccggttgcaagctatattgatattggtaaacaggcaggcttcctgttttatgttccggcacatcataccagcaaaatttgtccgtggaccggttttgtggactggctgaaaccgcgttatgatggcattgataaagcgaaagcattctttacctgtttcgaaagcatccatttcaacacgcagaaaaactattttgagttcgccttcgactatgagaaatttcgcggtaacattaatcatctgccggaaggtctgaaacgtaccagctggaccctgtgtagccataatagcctgcgtgatattgccacgaaagataaaaatggtaactggccgtataagcagatcaatctgacagcagaactgcttgaaattctgaaaaccctgaatccgcgtaatggcgaaaacctggttgaacgtattatcgagatgaacgacaaaaagttcttcgagagcctgatgtgggcactgcgtgttctgctgcaactgcgttatggttatatcaaacgtaataacgagggcatcatcatcgaagaggttgattatattctgagtccggtggcaaatgaaaacggcgaattttttgatagccgcaactttgtgaatatcgagaaagccgattttcccaaagatgcagatgcaaatggtgcatataacattgcacgtaaaggtctgctgctgattgcacagaatattaacaacgccaaaatcaacgataaaggcgaggttaaatgtgacctgcagattgataaaacaacctggtttaactgggttcagagcaaaagctaa

SEQ ID NO: 34 - DNA, 1191 bp, Escherichia coli
  Nucleotide sequence of the araC-ParaBAD inducible promotor system
tatggagaaacagtagagagttgcgataaaaagcgtcaggtaggatccgctaatcttatggataaaaatgctatggcatagcaaagtgtgacgccgtgcaaataatcaatgtggacttttctgccgtgattatagacacttttgttacgcgtttttgtcatggctttggtcccgctttgttacagaatgcttttaataagcggggttaccggtttggttagcgagaagagccagtaaaagacgcagtgacggcaatgtctgatgcaatatggacaattggtttcttctctgaatggcgggagtatgaaaagtatggctgaagcgcaaaatgatcccctgctgccgggatactcgtttaatgcccatctggtggcgggtttaacgccgattgaggccaacggttatctcgatttttttatcgaccgaccgctgggaatgaaaggttatattctcaatctcaccattcgcggtcagggggtggtgaaaaatcagggacgagaatttgtttgccgaccgggtgatattttgctgttcccgccaggagagattcatcactacggtcgtcatccggaggctcgcgaatggtatcaccagtgggtttactttcgtccgcgcgcctactggcatgaatggcttaactggccgtcaatatttgccaatacggggttctttcgcccggatgaagcgcaccagccgcatttcagcgacctgtttgggcaaatcattaacgccgggcaaggggaagggcgctattcggagctgctggcgataaatctgcttgagcaattgttactgcggcgcatggaagcgattaacgagtcgctccatccaccgatggataatcgggtacgcgaggcttgtcagtacatcagcgatcacctggcagacagcaattttgatatcgccagcgtcgcacagcatgtttgcttgtcgccgtcgcgtctgtcacatcttttccgccagcagttagggattagcgtcttaagctggcgcgaggaccaacgtatcagccaggcgaagctgcttttgagcaccacccggatgcctatcgccaccgtcggtcgcaatgttggttttgacgatcaactctatttctcgcgggtatttaaaaaatgcaccggggccagcccgagcgagttccgtgccggttgtgaagaaaaagtgaatgatgtagccgtcaagttgtcataa

SEQ ID NO: 35 - DNA, 177 bp, Escherichia coli
  Nucleotide sequence of the fdT expression terminator
aattttctgtatgaggttttgctaaacaactttcaacagtttcagcggagtgagaatagaaaggaacaactaaaggaattgcgaataataattttttcacgttgaaaatctccaaaaaaaaaggctccaaaaggagcctttaattgtatcggtttatcagcttgctttcgaggtgaa

SEQ ID NO: 36 - DNA, 10216 bp, Artificial Sequence
  CRISPR/BMC01-Ec vector system
caatcggcgttaaacccgccaccagatgggcattaaacgagtatcccggcagcaggggatcattttgcgcttcagccatacttttcatactcccgccattcagagaagaaaccaattgtccatattgcatcagacattgccgtcactgcgtcttttactggctcttctcgctaaccaaaccggtaaccccgcttattaaaagcattctgtaacaaagcgggaccaaagccatgacaaaaacgcgtaacaaaagtgtctataatcacggcagaaaagtccacattgattatttgcacggcgtcacactttgctatgccatagcatttttatccataagattagcggatcctacctgacgctttttatcgcaactctctactgtttctccatacccgttttttggtaccgggccccccctcgagtttattttaggaggcaaaaatgatcttcaacaacttcacccagaaattcagcctgagcaaaaccctgcgttttgaactgcgtccggttgatgccggtggtaatgttattaccgatctgaccattttcgaagaaaccatcaaaaacgatcagaaacgctatgaagcatacctggcaattaaaccgctggttgatgaaacccataaacactttattcagaccgttctgagtggtctgacagatctgattaaatccgatgagatgaagaactacctggaacacaaaaatctgatccgtcagaaagatgtggaagagaaagttaaaaccaaaagcatcgacgtgatcaacaaaatcgaaaaagattggcgtaaacgtgtgagcgatagctttaccaaacatccgcagtacaaaaagatgttcgataaaaccctgtttgccgatgaaagtccgctgtataaactggccgaaaatgattttcagcgtagccagattaaaatcttcgagaaatttaccggctacttcaacggctttcatgagaatcgtaaaaatctgtatgtggcggaaaaacagggcaccgcaattgcaaatcgtgtgattaatgaaaacctgccgaaatttatcgagaacgccaataaactgaaacgtgcctttgaaaaatatcccgaatttctgtccaaaatcagcgaggataaaagctttcaggcactgctgattaaaaaccagctgagcctggaaaaactgctgcagccgctgacctttaatctgctgatttctcagaccggtatcgatagctataatgaagtgttaggtggttacacaccggaaaatagcgaaccgattaaaggcctgaatcaactgattaatctgtaccgccagaaaattaacctggcacgtaacgattttccgaatctggcaccgctgtacaaacagctgctgagcgatcgtgaaaccaatagcgttgtgtataaacctctggaaaatgtggcagatgtttatagcagtgtgtttgaactgtgtcagaacctgctgagcaaacagagcgatattaataaatggatcgaggatatcaacatcagcagcggtcagatttggatctataaaagccatctgagcggtctgtcagttatgctgtttggtgaaagtggttggggtctgattccgcgtattctgaatattagcgaagatgatgaagaagagatcatcaaatccaaaagcaaaaagagccagcaagagtatttcagctttgcggaaattggtaacgccatcaacaactatagctttgaggatgtgaacattaaagcactggcaaaacagggtctgtgtctgtggcagaaacaaggtaatgaacgtctgatcaaattcggcaaactgtttagccagatgcagaatgaactgcagagcccgaaagaaaaatgggatagcaccgaaaaagagaaaatcaaagaactgctggatacaggcctggaatttgttcattggctgaaagttattagcaaccagccggaagataaagatgaagtcttttatgccgaatggcaggcactgaccgatacctggcgtggtctgccgaaactgtatgatcgtgttcgtaattttgccaccaaaaaagattacagccagaacaagctgaagatcaactttgataaaggcaccctgctgaatggttgggataccaataaagaaaccgataatctgggtatcctgctggaaaataaaggccagtattatctgggcatcatgaaagatagcagcatctttgattatcagtgggacattgacaattttcagaacccgaatagcaaacagtcagtggccaaaaaaaacctgcatgaagcaattgttagcgataacacccaggattgttggagcaaaattgtgtacaaactgttaccgggtccgaataaaatgctgccgaaagtgttttttagtgacaagcgccagaaatactttggtgcggatgaaaaagtgatcgacattaacgaaaatggccgtcataaaaaaggcgacaactttaacattagcgattgccactatctgatcgacttctataaaaccgccatcaataaacatccggaatggtcccagttcaacttcaaatttagcgcgaccaaaagctacgaagatatcagccagttttatcacgaagttcagaatcagggttatcgcatcgagtttgatcatatccgcaaagactatatccagaaaatggtgagcgaaggtaaactgttcctgtttaaaatccacagcaaagattttagcagctatgcaaaaggtcgtccgaatatgcataccatctattggcgtgccatttttaacccggaaaatctggccaatgttgtggttaaactgaatggtgaagccgaattcttttatcgcaaaagcagtaaagatcgcattatcagccatccgcaaggtctggaagttagcaataaaaacccgagcaatccgaaaaaaaccagtcgttttgcatacgacctgatcaaagataaacgtttcacgcaggacaagttttttttccatgttccgattacgctgaattttcgtgaaggtgaaggttatcgctttaaccagagcgttattcgtgagctgaaaaaatactatcagaccgataaagccaacctgcatatcattggtattgatcgtggtgaacgtcatctgctgtattattgcgttattaatgttgccagcggcaaaatcgttgaacagggtagcttcaatcagatcagcaccaattatacaccggaacaaattaccgatgatggcgaaatcattaaaggcgaaaccgtgaataaaaccaccgattatcataacctgcttaacaccaaagaaggtgatcgccagaaagcacgtaaaaattggcagaccattgaaaacatcaaagagctgaaagccggttatctgagcaatgtgattcataaaatcagccagctgatggtgaaatataacgcctttgttgttctggaagaactgaaatatggttttaaacgcggtcgcttcaaggttgagaaacaggtttatcagaaatttgagaaagccctgatcgacaagcttaactatctggtgtttaaagatcgtgcccctgccgaagttggtggtgttctgaatgcactgcagctggcacctccggttgcaagctatattgatattggtaaacaggcaggcttcctgttttatgttccggcacatcataccagcaaaatttgtccgtggaccggttttgtggactggctgaaaccgcgttatgatggcattgataaagcgaaagcattctttacctgtttcgaaagcatccatttcaacacgcagaaaaactattttgagttcgccttcgactatgagaaatttcgcggtaacattaatcatctgccggaaggtctgaaacgtaccagctggaccctgtgtagccataatagcctgcgtgatattgccacgaaagataaaaatggtaactggccgtataagcagatcaatctgacagcagaactgcttgaaattctgaaaaccctgaatccgcgtaatggcgaaaacctggttgaacgtattatcgagatgaacgacaaaaagttcttcgagagcctgatgtgggcactgcgtgttctgctgcaactgcgttatggttatatcaaacgtaataacgagggcatcatcatcgaagaggttgattatattctgagtccggtggcaaatgaaaacggcgaattttttgatagccgcaactttgtgaatatcgagaaagccgattttcccaaagatgcagatgcaaatggtgcatataacattgcacgtaaaggtctgctgctgattgcacagaatattaacaacgccaaaatcaacgataaaggcgaggttaaatgtgacctgcagattgataaaacaacctggtttaactgggttcagagcaaaagctaatggtctagaggtcgaaattcaaattgtgagcggataacaatttgaattttctgtatgaggttttgctaaacaactttcaacagtttcagtggagtgagaatagaaaggaacaactaaaggaattgcgaataataattttttcacgttgaaaatctccaaaaaaaaaggctccaaaaggagcctttaattgtatcggtttatcagcttgctttcgaggtgaattttgaccctctagcgaaaatgcaagagcaaagacgaaaacatgccacacatgaggaataccgattctctcattaacatattcaggccagttatctgggcttaaaagcagaagtccaacccagataacgatcatatacatggttctctccagaggttcattactgaacactcgtccgagaataacgagtggatcccctccaattcgccctatagtgagtcgtattacgcgcgctcactggccgtcgttttacaacgtcgtgactgggaaaaccctggcgttacccaacttaatcgccttgcagcacatccccctttcgccagctggcgtaatagcgaagaggcccgcaccgatcgcccttcccaacagttgcgcagcctgaatggcgaatggaaattgtaagcgttaatattttgttaaaattcgcgttaaatttttgttaaatcagctcattttttaaccaataggccgactgcgatgagtggcagggcggggcgtaatttttttaaggcagttattggtgcccttaaacgcctggtgctacgcctgaataagtgataataagcggatgaatggcagaaattcgaaagcaaattcgacccggtcgtcggttcagggcagggtcgttaaatagccgcttatgtctattgctggtttaccggtttattgactaccggaagcagtgtgaccgtgtgcttctcaaatgcctgaggccagtttgctcaggctctccccgtggaggtaataattgacgatatgatcatttattctgcctcccagagcctgataaaaacggtgaatccgttagcgaggtgccgccggcttccattcaggtcgaggtggcccggctccatgcaccgcgacgcaacgcggggaggcagacaaggtatagggcggcgaggcggctacagccgatagtctggaacagcgcacttacgggttgctgcgcaacccaagtgctaccggcgcggcagcgtgacccgtgtcggcggctccaacggctcgccatcgtccagaaaacacggctcatcgggcatcggcaggcgctgctgcccgcgccgttcccattcctccgtttcggtcaaggctggcaggtctggttccatgcccggaatgccgggctggctgggcggctcctcgccggggccggtcggtagttgctgctcgcccggatacagggtcgggatgcggcgcaggtcgccatgccccaacagcgattcgtcctggtcgtcgtgatcaaccaccacggcggcactgaacaccgacaggcgcaactggtcgcggggctggccccacgccacgcggtcattgaccacgtaggccgacacggtgccggggccgttgagcttcacgacggagatccagcgctcggccaccaagtccttgactgcgtattggaccgtccgcaaagaacgtccgatgagcttggaaagtgtcttttggctgaccaccacggcgttctggtggcccatctgcgccacgaggtgatgcagcagcattgccgccgtgggtttcctcgcaataagcccggcccacgcctcatgcgctttgcgttccgtttgcacccagtgaccgggcttgttcttggcttgaatgccgatttctctggactgcgtggccatgcttatctccatgcggtagggtgccgcacggttgcggcaccatgcgcaatcagctgcaacttttcggcagcgcgacaacaattatgcgttgcgtaaaagtggcagtcaattacagattttctttaacctacgcaatgagctattgcggggggtgccgcaatgagctgttgcgtaccccccttttttaagttgttgatttttaagtctttcgcatttcgccctatatctagttctttggtgcccaaagaagggcacccctgcggggttcccccacgccttcggcgcggctccccctccggcaaaaagtggcccctccggggcttgttgatcgactgcgcggccttcggccttgcccaaggtggcgctgcccccttggaacccccgcactcgccgccgtgaggctcggggggcaggcgggcgggcttcgccttcgactgcccccactcgcataggcttgggtcgttccaggcgcgtcaaggccaagccgctgcgcggtcgctgcgcgagccttgacccgccttccacttggtgtccaaccggcaagcgaagcgcgcaggccgcaggccggaggcttttccccagagaaaattaaaaaaattgatggggcaaggccgcaggccgcgcagttggagccggtgggtatgtggtcgaaggctgggtagccggtgggcaatccctgtggtcaagctcgtgggcaggcgcagcctgtccatcagcttgtccagcagggttgtccacgggccgagcgaagcgagccagccggtggccgctcgcggccatcgtccacatatccacgggctggcaagggagcgcagcgaccgcgcagggcgaagcccggagagcaagcccgtagggcgccgcagccgccgtaggcggtcacgactttgcgaagcaaagtctagtgagtatactcaagcattgagtggcccgccggaggcaccgccttgcgctgcccccgtcgagccggttggacaccaaaagggaggggcaggcatggcggcatacgcgatcatgcgatgcaagaagctggcgaaaatgggcaacgtggcggccagtctcaagcacgcctaccgcgagcgcgagacgcccaacgctgacgccagcaggacgccagagaacgagcactgggcggccagcagcaccgatgaagcgatgggccgactgcgcgagttgctgccagagaagcggcgcaaggacgctgtgttggcggtcgagtacgtcatgacggccagcccggaatggtggaagtcggccagccaagaacagcaggcggcgttcttcgagaaggcgcacaagtggctggcggacaagtacggggcggatcgcatcgtgacggccagcatccaccgtgacgaaaccagcccgcacatgaccgcgttcgtggtgccgctgacgcaggacggcaggctgtcggccaaggagttcatcggcaacaaagcgcagatgacccgcgaccagaccacgtttgcggccgctgtggccgatctagggctgcaacggggcatcgagggcagcaaggcacgtcacacgcgcattcaggcgttctacgaggccctggagcggccaccagtgggccacgtcaccatcagcccgcaagcggtcgagccacgcgcctatgcaccgcagggattggccgaaaagctgggaatctcaaagcgcgttgagacgccggaagccgtggccgaccggctgacaaaagcggttcggcaggggtatgagcctgccctacaggccgccgcaggagcgcgtgagatgcgcaagaaggccgatcaagcccaagagacggcccgagaccttcgggagcgcctgaagcccgttctggacgccctggggccgttgaatcgggatatgcaggccaaggccgccgcgatcatcaaggccgtgggcgaaaagctgctgacggaacagcgggaagtccagcgccagaaacaggcccagcgccagcaggaacgcgggcgcgcacatttccccgaaaagtgccacctgaaccccagagtcccgctcagaagaactcgtcaagaaggcgatagaaggcgatgcgctgcgaatcgggagcggcgataccgtaaagcacgaggaagcggtcagcccattcgccgccaagctcttcagcaatatcacgggtagccaacgctatgtcctgatagcggtccgccacacccagccggccacagtcgatgaatccagaaaagcggccattttccaccatgatattcggcaagcaggcatcgccatgggtcacgacgagatcctcgccgtcgggcatccgcgccttgagcctggcgaacagttcggctggcgcgagcccctgatgctcttcgtccagatcatcctgatcgacaagaccggcttccatccgagtacgtgctcgctcgatgcgatgtttcgcttggtggtcgaatgggcaggtagccggatcaagcgtatgcagccgccgcattgcatcagccatgatggatactttctcggcaggagcaaggtgagatgacaggagatcctgccccggcacttcgcccaatagcagccagtcccttcccgcttcagtgacaacgtcgagcacagctgcgcaaggaacgcccgtcgtggccagccacgatagccgcgctgcctcgtcttggagttcattcagggcaccggacaggtcggtcttgacaaaaagaaccgggcgcccctgcgctgacagccggaacacggcggcatcagagcagccgattgtctgttgtgcccagtcatagccgaatagcctctccacccaagcggccggagaacctgcgtgcaatccatcttgttcaatcatgcgaaacgatcctcatcctgtctcttgatcagatcttgatcccctgcgccatcagatccttggcggcaagaaagccatccagtttactttgcagggcttcccaaccttaccagagggcgccccagctggcaattccggttcgcttgctgtccataaaaccgcccagtctagctatcgccatgtaagcccactgcaagctacctgctttctctttgcgcttgcgttttcccttgtccagatagcccagtagctgacattcatccggggtcagcaccgtttctgcggactggctttctacgtgttccgcttcctttagcagcccttgcgccctgagtgcttgcggcagcgtgaagctagctgcataatgtgcctgtcaaatggacgaagcagggattctgcaaaccctatgctactccgtcaagccgtcaattgtctgattcgttaccaattatgacaacttgacggctacatcattcactttttcttcacaaccggcacggaactcgctcgggctggccccggtgcattttttaaatacccgcgagaaatagagttgatcgtcaaaaccaacattgcgaccgacggtggcgataggcatccgggtggtgctcaaaagcagcttcgcctggctgatacgttggtcctcgcgccagcttaagacgctaatccctaactgctggcggaaaagatgtgacagacgcgacggcgacaagcaaacatgctgtgcgacgctggcgatatcaaaattgctgtctgccaggtgatcgctgatgtactgacaagcctcgcgtacccgattatccatcggtggatggagcgactcgttaatcgcttccatgcgccgcagtaacaattgctcaagcagatttatcgccagcagctccgaatagcgcccttccccttgcccggcgttaatgatttgcccaaacaggtcgctgaaatgcggctggtgcgcttcatccgggcgaaagaaccccgtattggcaaatattgacggccagttaagccattcatgccagtaggcgcgcggacgaaagtaaacccactggtgataccattcgcgagcctccggatgacgaccgtagtgatgaatctctcctggcgggaacagcaaaatatcacccggtcggcaaacaaattctcgtccctgatttttcaccaccccctgaccgcgaatggtgagattgagaatataacctttcattcccagcggtcggtcgataaaaaaatcgagataaccgttggcct

SEQ ID NO: 37 - DNA, 10300 bp, Artificial Sequence
  CRISPR/BMC03-Ec vector system
caatcggcgttaaacccgccaccagatgggcattaaacgagtatcccggcagcaggggatcattttgcgcttcagccatacttttcatactcccgccattcagagaagaaaccaattgtccatattgcatcagacattgccgtcactgcgtcttttactggctcttctcgctaaccaaaccggtaaccccgcttattaaaagcattctgtaacaaagcgggaccaaagccatgacaaaaacgcgtaacaaaagtgtctataatcacggcagaaaagtccacattgattatttgcacggcgtcacactttgctatgccatagcatttttatccataagattagcggatcctacctgacgctttttatcgcaactctctactgtttctccatacccgttttttggtaccgggccccccctcgagtttattttaggaggcaaaaatggaaaagaacctgaattacctggaacgcttcaccaaacattacaacaccaaaaagaccctgaagaacaaactgattccgtatggtaataccgcagagaacatgatcaaaaacaacatcatcagcaacgagaagcagattattctgagcgcaaagaaacagaaacagagcattgattttctgcaaaaagagtacatcgagaacaagctgagcgaaattaccctgccgtatctgaatgattattacaacgagttcattaaaaacaagaaagagcgcgataccgacgtcattgataacattgaaattgccatgcgcaagcacattagcaaaagcctgaccgaaaatggcaaccacaagaaatatctgaacaaagaggtgtttgatatcatcagcgagaagaaagaactgtattatgacgtgacctttaaacgcaatgcaacctatctgagcgattattttcagagccgtgtgaacctgtataaagacagcaataaaagcagcaccattgccagccgttgcattaacattaatctgccgattttcgccaaaaacatcgtgctgtttaacttcatcaagaacaaggcgaacatcatcttcgatgacctgaaagaaattaccgatgatgagtataccctggatagcatttttagcatcgatttctttaacatggtgctgagccagaaaggcatcgattactataataccattttaggtggcatgaccaaagaggatggcaaaaagattaaaggcatcaacgagtacatcaacctgtacaatcagaacgtgaaagacgagaaaaacaaactgccttatccgaagaaactgaagaaacagctgctgagcgatatcaatagctatagcgcacgctttgaaaaattcgataccgaacaagaaatggtgaaaagcattaaaagcctggtggaaaatgacctgtttcagggtgaactgtttgataaaaaggtggatatcctgaaagagacagaacgtctgctggaacgtattagcgaatatgatagcaatgccctgtttatcaccgaaaagaacattagctatatcagcatcgacatcttcaacgacaaattctttatcaaaaccgccatcgagtacttctacgagaataacatttgtccggattaccgcaaaatctatgataacgccagcaaaaacaagcgtaaacagctgggtaaagaaaagaataaggtgatcaagcagaaaagctttagcatcagctttctgcaggatgccattaccttctatatcaaagatagcggcatcaacaagatcagcgaaaactgcattatcaactacttcaagaagcacaccatcaaactgaccgagctgtttggtaaagtgtatgaggattacaacgtgatcaaaccgattctggaacagcatctggttgaatatgaaggtaaaagcatcagcaaggatagcatcaaacgcagcaaaatcaaactgtttagcgaaaacctgaaaaacatcttctatttcattcgtccgctgaacattattgaagaggccctgaattatgataccagcttttataccccgttcaacatcctgtttgaagagatcaaaaagtttaacaaactgtacgataaaatccgcaactttatcaccaagaaaccgttcaacgatgaggaaattaacctgtattttggcattccgaatttaggcggtggttttattgatagccagaccgataaaagcaataacggcacccagtattgtacctacctgtttcgtaaaaagaaccaactgctgaactgggaatattttgtgggcattagcaagaataaacacctgttccgcgaaaaagaaaacatcgaactgaatagtgatgaaacgagctttcagcgttatagtttctataccccgaaagacaaaagcatttatggcagcagctattttagcgccaatgagaaaaactacaaggacgacaaacaagagttcatcaacatcattaacaacatcgtgaataacagcggtaacgaactggcaattaaagagctgaagaaatatatcaacaacagcaccgaaaatagcgaaaccccgaatggttgtctgagcgttctgaaaaataagtgcaacgagatttacaacctggtgatcaaccacgatgacttcaaagagaaaaacgaggacatcatcaataaacttaaaaacaccctgtcgaagctgagcaaagttccgcaggcaaaagaactgatcaacaaaaagtataacctgttcagcgagatcattagcgatattagtgaaatttgtctgaccagcacgcagcgttattatccgatcgatgatgaagaactgaacagcgcactgaacgatgaaaataaaccgctgtacttctttaaaatcagcaacaaagatctgagtgccgatgaaaacattctgaatggtaaacgcaaaagcaaaggcaaagataacatccataccatgattctgcgtgccatgatggatgataatgtgaccaacattattccgaccagctgcaaaattagcatgcgtgaagcaagcatcaaaaaggatgatctggttatccataaagccaacgaaccgattaagctgaaaaactcactggccaataagaaagaaagcaccttcagctatgatatcaccaaagatcgtcgttatagccgtgatgaattctttttcagcattaccgccagcattaacagcgattgcaaagagaacgattattactttaaccagaaagtgaacgagtacctgaagaataatagcaagattaacctgctggcagttgatctgggtgaaaccaatattatcaccattagcgtgattgatcagaaaggtaacatcatactgcagaaggatctggacaagtttatcaacaaagagaagaatatcattaccgatttcaacctgctgctgagtaatcgtagcaaagaacgtgatattgcaaaacgcgattggcaagaacagcagcagattaagaatctgaaagaaggtatgattagctgcatcatccacgaaatttgcaaactgatgattgaacataacgccatcctgatcatggaagatctggatgccaatttcaaaaatcgcaaaaagcgcatcgagaaagccatctatcagaaatttgaaatcgcgatcctggaaaagctgaataacctggtgtttaaagatatcccgattaatgaagttggcagcgttaccaaaccgctgcagctgagtgataaattcgaaacctatgaaaaagtgggtaaccagagcggctttgtctttaaagttagcccgttttataccagcattattgatccgaccaccggctttataaacctgtttaagaaaaacttcgaaagcgtgaaatacagcattgagttcttcagcaaatttgagagcattcgctataacaccaaagaaaaatacttcgagttcgccttcgactataagaatttcaaagaaatcaaatacaccgagaacattaaaaccgattgggttgcatgtaccaccaacattgatcgctatgagtatgacaagaagaacaagatctacaagaagtacgacgttaccaccgatctgaaaaacctgttcgaaaacgaagagatctattatcagaagggcgaaaatatcctggatgtgattctgaagaagaataaccgcgaattctttgagaaactgacgaacctgctgaaaatcaccatgctgtttcgttatcgtaatagccatctgaaactggactatattagcagtccggtgaaaaatagcaatggcgagttctttagcacagaaaatggcctggaaaactatccgattgatagcgataccaatggtgcgtatcatattgcactgaaaggcaaaatgattctggatcgcattaatagcaattcgagcgaaaaactggatacctacatcagcattgaagattggctgaaattcatccagaagtttagcgtcaacaaaatcacggaaaccaaaaagaacaaaaagatcaacatcaaatatgtgtaatggtctagaggtcgaaattcaaattgtgagcggataacaatttgaattttctgtatgaggttttgctaaacaactttcaacagtttcagtggagtgagaatagaaaggaacaactaaaggaattgcgaataataattttttcacgttgaaaatctccaaaaaaaaaggctccaaaaggagcctttaattgtatcggtttatcagcttgctttcgaggtgaattttgaccctctagcgaaaatgcaagagcaaagacgaaaacatgccacacatgaggaataccgattctctcattaacatattcaggccagttatctgggcttaaaagcagaagtccaacccagataacgatcatatacatggttctctccagaggttcattactgaacactcgtccgagaataacgagtggatcccctccaattcgccctatagtgagtcgtattacgcgcgctcactggccgtcgttttacaacgtcgtgactgggaaaaccctggcgttacccaacttaatcgccttgcagcacatccccctttcgccagctggcgtaatagcgaagaggcccgcaccgatcgcccttcccaacagttgcgcagcctgaatggcgaatggaaattgtaagcgttaatattttgttaaaattcgcgttaaatttttgttaaatcagctcattttttaaccaataggccgactgcgatgagtggcagggcggggcgtaatttttttaaggcagttattggtgcccttaaacgcctggtgctacgcctgaataagtgataataagcggatgaatggcagaaattcgaaagcaaattcgacccggtcgtcggttcagggcagggtcgttaaatagccgcttatgtctattgctggtttaccggtttattgactaccggaagcagtgtgaccgtgtgcttctcaaatgcctgaggccagtttgctcaggctctccccgtggaggtaataattgacgatatgatcatttattctgcctcccagagcctgataaaaacggtgaatccgttagcgaggtgccgccggcttccattcaggtcgaggtggcccggctccatgcaccgcgacgcaacgcggggaggcagacaaggtatagggcggcgaggcggctacagccgatagtctggaacagcgcacttacgggttgctgcgcaacccaagtgctaccggcgcggcagcgtgacccgtgtcggcggctccaacggctcgccatcgtccagaaaacacggctcatcgggcatcggcaggcgctgctgcccgcgccgttcccattcctccgtttcggtcaaggctggcaggtctggttccatgcccggaatgccgggctggctgggcggctcctcgccggggccggtcggtagttgctgctcgcccggatacagggtcgggatgcggcgcaggtcgccatgccccaacagcgattcgtcctggtcgtcgtgatcaaccaccacggcggcactgaacaccgacaggcgcaactggtcgcggggctggccccacgccacgcggtcattgaccacgtaggccgacacggtgccggggccgttgagcttcacgacggagatccagcgctcggccaccaagtccttgactgcgtattggaccgtccgcaaagaacgtccgatgagcttggaaagtgtcttttggctgaccaccacggcgttctggtggcccatctgcgccacgaggtgatgcagcagcattgccgccgtgggtttcctcgcaataagcccggcccacgcctcatgcgctttgcgttccgtttgcacccagtgaccgggcttgttcttggcttgaatgccgatttctctggactgcgtggccatgcttatctccatgcggtagggtgccgcacggttgcggcaccatgcgcaatcagctgcaacttttcggcagcgcgacaacaattatgcgttgcgtaaaagtggcagtcaattacagattttctttaacctacgcaatgagctattgcggggggtgccgcaatgagctgttgcgtaccccccttttttaagttgttgatttttaagtctttcgcatttcgccctatatctagttctttggtgcccaaagaagggcacccctgcggggttcccccacgccttcggcgcggctccccctccggcaaaaagtggcccctccggggcttgttgatcgactgcgcggccttcggccttgcccaaggtggcgctgcccccttggaacccccgcactcgccgccgtgaggctcggggggcaggcgggcgggcttcgccttcgactgcccccactcgcataggcttgggtcgttccaggcgcgtcaaggccaagccgctgcgcggtcgctgcgcgagccttgacccgccttccacttggtgtccaaccggcaagcgaagcgcgcaggccgcaggccggaggcttttccccagagaaaattaaaaaaattgatggggcaaggccgcaggccgcgcagttggagccggtgggtatgtggtcgaaggctgggtagccggtgggcaatccctgtggtcaagctcgtgggcaggcgcagcctgtccatcagcttgtccagcagggttgtccacgggccgagcgaagcgagccagccggtggccgctcgcggccatcgtccacatatccacgggctggcaagggagcgcagcgaccgcgcagggcgaagcccggagagcaagcccgtagggcgccgcagccgccgtaggcggtcacgactttgcgaagcaaagtctagtgagtatactcaagcattgagtggcccgccggaggcaccgccttgcgctgcccccgtcgagccggttggacaccaaaagggaggggcaggcatggcggcatacgcgatcatgcgatgcaagaagctggcgaaaatgggcaacgtggcggccagtctcaagcacgcctaccgcgagcgcgagacgcccaacgctgacgccagcaggacgccagagaacgagcactgggcggccagcagcaccgatgaagcgatgggccgactgcgcgagttgctgccagagaagcggcgcaaggacgctgtgttggcggtcgagtacgtcatgacggccagcccggaatggtggaagtcggccagccaagaacagcaggcggcgttcttcgagaaggcgcacaagtggctggcggacaagtacggggcggatcgcatcgtgacggccagcatccaccgtgacgaaaccagcccgcacatgaccgcgttcgtggtgccgctgacgcaggacggcaggctgtcggccaaggagttcatcggcaacaaagcgcagatgacccgcgaccagaccacgtttgcggccgctgtggccgatctagggctgcaacggggcatcgagggcagcaaggcacgtcacacgcgcattcaggcgttctacgaggccctggagcggccaccagtgggccacgtcaccatcagcccgcaagcggtcgagccacgcgcctatgcaccgcagggattggccgaaaagctgggaatctcaaagcgcgttgagacgccggaagccgtggccgaccggctgacaaaagcggttcggcaggggtatgagcctgccctacaggccgccgcaggagcgcgtgagatgcgcaagaaggccgatcaagcccaagagacggcccgagaccttcgggagcgcctgaagcccgttctggacgccctggggccgttgaatcgggatatgcaggccaaggccgccgcgatcatcaaggccgtgggcgaaaagctgctgacggaacagcgggaagtccagcgccagaaacaggcccagcgccagcaggaacgcgggcgcgcacatttccccgaaaagtgccacctgaaccccagagtcccgctcagaagaactcgtcaagaaggcgatagaaggcgatgcgctgcgaatcgggagcggcgataccgtaaagcacgaggaagcggtcagcccattcgccgccaagctcttcagcaatatcacgggtagccaacgctatgtcctgatagcggtccgccacacccagccggccacagtcgatgaatccagaaaagcggccattttccaccatgatattcggcaagcaggcatcgccatgggtcacgacgagatcctcgccgtcgggcatccgcgccttgagcctggcgaacagttcggctggcgcgagcccctgatgctcttcgtccagatcatcctgatcgacaagaccggcttccatccgagtacgtgctcgctcgatgcgatgtttcgcttggtggtcgaatgggcaggtagccggatcaagcgtatgcagccgccgcattgcatcagccatgatggatactttctcggcaggagcaaggtgagatgacaggagatcctgccccggcacttcgcccaatagcagccagtcccttcccgcttcagtgacaacgtcgagcacagctgcgcaaggaacgcccgtcgtggccagccacgatagccgcgctgcctcgtcttggagttcattcagggcaccggacaggtcggtcttgacaaaaagaaccgggcgcccctgcgctgacagccggaacacggcggcatcagagcagccgattgtctgttgtgcccagtcatagccgaatagcctctccacccaagcggccggagaacctgcgtgcaatccatcttgttcaatcatgcgaaacgatcctcatcctgtctcttgatcagatcttgatcccctgcgccatcagatccttggcggcaagaaagccatccagtttactttgcagggcttcccaaccttaccagagggcgccccagctggcaattccggttcgcttgctgtccataaaaccgcccagtctagctatcgccatgtaagcccactgcaagctacctgctttctctttgcgcttgcgttttcccttgtccagatagcccagtagctgacattcatccggggtcagcaccgtttctgcggactggctttctacgtgttccgcttcctttagcagcccttgcgccctgagtgcttgcggcagcgtgaagctagctgcataatgtgcctgtcaaatggacgaagcagggattctgcaaaccctatgctactccgtcaagccgtcaattgtctgattcgttaccaattatgacaacttgacggctacatcattcactttttcttcacaaccggcacggaactcgctcgggctggccccggtgcattttttaaatacccgcgagaaatagagttgatcgtcaaaaccaacattgcgaccgacggtggcgataggcatccgggtggtgctcaaaagcagcttcgcctggctgatacgttggtcctcgcgccagcttaagacgctaatccctaactgctggcggaaaagatgtgacagacgcgacggcgacaagcaaacatgctgtgcgacgctggcgatatcaaaattgctgtctgccaggtgatcgctgatgtactgacaagcctcgcgtacccgattatccatcggtggatggagcgactcgttaatcgcttccatgcgccgcagtaacaattgctcaagcagatttatcgccagcagctccgaatagcgcccttccccttgcccggcgttaatgatttgcccaaacaggtcgctgaaatgcggctggtgcgcttcatccgggcgaaagaaccccgtattggcaaatattgacggccagttaagccattcatgccagtaggcgcgcggacgaaagtaaacccactggtgataccattcgcgagcctccggatgacgaccgtagtgatgaatctctcctggcgggaacagcaaaatatcacccggtcggcaaacaaattctcgtccctgatttttcaccaccccctgaccgcgaatggtgagattgagaatataacctttcattcccagcggtcggtcgataaaaaaatcgagataaccgttggcct

SEQ ID NO: 38 - DNA, 10303 bp, Artificial Sequence
  CRISPR/BMC04-Ec vector system
caatcggcgttaaacccgccaccagatgggcattaaacgagtatcccggcagcaggggatcattttgcgcttcagccatacttttcatactcccgccattcagagaagaaaccaattgtccatattgcatcagacattgccgtcactgcgtcttttactggctcttctcgctaaccaaaccggtaaccccgcttattaaaagcattctgtaacaaagcgggaccaaagccatgacaaaaacgcgtaacaaaagtgtctataatcacggcagaaaagtccacattgattatttgcacggcgtcacactttgctatgccatagcatttttatccataagattagcggatcctacctgacgctttttatcgcaactctctactgtttctccatacccgttttttggtaccgggccccccctcgagtttattttaggaggcaaaaatgaaaaacctgaccgaattcaccggtctgtatccggttagcaaaaccctgcgttttgaactgaaaccgaccgatgattttaactgggaaacctttctggaaagcaccatctttaaacatgatcaagaacgtgcagaagcctatccgattgttaaagttattgtggaccagttccacaagtggtttattgaagatgcactgaacaaaagcacgatcaattggaatagcctgtatgatgcatatttcgcaccgaaaaatgaaaacagcgttgaaaatctgcgcaaagagcaggataaaatccgcaaagaaattgtggatacctacttcaagaaacacgactggtggaaatatgtgagcaaagatcatagcaagctgttcaaaattgaactgcctgcactgctgagtgatgatgcatttatctatgagatcaacgacaagtatccgaactatacccaagaaattctgattgatgcactggccaaatttcagaactttagcgtttatttcggtggctatttcaaaaaccgcgacaacatgtataaaagtgatgcacagagcaccagcattgccaatcgtattgttaatgagaacttcaccaaattcgccgacaacatcaaaatctataaccgcctgaaagaaaactgtctgagcgaactgcagaaagtcgaactggattttaccgatgaactgaccggtctgacctttgatgatatctttagcccgagctacttcaacaaatgtctgacccagaaaggcatcgaaaaactgaatctgtatattggtggtaagaccggcaaaaacaaagaggataaagtttttggcattaaccgcgtgggtaatgaattcctgcagtttaacaaagagagcaagctgaaactgaaagacctgaaaatggtgaaactgtacaagcagattctgagcgatcgtgaacagccgagctttctgccggaacagtttcgtaatgaagatgagctgattaaaagcatcgaggattttcataacctgatcaccgaacagaaactgtttgaacgtctgctgaaattgatgggtcgtctgaaaaatggcgaatgtgaagatctgaataaaatccatgttgtgggtagctcactgacccagctgagcaaagttctgtatggtaattgggaagttctgggcaccgcactgcgcaataaattccagaccaataaaaccaaaaaggacaagctggaaagcgagaaagatatccaagaatggatggaacgtaaaagctttagcctggcacagattattgaagttgaaagcagcctgcaggatgacaaaagcattaaagtgattgacctgttcaccacctttaatgcatggcagaaagttaacgaaaaaccgcagctggttgatctgattaaactgtgcaaagatgattttcagacccgttttcgtgcagtgaaagatctgattgaaaaaggtgagcagattcagggcaatgaaagcgcaaaagaagaaattaaagccgtcctggataactatcagaacctgctgcatgttgtgaaactgctgaatctgggtaagaaagaaagctatctggataaggatgaaaccttctataacgagtacaaagaaatcctgagcagcaccgaaagcgataatgtttgtctggaagatattatcccgctgtataacaaagttcgtagctttctgacccgtaaactgggtgatgaaggtaaaatgctgctgaagtttgattgtagcaccctggcagatggttgggatgttggtaaagaaagcgccaataatagcaccattctgatcgataacagcaaatactatctgatcatcacgaacccggaaaataaaccggatctgagcaccgcaattaccagcaataccgataatgtgtacaaaaagattgtgtatcgccagattgcagatccgaccaaagatctgccgaatctgatggttattgatggtaaaacccagcgcaaaaccggcaataaagatgatgatggtattaatcgtgttctggaccagctgaaagataaatatctgccgcaagaagtgaatcgcattcgcaaactgggtagctatctgaaaaccagcgaacatttcaacaaaaaggatagccaggtttatctggcctattatatgcagcgcctgatcgaatataaacagggcgaaatggaattcagctttaagaacagcgaagagtatgatagctatagcgatttcctggatgatatcaccaagcagaaatattcactgagctttgtgaacgtgtcgaaagaaattatcacacagtggattagcgagggcaaaattttcctgtttcagatctacaacaaggacttcgaagaaaaagcaaccggtacaccgaatctgcataccctgtattggaaagaactgtttagcgaagagaacctgaaagacatcgtgtataaactgaatggtgaagcggaactgttctaccgtaaaaagatggatggtaaaccgttcacgcataacaaaggtgcagttctggtgaataaaacctttgcagatggtagtccggtggaaccggaacattataaagaatatgtggaatacatcaccggcaaggtgattgagaaacagctgagtaaagaagccaaagacaaactgcatctggtgaaaaccaataaagcgaaactggacatcatcaaggacaaacgctattttcagcacaaactgctgtttcatgttccgatcaccatcaactttaaaagcgaaggtgttccgaaattcaacgattacaccctgaattatctgcgcgagaacaagaaagacattaacatcattggtatcgatcgcggtgaacgcaatctgatttatgttagcgttattaatcagaaaggcgagaacattatccctccgaaacatttcaatatcgtggaaagtgatatgttcggcatggaagataaacgcaaattcaactacctggaaaagctgattcagaaagaaggtaatcgcgacgacgcacgtaaaaattggagtaaaattgaaacgatcaaagaccttaaaaccggctatctgagcctggttgttcatgaaattgcaaaactggttgttgaacatcatgccattgtggtgctggaagatcttaactatggttttaaacgcggtcgctttaatgtggaacgtcagatttaccagaattttgagaaaatgctgatcgagaagctgaacctgcttgtgtttaaaaacaatagcaacagtccggattatggcaatattctgaatggtctgcagctgaccgcaccgtttggtagctttaaagaactgggtaaacagagcggttggctgttttatgttaatgcaagctataccagcaaaatcgatccgcagaccggctttgcaaacctgtttaatatgaaagacgccaagaaggataccaagagctttttcgagaaaatcaccgagatcaaatatgacgacggcatgttcaaattcaccttcgattatcgtaacggctttagcattgttcagaccgactataaaaacatttggaccgtttgcaccaacgacaaacgtattctggtttccaaagataacatctcgggcaaatttaagcacgagtatgtggatattaccgaaagcatcaaaaacctgttcatcaacaacaacattaacgactatcatagcatcagcaaagaaaccatcctgtccatcaaagaaaagaagttctttgacgacctgttcttttacttcaaactgagcctgcagatgcgtaatagcattccgaatagcgatatcgattatctgatttcaccggtgcagattaaaggcaaaccgttctttgatagccgtattccgaacaatattaacatcgttgatgcagatgcaaatggtgcctatcatattgcactgaaaggcctgtatctggtgattaatgattttcccacagagaaaaagggcaaaagcgagtacctgaaaaagatcaccaatgaagattggtttgaattcgcacagcgtcgtagcctgaaataatggtctagaggtcgaaattcaaattgtgagcggataacaatttgaattttctgtatgaggttttgctaaacaactttcaacagtttcagtggagtgagaatagaaaggaacaactaaaggaattgcgaataataattttttcacgttgaaaatctccaaaaaaaaaggctccaaaaggagcctttaattgtatcggtttatcagcttgctttcgaggtgaattttgaccctctagcgaaaatgcaagagcaaagacgaaaacatgccacacatgaggaataccgattctctcattaacatattcaggccagttatctgggcttaaaagcagaagtccaacccagataacgatcatatacatggttctctccagaggttcattactgaacactcgtccgagaataacgagtggatcccctccaattcgccctatagtgagtcgtattacgcgcgctcactggccgtcgttttacaacgtcgtgactgggaaaaccctggcgttacccaacttaatcgccttgcagcacatccccctttcgccagctggcgtaatagcgaagaggcccgcaccgatcgcccttcccaacagttgcgcagcctgaatggcgaatggaaattgtaagcgttaatattttgttaaaattcgcgttaaatttttgttaaatcagctcattttttaaccaataggccgactgcgatgagtggcagggcggggcgtaatttttttaaggcagttattggtgcccttaaacgcctggtgctacgcctgaataagtgataataagcggatgaatggcagaaattcgaaagcaaattcgacccggtcgtcggttcagggcagggtcgttaaatagccgcttatgtctattgctggtttaccggtttattgactaccggaagcagtgtgaccgtgtgcttctcaaatgcctgaggccagtttgctcaggctctccccgtggaggtaataattgacgatatgatcatttattctgcctcccagagcctgataaaaacggtgaatccgttagcgaggtgccgccggcttccattcaggtcgaggtggcccggctccatgcaccgcgacgcaacgcggggaggcagacaaggtatagggcggcgaggcggctacagccgatagtctggaacagcgcacttacgggttgctgcgcaacccaagtgctaccggcgcggcagcgtgacccgtgtcggcggctccaacggctcgccatcgtccagaaaacacggctcatcgggcatcggcaggcgctgctgcccgcgccgttcccattcctccgtttcggtcaaggctggcaggtctggttccatgcccggaatgccgggctggctgggcggctcctcgccggggccggtcggtagttgctgctcgcccggatacagggtcgggatgcggcgcaggtcgccatgccccaacagcgattcgtcctggtcgtcgtgatcaaccaccacggcggcactgaacaccgacaggcgcaactggtcgcggggctggccccacgccacgcggtcattgaccacgtaggccgacacggtgccggggccgttgagcttcacgacggagatccagcgctcggccaccaagtccttgactgcgtattggaccgtccgcaaagaacgtccgatgagcttggaaagtgtcttttggctgaccaccacggcgttctggtggcccatctgcgccacgaggtgatgcagcagcattgccgccgtgggtttcctcgcaataagcccggcccacgcctcatgcgctttgcgttccgtttgcacccagtgaccgggcttgttcttggcttgaatgccgatttctctggactgcgtggccatgcttatctccatgcggtagggtgccgcacggttgcggcaccatgcgcaatcagctgcaacttttcggcagcgcgacaacaattatgcgttgcgtaaaagtggcagtcaattacagattttctttaacctacgcaatgagctattgcggggggtgccgcaatgagctgttgcgtaccccccttttttaagttgttgatttttaagtctttcgcatttcgccctatatctagttctttggtgcccaaagaagggcacccctgcggggttcccccacgccttcggcgcggctccccctccggcaaaaagtggcccctccggggcttgttgatcgactgcgcggccttcggccttgcccaaggtggcgctgcccccttggaacccccgcactcgccgccgtgaggctcggggggcaggcgggcgggcttcgccttcgactgcccccactcgcataggcttgggtcgttccaggcgcgtcaaggccaagccgctgcgcggtcgctgcgcgagccttgacccgccttccacttggtgtccaaccggcaagcgaagcgcgcaggccgcaggccggaggcttttccccagagaaaattaaaaaaattgatggggcaaggccgcaggccgcgcagttggagccggtgggtatgtggtcgaaggctgggtagccggtgggcaatccctgtggtcaagctcgtgggcaggcgcagcctgtccatcagcttgtccagcagggttgtccacgggccgagcgaagcgagccagccggtggccgctcgcggccatcgtccacatatccacgggctggcaagggagcgcagcgaccgcgcagggcgaagcccggagagcaagcccgtagggcgccgcagccgccgtaggcggtcacgactttgcgaagcaaagtctagtgagtatactcaagcattgagtggcccgccggaggcaccgccttgcgctgcccccgtcgagccggttggacaccaaaagggaggggcaggcatggcggcatacgcgatcatgcgatgcaagaagctggcgaaaatgggcaacgtggcggccagtctcaagcacgcctaccgcgagcgcgagacgcccaacgctgacgccagcaggacgccagagaacgagcactgggcggccagcagcaccgatgaagcgatgggccgactgcgcgagttgctgccagagaagcggcgcaaggacgctgtgttggcggtcgagtacgtcatgacggccagcccggaatggtggaagtcggccagccaagaacagcaggcggcgttcttcgagaaggcgcacaagtggctggcggacaagtacggggcggatcgcatcgtgacggccagcatccaccgtgacgaaaccagcccgcacatgaccgcgttcgtggtgccgctgacgcaggacggcaggctgtcggccaaggagttcatcggcaacaaagcgcagatgacccgcgaccagaccacgtttgcggccgctgtggccgatctagggctgcaacggggcatcgagggcagcaaggcacgtcacacgcgcattcaggcgttctacgaggccctggagcggccaccagtgggccacgtcaccatcagcccgcaagcggtcgagccacgcgcctatgcaccgcagggattggccgaaaagctgggaatctcaaagcgcgttgagacgccggaagccgtggccgaccggctgacaaaagcggttcggcaggggtatgagcctgccctacaggccgccgcaggagcgcgtgagatgcgcaagaaggccgatcaagcccaagagacggcccgagaccttcgggagcgcctgaagcccgttctggacgccctggggccgttgaatcgggatatgcaggccaaggccgccgcgatcatcaaggccgtgggcgaaaagctgctgacggaacagcgggaagtccagcgccagaaacaggcccagcgccagcaggaacgcgggcgcgcacatttccccgaaaagtgccacctgaaccccagagtcccgctcagaagaactcgtcaagaaggcgatagaaggcgatgcgctgcgaatcgggagcggcgataccgtaaagcacgaggaagcggtcagcccattcgccgccaagctcttcagcaatatcacgggtagccaacgctatgtcctgatagcggtccgccacacccagccggccacagtcgatgaatccagaaaagcggccattttccaccatgatattcggcaagcaggcatcgccatgggtcacgacgagatcctcgccgtcgggcatccgcgccttgagcctggcgaacagttcggctggcgcgagcccctgatgctcttcgtccagatcatcctgatcgacaagaccggcttccatccgagtacgtgctcgctcgatgcgatgtttcgcttggtggtcgaatgggcaggtagccggatcaagcgtatgcagccgccgcattgcatcagccatgatggatactttctcggcaggagcaaggtgagatgacaggagatcctgccccggcacttcgcccaatagcagccagtcccttcccgcttcagtgacaacgtcgagcacagctgcgcaaggaacgcccgtcgtggccagccacgatagccgcgctgcctcgtcttggagttcattcagggcaccggacaggtcggtcttgacaaaaagaaccgggcgcccctgcgctgacagccggaacacggcggcatcagagcagccgattgtctgttgtgcccagtcatagccgaatagcctctccacccaagcggccggagaacctgcgtgcaatccatcttgttcaatcatgcgaaacgatcctcatcctgtctcttgatcagatcttgatcccctgcgccatcagatccttggcggcaagaaagccatccagtttactttgcagggcttcccaaccttaccagagggcgccccagctggcaattccggttcgcttgctgtccataaaaccgcccagtctagctatcgccatgtaagcccactgcaagctacctgctttctctttgcgcttgcgttttcccttgtccagatagcccagtagctgacattcatccggggtcagcaccgtttctgcggactggctttctacgtgttccgcttcctttagcagcccttgcgccctgagtgcttgcggcagcgtgaagctagctgcataatgtgcctgtcaaatggacgaagcagggattctgcaaaccctatgctactccgtcaagccgtcaattgtctgattcgttaccaattatgacaacttgacggctacatcattcactttttcttcacaaccggcacggaactcgctcgggctggccccggtgcattttttaaatacccgcgagaaatagagttgatcgtcaaaaccaacattgcgaccgacggtggcgataggcatccgggtggtgctcaaaagcagcttcgcctggctgatacgttggtcctcgcgccagcttaagacgctaatccctaactgctggcggaaaagatgtgacagacgcgacggcgacaagcaaacatgctgtgcgacgctggcgatatcaaaattgctgtctgccaggtgatcgctgatgtactgacaagcctcgcgtacccgattatccatcggtggatggagcgactcgttaatcgcttccatgcgccgcagtaacaattgctcaagcagatttatcgccagcagctccgaatagcgcccttccccttgcccggcgttaatgatttgcccaaacaggtcgctgaaatgcggctggtgcgcttcatccgggcgaaagaaccccgtattggcaaatattgacggccagttaagccattcatgccagtaggcgcgcggacgaaagtaaacccactggtgataccattcgcgagcctccggatgacgaccgtagtgatgaatctctcctggcgggaacagcaaaatatcacccggtcggcaaacaaattctcgtccctgatttttcaccaccccctgaccgcgaatggtgagattgagaatataacctttcattcccagcggtcggtcgataaaaaaatcgagataaccgttggcct

SEQ ID NO: 39 - DNA, 10153 bp, Artificial Sequence
  CRISPR/BMC09-Ec vector system
caatcggcgttaaacccgccaccagatgggcattaaacgagtatcccggcagcaggggatcattttgcgcttcagccatacttttcatactcccgccattcagagaagaaaccaattgtccatattgcatcagacattgccgtcactgcgtcttttactggctcttctcgctaaccaaaccggtaaccccgcttattaaaagcattctgtaacaaagcgggaccaaagccatgacaaaaacgcgtaacaaaagtgtctataatcacggcagaaaagtccacattgattatttgcacggcgtcacactttgctatgccatagcatttttatccataagattagcggatcctacctgacgctttttatcgcaactctctactgtttctccatacccgttttttggtaccgggccccccctcgagtttattttaggaggcaaaaatgaagaacagcctggaagatttcaccaatctgtatagcctgcagaaaaccctgcgttttgaactgaaaccgattggtaatacccagagcatgctggaagaagatggcgtttttgataccgatgaaaaacgcaaaatcgcctacagcaaaaccaaaccgtatattgatcgtctgcaccgcgaatttattgaagaaagtctgtcagatgcccagatcagcaaactggatgaatatttcaaagcctacgtggactacaaaaaggacaagaaagataccaaacgcttcaaccgcatcaaacagtttaaaagcgttctgcgtaaagaagtggtggatcactttaacaaacagggtaaagaatggaccaccgtgaaatttgcacatctgaaaatcaaaaagaaagatctggaagtgctgttcgaaaaacagctgccgaatattctgaaagaagaatacggcaccgaaaaagaaacccagattattgatgaagatagcggtgaagtgaccagcatttttgatatgtggaatggctttatgggctatttcacgaaatttttcgaaacccgcaagaacttctataaaagtgatggcaccagcaccgcaattgcaacccgcattattgatcagaatctggatcgctttatcgagaacatcctgatctatgatagcatcaaaccgaaaatcgataccagcgaagttcgcgaatttttcaatctggaaagcgataccatctttagcatggaattctataataactgtctgctgcaggcaggcattgatcagtataacaattttcttggtggcaaaaccctggaaaacggtcgtaaaattcgtggcattaacgagctgattaacaaatatcgtcaagagaacccggaagataaaatcccgtttctgaaaaagctggataagcagatccatagcgagaaagagaaatttatccagcagatcgaaacactggaagatctgaaagaggaactgcagaaattttacaatagcagcaacgagaagatcaaaattctggataatctgctgagccgcatcgaagaatttaaaccggaaggtatcttcattagcaaacaggcctttaataccattagccgtcgttggaccgatcagagcgaagcatttgaaaccagcctgtttgaaagccttaaagaagaaaaaccgattaccggcaccgcaaagaaaaaggatgatggttataacttcccggaattcattagtctgcagagcattcgtaataccctgaaaaaggttcagggtgaagaacgtttttggaaagaacgttattatcgcgacaatagcgaaagcggtattctggcaggtaatgaagaaatttggacccagtttctgatgatcttcaaaagcgaattcaacagcaaattcgaacgcaatgatcctgaagataatggcaccattggctacaacctgtttaaagaggatctggaaaaactgctgaaagacctgaaaattaccaaagacaccaagagcatcattaaacgctttgcagatgaagccctgcatatttatcaggtgggtaaatactttgcgctggaaaaagatcgtgtttggattagcagctatgatgatctgcttgataccttttataccgatccgaataccggttatctgagcttttatgaaggtgcctatgagcagattgttcagccgtataatatgatccgtaattatctgacccgtaaaccgtacagtgatgagaaatggaaactgaactttgaaaatccgacactggcaaatggttgggacaaaaacaaagaaaccgataacagcagtatcatgctgcgcaaagaaggtgcatattatctgggtatcatgaagaaaggcaagaacaaactgttcgaagaacgtaatcgtcagctgtttgaaccgaaaaatggtgaggatacgtatgagaaactgagctataaactgttcccggatcctgcaaaaatgattccgaaagtttgcttcagcaacaaaaacatccagatgtttagcccgagcaccgaaatcatgaatatctataatggcgaaaccttcaagaaaaactccgatgattttagcgttagcagcatgcagaaactgattgccttctataccaaatgtctgagccagtatgaaggctggaaatactatgacttcaaatatatcaaaagtccggatcagtacaaggataacatcggcgagttttataacgatgttgccaaaagcggttatcgtgtgtggtttgaaaacattagccagagctatgtggatagcaaaaataccatgggtgaactgtacctgttcaagatccataacaaagactggaaccagaaagataaaaagaccaaagtgggcagcaaaaacctgcatacccattattttgaagaactgttcagccaggacaacatcgaaaataactttccgctgaaactgaatggtgaagccgaagtgttttatcgtccgaaaaccaatcctgaaaaactgggcaccaaaaaggatagtaaaggtcgtgaagtgattgatcgtaaacgttatgcaagcgataaggtgctgtttcatgttccgattacactgaatcgtacaccggttaccaccaccaaactgaataaagaaattaatggcttcctggccaacaatccgagcattaacattattggtgttgatcgcggtgaaaaacacctggtgtattattcagtggtgaatcagcgtggtaagatgctggaaagtggtagctttaacacaattaacggcgtggattatcacggcaaattggaagaacgtgcagatcgtcgtgaacaggcacgtcgtgattggcaggatgttgaaggcattaaaaacctgaagaagggctatattagcctggttgttcgtgaactggccaatctgagcatcaaatataacgccattatcgtgatggaagatcttaacatgcgctttaagcagattcgtggtggtatcgaaaaatcagcatatcagcagttagaaaaagccctgatcgaaaagctgaattacctggtgaataaaaccgaaaccgatccgcagaaaacaggtcatatcctgaaagcctatcagctgaccagtccgattaaaagctttaaagagatgggtaaacagaccggcatcattttctatacccaggcaagctataccagcgttacagatccgatcaccggttggcgtccgaatctgtatctgaaatatagcagcgcaagcaaagcgaaaagcgacattctgaaattcagcaagattagctacaacaccaacaacaaccgctttgagtttacctatgatctgcgcaattttgtgaacatgaaggcctatcctcagaaaaccgcatggaccatttgtagcaatgttgaacgttttcgttgggatcgcaaaggcaataagaataacggtgagtacatccagtataaggatctgaccgaaaactttaagaccttcttcgaggaagtcagcattaactataaaggcgatattctgttccagatcaagaacctgagcgaaaaaggtaacgaaaaattctttcgcgacctgatcttttacattagcctgattagtcagattcgcaacacccagaaagacaagaagggtgacgaaaacgattttattctgagtccggttgaaccgttctttgatagccgtaaaagcagcacctttggtgaaaatctgccgctgaacggtgatgcaaatggtgcatacaatattgcacgcaagggcattattatgctgaacaaaatttcaaaaggcagcaagaataaagtcaaagaggatattggttggggagatctgtatattccgcataccgaatgggatgattttgcaaccggtagcatttaatggtctagaggtcgaaattcaaattgtgagcggataacaatttgaattttctgtatgaggttttgctaaacaactttcaacagtttcagtggagtgagaatagaaaggaacaactaaaggaattgcgaataataattttttcacgttgaaaatctccaaaaaaaaaggctccaaaaggagcctttaattgtatcggtttatcagcttgctttcgaggtgaattttgaccctctagcgaaaatgcaagagcaaagacgaaaacatgccacacatgaggaataccgattctctcattaacatattcaggccagttatctgggcttaaaagcagaagtccaacccagataacgatcatatacatggttctctccagaggttcattactgaacactcgtccgagaataacgagtggatcccctccaattcgccctatagtgagtcgtattacgcgcgctcactggccgtcgttttacaacgtcgtgactgggaaaaccctggcgttacccaacttaatcgccttgcagcacatccccctttcgccagctggcgtaatagcgaagaggcccgcaccgatcgcccttcccaacagttgcgcagcctgaatggcgaatggaaattgtaagcgttaatattttgttaaaattcgcgttaaatttttgttaaatcagctcattttttaaccaataggccgactgcgatgagtggcagggcggggcgtaatttttttaaggcagttattggtgcccttaaacgcctggtgctacgcctgaataagtgataataagcggatgaatggcagaaattcgaaagcaaattcgacccggtcgtcggttcagggcagggtcgttaaatagccgcttatgtctattgctggtttaccggtttattgactaccggaagcagtgtgaccgtgtgcttctcaaatgcctgaggccagtttgctcaggctctccccgtggaggtaataattgacgatatgatcatttattctgcctcccagagcctgataaaaacggtgaatccgttagcgaggtgccgccggcttccattcaggtcgaggtggcccggctccatgcaccgcgacgcaacgcggggaggcagacaaggtatagggcggcgaggcggctacagccgatagtctggaacagcgcacttacgggttgctgcgcaacccaagtgctaccggcgcggcagcgtgacccgtgtcggcggctccaacggctcgccatcgtccagaaaacacggctcatcgggcatcggcaggcgctgctgcccgcgccgttcccattcctccgtttcggtcaaggctggcaggtctggttccatgcccggaatgccgggctggctgggcggctcctcgccggggccggtcggtagttgctgctcgcccggatacagggtcgggatgcggcgcaggtcgccatgccccaacagcgattcgtcctggtcgtcgtgatcaaccaccacggcggcactgaacaccgacaggcgcaactggtcgcggggctggccccacgccacgcggtcattgaccacgtaggccgacacggtgccggggccgttgagcttcacgacggagatccagcgctcggccaccaagtccttgactgcgtattggaccgtccgcaaagaacgtccgatgagcttggaaagtgtcttttggctgaccaccacggcgttctggtggcccatctgcgccacgaggtgatgcagcagcattgccgccgtgggtttcctcgcaataagcccggcccacgcctcatgcgctttgcgttccgtttgcacccagtgaccgggcttgttcttggcttgaatgccgatttctctggactgcgtggccatgcttatctccatgcggtagggtgccgcacggttgcggcaccatgcgcaatcagctgcaacttttcggcagcgcgacaacaattatgcgttgcgtaaaagtggcagtcaattacagattttctttaacctacgcaatgagctattgcggggggtgccgcaatgagctgttgcgtaccccccttttttaagttgttgatttttaagtctttcgcatttcgccctatatctagttctttggtgcccaaagaagggcacccctgcggggttcccccacgccttcggcgcggctccccctccggcaaaaagtggcccctccggggcttgttgatcgactgcgcggccttcggccttgcccaaggtggcgctgcccccttggaacccccgcactcgccgccgtgaggctcggggggcaggcgggcgggcttcgccttcgactgcccccactcgcataggcttgggtcgttccaggcgcgtcaaggccaagccgctgcgcggtcgctgcgcgagccttgacccgccttccacttggtgtccaaccggcaagcgaagcgcgcaggccgcaggccggaggcttttccccagagaaaattaaaaaaattgatggggcaaggccgcaggccgcgcagttggagccggtgggtatgtggtcgaaggctgggtagccggtgggcaatccctgtggtcaagctcgtgggcaggcgcagcctgtccatcagcttgtccagcagggttgtccacgggccgagcgaagcgagccagccggtggccgctcgcggccatcgtccacatatccacgggctggcaagggagcgcagcgaccgcgcagggcgaagcccggagagcaagcccgtagggcgccgcagccgccgtaggcggtcacgactttgcgaagcaaagtctagtgagtatactcaagcattgagtggcccgccggaggcaccgccttgcgctgcccccgtcgagccggttggacaccaaaagggaggggcaggcatggcggcatacgcgatcatgcgatgcaagaagctggcgaaaatgggcaacgtggcggccagtctcaagcacgcctaccgcgagcgcgagacgcccaacgctgacgccagcaggacgccagagaacgagcactgggcggccagcagcaccgatgaagcgatgggccgactgcgcgagttgctgccagagaagcggcgcaaggacgctgtgttggcggtcgagtacgtcatgacggccagcccggaatggtggaagtcggccagccaagaacagcaggcggcgttcttcgagaaggcgcacaagtggctggcggacaagtacggggcggatcgcatcgtgacggccagcatccaccgtgacgaaaccagcccgcacatgaccgcgttcgtggtgccgctgacgcaggacggcaggctgtcggccaaggagttcatcggcaacaaagcgcagatgacccgcgaccagaccacgtttgcggccgctgtggccgatctagggctgcaacggggcatcgagggcagcaaggcacgtcacacgcgcattcaggcgttctacgaggccctggagcggccaccagtgggccacgtcaccatcagcccgcaagcggtcgagccacgcgcctatgcaccgcagggattggccgaaaagctgggaatctcaaagcgcgttgagacgccggaagccgtggccgaccggctgacaaaagcggttcggcaggggtatgagcctgccctacaggccgccgcaggagcgcgtgagatgcgcaagaaggccgatcaagcccaagagacggcccgagaccttcgggagcgcctgaagcccgttctggacgccctggggccgttgaatcgggatatgcaggccaaggccgccgcgatcatcaaggccgtgggcgaaaagctgctgacggaacagcgggaagtccagcgccagaaacaggcccagcgccagcaggaacgcgggcgcgcacatttccccgaaaagtgccacctgaaccccagagtcccgctcagaagaactcgtcaagaaggcgatagaaggcgatgcgctgcgaatcgggagcggcgataccgtaaagcacgaggaagcggtcagcccattcgccgccaagctcttcagcaatatcacgggtagccaacgctatgtcctgatagcggtccgccacacccagccggccacagtcgatgaatccagaaaagcggccattttccaccatgatattcggcaagcaggcatcgccatgggtcacgacgagatcctcgccgtcgggcatccgcgccttgagcctggcgaacagttcggctggcgcgagcccctgatgctcttcgtccagatcatcctgatcgacaagaccggcttccatccgagtacgtgctcgctcgatgcgatgtttcgcttggtggtcgaatgggcaggtagccggatcaagcgtatgcagccgccgcattgcatcagccatgatggatactttctcggcaggagcaaggtgagatgacaggagatcctgccccggcacttcgcccaatagcagccagtcccttcccgcttcagtgacaacgtcgagcacagctgcgcaaggaacgcccgtcgtggccagccacgatagccgcgctgcctcgtcttggagttcattcagggcaccggacaggtcggtcttgacaaaaagaaccgggcgcccctgcgctgacagccggaacacggcggcatcagagcagccgattgtctgttgtgcccagtcatagccgaatagcctctccacccaagcggccggagaacctgcgtgcaatccatcttgttcaatcatgcgaaacgatcctcatcctgtctcttgatcagatcttgatcccctgcgccatcagatccttggcggcaagaaagccatccagtttactttgcagggcttcccaaccttaccagagggcgccccagctggcaattccggttcgcttgctgtccataaaaccgcccagtctagctatcgccatgtaagcccactgcaagctacctgctttctctttgcgcttgcgttttcccttgtccagatagcccagtagctgacattcatccggggtcagcaccgtttctgcggactggctttctacgtgttccgcttcctttagcagcccttgcgccctgagtgcttgcggcagcgtgaagctagctgcataatgtgcctgtcaaatggacgaagcagggattctgcaaaccctatgctactccgtcaagccgtcaattgtctgattcgttaccaattatgacaacttgacggctacatcattcactttttcttcacaaccggcacggaactcgctcgggctggccccggtgcattttttaaatacccgcgagaaatagagttgatcgtcaaaaccaacattgcgaccgacggtggcgataggcatccgggtggtgctcaaaagcagcttcgcctggctgatacgttggtcctcgcgccagcttaagacgctaatccctaactgctggcggaaaagatgtgacagacgcgacggcgacaagcaaacatgctgtgcgacgctggcgatatcaaaattgctgtctgccaggtgatcgctgatgtactgacaagcctcgcgtacccgattatccatcggtggatggagcgactcgttaatcgcttccatgcgccgcagtaacaattgctcaagcagatttatcgccagcagctccgaatagcgcccttccccttgcccggcgttaatgatttgcccaaacaggtcgctgaaatgcggctggtgcgcttcatccgggcgaaagaaccccgtattggcaaatattgacggccagttaagccattcatgccagtaggcgcgcggacgaaagtaaacccactggtgataccattcgcgagcctccggatgacgaccgtagtgatgaatctctcctggcgggaacagcaaaatatcacccggtcggcaaacaaattctcgtccctgatttttcaccaccccctgaccgcgaatggtgagattgagaatataacctttcattcccagcggtcggtcgataaaaaaatcgagataaccgttggcct

SEQ ID NO: 40 - DNA, 10486 bp, Artificial Sequence
  CRISPR/BMC13-Ec vector system
ccatgcttatctccatgcggtagggtgccgcacggttgcggcaccatgcgcaatcagctgcaacttttcggcagcgcgacaacaattatgcgttgcgtaaaagtggcagtcaattacagattttctttaacctacgcaatgagctattgcggggggtgccgcaatgagctgttgcgtaccccccttttttaagttgttgatttttaagtctttcgcatttcgccctatatctagttctttggtgcccaaagaagggcacccctgcggggttcccccacgccttcggcgcggctccccctccggcaaaaagtggcccctccggggcttgttgatcgactgcgcggccttcggccttgcccaaggtggcgctgcccccttggaacccccgcactcgccgccgtgaggctcggggggcaggcgggcgggcttcgccttcgactgcccccactcgcataggcttgggtcgttccaggcgcgtcaaggccaagccgctgcgcggtcgctgcgcgagccttgacccgccttccacttggtgtccaaccggcaagcgaagcgcgcaggccgcaggccggaggcttttccccagagaaaattaaaaaaattgatggggcaaggccgcaggccgcgcagttggagccggtgggtatgtggtcgaaggctgggtagccggtgggcaatccctgtggtcaagctcgtgggcaggcgcagcctgtccatcagcttgtccagcagggttgtccacgggccgagcgaagcgagccagccggtggccgctcgcggccatcgtccacatatccacgggctggcaagggagcgcagcgaccgcgcagggcgaagcccggagagcaagcccgtagggcgccgcagccgccgtaggcggtcacgactttgcgaagcaaagtctagtgagtatactcaagcattgagtggcccgccggaggcaccgccttgcgctgcccccgtcgagccggttggacaccaaaagggaggggcaggcatggcggcatacgcgatcatgcgatgcaagaagctggcgaaaatgggcaacgtggcggccagtctcaagcacgcctaccgcgagcgcgagacgcccaacgctgacgccagcaggacgccagagaacgagcactgggcggccagcagcaccgatgaagcgatgggccgactgcgcgagttgctgccagagaagcggcgcaaggacgctgtgttggcggtcgagtacgtcatgacggccagcccggaatggtggaagtcggccagccaagaacagcaggcggcgttcttcgagaaggcgcacaagtggctggcggacaagtacggggcggatcgcatcgtgacggccagcatccaccgtgacgaaaccagcccgcacatgaccgcgttcgtggtgccgctgacgcaggacggcaggctgtcggccaaggagttcatcggcaacaaagcgcagatgacccgcgaccagaccacgtttgcggccgctgtggccgatctagggctgcaacggggcatcgagggcagcaaggcacgtcacacgcgcattcaggcgttctacgaggccctggagcggccaccagtgggccacgtcaccatcagcccgcaagcggtcgagccacgcgcctatgcaccgcagggattggccgaaaagctgggaatctcaaagcgcgttgagacgccggaagccgtggccgaccggctgacaaaagcggttcggcaggggtatgagcctgccctacaggccgccgcaggagcgcgtgagatgcgcaagaaggccgatcaagcccaagagacggcccgagaccttcgggagcgcctgaagcccgttctggacgccctggggccgttgaatcgggatatgcaggccaaggccgccgcgatcatcaaggccgtgggcgaaaagctgctgacggaacagcgggaagtccagcgccagaaacaggcccagcgccagcaggaacgcgggcgcgcacatttccccgaaaagtgccacctgaaccccagagtcccgctcagaagaactcgtcaagaaggcgatagaaggcgatgcgctgcgaatcgggagcggcgataccgtaaagcacgaggaagcggtcagcccattcgccgccaagctcttcagcaatatcacgggtagccaacgctatgtcctgatagcggtccgccacacccagccggccacagtcgatgaatccagaaaagcggccattttccaccatgatattcggcaagcaggcatcgccatgggtcacgacgagatcctcgccgtcgggcatccgcgccttgagcctggcgaacagttcggctggcgcgagcccctgatgctcttcgtccagatcatcctgatcgacaagaccggcttccatccgagtacgtgctcgctcgatgcgatgtttcgcttggtggtcgaatgggcaggtagccggatcaagcgtatgcagccgccgcattgcatcagccatgatggatactttctcggcaggagcaaggtgagatgacaggagatcctgccccggcacttcgcccaatagcagccagtcccttcccgcttcagtgacaacgtcgagcacagctgcgcaaggaacgcccgtcgtggccagccacgatagccgcgctgcctcgtcttggagttcattcagggcaccggacaggtcggtcttgacaaaaagaaccgggcgcccctgcgctgacagccggaacacggcggcatcagagcagccgattgtctgttgtgcccagtcatagccgaatagcctctccacccaagcggccggagaacctgcgtgcaatccatcttgttcaatcatgcgaaacgatcctcatcctgtctcttgatcagatcttgatcccctgcgccatcagatccttggcggcaagaaagccatccagtttactttgcagggcttcccaaccttaccagagggcgccccagctggcaattccggttcgcttgctgtccataaaaccgcccagtctagctatcgccatgtaagcccactgcaagctacctgctttctctttgcgcttgcgttttcccttgtccagatagcccagtagctgacattcatccggggtcagcaccgtttctgcggactggctttctacgtgttccgcttcctttagcagcccttgcgccctgagtgcttgcggcagcgtgaagctagctgcataatgtgcctgtcaaatggacgaagcagggattctgcaaaccctatgctactccgtcaagccgtcaattgtctgattcgttaccaattatgacaacttgacggctacatcattcactttttcttcacaaccggcacggaactcgctcgggctggccccggtgcattttttaaatacccgcgagaaatagagttgatcgtcaaaaccaacattgcgaccgacggtggcgataggcatccgggtggtgctcaaaagcagcttcgcctggctgatacgttggtcctcgcgccagcttaagacgctaatccctaactgctggcggaaaagatgtgacagacgcgacggcgacaagcaaacatgctgtgcgacgctggcgatatcaaaattgctgtctgccaggtgatcgctgatgtactgacaagcctcgcgtacccgattatccatcggtggatggagcgactcgttaatcgcttccatgcgccgcagtaacaattgctcaagcagatttatcgccagcagctccgaatagcgcccttccccttgcccggcgttaatgatttgcccaaacaggtcgctgaaatgcggctggtgcgcttcatccgggcgaaagaaccccgtattggcaaatattgacggccagttaagccattcatgccagtaggcgcgcggacgaaagtaaacccactggtgataccattcgcgagcctccggatgacgaccgtagtgatgaatctctcctggcgggaacagcaaaatatcacccggtcggcaaacaaattctcgtccctgatttttcaccaccccctgaccgcgaatggtgagattgagaatataacctttcattcccagcggtcggtcgataaaaaaatcgagataaccgttggcctcaatcggcgttaaacccgccaccagatgggcattaaacgagtatcccggcagcaggggatcattttgcgcttcagccatacttttcatactcccgccattcagagaagaaaccaattgtccatattgcatcagacattgccgtcactgcgtcttttactggctcttctcgctaaccaaaccggtaaccccgcttattaaaagcattctgtaacaaagcgggaccaaagccatgacaaaaacgcgtaacaaaagtgtctataatcacggcagaaaagtccacattgattatttgcacggcgtcacactttgctatgccatagcatttttatccataagattagcggatcctacctgacgctttttatcgcaactctctactgtttctccatacccgttttttggtaccgggccccccctcgagtttattttaggaggcaaaaatgagcaccaaaaccatctttagcgatttcaccaatctgtacgaactgagcaaaaccctgcgttttgaactgaaaccggttggtgaaaccgaaaatctgctgaatgaaaatcaggtgttcctgaccgataaaatccgccagaaaaaatacgaagagatcaaaccgtttctggatgaatttcacctggactttattcacttttgtctgagcgatctgcatctggattataccgaatacaaaaaaagcctggacaactaccagaaggacaaaaaaaacaaagatctggaaaaaaagaaagagaacgaagagaaaaaactgcgcgagcagattgtgggtaaatttgatagcaaagtggaagattttctgaaaacctttggcaaggtggaaaaaatcaaaggcaaaaaggacaacgagaagttcaaagttagcctgggtaaagattgggagatcgaatttagcaaaaacaactacgaattcctgttcgagatcggcattttcgatctgatgaagaaaaagtttgaaggcaacggcgatatttatgtggcagataaagaaaccggtgagatctatcaggatgaaaaaaccggtaaagacatcaccatcttcgatgattggaatggttggctgggttatctgaccaaatttttcgaaacccgcaaaaacctgtataaaagtgatggcaccagcaccgcaattgcaacccgtattatcaatgaaaacctgaagaaatactgcgagaacctggacatctataacaaactgagccagattgagaacctgaaaaacaaattccaaaacctggaagccgatttcggcattaaactggaaaaattctttagcctggaaaattacaacagctgcatcctgcagaatggcatcgaaaactataatgatattcgcggtggtaagctggaaaagaacaataacaaaattccgggtatcaacgagtacatcaataaataccgtcaggatagcggtgaaaaactgccgtttctgcaaaaactggataagcagattctggcaggcggtaaagaaaactttattgagcagatagaaaacgagccgagctttgaaaaatgcctgaagaacttttacaacaacagcatcaagaaggtggatattctgacccagatttttcaggatctgagcacctataccaacgaggactataaaaccatttatttcagcaaagaggccttcaataccctgagccataaattcaccgatcaggtgctgaattttgagaaactggtttttgaagaactgctgctgaataagctggtcgagaaaaaagacttcgacaaaaaagaagaaaaatacaagttcccggatttcatcccgctgttctatgttaaaaaaggccttgaaaactatcacaccaagaacctgttctataaaagccgctattatgagaacgaaattatcgaagaggataacgacaacatctggcagaaattttgcaccatcctgaactatgaattccagagcctgctgagcaataccattattaaccagaatggcgaagaaatcgaagtgggttttaccatcagtaagaacaagcttgagaagatcctggacaattttagtctgggcgaaaataacaacggcatcatcaaagattttgccgacatcagcaaaacgatttatcagatgggtaaatacttcgcccttgaaaaaaaacgcgaatggaacaacaacttcgacctgaacgatgatttttacaaaaccgagtatagccaagaaaacgaaaaatacggttatctggaattttacaacgaggcctatgagcagattattgtgccgtataatctgatgcgcaactttatcgcaaaaaagccgtgggaagataacaagaaatggaaactgaacttcgaaaatagcagtctgctgaaaggttgggataaagaattcgaaagctatggcagctacatctttgagaaagcaggtctgtattatctgggcatcattaatggcaccaaactgaacaaaaacgagatcgagaaactgtacaattataacgccaataatggtgccaaacgcttcgtgtatgatttccagaaaccggacaacaaaaatacaccgcgtctgtttattcgtagcaaaggcgataactttgcaccgagcgttaaagaactgaatctgccgattaataacatcatcgaaatctatgataaagagctgtacaagaaagataaagagaagccgaacaagcataaagaaagcctgatgaaactgatcgactatttcaaactgggctttcgcaaacacatcagctataaacactttaacttcgtgtggaaagaaagcaacaaatatgacaacattgccgatttttatcgcgacgttgaaaaaagctgctataaaccgtattgggaagaggacatcaacttcgatgaactgaagaatctgacgaaagaaaaacgcatgtacctgtttcagatctacaataagaacttcgagctggatgaaagcattagcaccgatgattacacgtttaaaggcaatggtaaagatagcgtgcacaccatgtatttcaaaggcctgtttagcaaagataaccttgagaataaaaacggcgtcaacctgaaactgagcggtggtggtgaactgttttttcgtccgaaaagcattgagaaaaaaatcgacaagaaccgcaaaagcaaacgcgaaatcattgagaacaaacgctacagcaaagacaaaatcctgctgcattttccgattcaggtgaacttcaaagaaaacaagaccagcaacttcaacaactacatcaacaattttctggccaacaatcccgacattaacattattggtattgaccgtggcgaaaaacacctggcatattatagcgttatcaaccagaaacaagagattattgaaagcggcagcctgaactacatctatcagaaagacaaagatggcaaaatcattcagaaaagcgagaaaaagattcaagaggtgcgtaatgatgaaggcaagatcattgattatgaactggttgaaaccggcaaactggtggattatgaagattatggtatcctgctggactacaaagaaaaaaagcgtcgtctgcagcgtcagagctggaaagaagttgaacaaatcaaggatctgaagaagggctatattagcgcagttgttcgtaaaattgcggatctgattatcgaacataacgccatcgtgatctttgaggacctgaatatgcgctttaaacaaatccgtggtggtattgaaaaatccgtgtatcagcagttagaaaaagccctgattgataagctgaacttcctggttaacaaaggcgagaaagatagtgaacaggcaggtaatttactgaaagcgtttcagctgaccgcaccgattggcacctttaaagatatgggtaaacagaccggcattatcttttatacccaggcacgttataccagcaaaattgatccgctgaccggttggcgtccgaatctgtatatcaaaaaacagagtgccgagctgaacaaagagagcattctgaaattcgatagcatcatctggaataaagaaaaagagtacttcgaaatcacctatgacctggaaaagtttcagagcgaaagtaccaaaaatctgaaagagaagaaagaagagaagctggaacgtaccaaatggaccctgagcacccgtgttgaacgttttaaatggaataagaaccttaataacaacaaaggtggctacgaacacttcgagaatctgaacatccatttcaaagaactgtttgagaaatatggcctggatattagcggtgatatcctgaagcaaatccataatctggaaaccaaaggtaacgaagcctttttcagccattttctggacctgtttaaactggtgtgtcagattcgtaataccaaccaggataaaaagggtaacgagaacgatttcatttacagtccggtgtttccgtttttcgatagccgtaaacagaataccgttggcgttaaaaatggtgatgataacggtgcattcaacattgcacgtaaaggcattattatcctggaacgcattggcaagtggaagaaagaaaacgatatgaagattcagaaaggtgaaaaagagatgtatccggacctgttcattagcaatattggctgggataatttcacgcagaatcataacattcgcgataattaatggtctagaggtcgaaattcaaattgtgagcggataacaatttgaattttctgtatgaggttttgctaaacaactttcaacagtttcagtggagtgagaatagaaaggaacaactaaaggaattgcgaataataattttttcacgttgaaaatctccaaaaaaaaaggctccaaaaggagcctttaattgtatcggtttatcagcttgctttcgaggtgaattttgaccctctagcgaaaatgcaagagcaaagacgaaaacatgccacacatgaggaataccgattctctcattaacatattcaggccagttatctgggcttaaaagcagaagtccaacccagataacgatcatatacatggttctctccagaggttcattactgaacactcgtccgagaataacgagtggatcccctccaattcgccctatagtgagtcgtattacgcgcgctcactggccgtcgttttacaacgtcgtgactgggaaaaccctggcgttacccaacttaatcgccttgcagcacatccccctttcgccagctggcgtaatagcgaagaggcccgcaccgatcgcccttcccaacagttgcgcagcctgaatggcgaatggaaattgtaagcgttaatattttgttaaaattcgcgttaaatttttgttaaatcagctcattttttaaccaataggccgactgcgatgagtggcagggcggggcgtaatttttttaaggcagttattggtgcccttaaacgcctggtgctacgcctgaataagtgataataagcggatgaatggcagaaattcgaaagcaaattcgacccggtcgtcggttcagggcagggtcgttaaatagccgcttatgtctattgctggtttaccggtttattgactaccggaagcagtgtgaccgtgtgcttctcaaatgcctgaggccagtttgctcaggctctccccgtggaggtaataattgacgatatgatcatttattctgcctcccagagcctgataaaaacggtgaatccgttagcgaggtgccgccggcttccattcaggtcgaggtggcccggctccatgcaccgcgacgcaacgcggggaggcagacaaggtatagggcggcgaggcggctacagccgatagtctggaacagcgcacttacgggttgctgcgcaacccaagtgctaccggcgcggcagcgtgacccgtgtcggcggctccaacggctcgccatcgtccagaaaacacggctcatcgggcatcggcaggcgctgctgcccgcgccgttcccattcctccgtttcggtcaaggctggcaggtctggttccatgcccggaatgccgggctggctgggcggctcctcgccggggccggtcggtagttgctgctcgcccggatacagggtcgggatgcggcgcaggtcgccatgccccaacagcgattcgtcctggtcgtcgtgatcaaccaccacggcggcactgaacaccgacaggcgcaactggtcgcggggctggccccacgccacgcggtcattgaccacgtaggccgacacggtgccggggccgttgagcttcacgacggagatccagcgctcggccaccaagtccttgactgcgtattggaccgtccgcaaagaacgtccgatgagcttggaaagtgtcttttggctgaccaccacggcgttctggtggcccatctgcgccacgaggtgatgcagcagcattgccgccgtgggtttcctcgcaataagcccggcccacgcctcatgcgctttgcgttccgtttgcacccagtgaccgggcttgttcttggcttgaatgccgatttctctggactgcgtgg

SEQ ID NO: 41 - DNA, 165 bp, Bacillus megaterium
  Nucleotide sequence of the PsacB RNA polymerase II promotor from Bacillus megaterium
gcccatgcaacagaaactataaaaaatacagagaatgaaaagaaacagatagattttttagttctttaggcccgtagtctgcaaatccttttatgattttctatcaaacaaaagaggaaaatagaccagttgcaatccaaacgagagtctaatagaatgaggtcg

SEQ ID NO: 42 - DNA, 169 bp, Escherichia coli
  Nucleotide sequence of the transcription T1 and T2 termination region of the E. coli rrnB gene
tttgcctggcggcagtagcgcggtggtcccacctgaccccatgccgaactcagaagtgaaacgccgtagcgccgatggtagtgtggggtctccccatgcgagagtagggaactgccaggcatcaaataaaacgaaaggctcagtcgaaagactgggcctttcgttttat

SEQ ID NO: 43 - DNA, 24 bp, Artificial Sequence
  MalQ target-specific 24 bps spacer sequence
gtggcggtacgttgatgcatcgcg

SEQ ID NO: 44 - DNA, 5039 bp, Artificial Sequence
  Nucleotide sequence of the CRISPR/gRNA-Ec vector system
gacgaaagggcctcgtgatacgcctatttttataggttaatgtcatgataataatggtttcttagacgtcaggtggcacttttcggggaaatgtgcgcggaacccctatttgtttatttttctaaatacattcaaatatgtatccgctcatgagacaataaccctgataaatgcttcaataatattgaaaaaggaagagtatgagtattcaacatttccgtgtcgcccttattcccttttttgcggcattttgccttcctgtttttgctcacccagaaacgctggtgaaagtaaaagatgctgaagatcagttgggtgcacgagtgggttacatcgaactggatctcaacagcggtaagatccttgagagttttcgccccgaagaacgttttccaatgatgagcacttttaaagttctgctatgtggcgcggtattatcccgtattgacgccgggcaagagcaactcggtcgccgcatacactattctcagaatgacttggttgagtactcaccagtcacagaaaagcatcttacggatggcatgacagtaagagaattatgcagtgctgccataaccatgagtgataacactgcggccaacttacttctgacaacgatcggaggaccgaaggagctaaccgcttttttgcacaacatgggggatcatgtaactcgccttgatcgttgggaaccggagctgaatgaagccataccaaacgacgagcgtgacaccacgatgcctgtagcaatggcaacaacgttgcgcaaactattaactggcgaactacttactctagcttcccggcaacaattaatagactggatggaggcggataaagttgcaggaccacttctgcgctcggcccttccggctggctggtttattgctgataaatctggagccggtgagcgtgggtctcgcggtatcattgcagcactggggccagatggtaagccctcccgtatcgtagttatctacacgacggggagtcaggcaactatggatgaacgaaatagacagatcgctgagataggtgcctcactgattaagcattggtaactgtcagaccaagtttactcatatatactttagattgatttaaaacttcatttttaatttaaaaggatctaggtgaagatcctttttgataatctcatgaccaaaatcccttaacgtgagttttcgttccactgagcgtcagaccccgtagaaaagatcaaaggatcttcttgagatcctttttttctgcgcgtaatctgctgcttgcaaacaaaaaaaccaccgctaccagcggtggtttgtttgccggatcaagagctaccaactctttttccgaaggtaactggcttcagcagagcgcagataccaaatactgtccttctagtgtagccgtagttaggccaccacttcaagaactctgtagcaccgcctacatacctcgctctgctaatcctgttaccagtggctgctgccagtggcgataagtcgtgtcttaccgggttggactcaagacgatagttaccggataaggcgcagcggtcgggctgaacggggggttcgtgcacacagcccagcttggagcgaacgacctacaccgaactgagatacctacagcgtgagctatgagaaagcgccacgcttcccgaagggagaaaggcggacaggtatccggtaagcggcagggtcggaacaggagagcgcacgagggagcttccagggggaaacgcctggtatctttatagtcctgtcgggtttcgccacctctgacttgagcgtcgatttttgtgatgctcgtcaggggggcggagcctatggaaaaacgccagcaacgcggcctttttacggttcctggccttttgctggccttttgctcacatgttctttcctgcgttatcccctgattctgtggataaccgtattaccgcctttgagtgagctgataccgctcgccgcagccgaacgaccgagcgcagcgagtcagtgagcgaggaagcggaagagcgcccaatacgcaaaccgcctctccccgcgcgttggccgattcattaatgcagctggcacgacaggtttcccgactggaaagcgggcagtgagcgcaacgcaattaatgtgagttagctcactcattaggcaccccaggctttacactttatgcttccggctcgtatgttgtgtggaattgtgagcggataacaatttcacacaggaaacagctatgaccatgattacgccaagctcggaattaaccctcactaaagggaacaaaagctggagctctgcagcccatgcaacagaaactataaaaaatacagagaatgaaaagaaacagatagattttttagttctttaggcccgtagtctgcaaatccttttatgattttctatcaaacaaaagaggaaaatagaccagttgcaatccaaacgagagtctaatagaatgaggtcggatttctactattgtagatgtggcggtacgttgatgcatcgcgggccggcatggtcccagcctcctcgctggcgccggctgggcaacatgcttcggcatggcgaatgggactttttttttgcctggcggcagtagcgcggtggtcccacctgaccccatgccgaactcagaagtgaaacgccgtagcgccgatggtagtgtggggtctccccatgcgagagtagggaactgccaggcatcaaataaaacgaaaggctcagtcgaaagactgggcctttcgttttatggtacccaattcgccctatagtgagtcgtattacaattcactggccgtcgttttacaacgtcgtgactgggaaaaccctggcgttacccaacttaatcgccttgcagcacatccccctttcgccagctggcgtaatagcgaagaggcccgcaccgatcgcccttcccaacagttgcgcagcctgaaaggcaggccgggccgtggtggccacggcctctaggccagatccagcggcatctgggttagtcgagcgcgggccgcttcccatgtctcaccagggcgagcctgtttcgcgatctcagcatctgaaatcttcccggccttgcgcttcgctggggccttacccaccgccttggcgggcttcttcggtccaaaactgaacaacagatgtgtgaccttgcgcccggtctttcgctgcgcccactccacctgtagcgggctgtgctcgttgatctgcgtcacggctggatcaagcactcgcaacttgaagtccttgatcgagggataccggccttccagttgaaaccactttcgcagctggtcaatttctatttcgcgctggccgatgctgtcccattgcatgagcagctcgtaaagcctgatcgcgtgggtgctgtccatcttggccacgtcagccaaggcgtatttggtgaactgtttggtgagttccgtcaggtacggcagcatgtctttggtgaacctgagttctacacggccctcaccctcccggtagatgattgtttgcacccagccggtaatcatcacactcggtcttttccccttgccattgggctcttgggttaaccggacttcccgccgtttcaggcgcagggccgcttctttgagctggttgtaggaagattcgatagggacacccgccatcgtcgctatgtcctccgccgtcactgaatacatcacttcatcggtgacaggctcgctcctcttcacctggctaatacaggccagaacgatccgctgttcctgaacactgaggcgatacgcggcctcgaccagggcattgcttttgtaaaccattgggggtgaggccacgttcgacattccttgtgtataaggggacactgtatctgcgtcccacaatacaacaaatccgtccctttacaacaacaaatccgtcccttcttaacaacaaatccgtcccttaatggcaacaaatccgtccctttttaaactctacaggccacggattacgtggcctgtagacgtcctaaaaggtttaaaagggaaaaggaagaaaagggtggaaacgcaaaaaacgcaccactacgtggccccgttggggccgcatttgtgcccctgaaggggcgggggaggcgtctgggcaatccccgttttaccagtcccctatcgccgcctgagagggcgcaggaagcgagtaatcagggtatcgaggcggattcacccttggcgtccaaccagcggcaccagcggcgcctgagaggcctacagagcggttggacaccaaggggaggggctaagaccggtttatcagtcccctttccctcgtttctttccaacgcgatagcccagcaaggccgccaccgttgccaccgtcaccccagcaagcacagccagtggcgtgtaattggggtctgacgctcagtggaacgaaaactcacgttaagggattttggtcatgagattatcaaaaaggatcttcacctagatccttttaaattaaaaatgaagttttaaatcaatctaaagtatatatgagtaaacttggtctgacagttaccaatgcttaatcagtgaggcacctatctcagcgatctgtctatttcgttcatccatagttgcctgactccccgtcgtgtagataactacgatacgggagggcttaccatctggccccagtgctgcaatgataccgcgagatccacgctcaccggctccagatttatcagcaataaaccagccagccggaagggccgagcgcagaagtggtcctgcaactttatccgcctccatccagtctattaattgttgccgggaagctagagtaagtagttcgccagttaatagtttgcgcaacgttgttgccattgccgcctgatgcggtattttctccttacgcatctgtgcggtatttcacaccgcatatggtgcactctcagtacaatctgctctgatgccgcatagttaagccagccccgacacccgccaacacccgctgacgcgccctgacgggcttgtctgctcccggcatccgcttacagacaagctgtgaccgtctccgggagctgcatgtgtcagaggttttcaccgtcatcaccgaaacgcgcga

SEQ ID NO: 45 - DNA, 674 bp, Escherichia coli
  Nucleotide sequence of the pMB1 derived high copy replicon (pUC) for episomal vector propagation in E. coli
atgtgagcaaaaggccagcaaaaggccaggaaccgtaaaaaggccgcgttgctggcgtttttccataggctccgcccccctgacgagcatcacaaaaatcgacgctcaagtcagaggtggcgaaacccgacaggactataaagataccaggcgtttccccctggaagctccctcgtgcgctctcctgttccgaccctgccgcttaccggatacctgtccgcctttctcccttcgggaagcgtggcgctttctcatagctcacgctgtaggtatctcagttcggtgtaggtcgttcgctccaagctgggctgtgtgcacgaaccccccgttcagcccgaccgctgcgccttatccggtaactatcgtcttgagtccaacccggtaagacacgacttatcgccactggcagcagccactggtaacaggattagcagagcgaggtatgtaggcggtgctacagagttcttgaagtggtggcctaactacggctacactagaaggacagtatttggtatctgcgctctgctgaagccagttaccttcggaaaaagagttggtagctcttgatccggcaaacaaaccaccgctggtagcggtggtttttttgtttgcaagcagcagattacgcgcagaaaaaaaggatctcaagaagatcctttgatcttttctacggg

SEQ ID NO: 46 - DNA, 1884 bp, Pseudomonas
  Nucleotide sequence of the pRO1614 derived replicon region for episomal vector propagation in the genus Pseudomonas
gcaatggcaacaacgttgcgcaaactattaactggcgaactacttactctagcttcccggcaacaattaatagactggatggaggcggataaagttgcaggaccacttctgcgctcggcccttccggctggctggtttattgctgataaatctggagccggtgagcgtggatctcgcggtatcattgcagcactggggccagatggtaagccctcccgtatcgtagttatctacacgacggggagtcaggcaactatggatgaacgaaatagacagatcgctgagataggtgcctcactgattaagcattggtaactgtcagaccaagtttactcatatatactttagattgatttaaaacttcatttttaatttaaaaggatctaggtgaagatcctttttgataatctcatgaccaaaatcccttaacgtgagttttcgttccactgagcgtcagaccccaattacacgccactggctgtgcttgctggggtgacggtggcaacggtggcggccttgctgggctatcgcgttggaaagaaacgagggaaaggggactgataaaccggtcttagcccctccccttggtgtccaaccgctctgtaggcctctcaggcgccgctggtgccgctggttggacgccaagggtgaatccgcctcgataccctgattactcgcttcctgcgccctctcaggcggcgataggggactggtaaaacggggattgcccagacgcctcccccgccccttcaggggcacaaatgcggccccaacggggccacgtagtggtgcgttttttgcgtttccacccttttcttccttttcccttttaaaccttttaggacgtctacaggccacgtaatccgtggcctgtagagtttaaaaagggacggatttgttgccattaagggacggatttgttgttaagaagggacggatttgttgttgtaaagggacggatttgttgtattgtgggacgcagatacagtgtccccttatacacaaggaatgtcgaacgtggcctcacccccaatggtttacaaaagcaatgccctggtcgaggccgcgtatcgcctcagtgttcaggaacagcggatcgttctggcctgtattagccaggtgaagaggagcgagcctgtcaccgatgaagtgatgtattcagtgacggcggaggacatagcgacgatggcgggtgtccctatcgaatcttcctacaaccagctcaaagaagcggccctgcgcctgaaacggcgggaagtccggttaacccaagagcccaatggcaaggggaaaagaccgagtgtgatgattaccggctgggtgcaaacaatcatctaccgggagggtgagggccgtgtagaactcaggttcaccaaagacatgctgccgtacctgacggaactcaccaaacagttcaccaaatacgccttggctgacgtggccaagatggacagcacccacgcgatcaggctttacgagctgctcatgcaatgggacagcatcggccagcgcgaaatagaaattgaccagctgcgaaagtggtttcaactggaaggccggtatccctcgatcaaggacttcaagttgcgagtgcttgatccagccgtgacgcagatcaacgagcacagcccgctacaggtggagtgggcgcagcgaaagaccgggcgcaaggtcacacatctgttgttcagttttggaccgaagaagcccgccaaggcggtgggtaaggccccagcgaagcgcaaggccgggaagatttcagatgctgagatcgcgaaacaggctcgccctggtgagacatgggaagcggcccgcgctcgactaacccagatgccgctggatctggcctagaggccgtggccaccacggcccggcctgcctttc

SEQ ID NO: 47 - DNA, 570 bp, Streptomyces noursei
  Nucleotide sequence of the nourseothricin acetyltransferase gene (nat1)
atgaccactcttgacgacacggcttaccggtaccgcaccagtgtcccgggggacgccgaggccatcgaggcactggatgggtccttcaccaccgacaccgtcttccgcgtcaccgccaccggggacggcttcaccctgcgggaggtgccggtggacccgcccctgaccaaggtgttccccgacgacgaatcggacgacgaatcggacgccggggaggacggcgacccggactcccggacgttcgtcgcgtacggggacgacggcgacctggcgggcttcgtggtcgtctcgtactccggctggaaccgccggctgaccgtcgaggacatcgaggtcgccccggagcaccgggggcacggggtcgggcgcgcgttgatggggctcgcgacggagttcgcccgcgagcggggcgccgggcacctctggctggaggtcaccaacgtcaacgcaccggcgatccacgcgtaccggcggatggggttcaccctctgcggcctggacaccgccctgtacgacggcaccgcctcggacggcgagcaggcgctctacatgagcatgccctgcccctga

SEQ ID NO: 48 - DNA, 90 bp, Bacillus subtilis
  N-terminal 90 bps nucleotide coding sequence fragment of the veg protein gene from Bacillus subtilis
atggcgaagacgttgtccgatattaaaagatcgcttgatgggaatttaggtaaaaggctgacgttaaaagcaaacggtggccggatccat

SEQ ID NO: 49 - DNA, 660 bp, Artificial Sequence
  Nucleotide sequence of the veg-nat1 gene fusion
atggcgaagacgttgtccgatattaaaagatcgcttgatgggaatttaggtaaaaggctgacgttaaaagcaaacggtggccggatccatatgaccactcttgacgacacggcttaccggtaccgcaccagtgtcccgggggacgccgaggccatcgaggcactggatgggtccttcaccaccgacaccgtcttccgcgtcaccgccaccggggacggcttcaccctgcgggaggtgccggtggacccgcccctgaccaaggtgttccccgacgacgaatcggacgacgaatcggacgccggggaggacggcgacccggactcccggacgttcgtcgcgtacggggacgacggcgacctggcgggcttcgtggtcgtctcgtactccggctggaaccgccggctgaccgtcgaggacatcgaggtcgccccggagcaccgggggcacggggtcgggcgcgcgttgatggggctcgcgacggagttcgcccgcgagcggggcgccgggcacctctggctggaggtcaccaacgtcaacgcaccggcgatccacgcgtaccggcggatggggttcaccctctgcggcctggacaccgccctgtacgacggcaccgcctcggacggcgagcaggcgctctacatgagcatgccctgcccctga

SEQ ID NO: 50 - DNA, 822 bp, Bacillus subtilis
  Nucleotide sequence of the 5’-UTR region upstream to the veg-nat1 gene fusion, containing the Veg RNA polymerase II promoter from Bacillus subtilis
atgcgagccatttggacgggttcgatcgccttcgggctggtgaacgtgccggtcaaggtgtacagcgctaccgcagaccacgacatcaggttccaccaggtgcacgccaaggacaacggacgcatccggtacaagcgcgtctgcgaggcgtgtggcgaggtggtcgactaccgcgatcttgcccgggcctacgagtccggcgacggccaaatggtggcgatcaccgacgacgacatcgccagcttgcctgaagaacgcagccgggagatcgaggtgttggagttcgtccccgccgccgacgtggacccgatgatgttcgaccgcagctactttttggagcctgattcgaagtcgtcgaaatcgtatgtgctgctggctaagacactcgccgagaccgaccggatggcgatcgtgcatttcacgctgcgcaacaagaccaggctggcggcgttgcgcgtcaaggatttcggcaagcgagaggtgatgatggtgcacacgttgctgtggcccgatgagatccgcgaccccgacttcccggtgctggaccagaaggtggagatcaaacccgcggaactcaagatggccggccaggtggtggactcgatggccgacgacttcaatccggaccgctaccacgacacctaccaggagcagttacaggagctgatcgacaccaaactcgaaggtgggcaggcatttaccgccgaggaccaaccgaggttgctggacgagcccgaagacgtctccgacctgctcgccaagctggaggccagcgtgaaggcgcgctcgaaggccaactcaaacgtcccaacgcctccgtga

SEQ ID NO: 51 - DNA, 822 bp, Mycobacterium tuberculosis; identical to SEQ ID NO: 50
  Nucleotide sequence of the ku gene from Mycobacterium tuberculosis

SEQ ID NO: 52 - DNA, 2280 bp, Mycobacterium tuberculosis
  Nucleotide sequence of the ligD gene from Mycobacterium tuberculosis
atgggttcggcgtcggagcaacgggtgacgctgaccaacgccgacaaggtgctctatcccgccaccgggaccacaaagtccgatatcttcgactactacgccggtgttgccgaagtcatgctcggccacatcgcgggacggccggcgacgcgcaagcgctggcctaacggcgtcgaccaacccgcgttcttcgaaaagcagttggcgttgtcggcgccgccttggctgtcacgtgcaacggtggcgcaccggtccgggacgacgacctatccgatcatcgatagcgcaaccgggctggcctggatcgcccaacaggcggcgctggaggtgcacgtgccgcagtggcggtttgtcgccgagcccggatcaggtgagttaaatccgggcccggcaacgcgtttggtgttcgacctggacccgggcgaaggcgtgatgatggcccagctggccgaggtggcgcgcgcggttcgtgatcttctcgccgatatcgggttggtcaccttcccggtcaccagcggcagcaagggattgcatctgtacacaccgctggatgagccggtgagcagcaggggagccacggtgttggccaagcgcgtcgcgcagcgattggagcaggcgatgcccgcgttggtcacctcgaccatgaccaaaagcctgcgggccgggaaggtgtttgtggactggagccagaacagcggctcgaagaccaccatcgcgccgtactcactacgtggccggacgcatccgaccgtcgcggcgccacgcacctgggcggagctcgacgaccccgcactgcgtcagctctcctacgacgaggtgctgacccggattgcccgcgacggcgatctgctcgagcggctggatgccgacgctccggtagcggaccggttgacccgataccgccgcatgcgcgacgcatcgaaaactcccgagccgattcccacggcgaaacccgttaccggagacggcaatacgttcgtcatccaggagcatcacgcgcgtcggccgcactacgatttccggctggaatgcgacggcgtgctggtctcgtgggcggtaccgaaaaacctgcccgacaacacatcggttaaccatctagcgatacacaccgaggaccacccgctggaatacgccacgttcgagggcgcgattcccagcggggagtacggcgccggcaaggtgatcatctgggactccggcacttacgacaccgagaagttccacgatgacccgcacacgggggaggtcatcgtgaatctgcacggcggccggatctctgggcgttatgcgctgattcggaccaacggcgatcggtggctggcgcaccgcctaaagaatcagaaagaccagaaggtgttcgagttcgacaatctggccccaatgcttgccacgcacggcacggtggccggtctaaaggccagccagtgggcgttcgaaggcaagtgggacggctaccggttgctggttgaggctgaccacggcgccgtgcggctgcggtcccgcagcgggcgcgatgtcaccgccgagtatccgcaattgcgggcattggcggaggatctcgccgatcaccacgtggtgctggacggcgaggccgtcgtacttgactcctctggtgtgcccagcttcagccagatgcagaatcggggccgcgacacccgtgtcgagttctgggcgttcgacctgctctacctcgacggccgcgcgctgctaggcacccgctaccaagaccggcgtaagctgctcgaaaccctagctaacgcaaccagtctcaccgttcccgagctgctgcccggtgacggcgcccaagcgtttgcgtgctcgcgcaagcacggctgggagggcgtgatcgccaagaggcgtgactcgcgctatcagccgggccggcgctgcgcgtcgtgggtcaaggacaagcactggaacacccaggaagtcgtcattggtggctggcgcgccggggaaggcgggcgcagcagtggcgtcgggtcgctgctcatgggcatccccggtccaggtgggctgcagttcgccgggcgggtcggtaccggcctcagcgaacgcgaactggccaacctcaaggagatgctggcgccgctgcataccgacgagtcccccttcgacgtaccactgcccgcgcgtgacgccaagggcatcacatatgtcaagccggcgctggttgcagaggtgcgctacagcgagtggactccggagggccggctgcgtcaatcaagctggcgtgggctgcggccggacaagaaacccagtgaggtggtgcgcgaatga

SEQ ID NO: 53 - DNA, 176 bp, Bacillus subtilis
  Nucleotide sequence of the 5’-UTR region upstream to the ligD coding sequence, containing the Veg RNA polymerase II promoter from Bacillus subtilis
ctcatgtttgacagcttatcatcgaattataggaatagagcaaacaagcaaaggaaattttgtcaaaataattttattgacaacgtcttattaacgttgatataatttaaattttatttgacaaaaatgggctcgtgttgtacaataaatgtaactagttaaggaggtaataatat

SEQ ID NO: 54 - DNA, 47 bp, T7 bacteriophage
  Nucleotide sequence of the T7 transcription terminator
tagcataaccccttggggcctctaaacgggtcttgaggggttttttg

SEQ ID NO: 55 - DNA, 362 bp, Bacillus megaterium
  Nucleotide sequence of the 5’-UTR region upstream to the ku gene, containing the SacB RNA polymerase II promoter from Bacillus megaterium
cccatgcaacagaaactataaaaaatacagagaatgaaaagaaacagatagattttttagttctttaggcccgtagtctgcaaatccttttatgattttctatcaaacaaaagaggaaaatagaccagttgcaatccaaacgagagtctaatagaatgaggtcgaaaagtaaatcgcgcgggtttgttactgataaagcaggcaagacctaaaatgtgtaaagggcaaagtgtatactttggcgtcaccccttacatattttaggtctttttttattgtgcgtaactaacttgccatcttcaaacaggagggctggaagaagcagaccgctaacacagtacataaaaaaggagacatgaacg

SEQ ID NO: 56 - DNA, 8883 bp, Artificial Sequence
  Nucleotide sequence of the pUCP-SK-Pveg-LigD_PsacB-Ku NHEJ vector system
gcaatggcaacaacgttgcgcaaactattaactggcgaactacttactctagcttcccggcaacaattaatagactggatggaggcggataaagttgcaggaccacttctgcgctcggcccttccggctggctggtttattgctgataaatctggagccggtgagcgtggatctcgcggtatcattgcagcactggggccagatggtaagccctcccgtatcgtagttatctacacgacggggagtcaggcaactatggatgaacgaaatagacagatcgctgagataggtgcctcactgattaagcattggtaactgtcagaccaagtttactcatatatactttagattgatttaaaacttcatttttaatttaaaaggatctaggtgaagatcctttttgataatctcatgaccaaaatcccttaacgtgagttttcgttccactgagcgtcagaccccaattacacgccactggctgtgcttgctggggtgacggtggcaacggtggcggccttgctgggctatcgcgttggaaagaaacgagggaaaggggactgataaaccggtcttagcccctccccttggtgtccaaccgctctgtaggcctctcaggcgccgctggtgccgctggttggacgccaagggtgaatccgcctcgataccctgattactcgcttcctgcgccctctcaggcggcgataggggactggtaaaacggggattgcccagacgcctcccccgccccttcaggggcacaaatgcggccccaacggggccacgtagtggtgcgttttttgcgtttccacccttttcttccttttcccttttaaaccttttaggacgtctacaggccacgtaatccgtggcctgtagagtttaaaaagggacggatttgttgccattaagggacggatttgttgttaagaagggacggatttgttgttgtaaagggacggatttgttgtattgtgggacgcagatacagtgtccccttatacacaaggaatgtcgaacgtggcctcacccccaatggtttacaaaagcaatgccctggtcgaggccgcgtatcgcctcagtgttcaggaacagcggatcgttctggcctgtattagccaggtgaagaggagcgagcctgtcaccgatgaagtgatgtattcagtgacggcggaggacatagcgacgatggcgggtgtccctatcgaatcttcctacaaccagctcaaagaagcggccctgcgcctgaaacggcgggaagtccggttaacccaagagcccaatggcaaggggaaaagaccgagtgtgatgattaccggctgggtgcaaacaatcatctaccgggagggtgagggccgtgtagaactcaggttcaccaaagacatgctgccgtacctgacggaactcaccaaacagttcaccaaatacgccttggctgacgtggccaagatggacagcacccacgcgatcaggctttacgagctgctcatgcaatgggacagcatcggccagcgcgaaatagaaattgaccagctgcgaaagtggtttcaactggaaggccggtatccctcgatcaaggacttcaagttgcgagtgcttgatccagccgtgacgcagatcaacgagcacagcccgctacaggtggagtgggcgcagcgaaagaccgggcgcaaggtcacacatctgttgttcagttttggaccgaagaagcccgccaaggcggtgggtaaggccccagcgaagcgcaaggccgggaagatttcagatgctgagatcgcgaaacaggctcgccctggtgagacatgggaagcggcccgcgctcgactaacccagatgccgctggatctggcctagaggccgtggccaccacggcccggcctgcctttcaggctgcgcaactgttgggaagggcgatcggtgcgggcctcttcgctattacgccagctggcgaaagggggatgtgctgcaaggcgattaagttgggtaacgccagggttttcccagtcacgacgttgtaaaacgacggccagtgaattgtaatacgactcactatagggcgaattgggtaccgggccccccctcgaggtcgacggtatcgataagcttgatatcgaattctcatgtttgacagcttatcatcgaattataggaatagagcaaacaagcaaaggaaattttgtcaaaataattttattgacaacgtcttattaacgttgatataatttaaattttatttgacaaaaatgggctcgtgttgtacaataaatgtaactagttaaggaggtaataatatatgggttcggcgtcggagcaacgggtgacgctgaccaacgccgacaaggtgctctatcccgccaccgggaccacaaagtccgatatcttcgactactacgccggtgttgccgaagtcatgctcggccacatcgcgggacggccggcgacgcgcaagcgctggcctaacggcgtcgaccaacccgcgttcttcgaaaagcagttggcgttgtcggcgccgccttggctgtcacgtgcaacggtggcgcaccggtccgggacgacgacctatccgatcatcgatagcgcaaccgggctggcctggatcgcccaacaggcggcgctggaggtgcacgtgccgcagtggcggtttgtcgccgagcccggatcaggtgagttaaatccgggcccggcaacgcgtttggtgttcgacctggacccgggcgaaggcgtgatgatggcccagctggccgaggtggcgcgcgcggttcgtgatcttctcgccgatatcgggttggtcaccttcccggtcaccagcggcagcaagggattgcatctgtacacaccgctggatgagccggtgagcagcaggggagccacggtgttggccaagcgcgtcgcgcagcgattggagcaggcgatgcccgcgttggtcacctcgaccatgaccaaaagcctgcgggccgggaaggtgtttgtggactggagccagaacagcggctcgaagaccaccatcgcgccgtactcactacgtggccggacgcatccgaccgtcgcggcgccacgcacctgggcggagctcgacgaccccgcactgcgtcagctctcctacgacgaggtgctgacccggattgcccgcgacggcgatctgctcgagcggctggatgccgacgctccggtagcggaccggttgacccgataccgccgcatgcgcgacgcatcgaaaactcccgagccgattcccacggcgaaacccgttaccggagacggcaatacgttcgtcatccaggagcatcacgcgcgtcggccgcactacgatttccggctggaatgcgacggcgtgctggtctcgtgggcggtaccgaaaaacctgcccgacaacacatcggttaaccatctagcgatacacaccgaggaccacccgctggaatacgccacgttcgagggcgcgattcccagcggggagtacggcgccggcaaggtgatcatctgggactccggcacttacgacaccgagaagttccacgatgacccgcacacgggggaggtcatcgtgaatctgcacggcggccggatctctgggcgttatgcgctgattcggaccaacggcgatcggtggctggcgcaccgcctaaagaatcagaaagaccagaaggtgttcgagttcgacaatctggccccaatgcttgccacgcacggcacggtggccggtctaaaggccagccagtgggcgttcgaaggcaagtgggacggctaccggttgctggttgaggctgaccacggcgccgtgcggctgcggtcccgcagcgggcgcgatgtcaccgccgagtatccgcaattgcgggcattggcggaggatctcgccgatcaccacgtggtgctggacggcgaggccgtcgtacttgactcctctggtgtgcccagcttcagccagatgcagaatcggggccgcgacacccgtgtcgagttctgggcgttcgacctgctctacctcgacggccgcgcgctgctaggcacccgctaccaagaccggcgtaagctgctcgaaaccctagctaacgcaaccagtctcaccgttcccgagctgctgcccggtgacggcgcccaagcgtttgcgtgctcgcgcaagcacggctgggagggcgtgatcgccaagaggcgtgactcgcgctatcagccgggccggcgctgcgcgtcgtgggtcaaggacaagcactggaacacccaggaagtcgtcattggtggctggcgcgccggggaaggcgggcgcagcagtggcgtcgggtcgctgctcatgggcatccccggtccaggtgggctgcagttcgccgggcgggtcggtaccggcctcagcgaacgcgaactggccaacctcaaggagatgctggcgccgctgcataccgacgagtcccccttcgacgtaccactgcccgcgcgtgacgccaagggcatcacatatgtcaagccggcgctggttgcagaggtgcgctacagcgagtggactccggagggccggctgcgtcaatcaagctggcgtgggctgcggccggacaagaaacccagtgaggtggtgcgcgaatgataagttggctgctgccaccgctgagcaataactagcataaccccttggggcctctaaacgggtcttgaggggttttttgcccatgcaacagaaactataaaaaatacagagaatgaaaagaaacagatagattttttagttctttaggcccgtagtctgcaaatccttttatgattttctatcaaacaaaagaggaaaatagaccagttgcaatccaaacgagagtctaatagaatgaggtcgaaaagtaaatcgcgcgggtttgttactgataaagcaggcaagacctaaaatgtgtaaagggcaaagtgtatactttggcgtcaccccttacatattttaggtctttttttattgtgcgtaactaacttgccatcttcaaacaggagggctggaagaagcagaccgctaacacagtacataaaaaaggagacatgaacgatgcgagccatttggacgggttcgatcgccttcgggctggtgaacgtgccggtcaaggtgtacagcgctaccgcagaccacgacatcaggttccaccaggtgcacgccaaggacaacggacgcatccggtacaagcgcgtctgcgaggcgtgtggcgaggtggtcgactaccgcgatcttgcccgggcctacgagtccggcgacggccaaatggtggcgatcaccgacgacgacatcgccagcttgcctgaagaacgcagccgggagatcgaggtgttggagttcgtccccgccgccgacgtggacccgatgatgttcgaccgcagctactttttggagcctgattcgaagtcgtcgaaatcgtatgtgctgctggctaagacactcgccgagaccgaccggatggcgatcgtgcatttcacgctgcgcaacaagaccaggctggcggcgttgcgcgtcaaggatttcggcaagcgagaggtgatgatggtgcacacgttgctgtggcccgatgagatccgcgaccccgacttcccggtgctggaccagaaggtggagatcaaacccgcggaactcaagatggccggccaggtggtggactcgatggccgacgacttcaatccggaccgctaccacgacacctaccaggagcagttacaggagctgatcgacaccaaactcgaaggtgggcaggcatttaccgccgaggaccaaccgaggttgctggacgagcccgaagacgtctccgacctgctcgccaagctggaggccagcgtgaaggcgcgctcgaaggccaactcaaacgtcccaacgcctccgtgacgaaattcaaattgtgagcggcgaaattcaaattgtgagcggataacaatttgaattttctgtatgaggttttgctaaacaactttcaacagtttcagtggagtgagaatagaaaggaacaactaaaggaattgcgaataataattttttcacgttgaaaatctccaaaaaaaaaggctccaaaaggagcctttaattgtatcggtttatcagcttgctttcgaggtgaattttgaccctctagcgaaaatgcaagagcaaagacgaaaacatgccacacatgaggaataccgattctctcattaacatattcaggccagttatctgggcttaaaagcagaagtccaacccagataacgatcatatacatggttctctccagaggttcattactgaacactcgtccgagaataacgagtggatccactagttctagagcggccgccaccgcggtggagctccagcttttgttccctttagtgagggttaattccgagcttggcgtaatcatggtcatagctgtttcctgtgtgaaattgttatccgctcacaattccacacaacatacgagccggaagcataaagtgtaaagcctggggtgcctaatgagtgagctaactcacattaattgcgttgcgctcactgcccgctttccagtcgggaaacctgtcgtgccagctgcattaatgaatcggccaacgcgcggggagaggcggtttgcgtattgggcgctcttccgcttcctcgctcactgactcgctgcgctcggtcgttcggctgcggcgagcggtatcagctcactcaaaggcggtaatacggttatccacagaatcaggggataacgcaggaaagaacatgtgagcaaaaggccagcaaaaggccaggaaccgtaaaaaggccgcgttgctggcgtttttccataggctccgcccccctgacgagcatcacaaaaatcgacgctcaagtcagaggtggcgaaacccgacaggactataaagataccaggcgtttccccctggaagctccctcgtgcgctctcctgttccgaccctgccgcttaccggatacctgtccgcctttctcccttcgggaagcgtggcgctttctcatagctcacgctgtaggtatctcagttcggtgtaggtcgttcgctccaagctgggctgtgtgcacgaaccccccgttcagcccgaccgctgcgccttatccggtaactatcgtcttgagtccaacccggtaagacacgacttatcgccactggcagcagccactggtaacaggattagcagagcgaggtatgtaggcggtgctacagagttcttgaagtggtggcctaactacggctacactagaaggacagtatttggtatctgcgctctgctgaagccagttaccttcggaaaaagagttggtagctcttgatccggcaaacaaaccaccgctggtagcggtggtttttttgtttgcaagcagcagattacgcgcagaaaaaaaggatctcaagaagatcctttgatcttttctacggggtctgacgctcagtggaacgaaaactcacgttaagggattttggtcatgagattatcaaaaaggatcttcacctagatccttttaaattaaaaatgaagttttaaatcaatctaaagtatatatgagtaaacttggtctgacagttaccaatgcttaatcagtgaggcacctatctcagcgatctgtctatttcgttcatccatagttgcctgactccccgtcgtgtagataactacgatacgggagggcttaccatctggccccagtgctgcaatgataccgccggtcatttcgaaccccagagtcccgcccatggtcaggggcagggcatgctcatgtagagcgcctgctcgccgtccgaggcggtgccgtcgtacagggcggtgtccaggccgcagagggtgaaccccatccgccggtacgcgtggatcgccggtgcgttgacgttggtgacctccagccagaggtgcccggcgccccgctcgcgggcgaactccgtcgcgagccccatcaacgcgcgcccgaccccgtgcccccggtgctccggggcgacctcgatgtcctcgacggtcagccggcggttccagccggagtacgagacgaccacgaagcccgccaggtcgccgtcgtccccgtacgcgacgaacgtccgggagtccgggtcgccgtcctccccggcgtccgattcgtcgtccgattcgtcgtcggggaacaccttggtcaggggcgggtccaccggcacctcccgcagggtgaagccgtccccggtggcggtgacgcggaagacggtgtcggtggtgaaggacccatccagtgcctcgatggcctcggcgtcccccgggacactggtgcggtaccggtaagccgtgtcgtcaagagtggtcatatggatccggccaccgtttgcttttaacgtcagccttttacctaaattcccatcaagcgatcttttaatatcggacaacgtcttcgccattgcatccacctcactacatttattgtacaacacgagcccatttttgtcaaataaaatttaaattatatcaacgttaataagacgttgtcaataaaattattttgacaaaatttcctttgcttgtttgctctattcctataattcgatgataagctgtcaaacatgagagatcttgatcccctgcgccatcagatccttggcggcaagaaagccatccagtttactttgcagggcttcccaaccttaccagagggcgccccagctggcaattccggttcgcttgctgtccataaaaccgcccagtctagctatcgccatgtaagcccactgcaagctacctgctttctctttgcgcttgcgttttcccttgtccagatagcccagtagctgacattcatccggggtcagcaccgtttctgcggactggctttctacgtgttccgcttcctttagcagcccttgcgccctgagtgcttgcggcagcgtgaagtatgcggtgtgaaataccgcacagatgcgtaaggagaaaataccgcatcaggcg

SEQ ID NO: 57 - DNA, 9652 bp, Artificial Sequence
  CRISPR/BMC02-Ec vector system
caatcggcgttaaacccgccaccagatgggcattaaacgagtatcccggcagcaggggatcattttgcgcttcagccatacttttcatactcccgccattcagagaagaaaccaattgtccatattgcatcagacattgccgtcactgcgtcttttactggctcttctcgctaaccaaaccggtaaccccgcttattaaaagcattctgtaacaaagcgggaccaaagccatgacaaaaacgcgtaacaaaagtgtctataatcacggcagaaaagtccacattgattatttgcacggcgtcacactttgctatgccatagcatttttatccataagattagcggatcctacctgacgctttttatcgcaactctctactgtttctccatacccgttttttggtaccgggccccccctcgagtttattttaggaggcaaaaatgccgaaagaggattttgataaagcctgcatttatctgagcaacttcgataaattcagcacctattttgtgggctttaatcagaatcgcgaaaacctgtataccgatgaagaacaggcaaccgcaattccgtatcgtattatcaatgataacatggtgcgccactttgataactgccgtaaatttgagaagatcgtgaaaaagtatggcgacattagcaatgttctgagcacctataaagaatttttcgcaccggattgcttcaaaaacaaactgaatcagagccagatcgaccactataataacaccattggtcataccgcagatgatatttatggtgtgggtattaaccagatcctgagcaaatacaaacaggacaataaactgaatagcagcgatctgccgctgattagcaaactgtataaacaaattctgagcgacaccgaaagctatgccattgaaaattttgccgacgacaaaatgatgctgaacgccgttgataaagaatacagccgcattaaagaaaacgacgtgttcattaacatcgaaacctgcatgaatgaatacctgacactggaaaatagccacatgatctatctgaaaaatgatagcagcctgaccgacatcagtaataaactgtgggaagattgggcctttgtgaaaaatgccattcagaagtacagcaaagaaattctgtgtctgtccgacaaaaagatcgaggatatgctgaaaatgagccactatagcattagctttgttcagaacagcgtgtattattacgtggataactatatggaaagctgcgaggataaacgcaaaagcatcatcgattacatcaagaccttctatagcatcaaatacaacaacgtgtttagctgctataaagaggcagaagcagttctgcgtctggatagcattcataaaaatcgtcgtagtccggtggataaaaatggtattggtggtgaaggttttgcccagattgagaaaatcaaaaactttctggacagcatcctggaagtgaagaattttctgaatccgctgtatctgatcaaaagcggtaaaatggcagaaatcgaagataagagcgaagagttttataatcgcttcaacgagctgtataatagcctgagcgataccacctatctgtataacaaagtgcgtaactacctgaccaaaaagccgtacaagaaagaaaaattcaaaatgaactttgaaaacagcaccctgctgagcggttgggatgttaataaagaaaattgctccaacagcatcatcctgattcgcaatggtaaatactatctggggatcatcgataaacagtgcggcaatatgttcaacttcaaaatcgatgccgaagataacgagaaaaagcgcaaagaaaaagaagatctggcggaagatattctgagtgatggtagcgatagctactatgagaaaatggtgtataaactgctgccggatccgagcaaaatgctgccgaaagtgtttttcagcaacaagagcattgatttctatgcaccgagcgaggacattaaatacattcgtgaaaatggcctgttcaagaaagacgccaaaaataagaaagccctgtatatctggatcgaatttatgcagaacagcctgaaaaagcatccggaatggtccaactattttaactttaacttcaaaccgagcaccgagtatgcagatgttagcgaattctataaacaggttagcgatcagggttattccctgagctttgataagatcaaagatagctatatcgagagcaagatcaaaagtggtgaactgtttctgttcgagatctacaacaaagatttcagcccgtatagcaaaggtaatccgaacctgcataccatctattggaaatccatctttgacaaagagaacctgagcaacgttgtgattaaactgaacggtcaggccgaaatctttttccgtccggcaagcctgaaacgtaatgaagttgttgttcatcgtgcgaaagaaaacatcctgaataaaaacccgctgaacccgaagaaagaatccatgtttgaatacgacatcgtgaaagataaacgctacacccaggacaaattctttttccattgtccgattacgctgaactttaaaagcggcaatgttggcaaattcaacgacaaagttaaccagtttctgaagaataacccggatgtgaatgtgattggttttgatcgtggtgaacgtcatctgctgtattgtaatgtgctgaaccagaaaggcgaaatcattgaacagaaaagctttaacgtgatcgagaacaaaaacaacggcattacccagaaagtggattatcataatctgctggatcgtaaagagaaagaacgcgacgcaagccgtaaaagctggtcaacaattgaaaacatcaaagagctgaaagagggctatctgtcaaacgttgttcatgaaattagcgagctgatcatcaagtataatgcgattctggttcttgaggatctgaacttcgaatttaagaaaggtcgcttcaagatcgagaaacaggtgtatcagaaattcgaaaaagccctgattgacaagctgagctatatggtgtttaagaaagaagagagcaacaaaccgggtcatagcctgatggcatatcagctggcaagcccgtttgaaagcttccaaaaactgggtaaacagtgtggctttatcttctatgtgaacagcaactacaccagcaaaattgatccggttaccggttttgtgaatctgctgaagatcaaatatgagagcgtggacaaaagctgcaaattcatcaacgataagttcgatgatatccgctataatgccgatcgcgaatattttgagtttaccttcgataatggcaaatggaccgcatgtagtcatggtaaagaacgttatcgctataatcgcaacgacaagaaatacaactgtttcgacgttaccgaagaactgaaaagcctgtttaacaaatacgagatcgatttcaaagcaggcacggatattaagaaaagcatttgtcaggtgcaggacaagaactttcatagcgaactgctgtttaatctgagcctgattgttcagctgcgtcatacctataaaaacggcgatatcgagaaagactttattctgtcaccgattatggataaagaaaccggcaaatttttcgacagccgtgaatatgaaaatctggaaaacagcctgctgccgaccaatgcagatagcaatggtgcatataacattgcacgtaaaggtctgctgaccctgcgtcagatcgataaagatggtaaaccgtccaacatctccaataaagaatggtttgattttgtgcagaaataatggtctagaggtcgaaattcaaattgtgagcggataacaatttgaattttctgtatgaggttttgctaaacaactttcaacagtttcagtggagtgagaatagaaaggaacaactaaaggaattgcgaataataattttttcacgttgaaaatctccaaaaaaaaaggctccaaaaggagcctttaattgtatcggtttatcagcttgctttcgaggtgaattttgaccctctagcgaaaatgcaagagcaaagacgaaaacatgccacacatgaggaataccgattctctcattaacatattcaggccagttatctgggcttaaaagcagaagtccaacccagataacgatcatatacatggttctctccagaggttcattactgaacactcgtccgagaataacgagtggatcccctccaattcgccctatagtgagtcgtattacgcgcgctcactggccgtcgttttacaacgtcgtgactgggaaaaccctggcgttacccaacttaatcgccttgcagcacatccccctttcgccagctggcgtaatagcgaagaggcccgcaccgatcgcccttcccaacagttgcgcagcctgaatggcgaatggaaattgtaagcgttaatattttgttaaaattcgcgttaaatttttgttaaatcagctcattttttaaccaataggccgactgcgatgagtggcagggcggggcgtaatttttttaaggcagttattggtgcccttaaacgcctggtgctacgcctgaataagtgataataagcggatgaatggcagaaattcgaaagcaaattcgacccggtcgtcggttcagggcagggtcgttaaatagccgcttatgtctattgctggtttaccggtttattgactaccggaagcagtgtgaccgtgtgcttctcaaatgcctgaggccagtttgctcaggctctccccgtggaggtaataattgacgatatgatcatttattctgcctcccagagcctgataaaaacggtgaatccgttagcgaggtgccgccggcttccattcaggtcgaggtggcccggctccatgcaccgcgacgcaacgcggggaggcagacaaggtatagggcggcgaggcggctacagccgatagtctggaacagcgcacttacgggttgctgcgcaacccaagtgctaccggcgcggcagcgtgacccgtgtcggcggctccaacggctcgccatcgtccagaaaacacggctcatcgggcatcggcaggcgctgctgcccgcgccgttcccattcctccgtttcggtcaaggctggcaggtctggttccatgcccggaatgccgggctggctgggcggctcctcgccggggccggtcggtagttgctgctcgcccggatacagggtcgggatgcggcgcaggtcgccatgccccaacagcgattcgtcctggtcgtcgtgatcaaccaccacggcggcactgaacaccgacaggcgcaactggtcgcggggctggccccacgccacgcggtcattgaccacgtaggccgacacggtgccggggccgttgagcttcacgacggagatccagcgctcggccaccaagtccttgactgcgtattggaccgtccgcaaagaacgtccgatgagcttggaaagtgtcttttggctgaccaccacggcgttctggtggcccatctgcgccacgaggtgatgcagcagcattgccgccgtgggtttcctcgcaataagcccggcccacgcctcatgcgctttgcgttccgtttgcacccagtgaccgggcttgttcttggcttgaatgccgatttctctggactgcgtggccatgcttatctccatgcggtagggtgccgcacggttgcggcaccatgcgcaatcagctgcaacttttcggcagcgcgacaacaattatgcgttgcgtaaaagtggcagtcaattacagattttctttaacctacgcaatgagctattgcggggggtgccgcaatgagctgttgcgtaccccccttttttaagttgttgatttttaagtctttcgcatttcgccctatatctagttctttggtgcccaaagaagggcacccctgcggggttcccccacgccttcggcgcggctccccctccggcaaaaagtggcccctccggggcttgttgatcgactgcgcggccttcggccttgcccaaggtggcgctgcccccttggaacccccgcactcgccgccgtgaggctcggggggcaggcgggcgggcttcgccttcgactgcccccactcgcataggcttgggtcgttccaggcgcgtcaaggccaagccgctgcgcggtcgctgcgcgagccttgacccgccttccacttggtgtccaaccggcaagcgaagcgcgcaggccgcaggccggaggcttttccccagagaaaattaaaaaaattgatggggcaaggccgcaggccgcgcagttggagccggtgggtatgtggtcgaaggctgggtagccggtgggcaatccctgtggtcaagctcgtgggcaggcgcagcctgtccatcagcttgtccagcagggttgtccacgggccgagcgaagcgagccagccggtggccgctcgcggccatcgtccacatatccacgggctggcaagggagcgcagcgaccgcgcagggcgaagcccggagagcaagcccgtagggcgccgcagccgccgtaggcggtcacgactttgcgaagcaaagtctagtgagtatactcaagcattgagtggcccgccggaggcaccgccttgcgctgcccccgtcgagccggttggacaccaaaagggaggggcaggcatggcggcatacgcgatcatgcgatgcaagaagctggcgaaaatgggcaacgtggcggccagtctcaagcacgcctaccgcgagcgcgagacgcccaacgctgacgccagcaggacgccagagaacgagcactgggcggccagcagcaccgatgaagcgatgggccgactgcgcgagttgctgccagagaagcggcgcaaggacgctgtgttggcggtcgagtacgtcatgacggccagcccggaatggtggaagtcggccagccaagaacagcaggcggcgttcttcgagaaggcgcacaagtggctggcggacaagtacggggcggatcgcatcgtgacggccagcatccaccgtgacgaaaccagcccgcacatgaccgcgttcgtggtgccgctgacgcaggacggcaggctgtcggccaaggagttcatcggcaacaaagcgcagatgacccgcgaccagaccacgtttgcggccgctgtggccgatctagggctgcaacggggcatcgagggcagcaaggcacgtcacacgcgcattcaggcgttctacgaggccctggagcggccaccagtgggccacgtcaccatcagcccgcaagcggtcgagccacgcgcctatgcaccgcagggattggccgaaaagctgggaatctcaaagcgcgttgagacgccggaagccgtggccgaccggctgacaaaagcggttcggcaggggtatgagcctgccctacaggccgccgcaggagcgcgtgagatgcgcaagaaggccgatcaagcccaagagacggcccgagaccttcgggagcgcctgaagcccgttctggacgccctggggccgttgaatcgggatatgcaggccaaggccgccgcgatcatcaaggccgtgggcgaaaagctgctgacggaacagcgggaagtccagcgccagaaacaggcccagcgccagcaggaacgcgggcgcgcacatttccccgaaaagtgccacctgaaccccagagtcccgctcagaagaactcgtcaagaaggcgatagaaggcgatgcgctgcgaatcgggagcggcgataccgtaaagcacgaggaagcggtcagcccattcgccgccaagctcttcagcaatatcacgggtagccaacgctatgtcctgatagcggtccgccacacccagccggccacagtcgatgaatccagaaaagcggccattttccaccatgatattcggcaagcaggcatcgccatgggtcacgacgagatcctcgccgtcgggcatccgcgccttgagcctggcgaacagttcggctggcgcgagcccctgatgctcttcgtccagatcatcctgatcgacaagaccggcttccatccgagtacgtgctcgctcgatgcgatgtttcgcttggtggtcgaatgggcaggtagccggatcaagcgtatgcagccgccgcattgcatcagccatgatggatactttctcggcaggagcaaggtgagatgacaggagatcctgccccggcacttcgcccaatagcagccagtcccttcccgcttcagtgacaacgtcgagcacagctgcgcaaggaacgcccgtcgtggccagccacgatagccgcgctgcctcgtcttggagttcattcagggcaccggacaggtcggtcttgacaaaaagaaccgggcgcccctgcgctgacagccggaacacggcggcatcagagcagccgattgtctgttgtgcccagtcatagccgaatagcctctccacccaagcggccggagaacctgcgtgcaatccatcttgttcaatcatgcgaaacgatcctcatcctgtctcttgatcagatcttgatcccctgcgccatcagatccttggcggcaagaaagccatccagtttactttgcagggcttcccaaccttaccagagggcgccccagctggcaattccggttcgcttgctgtccataaaaccgcccagtctagctatcgccatgtaagcccactgcaagctacctgctttctctttgcgcttgcgttttcccttgtccagatagcccagtagctgacattcatccggggtcagcaccgtttctgcggactggctttctacgtgttccgcttcctttagcagcccttgcgccctgagtgcttgcggcagcgtgaagctagctgcataatgtgcctgtcaaatggacgaagcagggattctgcaaaccctatgctactccgtcaagccgtcaattgtctgattcgttaccaattatgacaacttgacggctacatcattcactttttcttcacaaccggcacggaactcgctcgggctggccccggtgcattttttaaatacccgcgagaaatagagttgatcgtcaaaaccaacattgcgaccgacggtggcgataggcatccgggtggtgctcaaaagcagcttcgcctggctgatacgttggtcctcgcgccagcttaagacgctaatccctaactgctggcggaaaagatgtgacagacgcgacggcgacaagcaaacatgctgtgcgacgctggcgatatcaaaattgctgtctgccaggtgatcgctgatgtactgacaagcctcgcgtacccgattatccatcggtggatggagcgactcgttaatcgcttccatgcgccgcagtaacaattgctcaagcagatttatcgccagcagctccgaatagcgcccttccccttgcccggcgttaatgatttgcccaaacaggtcgctgaaatgcggctggtgcgcttcatccgggcgaaagaaccccgtattggcaaatattgacggccagttaagccattcatgccagtaggcgcgcggacgaaagtaaacccactggtgataccattcgcgagcctccggatgacgaccgtagtgatgaatctctcctggcgggaacagcaaaatatcacccggtcggcaaacaaattctcgtccctgatttttcaccaccccctgaccgcgaatggtgagattgagaatataacctttcattcccagcggtcggtcgataaaaaaatcgagataaccgttggcct

SEQ ID NO: 58 - DNA, 10021 bp, Artificial Sequence
  CRISPR/BMC05-Ec vector system
caatcggcgttaaacccgccaccagatgggcattaaacgagtatcccggcagcaggggatcattttgcgcttcagccatacttttcatactcccgccattcagagaagaaaccaattgtccatattgcatcagacattgccgtcactgcgtcttttactggctcttctcgctaaccaaaccggtaaccccgcttattaaaagcattctgtaacaaagcgggaccaaagccatgacaaaaacgcgtaacaaaagtgtctataatcacggcagaaaagtccacattgattatttgcacggcgtcacactttgctatgccatagcatttttatccataagattagcggatcctacctgacgctttttatcgcaactctctactgtttctccatacccgttttttggtaccgggccccccctcgagtttattttaggaggcaaaaatgcgctgggatgaaaaactgcagacctttctgaatgatcaagaaatcgaagatgcctaccaggttctgaaaccggtgtttgataaactgcacgaaaactttattatcggcagcctggaaaataccaacaacaaaaagctgttcagcttcgacaaatacctgaaactgaaaaacgatctgctgcacgtgaataagaaagaacaagagagcgactacaaaaagaaagagaaagaatttgaaaccgagggtaaactgctgcgtaatacctttgcaaccgtttggattaatgagggcaaaaacttcaagaacaccattgttggtggtgaaaacgatcgcgaaattctgaaagaaggtggctataaaatcctgaccgaagcaggtattctgaaatatatcaagatgaacatcgataaatttgtggaactgaagctgaaaacccgtgaagatattctgtggaagaaagaaaatcgcaacctggttgaaatggcagatctggaaaaatcactgggcaccattgaaagctggggtgtttttgaaggtttcttcacctatttcagcggctttaatcagaaccgcgaaaactattatagcaccgatgaaaaagcaaccgcagttgcaagccgtgttattgatgaaaatctgccgaaatttagcgacaacgtgctggaattcaataaaaagaacgatgtgtacatcggcatctttagctttctgaaaggcaaaaacattgtgctgaaaggtaaaagcggtaatggtgaagaacaggacctgctgccgattaccgaaaagatttttgaaatcgagtactttaaaaactgcctgagcgaaggtgaaatcgaacgttataatagcgatattggcaacgccaactttctgatcaatctgtataaccagcagcaggacaagaaagaaaacaaactgcgtatcttcaagaccctgtataaacaaattggctgcggtatcaaaggcgattttattcagctgatcaaaaccgatgatgagctgaagaagatctttgaggatctgaaaattaccggtgacaacttctttaagaatacccagaacctgaaagagattatcctgtcgctggaaaacttcagcggtatttattggagcgataaagcactgaataccgtgagcggtaaatactttgcaaattgggcaagcctgaaagaactgctgaaaaatgccaaaatctttaagaaagaaaaagacgagatcaaaatcccgcagaccattgaactgagcgacctgtttggtgttctggatagcaatgaactgatcttcaaagaaagcttcaacgagaacgacgagctgaaacaaatcatcctgaaaagctatgagaaaaacagcatcaagctgctgaagatgattttcgtggatgttgaagagaaccagaaaatctttggcaatctgaaagatggtctgccgatcaacgatttcaagaaagatgaaaacacccagatcatcaaaacctggctggatggcctgctgaataccaatcagatcctgaaatacttcaaagtgcgcgagagcaaaatcaaaggtgcaccgctgaatccggaagttagcgaacgtctgaataagattctgaatgttgaaaatccgaccgtgatctatgatgtggttcgtaattatctgaccaaaaagccgaccgaaggcctgaataaactgaaacttaattttgataatgccgtgctggcagccggttgggatgttaataaagaaagcgaacgtggttgcctgattctgaaggatggtgataataagaaatatctggccatcctgaccaacaagacccagaaatttttcggtgagaaggtgaagtacaaagaattcgtgggtgatgaaaactggcagaaaatggattataaactgttaccgggtccgaataagatgctgccgaaagttctgctgcctaaaagcgatcgttacaaatttggtgccacagacgaaatcctgaagatttataacgaaggcggtttcaagaagaacgaaccgacctttaccaaagcaaaactggccaaaattgtggactttttcaaagacggcctgaaaaattacccgagcgcaaaaagcagctggtataacctgtttgcatttgattttagcgataccgagaaatacgaaagcatcgatcgtttctataccgaggttgaaaaacagggctataaactgagctggtcagccattagcaaaaatttcatcttcgaaaaagtggacgcaggcgatatgtacctgtttgaaattcgcaacaaagataacaacctgaagaacggtaaagcaaaaaccggtgccaaaaatctgcataccatttattggggtacgatctttggtgaaagcgagaacaaaccgaaactgaatggcgaagcagaaatcttttatcgtccggttgttaaagacctgatcaaagacaaggataaaaacggcgatattatcaaagccagcgaaaaacgctttgagcaagaaaaatttgtgtttcattgcccgatcacgctgaacttttgtctgaaaagcacacgcctgaatgatgtgattaaccagattatgatcgagaataaaaaggatgtgtgctttattggcattgaccgtggcgaaaaacatctggcatattatagcgttgtgaatcagaaaggggaaattctggaacagggtagctttaatgaaattaacggtcagaactacgccaagaaactggaagagaaagcaggtcatcgtgatgaagcacgtaaaaactggaaaaccattggcacgatcaaagaactgaagaatggttatattagccaggtggttcgtcgtattgttgatctggcagtgaaatataacgcctacattgttctggaagatctgaatagcggttttaaacgtggtcgtcagaaaattgagaaaagcgtgtatcagaaattagaactggcactggctaaaaagctgaatttcctggttgacaaaagcaagaaagacggtgaaattggtagcgtgcagaaagcactgcagctgacccctccggcaaccaattttgcagatattgaaaaagcgaaacagtttggcatcatgctgtatgttcgtgcgaattacaccagccagaccgatccggttaccggttggcgtaaaaccatttactttaaatcaaccacgcaagagaacttaaagaaagaaatctgcgagaaattctccgagatcggctttgatggtaacgattattacttcgagtataaggatgaaaacgccgagaagaaatggaccatgtatagcggtgttagcggtaaaagcctggatcgctttcgtggtaagaaagatacccatggtatttggaaagtggaaaagcaggatattgtcgagctgttaaagaagattttcggtcagcagaccagcgttgttggtgacctgaaaaccaaaattaccaacgataatgtgaacgatctgaaatacaccatcgatctgattcagcagattcgcaatacgggttttaacgagatcgataacgactttattctgagtccggttcgtgatgagaaaggcaatcattttgatagccgtaaagatggtgcaattctgagcaatggtgatgcaaatggtgcatataacattgcccgtaaaggtgtgctggcatttgaacgtattaatgcaaaaccggaaaagcccgaactgtatattgccgatgttgaatgggataaatggctgcagagcaaataatggtctagaggtcgaaattcaaattgtgagcggataacaatttgaattttctgtatgaggttttgctaaacaactttcaacagtttcagtggagtgagaatagaaaggaacaactaaaggaattgcgaataataattttttcacgttgaaaatctccaaaaaaaaaggctccaaaaggagcctttaattgtatcggtttatcagcttgctttcgaggtgaattttgaccctctagcgaaaatgcaagagcaaagacgaaaacatgccacacatgaggaataccgattctctcattaacatattcaggccagttatctgggcttaaaagcagaagtccaacccagataacgatcatatacatggttctctccagaggttcattactgaacactcgtccgagaataacgagtggatcccctccaattcgccctatagtgagtcgtattacgcgcgctcactggccgtcgttttacaacgtcgtgactgggaaaaccctggcgttacccaacttaatcgccttgcagcacatccccctttcgccagctggcgtaatagcgaagaggcccgcaccgatcgcccttcccaacagttgcgcagcctgaatggcgaatggaaattgtaagcgttaatattttgttaaaattcgcgttaaatttttgttaaatcagctcattttttaaccaataggccgactgcgatgagtggcagggcggggcgtaatttttttaaggcagttattggtgcccttaaacgcctggtgctacgcctgaataagtgataataagcggatgaatggcagaaattcgaaagcaaattcgacccggtcgtcggttcagggcagggtcgttaaatagccgcttatgtctattgctggtttaccggtttattgactaccggaagcagtgtgaccgtgtgcttctcaaatgcctgaggccagtttgctcaggctctccccgtggaggtaataattgacgatatgatcatttattctgcctcccagagcctgataaaaacggtgaatccgttagcgaggtgccgccggcttccattcaggtcgaggtggcccggctccatgcaccgcgacgcaacgcggggaggcagacaaggtatagggcggcgaggcggctacagccgatagtctggaacagcgcacttacgggttgctgcgcaacccaagtgctaccggcgcggcagcgtgacccgtgtcggcggctccaacggctcgccatcgtccagaaaacacggctcatcgggcatcggcaggcgctgctgcccgcgccgttcccattcctccgtttcggtcaaggctggcaggtctggttccatgcccggaatgccgggctggctgggcggctcctcgccggggccggtcggtagttgctgctcgcccggatacagggtcgggatgcggcgcaggtcgccatgccccaacagcgattcgtcctggtcgtcgtgatcaaccaccacggcggcactgaacaccgacaggcgcaactggtcgcggggctggccccacgccacgcggtcattgaccacgtaggccgacacggtgccggggccgttgagcttcacgacggagatccagcgctcggccaccaagtccttgactgcgtattggaccgtccgcaaagaacgtccgatgagcttggaaagtgtcttttggctgaccaccacggcgttctggtggcccatctgcgccacgaggtgatgcagcagcattgccgccgtgggtttcctcgcaataagcccggcccacgcctcatgcgctttgcgttccgtttgcacccagtgaccgggcttgttcttggcttgaatgccgatttctctggactgcgtggccatgcttatctccatgcggtagggtgccgcacggttgcggcaccatgcgcaatcagctgcaacttttcggcagcgcgacaacaattatgcgttgcgtaaaagtggcagtcaattacagattttctttaacctacgcaatgagctattgcggggggtgccgcaatgagctgttgcgtaccccccttttttaagttgttgatttttaagtctttcgcatttcgccctatatctagttctttggtgcccaaagaagggcacccctgcggggttcccccacgccttcggcgcggctccccctccggcaaaaagtggcccctccggggcttgttgatcgactgcgcggccttcggccttgcccaaggtggcgctgcccccttggaacccccgcactcgccgccgtgaggctcggggggcaggcgggcgggcttcgccttcgactgcccccactcgcataggcttgggtcgttccaggcgcgtcaaggccaagccgctgcgcggtcgctgcgcgagccttgacccgccttccacttggtgtccaaccggcaagcgaagcgcgcaggccgcaggccggaggcttttccccagagaaaattaaaaaaattgatggggcaaggccgcaggccgcgcagttggagccggtgggtatgtggtcgaaggctgggtagccggtgggcaatccctgtggtcaagctcgtgggcaggcgcagcctgtccatcagcttgtccagcagggttgtccacgggccgagcgaagcgagccagccggtggccgctcgcggccatcgtccacatatccacgggctggcaagggagcgcagcgaccgcgcagggcgaagcccggagagcaagcccgtagggcgccgcagccgccgtaggcggtcacgactttgcgaagcaaagtctagtgagtatactcaagcattgagtggcccgccggaggcaccgccttgcgctgcccccgtcgagccggttggacaccaaaagggaggggcaggcatggcggcatacgcgatcatgcgatgcaagaagctggcgaaaatgggcaacgtggcggccagtctcaagcacgcctaccgcgagcgcgagacgcccaacgctgacgccagcaggacgccagagaacgagcactgggcggccagcagcaccgatgaagcgatgggccgactgcgcgagttgctgccagagaagcggcgcaaggacgctgtgttggcggtcgagtacgtcatgacggccagcccggaatggtggaagtcggccagccaagaacagcaggcggcgttcttcgagaaggcgcacaagtggctggcggacaagtacggggcggatcgcatcgtgacggccagcatccaccgtgacgaaaccagcccgcacatgaccgcgttcgtggtgccgctgacgcaggacggcaggctgtcggccaaggagttcatcggcaacaaagcgcagatgacccgcgaccagaccacgtttgcggccgctgtggccgatctagggctgcaacggggcatcgagggcagcaaggcacgtcacacgcgcattcaggcgttctacgaggccctggagcggccaccagtgggccacgtcaccatcagcccgcaagcggtcgagccacgcgcctatgcaccgcagggattggccgaaaagctgggaatctcaaagcgcgttgagacgccggaagccgtggccgaccggctgacaaaagcggttcggcaggggtatgagcctgccctacaggccgccgcaggagcgcgtgagatgcgcaagaaggccgatcaagcccaagagacggcccgagaccttcgggagcgcctgaagcccgttctggacgccctggggccgttgaatcgggatatgcaggccaaggccgccgcgatcatcaaggccgtgggcgaaaagctgctgacggaacagcgggaagtccagcgccagaaacaggcccagcgccagcaggaacgcgggcgcgcacatttccccgaaaagtgccacctgaaccccagagtcccgctcagaagaactcgtcaagaaggcgatagaaggcgatgcgctgcgaatcgggagcggcgataccgtaaagcacgaggaagcggtcagcccattcgccgccaagctcttcagcaatatcacgggtagccaacgctatgtcctgatagcggtccgccacacccagccggccacagtcgatgaatccagaaaagcggccattttccaccatgatattcggcaagcaggcatcgccatgggtcacgacgagatcctcgccgtcgggcatccgcgccttgagcctggcgaacagttcggctggcgcgagcccctgatgctcttcgtccagatcatcctgatcgacaagaccggcttccatccgagtacgtgctcgctcgatgcgatgtttcgcttggtggtcgaatgggcaggtagccggatcaagcgtatgcagccgccgcattgcatcagccatgatggatactttctcggcaggagcaaggtgagatgacaggagatcctgccccggcacttcgcccaatagcagccagtcccttcccgcttcagtgacaacgtcgagcacagctgcgcaaggaacgcccgtcgtggccagccacgatagccgcgctgcctcgtcttggagttcattcagggcaccggacaggtcggtcttgacaaaaagaaccgggcgcccctgcgctgacagccggaacacggcggcatcagagcagccgattgtctgttgtgcccagtcatagccgaatagcctctccacccaagcggccggagaacctgcgtgcaatccatcttgttcaatcatgcgaaacgatcctcatcctgtctcttgatcagatcttgatcccctgcgccatcagatccttggcggcaagaaagccatccagtttactttgcagggcttcccaaccttaccagagggcgccccagctggcaattccggttcgcttgctgtccataaaaccgcccagtctagctatcgccatgtaagcccactgcaagctacctgctttctctttgcgcttgcgttttcccttgtccagatagcccagtagctgacattcatccggggtcagcaccgtttctgcggactggctttctacgtgttccgcttcctttagcagcccttgcgccctgagtgcttgcggcagcgtgaagctagctgcataatgtgcctgtcaaatggacgaagcagggattctgcaaaccctatgctactccgtcaagccgtcaattgtctgattcgttaccaattatgacaacttgacggctacatcattcactttttcttcacaaccggcacggaactcgctcgggctggccccggtgcattttttaaatacccgcgagaaatagagttgatcgtcaaaaccaacattgcgaccgacggtggcgataggcatccgggtggtgctcaaaagcagcttcgcctggctgatacgttggtcctcgcgccagcttaagacgctaatccctaactgctggcggaaaagatgtgacagacgcgacggcgacaagcaaacatgctgtgcgacgctggcgatatcaaaattgctgtctgccaggtgatcgctgatgtactgacaagcctcgcgtacccgattatccatcggtggatggagcgactcgttaatcgcttccatgcgccgcagtaacaattgctcaagcagatttatcgccagcagctccgaatagcgcccttccccttgcccggcgttaatgatttgcccaaacaggtcgctgaaatgcggctggtgcgcttcatccgggcgaaagaaccccgtattggcaaatattgacggccagttaagccattcatgccagtaggcgcgcggacgaaagtaaacccactggtgataccattcgcgagcctccggatgacgaccgtagtgatgaatctctcctggcgggaacagcaaaatatcacccggtcggcaaacaaattctcgtccctgatttttcaccaccccctgaccgcgaatggtgagattgagaatataacctttcattcccagcggtcggtcgataaaaaaatcgagataaccgttggcct

SEQ ID NO: 59 - DNA, 10153 bp, Artificial Sequence
  CRISPR/BMC07-Ec vector system
ccatgcttatctccatgcggtagggtgccgcacggttgcggcaccatgcgcaatcagctgcaacttttcggcagcgcgacaacaattatgcgttgcgtaaaagtggcagtcaattacagattttctttaacctacgcaatgagctattgcggggggtgccgcaatgagctgttgcgtaccccccttttttaagttgttgatttttaagtctttcgcatttcgccctatatctagttctttggtgcccaaagaagggcacccctgcggggttcccccacgccttcggcgcggctccccctccggcaaaaagtggcccctccggggcttgttgatcgactgcgcggccttcggccttgcccaaggtggcgctgcccccttggaacccccgcactcgccgccgtgaggctcggggggcaggcgggcgggcttcgccttcgactgcccccactcgcataggcttgggtcgttccaggcgcgtcaaggccaagccgctgcgcggtcgctgcgcgagccttgacccgccttccacttggtgtccaaccggcaagcgaagcgcgcaggccgcaggccggaggcttttccccagagaaaattaaaaaaattgatggggcaaggccgcaggccgcgcagttggagccggtgggtatgtggtcgaaggctgggtagccggtgggcaatccctgtggtcaagctcgtgggcaggcgcagcctgtccatcagcttgtccagcagggttgtccacgggccgagcgaagcgagccagccggtggccgctcgcggccatcgtccacatatccacgggctggcaagggagcgcagcgaccgcgcagggcgaagcccggagagcaagcccgtagggcgccgcagccgccgtaggcggtcacgactttgcgaagcaaagtctagtgagtatactcaagcattgagtggcccgccggaggcaccgccttgcgctgcccccgtcgagccggttggacaccaaaagggaggggcaggcatggcggcatacgcgatcatgcgatgcaagaagctggcgaaaatgggcaacgtggcggccagtctcaagcacgcctaccgcgagcgcgagacgcccaacgctgacgccagcaggacgccagagaacgagcactgggcggccagcagcaccgatgaagcgatgggccgactgcgcgagttgctgccagagaagcggcgcaaggacgctgtgttggcggtcgagtacgtcatgacggccagcccggaatggtggaagtcggccagccaagaacagcaggcggcgttcttcgagaaggcgcacaagtggctggcggacaagtacggggcggatcgcatcgtgacggccagcatccaccgtgacgaaaccagcccgcacatgaccgcgttcgtggtgccgctgacgcaggacggcaggctgtcggccaaggagttcatcggcaacaaagcgcagatgacccgcgaccagaccacgtttgcggccgctgtggccgatctagggctgcaacggggcatcgagggcagcaaggcacgtcacacgcgcattcaggcgttctacgaggccctggagcggccaccagtgggccacgtcaccatcagcccgcaagcggtcgagccacgcgcctatgcaccgcagggattggccgaaaagctgggaatctcaaagcgcgttgagacgccggaagccgtggccgaccggctgacaaaagcggttcggcaggggtatgagcctgccctacaggccgccgcaggagcgcgtgagatgcgcaagaaggccgatcaagcccaagagacggcccgagaccttcgggagcgcctgaagcccgttctggacgccctggggccgttgaatcgggatatgcaggccaaggccgccgcgatcatcaaggccgtgggcgaaaagctgctgacggaacagcgggaagtccagcgccagaaacaggcccagcgccagcaggaacgcgggcgcgcacatttccccgaaaagtgccacctgaaccccagagtcccgctcagaagaactcgtcaagaaggcgatagaaggcgatgcgctgcgaatcgggagcggcgataccgtaaagcacgaggaagcggtcagcccattcgccgccaagctcttcagcaatatcacgggtagccaacgctatgtcctgatagcggtccgccacacccagccggccacagtcgatgaatccagaaaagcggccattttccaccatgatattcggcaagcaggcatcgccatgggtcacgacgagatcctcgccgtcgggcatccgcgccttgagcctggcgaacagttcggctggcgcgagcccctgatgctcttcgtccagatcatcctgatcgacaagaccggcttccatccgagtacgtgctcgctcgatgcgatgtttcgcttggtggtcgaatgggcaggtagccggatcaagcgtatgcagccgccgcattgcatcagccatgatggatactttctcggcaggagcaaggtgagatgacaggagatcctgccccggcacttcgcccaatagcagccagtcccttcccgcttcagtgacaacgtcgagcacagctgcgcaaggaacgcccgtcgtggccagccacgatagccgcgctgcctcgtcttggagttcattcagggcaccggacaggtcggtcttgacaaaaagaaccgggcgcccctgcgctgacagccggaacacggcggcatcagagcagccgattgtctgttgtgcccagtcatagccgaatagcctctccacccaagcggccggagaacctgcgtgcaatccatcttgttcaatcatgcgaaacgatcctcatcctgtctcttgatcagatcttgatcccctgcgccatcagatccttggcggcaagaaagccatccagtttactttgcagggcttcccaaccttaccagagggcgccccagctggcaattccggttcgcttgctgtccataaaaccgcccagtctagctatcgccatgtaagcccactgcaagctacctgctttctctttgcgcttgcgttttcccttgtccagatagcccagtagctgacattcatccggggtcagcaccgtttctgcggactggctttctacgtgttccgcttcctttagcagcccttgcgccctgagtgcttgcggcagcgtgaagctagctgcataatgtgcctgtcaaatggacgaagcagggattctgcaaaccctatgctactccgtcaagccgtcaattgtctgattcgttaccaattatgacaacttgacggctacatcattcactttttcttcacaaccggcacggaactcgctcgggctggccccggtgcattttttaaatacccgcgagaaatagagttgatcgtcaaaaccaacattgcgaccgacggtggcgataggcatccgggtggtgctcaaaagcagcttcgcctggctgatacgttggtcctcgcgccagcttaagacgctaatccctaactgctggcggaaaagatgtgacagacgcgacggcgacaagcaaacatgctgtgcgacgctggcgatatcaaaattgctgtctgccaggtgatcgctgatgtactgacaagcctcgcgtacccgattatccatcggtggatggagcgactcgttaatcgcttccatgcgccgcagtaacaattgctcaagcagatttatcgccagcagctccgaatagcgcccttccccttgcccggcgttaatgatttgcccaaacaggtcgctgaaatgcggctggtgcgcttcatccgggcgaaagaaccccgtattggcaaatattgacggccagttaagccattcatgccagtaggcgcgcggacgaaagtaaacccactggtgataccattcgcgagcctccggatgacgaccgtagtgatgaatctctcctggcgggaacagcaaaatatcacccggtcggcaaacaaattctcgtccctgatttttcaccaccccctgaccgcgaatggtgagattgagaatataacctttcattcccagcggtcggtcgataaaaaaatcgagataaccgttggcctcaatcggcgttaaacccgccaccagatgggcattaaacgagtatcccggcagcaggggatcattttgcgcttcagccatacttttcatactcccgccattcagagaagaaaccaattgtccatattgcatcagacattgccgtcactgcgtcttttactggctcttctcgctaaccaaaccggtaaccccgcttattaaaagcattctgtaacaaagcgggaccaaagccatgacaaaaacgcgtaacaaaagtgtctataatcacggcagaaaagtccacattgattatttgcacggcgtcacactttgctatgccatagcatttttatccataagattagcggatcctacctgacgctttttatcgcaactctctactgtttctccatacccgttttttggtaccgggccccccctcgagtttattttaggaggcaaaaatggataacgcctttagcgatttcacccagaaatataccctgagcaaaaccctgcgttttgaactgcgtccggttggtaataccgaaaaaatgctggaagatgagaaagtgttcgagaaagacaaactgatccaagagaaatatatcaaaaccaaaccgtacttcgatctgctgcatcgtgaatttgttgaagaggcactgaaagatgttgatattagcggtctgcacaactactttgaaacctatcagaaatgggccaaagacaagaagaaataccagaaagaactgcagaacaaagagcagattctgcgcaaagaaattctggtttttctggatagcaccgccaaatattgggcagaaaaaaagtatagcgaactgcgcatcaaaaagaaggatatcgaaatctttttcgaagaggacgtgttcaccattctgaaaaaacgttatggtgaagatagcgaagcccagattattgatgaagttagcggtgaaaccgtgagcatttttgatagctggaaaggttttaccggctacttcaaaaaattccaagaaacccgcaaaaacctgtatcgtgatgatggcaccgcaaccgcacatgcaacccgtattattgatcagaatctgaaacgcttttgcgataacctggaaatcattaaacgtatcgcaggcatcatcgaatttagcgaagttgaaggcaacttcaaacatagcatgggtgatgtttttagcctgagcttctataacaaatgtctgctgcaggatggcatcaacttttataaccgtattttaggtggtgaggttctgcaggacggcaccaaactgaaaggtattaatgaactgatcaacaagtatcgccaggataacaaaggtgtgaaaatcccgtttctgaaactgctggataaacaaatcctgagcgaaaaagaagaatttctggacggcatcgaagatgataaagagctgctggcagtactgaaaaaattctatgaagtggccgagaaaaaaaccagcatcctgaaaagcctgattcaggattttgcacagaataaccgtcagtacaatctggaagaagtgtacattagcaaagaagcctttaataccattagccgcaaatggacccatgaaaccagcaaatttgaagagtggctgtacaatgtgatgaaaccgaataaaccgaccggtctgaaatacgacaaaaaagaggaaagctataagttcccggattttattccgctgagctatattcagaccgcactggaacaggcagatattgatggtgatttttggaaagaacactacagcgaaaatagcaaagccaatgatggttgtctgatgggagatgaaagcatttgggaacagtttatcaagatcttcgagtatgaattccagagcctgtttgaaaaagaaatcattgatcgtgaaaccggtcagccgaagaaaaatggttataactatgtgaaggacgacttcaaaggtctgctgaatggcgaaaactttagcgtcgaaatcatcaaagattttgccgataccgtgctgagcatttatcagatggccaaatactttgccatcgagaaaaagcgtaaatggctggatgaatatgataccggtgatttctatgaaaacccggaatttggctacaaactgttctatgatgatgcgtataaagaaatcgtgcagacctataataacctgcgcaattacctgaccaaaaaatcctatagcgaagagaaatggaagctgaattttgaaaatccgacactggcagatggttgggataaaaacaaagaaccggataattcagccgtgatcctgcgtaaagatggtcgttattatctgggcctgatgaaaaaaggctgcaacaaaattttcgacgaccgcaacaaagtggaatttagtggtggtgtggataaagacaaatacgagaaaatcgtgtacaagttctttccggatcaggcaaaaatgtttccgaaagtttgttttagcgcgaaaggcctggatttttttcagccgagcgaggaaattctgaacatctataaaaacagcgagttcaaaaaaggcgatacctttagcgttcagagcatgcagaaactgatcgatttctataaagattgcctgaccaagtatgaaggctggattgcctatgaattcaaacatctgaaaagcaccgatctgtatcgcaataacatcagcgaatttttcagtgatgttgccgaagatggctataaaatcacctttcaggatatcagcgataactacattgataaaaagaaccagtccgaggaactgtacctgttcgaaattcataacaaagactggaacctgaaagacgaggtgaaaaaaacaggtagcaaaaatctgcacaccctgtattttgaagcactgtttagccatgaaaacatccagaacaactttccgattaaactgaatggtcaggccgaagttttttatcgtccgaaaaccgatgaagagaaactggtgaagaaaaaggataaaaaaggccgtgaagtgatcgaccataaacgctatgcagaaaacaaaatcttctttcatgttccgctgacactgaatcgtggtaaaggtgatgcatatcagtttaacgccaagatcaataactttctggccaacaacagcgatattaatgttattggtgttgaccgtggcgaaaaacatctggcatattatagcgtgattaaccagaaaggcgaaaccctggatagcggtagcctgaatgttgtgaacaaaattaactatggcgagaaactgcaagagaaagccagcaatcgtaaacagagcattcgtgattggaaagcagttgagggcattaaaaacctgaaaaagggctatattagccaggttgttcgtaaactggccgatctggcaattgaacataatgcgatcatcatctttgaggatctgaacatgcgttttaagcagattcgtggtggtattgaaaaaagcgtgtatcagcagctggaaggtgcactgattgaaaaactgagctttctggtgaataaaggcgagaaagatccgaaacaggcaggtaatctgctgaaagcatatcagctggcagcaccgtttaccacctttaaagatatgggtaaacagaccggcatcatcttctatacccaggcaagctataccagtaaaattgatccgctgaccggctggcgtccgaatctgtatctgaaatatacaaatgccgaaaaaaccaaagaggacatcggcaactttagcaacatcgaattcaaaaacggcatctttgaatttacctacgatctgcgcaacttccagaaacagaaagagtatccgaaaaaaacggaatggaccctgtgtagctgtgttgaacgttttcgttggaatcgtgttctgaaccagaataaaggtggctatgatcattatgaggatatcacccataatttccgtgacctgtttgagaagtatgacatcaatttcatgagcgcagatatcaaaggtcagattgataccctggatgccaaaggcaatgaaaacttcttcaaagactttatcttcttcttcaacctgatctgccagattcgtaatacccagcaggacaaagatggtgatgaaaacgattttatcctgagtccgatcaaaccgttttttgattcacgtgacagcaagaaatttggcgaaaatctgccgaataatggcgacgataatggtgcatacaatattagccgtaagggcattatcatcctgaacaagattagcgaattcttcgatgaaaatggtggctgcgagaaaatgaaatggggtgatctgtatatcagccacaaagattgggatgattttgcccgtcagatctaatggtctagaggtcgaaattcaaattgtgagcggataacaatttgaattttctgtatgaggttttgctaaacaactttcaacagtttcagtggagtgagaatagaaaggaacaactaaaggaattgcgaataataattttttcacgttgaaaatctccaaaaaaaaaggctccaaaaggagcctttaattgtatcggtttatcagcttgctttcgaggtgaattttgaccctctagcgaaaatgcaagagcaaagacgaaaacatgccacacatgaggaataccgattctctcattaacatattcaggccagttatctgggcttaaaagcagaagtccaacccagataacgatcatatacatggttctctccagaggttcattactgaacactcgtccgagaataacgagtggatcccctccaattcgccctatagtgagtcgtattacgcgcgctcactggccgtcgttttacaacgtcgtgactgggaaaaccctggcgttacccaacttaatcgccttgcagcacatccccctttcgccagctggcgtaatagcgaagaggcccgcaccgatcgcccttcccaacagttgcgcagcctgaatggcgaatggaaattgtaagcgttaatattttgttaaaattcgcgttaaatttttgttaaatcagctcattttttaaccaataggccgactgcgatgagtggcagggcggggcgtaatttttttaaggcagttattggtgcccttaaacgcctggtgctacgcctgaataagtgataataagcggatgaatggcagaaattcgaaagcaaattcgacccggtcgtcggttcagggcagggtcgttaaatagccgcttatgtctattgctggtttaccggtttattgactaccggaagcagtgtgaccgtgtgcttctcaaatgcctgaggccagtttgctcaggctctccccgtggaggtaataattgacgatatgatcatttattctgcctcccagagcctgataaaaacggtgaatccgttagcgaggtgccgccggcttccattcaggtcgaggtggcccggctccatgcaccgcgacgcaacgcggggaggcagacaaggtatagggcggcgaggcggctacagccgatagtctggaacagcgcacttacgggttgctgcgcaacccaagtgctaccggcgcggcagcgtgacccgtgtcggcggctccaacggctcgccatcgtccagaaaacacggctcatcgggcatcggcaggcgctgctgcccgcgccgttcccattcctccgtttcggtcaaggctggcaggtctggttccatgcccggaatgccgggctggctgggcggctcctcgccggggccggtcggtagttgctgctcgcccggatacagggtcgggatgcggcgcaggtcgccatgccccaacagcgattcgtcctggtcgtcgtgatcaaccaccacggcggcactgaacaccgacaggcgcaactggtcgcggggctggccccacgccacgcggtcattgaccacgtaggccgacacggtgccggggccgttgagcttcacgacggagatccagcgctcggccaccaagtccttgactgcgtattggaccgtccgcaaagaacgtccgatgagcttggaaagtgtcttttggctgaccaccacggcgttctggtggcccatctgcgccacgaggtgatgcagcagcattgccgccgtgggtttcctcgcaataagcccggcccacgcctcatgcgctttgcgttccgtttgcacccagtgaccgggcttgttcttggcttgaatgccgatttctctggactgcgtgg

SEQ ID NO: 60 - DNA, 10336 bp, Artificial Sequence
  CRISPR/BMC08-Ec vector system
ccatgcttatctccatgcggtagggtgccgcacggttgcggcaccatgcgcaatcagctgcaacttttcggcagcgcgacaacaattatgcgttgcgtaaaagtggcagtcaattacagattttctttaacctacgcaatgagctattgcggggggtgccgcaatgagctgttgcgtaccccccttttttaagttgttgatttttaagtctttcgcatttcgccctatatctagttctttggtgcccaaagaagggcacccctgcggggttcccccacgccttcggcgcggctccccctccggcaaaaagtggcccctccggggcttgttgatcgactgcgcggccttcggccttgcccaaggtggcgctgcccccttggaacccccgcactcgccgccgtgaggctcggggggcaggcgggcgggcttcgccttcgactgcccccactcgcataggcttgggtcgttccaggcgcgtcaaggccaagccgctgcgcggtcgctgcgcgagccttgacccgccttccacttggtgtccaaccggcaagcgaagcgcgcaggccgcaggccggaggcttttccccagagaaaattaaaaaaattgatggggcaaggccgcaggccgcgcagttggagccggtgggtatgtggtcgaaggctgggtagccggtgggcaatccctgtggtcaagctcgtgggcaggcgcagcctgtccatcagcttgtccagcagggttgtccacgggccgagcgaagcgagccagccggtggccgctcgcggccatcgtccacatatccacgggctggcaagggagcgcagcgaccgcgcagggcgaagcccggagagcaagcccgtagggcgccgcagccgccgtaggcggtcacgactttgcgaagcaaagtctagtgagtatactcaagcattgagtggcccgccggaggcaccgccttgcgctgcccccgtcgagccggttggacaccaaaagggaggggcaggcatggcggcatacgcgatcatgcgatgcaagaagctggcgaaaatgggcaacgtggcggccagtctcaagcacgcctaccgcgagcgcgagacgcccaacgctgacgccagcaggacgccagagaacgagcactgggcggccagcagcaccgatgaagcgatgggccgactgcgcgagttgctgccagagaagcggcgcaaggacgctgtgttggcggtcgagtacgtcatgacggccagcccggaatggtggaagtcggccagccaagaacagcaggcggcgttcttcgagaaggcgcacaagtggctggcggacaagtacggggcggatcgcatcgtgacggccagcatccaccgtgacgaaaccagcccgcacatgaccgcgttcgtggtgccgctgacgcaggacggcaggctgtcggccaaggagttcatcggcaacaaagcgcagatgacccgcgaccagaccacgtttgcggccgctgtggccgatctagggctgcaacggggcatcgagggcagcaaggcacgtcacacgcgcattcaggcgttctacgaggccctggagcggccaccagtgggccacgtcaccatcagcccgcaagcggtcgagccacgcgcctatgcaccgcagggattggccgaaaagctgggaatctcaaagcgcgttgagacgccggaagccgtggccgaccggctgacaaaagcggttcggcaggggtatgagcctgccctacaggccgccgcaggagcgcgtgagatgcgcaagaaggccgatcaagcccaagagacggcccgagaccttcgggagcgcctgaagcccgttctggacgccctggggccgttgaatcgggatatgcaggccaaggccgccgcgatcatcaaggccgtgggcgaaaagctgctgacggaacagcgggaagtccagcgccagaaacaggcccagcgccagcaggaacgcgggcgcgcacatttccccgaaaagtgccacctgaaccccagagtcccgctcagaagaactcgtcaagaaggcgatagaaggcgatgcgctgcgaatcgggagcggcgataccgtaaagcacgaggaagcggtcagcccattcgccgccaagctcttcagcaatatcacgggtagccaacgctatgtcctgatagcggtccgccacacccagccggccacagtcgatgaatccagaaaagcggccattttccaccatgatattcggcaagcaggcatcgccatgggtcacgacgagatcctcgccgtcgggcatccgcgccttgagcctggcgaacagttcggctggcgcgagcccctgatgctcttcgtccagatcatcctgatcgacaagaccggcttccatccgagtacgtgctcgctcgatgcgatgtttcgcttggtggtcgaatgggcaggtagccggatcaagcgtatgcagccgccgcattgcatcagccatgatggatactttctcggcaggagcaaggtgagatgacaggagatcctgccccggcacttcgcccaatagcagccagtcccttcccgcttcagtgacaacgtcgagcacagctgcgcaaggaacgcccgtcgtggccagccacgatagccgcgctgcctcgtcttggagttcattcagggcaccggacaggtcggtcttgacaaaaagaaccgggcgcccctgcgctgacagccggaacacggcggcatcagagcagccgattgtctgttgtgcccagtcatagccgaatagcctctccacccaagcggccggagaacctgcgtgcaatccatcttgttcaatcatgcgaaacgatcctcatcctgtctcttgatcagatcttgatcccctgcgccatcagatccttggcggcaagaaagccatccagtttactttgcagggcttcccaaccttaccagagggcgccccagctggcaattccggttcgcttgctgtccataaaaccgcccagtctagctatcgccatgtaagcccactgcaagctacctgctttctctttgcgcttgcgttttcccttgtccagatagcccagtagctgacattcatccggggtcagcaccgtttctgcggactggctttctacgtgttccgcttcctttagcagcccttgcgccctgagtgcttgcggcagcgtgaagctagctgcataatgtgcctgtcaaatggacgaagcagggattctgcaaaccctatgctactccgtcaagccgtcaattgtctgattcgttaccaattatgacaacttgacggctacatcattcactttttcttcacaaccggcacggaactcgctcgggctggccccggtgcattttttaaatacccgcgagaaatagagttgatcgtcaaaaccaacattgcgaccgacggtggcgataggcatccgggtggtgctcaaaagcagcttcgcctggctgatacgttggtcctcgcgccagcttaagacgctaatccctaactgctggcggaaaagatgtgacagacgcgacggcgacaagcaaacatgctgtgcgacgctggcgatatcaaaattgctgtctgccaggtgatcgctgatgtactgacaagcctcgcgtacccgattatccatcggtggatggagcgactcgttaatcgcttccatgcgccgcagtaacaattgctcaagcagatttatcgccagcagctccgaatagcgcccttccccttgcccggcgttaatgatttgcccaaacaggtcgctgaaatgcggctggtgcgcttcatccgggcgaaagaaccccgtattggcaaatattgacggccagttaagccattcatgccagtaggcgcgcggacgaaagtaaacccactggtgataccattcgcgagcctccggatgacgaccgtagtgatgaatctctcctggcgggaacagcaaaatatcacccggtcggcaaacaaattctcgtccctgatttttcaccaccccctgaccgcgaatggtgagattgagaatataacctttcattcccagcggtcggtcgataaaaaaatcgagataaccgttggcctcaatcggcgttaaacccgccaccagatgggcattaaacgagtatcccggcagcaggggatcattttgcgcttcagccatacttttcatactcccgccattcagagaagaaaccaattgtccatattgcatcagacattgccgtcactgcgtcttttactggctcttctcgctaaccaaaccggtaaccccgcttattaaaagcattctgtaacaaagcgggaccaaagccatgacaaaaacgcgtaacaaaagtgtctataatcacggcagaaaagtccacattgattatttgcacggcgtcacactttgctatgccatagcatttttatccataagattagcggatcctacctgacgctttttatcgcaactctctactgtttctccatacccgttttttggtaccgggccccccctcgagtttattttaggaggcaaaaatgatgcagatcatgaagaacttcgacaaattcaccaatctgtacagcgttagcaaaaccctgcgttttgaactgcgtccggaaccgaaaacactggaatatatgcgtagcaatctgcgctttgataaaaacctgcagacctttctggcagatcaagaaattgaagatgcatatcaggcactgaaaccgatttttgatagcctgcatgaacgctttattaccgaaagcctggaaagcggtagcgcacagaaaattgattttagcaaatatctggaaaaatatcgcaacaaacgcgacctgggtattaaagcactggaaggcaccgaaaaactgctgcgtaataactttgccgaaatctataaagcaaccgccaaaagctggaaagaaaatgcaggtaaagatggcaaaggcaaagaggtgttcaaaaaagaaggctttaacatcctgaccgaaaaaggcattctggaatacatcgagaaaaacatcgatagctttagcgccattaaaagtccggaagaaattcgtggtgcactgggtgcatttgatggtttttttacctatttcaccggcttcaatcagaaccgcgaaaactattacgaaaccaaaaaagaggcaagcaccgcagttgcaacccgtattgttcatgaaaatctgccgaaattctgcgataacattctgatctttgatgaacgtgccgaggattatattggtgcatataaagccctgcagaaaatgggtcgtgcactggttaataaagaaggtggcgaactgccgagcattagcggtgacctgtttaaaatcaccttcttcaacaaatgcttcagccagaagcagatcgaagaatataacaccgcaattggtaatgccaatagcctggttaacctgttcaatcaggcaaaacgtgatgaagatggctacaaaaaactggcactgtttaagaccctgtataagcagattggctgcgataaaaaagatagcctgttttttgcagtgacccatgatcgtcgtgcagatgcagaaaaagcacgtgaaaatggtcaagaagcatttagcgtagaagaagttctggttctggcaaaacatgcgggtgaaaagtatttcaataaaggcaatgatgatggcgaagtgaataccacgcaagaatttatcagctatattaaggatcgcagcgattaccagggtatctattggagcaaagcagcactgaataccatcagcaacaaatatttcgataactggtatgagctgattgatcagctgaaagaagccaaagtttttaccaaaaccggtagcggtagtgaggataatgttaaaattccggatgccattgaactggaaggtttttttcaggtgctgaacaaaatccaggattggaaaaccgtgttcttcaaaaaaagcattaccgcagatccgcagaaactgggcattattgaaagcagcgaaaccgcaagcgcagcactgctgagcctgattttcgatgatgttgcaaaacacaccaaactgtttatcgatcagagcgaggatattctgaaagtggaaaattttgtgaaaccggaaaacaaagaggacattaaacgttggctggatcatagcctggcaattaatcagatgctgaagtattttctggtgaaagaaagccgtaccaaaggtgcaccgattgatccgacactgaccaaagcgctggataccctgctgcgttcacaggatgcagaatggtttaaatggtatgatgtgctgcgcaactacctgaccaaaaaaccgcaggatggcaccaaagaaaataaactgaaactgagctttgaaaatggcaccctggcaaatggttgggatgtgaataaagaaccggataacttttgcgtgatcctgcagaatccggaaggcaaaaaattcctggccattattgcacgtcaagaaggtcagaaaggttttaatcaggtgttcgccaaaaaacatgataacccgctgtataaagttgatgaaggtggtgtcttttggtccaagatggaatataaactgttaccgggtccgaataagatgctgcctaaatgtctgatgccgaaaagcaatcgtgaaaaatatggtgcaaccgaggaagtgctgaaaatttacaatcagggcagctttaaaaagaccgaaagcaacttcagcaaaaaagatctgagtcgcctgatcaacttctataaaagcgcactgcagcagtatgaagattggcgttgttttaactttagctttcgtgccaccgatagctatgaagatattggtcagttttatcgtgatgtggaaagccagggttataaactggattttcagagcattaataccgatgtgctggatgaactggtggaagaaggtaaaatctacctgttcgaaatcaaaaaccaggatagcaatcagggtaaaagcagcattcatcgtgataatctgcataccatgtattggaatgccctgtttcaagaagtactgaatcgtccgaaactgaatggtggtgcagaactgttctatcgtaaagcgctgtcaccggaaaaaatcaaagaactgggtagcgtggataaaaacggcaaacgtattattcgcaactatcggttcagcaaagagaagttcattttccatattccgatcacgctgaacttttgtctgagcgatacccgtgttaatgataccgttaatcaagaactgagccgtacctcaagcagtcattttctgggtattgatcgtggtgaaaaacacctggcatattactttctggttgatcagaacggcaaaattgtgctggacgaatatggtaaagcagttcagggcaccctgaatattccgtttctggataataatggtaacgtgcgcaaaattaaggccaaacgtcgtagcctggatgagaatggcaaagaaaaaatagaagaggtgtggtgcaaagactataacgaactgctggaagcacgtgccggtgatcgtgcatatgcccgtaaaaattggcagaccattggcaacattaaagaactgaaagagggctatattagccaggtggttcgtaaaattgttgatctggccattgaatatgaagcctttatcgttctggaagatctgaacgttggttttaaacgtggtcgtcagaaaatcgaaaaaagcgtgtatcagaaattagaactggccctggcgaaaaaactgaattttgttgttgacaaaagcgccaaaattggtggtctgaaaagcgttaccaatgcgctgcagctggcaccgcctgttagcaattttggtgatattgaaggtcgtaaacagttcggcattatgctgtatacccgtgcaaattataccagccagaccgatccggcaaccggctggcgtaaaagcatttatctgaaacgtggtagcgaagaaagcattcgcaagcagattattgatagcttcgaagaaattggctttgatggcgaggattactttttcacctataccgatagcgttgcaggtcgcacctggattctgtatagcggtaaaaatggtggtagtctggatcgcttttatggcaaacgtgataacgataaaaatcagtgggttagcatgcgccaggatgtgagcaaacagctggatggtatcctggccaattttgaaaaagatcgtagcattctggcccagattatcgatggtgaagtggatctgatcaaagtcgaacagaaatataccgcatgggaaagttttcgtagcaccattgatctgattcagcagattcgtaataccggcaccagcgaacgtgatggcgatttcattctgagtccggttcgtgatgaacgcggtattcattttgatagtcgtgatacacgtgaaggtatgccgaccagcggtgatgcaaatggtgcctataacattgcacgtaaaggtacgattatgggcgaacatattaaacgtgaatacagccgcatgttcatttccgatgaagaatgggatgcatggctggcaggtaaacaggtttgggaaaaatggctgaaagacaacgagaaaatcctgaaaaagaaataatggtctagaggtcgaaattcaaattgtgagcggataacaatttgaattttctgtatgaggttttgctaaacaactttcaacagtttcagtggagtgagaatagaaaggaacaactaaaggaattgcgaataataattttttcacgttgaaaatctccaaaaaaaaaggctccaaaaggagcctttaattgtatcggtttatcagcttgctttcgaggtgaattttgaccctctagcgaaaatgcaagagcaaagacgaaaacatgccacacatgaggaataccgattctctcattaacatattcaggccagttatctgggcttaaaagcagaagtccaacccagataacgatcatatacatggttctctccagaggttcattactgaacactcgtccgagaataacgagtggatcccctccaattcgccctatagtgagtcgtattacgcgcgctcactggccgtcgttttacaacgtcgtgactgggaaaaccctggcgttacccaacttaatcgccttgcagcacatccccctttcgccagctggcgtaatagcgaagaggcccgcaccgatcgcccttcccaacagttgcgcagcctgaatggcgaatggaaattgtaagcgttaatattttgttaaaattcgcgttaaatttttgttaaatcagctcattttttaaccaataggccgactgcgatgagtggcagggcggggcgtaatttttttaaggcagttattggtgcccttaaacgcctggtgctacgcctgaataagtgataataagcggatgaatggcagaaattcgaaagcaaattcgacccggtcgtcggttcagggcagggtcgttaaatagccgcttatgtctattgctggtttaccggtttattgactaccggaagcagtgtgaccgtgtgcttctcaaatgcctgaggccagtttgctcaggctctccccgtggaggtaataattgacgatatgatcatttattctgcctcccagagcctgataaaaacggtgaatccgttagcgaggtgccgccggcttccattcaggtcgaggtggcccggctccatgcaccgcgacgcaacgcggggaggcagacaaggtatagggcggcgaggcggctacagccgatagtctggaacagcgcacttacgggttgctgcgcaacccaagtgctaccggcgcggcagcgtgacccgtgtcggcggctccaacggctcgccatcgtccagaaaacacggctcatcgggcatcggcaggcgctgctgcccgcgccgttcccattcctccgtttcggtcaaggctggcaggtctggttccatgcccggaatgccgggctggctgggcggctcctcgccggggccggtcggtagttgctgctcgcccggatacagggtcgggatgcggcgcaggtcgccatgccccaacagcgattcgtcctggtcgtcgtgatcaaccaccacggcggcactgaacaccgacaggcgcaactggtcgcggggctggccccacgccacgcggtcattgaccacgtaggccgacacggtgccggggccgttgagcttcacgacggagatccagcgctcggccaccaagtccttgactgcgtattggaccgtccgcaaagaacgtccgatgagcttggaaagtgtcttttggctgaccaccacggcgttctggtggcccatctgcgccacgaggtgatgcagcagcattgccgccgtgggtttcctcgcaataagcccggcccacgcctcatgcgctttgcgttccgtttgcacccagtgaccgggcttgttcttggcttgaatgccgatttctctggactgcgtgg

SEQ ID NO: 61 - DNA, 10699 bp, Artificial Sequence
  CRISPR/BMC10-Ec vector system
caatcggcgttaaacccgccaccagatgggcattaaacgagtatcccggcagcaggggatcattttgcgcttcagccatacttttcatactcccgccattcagagaagaaaccaattgtccatattgcatcagacattgccgtcactgcgtcttttactggctcttctcgctaaccaaaccggtaaccccgcttattaaaagcattctgtaacaaagcgggaccaaagccatgacaaaaacgcgtaacaaaagtgtctataatcacggcagaaaagtccacattgattatttgcacggcgtcacactttgctatgccatagcatttttatccataagattagcggatcctacctgacgctttttatcgcaactctctactgtttctccatacccgttttttggtaccgggccccccctcgagtttattttaggaggcaaaaatgagcaccaaacgtagctttagcgatttcaccaatctgtatagcgttagcaaaaccctgcgttttgaactgaaaccgattggtaaaaccctggaaaatatgcgtgaacgcatctacaacgataaaaaggattatgatagcgctctgcagacctttctgcatgatcaggcaattgaagatgcctataaaacactgaaacccattctggatagcctgcacgaagaatttatcaataccagcctgaatagcagcaaagccaaaaacattgatctgagcgaatatctgaatgcctatcgtgaacgtggtaatgataccaaaaccggtgaagaaagcaaactgagcggtattgaaaaatcactgcgtaaagcaattggcgaaacctatctgacctgggcaaaaagctttaccgaacaggccaaaaatctgattggcatcattgaagatatctgggataccgaagaggaatgggatgaagaaaagaaaaccaaatggctgttcaaaaagaaaaacttcgaactgctgaccgaaagcggtattctggtttttattgagaaaaagctggataccatgaacatcagcgaacaagagaaaaccgatattaagaaagccctggaagaattcaaaggcttctttacctatttcagcggctataatcagaaccgcaaaaactactatgaaaccaaggcagagaaaaagaccgcaattgcaacccgtattgttcatgaaaatctgccgaaattttgcgacaacgtgattctgtttcatggctatcagaaaatcctgaaagatggtagcaaacgcgagtacaagaagaaagaggaatatctgggtatgtacgcctttctgaaactgcgtaatattgaaacctgcatcaaagatgcggaaagcggtgaaatgattgaactgtatgcaatcaccgaggatatcttcgatattagctttttcagcagctgtctggcacagcgtgaaattgatgaacataatcgtattatcggtggcatcgataaatacaaccgcattattggtcattataatgccctgatcaacctgtataatcaggcacgtaagaaagacgagaaatttaccaaactgtccccgttcaaagaactgtataaacaaatttggtgcggcaacaaaaagtggtcatggattaaagcgattacccatgataccgatgagcagattctggcagataccaatcatacaggtgaagcaattagcgttgaacgtattctgagcctggcaagcaaagcaggtaaaaagtattttcagccgtggaaaagcaccgatgatggtattaaaaccgttccggatttcctggattggctgcgtggtcagaccgattggaatggtatttattggagcaaagccgcaattaatagcatcagcaatgtgtattttccgaactggggtagcattaaagaaaccatgaaaggtgataaaacgctggtgagctatgataaaaagcgcgaagaacaaatcaaaatcaacgaagcagttgaactgagtggcctgtttgatattctggattcaaccgatggtgattggaaacaagaatgggtgctgtttaaagcaagcctgaccaaactgctggatgcaagcgcagaaaatgccgaagaaaattcaaaacgtgcccgtcgcaaagatattattgatcgtagcagcagcccgagccaggcactgctggcactgattaccgattttattgaagagaacatgaaacattttctggaccagagccataccattctgcgtctgaccgaatatagcagtccgaaaagcaaagaagccatcaaaagttggatggatctggccctgagcgttagccagaccattcgttattttcgtgtgaaagaatccaaaaccaaaggcgataccctgaatgcagaactggttggtattctgaccaatttactggatgcagaagatgcaacctggtttgagtggtatgatctgctgcgtaattatctgaccaaaaagccgcaggatgatgcgaaagaaaataaactgaaactgaactttgccaacagtaccctggcagcaggttgggatgttaataaagaaacggataatacctgcgtgatcctgcagaatccggaatggaaaacatatctggccgtgatgaacaaaaacaaaaagaacgtgttccagaaagaatggaatgaatggcgctggaagaagaaaacaaccaaactgaatccgctgtatgaaatcgattggggtgaaagctggaaaaagatggaatatgatttttggagcgacgtgagcaaaatgattccgaaatgtagcacccagctgaagaaagtgatcaagcactttaaagaaagcgacgaggattttatctttccgagcggttataaagttaccagcggtgaacgttttatcgaagaatgtcgtattaccaaagaacagttcgagctgaacaacaaagtgtataaacgtgatggcgatcgcattattagcgcctttcgttatgaactgagcgaaaccgaggaaaagacctatatcaaaagcttccaaaaaggctatctggatatgctgctgaagagtaataatctgccggaaaccgaacaagaaatctaccgcaagaaatatgaagatagcctgagcaaatggatcaacttctgcaaatacttcatctggaaatacccgaaaaccagcctgttcgaatatcagtttgatgaaaccgaccactataaaagcgtggacaaatttaacctggatgtggatatttggagctacaaactgaaagtggacaccaagattaacaaaaccatcctggataccctggtggaaaatggtgatatttacctgttcgagatcaaaaaccaggatagcaatattggcaaatgggagaaccataaaaacaacctgcataccacctactggaaatccatttttgaaagcgttcagaatcgtccgaaactgaatggtgaagccgaaatcttttatatgaaaccgctgagtccggaaaaactgcagaaaaagattgacaagaagggcaaagaaatcatcgatggttatcgttttagccgtgaacgcttcatttttcattgtccgattacgctgaatttttgcctgggcaatgagaagatcaacaacatcattaatttcgaactgagcccgaaaagcgatatctattttctgggtttagatcgcggtgaaaaacacctggtgtattattcaattgtggaccagaacggtaaaatgatcgaccagtggtctttcaacgagatcaagtggaaagattatcatgcgctgctgacaaaacgcgaatgggatcgtatggaaagccgtaaaaattggcagaccattagcaacattgccaagcttaaagagtggtatattagcctggtgatccatgagattatcgagaagctgaagctgaatccgtggtttattgttctggaagatctgaacaccggctttaaacgtggtcgtcagaaaattgaaaagagcatctaccagaaatttgaactggcactggctaaaaagctgaatttcgttgttgataaaagcgccaaactgggtgaagttggtagcgttaccaatgcactgcagctgacccctccggttagcaattatggcgatattgaaaatcgtaaacaggtgggcattatgctgtatacccgtgcaaattataccagccagaccgatccggcaaccggctggcgtaaaaccatttatctgaaaaccggtagcgaggaaaacatcaaagagcagattgttacccagtttagcgatattggctttgatggcaaagattattattttgaatataccgacaaaatcggcaaaacctggattctgtatagtggcaaaaatggcaaaagtctgacccgttttcgtggtgttcgtggtaaagaaaagaatgaatggaacattaaagagatcaacgtccgcaatatgctggatggtatttttgcgaactttgataaagatcgcagctttctgagccagatcctggatgaatgggttgaaattaagaaaatcgatgaacacaccgcatgggaaagcctgcgctttgcaatcgatctgattcagcagattcgtaacagtggcgataaaacccagtgggaagatgataactttctgtttagtccggttcgtgatgcacagggtaaccattttgatacccgtgaacagaaagaaggcctgccgaaagacgcagatgcaaatggtgcatataatattgcccgtaagtggatcatcatgaacgaacatattcgcattaacgaggataccaaagatctggacctgtttgttagtgatgaagaatgggatatgtggctgaccgatcgtgaaaaatggaaagaaatgctgcctatttttgcaagccgcaaagcaatggaaaaacgtcgcggtaaataatggtctagaggtcgaaattcaaattgtgagcggataacaatttgaattttctgtatgaggttttgctaaacaactttcaacagtttcagtggagtgagaatagaaaggaacaactaaaggaattgcgaataataattttttcacgttgaaaatctccaaaaaaaaaggctccaaaaggagcctttaattgtatcggtttatcagcttgctttcgaggtgaattttgaccctctagcgaaaatgcaagagcaaagacgaaaacatgccacacatgaggaataccgattctctcattaacatattcaggccagttatctgggcttaaaagcagaagtccaacccagataacgatcatatacatggttctctccagaggttcattactgaacactcgtccgagaataacgagtggatcccctccaattcgccctatagtgagtcgtattacgcgcgctcactggccgtcgttttacaacgtcgtgactgggaaaaccctggcgttacccaacttaatcgccttgcagcacatccccctttcgccagctggcgtaatagcgaagaggcccgcaccgatcgcccttcccaacagttgcgcagcctgaatggcgaatggaaattgtaagcgttaatattttgttaaaattcgcgttaaatttttgttaaatcagctcattttttaaccaataggccgactgcgatgagtggcagggcggggcgtaatttttttaaggcagttattggtgcccttaaacgcctggtgctacgcctgaataagtgataataagcggatgaatggcagaaattcgaaagcaaattcgacccggtcgtcggttcagggcagggtcgttaaatagccgcttatgtctattgctggtttaccggtttattgactaccggaagcagtgtgaccgtgtgcttctcaaatgcctgaggccagtttgctcaggctctccccgtggaggtaataattgacgatatgatcatttattctgcctcccagagcctgataaaaacggtgaatccgttagcgaggtgccgccggcttccattcaggtcgaggtggcccggctccatgcaccgcgacgcaacgcggggaggcagacaaggtatagggcggcgaggcggctacagccgatagtctggaacagcgcacttacgggttgctgcgcaacccaagtgctaccggcgcggcagcgtgacccgtgtcggcggctccaacggctcgccatcgtccagaaaacacggctcatcgggcatcggcaggcgctgctgcccgcgccgttcccattcctccgtttcggtcaaggctggcaggtctggttccatgcccggaatgccgggctggctgggcggctcctcgccggggccggtcggtagttgctgctcgcccggatacagggtcgggatgcggcgcaggtcgccatgccccaacagcgattcgtcctggtcgtcgtgatcaaccaccacggcggcactgaacaccgacaggcgcaactggtcgcggggctggccccacgccacgcggtcattgaccacgtaggccgacacggtgccggggccgttgagcttcacgacggagatccagcgctcggccaccaagtccttgactgcgtattggaccgtccgcaaagaacgtccgatgagcttggaaagtgtcttttggctgaccaccacggcgttctggtggcccatctgcgccacgaggtgatgcagcagcattgccgccgtgggtttcctcgcaataagcccggcccacgcctcatgcgctttgcgttccgtttgcacccagtgaccgggcttgttcttggcttgaatgccgatttctctggactgcgtggccatgcttatctccatgcggtagggtgccgcacggttgcggcaccatgcgcaatcagctgcaacttttcggcagcgcgacaacaattatgcgttgcgtaaaagtggcagtcaattacagattttctttaacctacgcaatgagctattgcggggggtgccgcaatgagctgttgcgtaccccccttttttaagttgttgatttttaagtctttcgcatttcgccctatatctagttctttggtgcccaaagaagggcacccctgcggggttcccccacgccttcggcgcggctccccctccggcaaaaagtggcccctccggggcttgttgatcgactgcgcggccttcggccttgcccaaggtggcgctgcccccttggaacccccgcactcgccgccgtgaggctcggggggcaggcgggcgggcttcgccttcgactgcccccactcgcataggcttgggtcgttccaggcgcgtcaaggccaagccgctgcgcggtcgctgcgcgagccttgacccgccttccacttggtgtccaaccggcaagcgaagcgcgcaggccgcaggccggaggcttttccccagagaaaattaaaaaaattgatggggcaaggccgcaggccgcgcagttggagccggtgggtatgtggtcgaaggctgggtagccggtgggcaatccctgtggtcaagctcgtgggcaggcgcagcctgtccatcagcttgtccagcagggttgtccacgggccgagcgaagcgagccagccggtggccgctcgcggccatcgtccacatatccacgggctggcaagggagcgcagcgaccgcgcagggcgaagcccggagagcaagcccgtagggcgccgcagccgccgtaggcggtcacgactttgcgaagcaaagtctagtgagtatactcaagcattgagtggcccgccggaggcaccgccttgcgctgcccccgtcgagccggttggacaccaaaagggaggggcaggcatggcggcatacgcgatcatgcgatgcaagaagctggcgaaaatgggcaacgtggcggccagtctcaagcacgcctaccgcgagcgcgagacgcccaacgctgacgccagcaggacgccagagaacgagcactgggcggccagcagcaccgatgaagcgatgggccgactgcgcgagttgctgccagagaagcggcgcaaggacgctgtgttggcggtcgagtacgtcatgacggccagcccggaatggtggaagtcggccagccaagaacagcaggcggcgttcttcgagaaggcgcacaagtggctggcggacaagtacggggcggatcgcatcgtgacggccagcatccaccgtgacgaaaccagcccgcacatgaccgcgttcgtggtgccgctgacgcaggacggcaggctgtcggccaaggagttcatcggcaacaaagcgcagatgacccgcgaccagaccacgtttgcggccgctgtggccgatctagggctgcaacggggcatcgagggcagcaaggcacgtcacacgcgcattcaggcgttctacgaggccctggagcggccaccagtgggccacgtcaccatcagcccgcaagcggtcgagccacgcgcctatgcaccgcagggattggccgaaaagctgggaatctcaaagcgcgttgagacgccggaagccgtggccgaccggctgacaaaagcggttcggcaggggtatgagcctgccctacaggccgccgcaggagcgcgtgagatgcgcaagaaggccgatcaagcccaagagacggcccgagaccttcgggagcgcctgaagcccgttctggacgccctggggccgttgaatcgggatatgcaggccaaggccgccgcgatcatcaaggccgtgggcgaaaagctgctgacggaacagcgggaagtccagcgccagaaacaggcccagcgccagcaggaacgcgggcgcgcacatttccccgaaaagtgccacctgaaccccagagtcccgctcagaagaactcgtcaagaaggcgatagaaggcgatgcgctgcgaatcgggagcggcgataccgtaaagcacgaggaagcggtcagcccattcgccgccaagctcttcagcaatatcacgggtagccaacgctatgtcctgatagcggtccgccacacccagccggccacagtcgatgaatccagaaaagcggccattttccaccatgatattcggcaagcaggcatcgccatgggtcacgacgagatcctcgccgtcgggcatccgcgccttgagcctggcgaacagttcggctggcgcgagcccctgatgctcttcgtccagatcatcctgatcgacaagaccggcttccatccgagtacgtgctcgctcgatgcgatgtttcgcttggtggtcgaatgggcaggtagccggatcaagcgtatgcagccgccgcattgcatcagccatgatggatactttctcggcaggagcaaggtgagatgacaggagatcctgccccggcacttcgcccaatagcagccagtcccttcccgcttcagtgacaacgtcgagcacagctgcgcaaggaacgcccgtcgtggccagccacgatagccgcgctgcctcgtcttggagttcattcagggcaccggacaggtcggtcttgacaaaaagaaccgggcgcccctgcgctgacagccggaacacggcggcatcagagcagccgattgtctgttgtgcccagtcatagccgaatagcctctccacccaagcggccggagaacctgcgtgcaatccatcttgttcaatcatgcgaaacgatcctcatcctgtctcttgatcagatcttgatcccctgcgccatcagatccttggcggcaagaaagccatccagtttactttgcagggcttcccaaccttaccagagggcgccccagctggcaattccggttcgcttgctgtccataaaaccgcccagtctagctatcgccatgtaagcccactgcaagctacctgctttctctttgcgcttgcgttttcccttgtccagatagcccagtagctgacattcatccggggtcagcaccgtttctgcggactggctttctacgtgttccgcttcctttagcagcccttgcgccctgagtgcttgcggcagcgtgaagctagctgcataatgtgcctgtcaaatggacgaagcagggattctgcaaaccctatgctactccgtcaagccgtcaattgtctgattcgttaccaattatgacaacttgacggctacatcattcactttttcttcacaaccggcacggaactcgctcgggctggccccggtgcattttttaaatacccgcgagaaatagagttgatcgtcaaaaccaacattgcgaccgacggtggcgataggcatccgggtggtgctcaaaagcagcttcgcctggctgatacgttggtcctcgcgccagcttaagacgctaatccctaactgctggcggaaaagatgtgacagacgcgacggcgacaagcaaacatgctgtgcgacgctggcgatatcaaaattgctgtctgccaggtgatcgctgatgtactgacaagcctcgcgtacccgattatccatcggtggatggagcgactcgttaatcgcttccatgcgccgcagtaacaattgctcaagcagatttatcgccagcagctccgaatagcgcccttccccttgcccggcgttaatgatttgcccaaacaggtcgctgaaatgcggctggtgcgcttcatccgggcgaaagaaccccgtattggcaaatattgacggccagttaagccattcatgccagtaggcgcgcggacgaaagtaaacccactggtgataccattcgcgagcctccggatgacgaccgtagtgatgaatctctcctggcgggaacagcaaaatatcacccggtcggcaaacaaattctcgtccctgatttttcaccaccccctgaccgcgaatggtgagattgagaatataacctttcattcccagcggtcggtcgataaaaaaatcgagataaccgttggcct

SEQ ID NO: 62 - DNA, 10282 bp, Artificial Sequence
  CRISPR/BMC11-Ec vector system
ccatgcttatctccatgcggtagggtgccgcacggttgcggcaccatgcgcaatcagctgcaacttttcggcagcgcgacaacaattatgcgttgcgtaaaagtggcagtcaattacagattttctttaacctacgcaatgagctattgcggggggtgccgcaatgagctgttgcgtaccccccttttttaagttgttgatttttaagtctttcgcatttcgccctatatctagttctttggtgcccaaagaagggcacccctgcggggttcccccacgccttcggcgcggctccccctccggcaaaaagtggcccctccggggcttgttgatcgactgcgcggccttcggccttgcccaaggtggcgctgcccccttggaacccccgcactcgccgccgtgaggctcggggggcaggcgggcgggcttcgccttcgactgcccccactcgcataggcttgggtcgttccaggcgcgtcaaggccaagccgctgcgcggtcgctgcgcgagccttgacccgccttccacttggtgtccaaccggcaagcgaagcgcgcaggccgcaggccggaggcttttccccagagaaaattaaaaaaattgatggggcaaggccgcaggccgcgcagttggagccggtgggtatgtggtcgaaggctgggtagccggtgggcaatccctgtggtcaagctcgtgggcaggcgcagcctgtccatcagcttgtccagcagggttgtccacgggccgagcgaagcgagccagccggtggccgctcgcggccatcgtccacatatccacgggctggcaagggagcgcagcgaccgcgcagggcgaagcccggagagcaagcccgtagggcgccgcagccgccgtaggcggtcacgactttgcgaagcaaagtctagtgagtatactcaagcattgagtggcccgccggaggcaccgccttgcgctgcccccgtcgagccggttggacaccaaaagggaggggcaggcatggcggcatacgcgatcatgcgatgcaagaagctggcgaaaatgggcaacgtggcggccagtctcaagcacgcctaccgcgagcgcgagacgcccaacgctgacgccagcaggacgccagagaacgagcactgggcggccagcagcaccgatgaagcgatgggccgactgcgcgagttgctgccagagaagcggcgcaaggacgctgtgttggcggtcgagtacgtcatgacggccagcccggaatggtggaagtcggccagccaagaacagcaggcggcgttcttcgagaaggcgcacaagtggctggcggacaagtacggggcggatcgcatcgtgacggccagcatccaccgtgacgaaaccagcccgcacatgaccgcgttcgtggtgccgctgacgcaggacggcaggctgtcggccaaggagttcatcggcaacaaagcgcagatgacccgcgaccagaccacgtttgcggccgctgtggccgatctagggctgcaacggggcatcgagggcagcaaggcacgtcacacgcgcattcaggcgttctacgaggccctggagcggccaccagtgggccacgtcaccatcagcccgcaagcggtcgagccacgcgcctatgcaccgcagggattggccgaaaagctgggaatctcaaagcgcgttgagacgccggaagccgtggccgaccggctgacaaaagcggttcggcaggggtatgagcctgccctacaggccgccgcaggagcgcgtgagatgcgcaagaaggccgatcaagcccaagagacggcccgagaccttcgggagcgcctgaagcccgttctggacgccctggggccgttgaatcgggatatgcaggccaaggccgccgcgatcatcaaggccgtgggcgaaaagctgctgacggaacagcgggaagtccagcgccagaaacaggcccagcgccagcaggaacgcgggcgcgcacatttccccgaaaagtgccacctgaaccccagagtcccgctcagaagaactcgtcaagaaggcgatagaaggcgatgcgctgcgaatcgggagcggcgataccgtaaagcacgaggaagcggtcagcccattcgccgccaagctcttcagcaatatcacgggtagccaacgctatgtcctgatagcggtccgccacacccagccggccacagtcgatgaatccagaaaagcggccattttccaccatgatattcggcaagcaggcatcgccatgggtcacgacgagatcctcgccgtcgggcatccgcgccttgagcctggcgaacagttcggctggcgcgagcccctgatgctcttcgtccagatcatcctgatcgacaagaccggcttccatccgagtacgtgctcgctcgatgcgatgtttcgcttggtggtcgaatgggcaggtagccggatcaagcgtatgcagccgccgcattgcatcagccatgatggatactttctcggcaggagcaaggtgagatgacaggagatcctgccccggcacttcgcccaatagcagccagtcccttcccgcttcagtgacaacgtcgagcacagctgcgcaaggaacgcccgtcgtggccagccacgatagccgcgctgcctcgtcttggagttcattcagggcaccggacaggtcggtcttgacaaaaagaaccgggcgcccctgcgctgacagccggaacacggcggcatcagagcagccgattgtctgttgtgcccagtcatagccgaatagcctctccacccaagcggccggagaacctgcgtgcaatccatcttgttcaatcatgcgaaacgatcctcatcctgtctcttgatcagatcttgatcccctgcgccatcagatccttggcggcaagaaagccatccagtttactttgcagggcttcccaaccttaccagagggcgccccagctggcaattccggttcgcttgctgtccataaaaccgcccagtctagctatcgccatgtaagcccactgcaagctacctgctttctctttgcgcttgcgttttcccttgtccagatagcccagtagctgacattcatccggggtcagcaccgtttctgcggactggctttctacgtgttccgcttcctttagcagcccttgcgccctgagtgcttgcggcagcgtgaagctagctgcataatgtgcctgtcaaatggacgaagcagggattctgcaaaccctatgctactccgtcaagccgtcaattgtctgattcgttaccaattatgacaacttgacggctacatcattcactttttcttcacaaccggcacggaactcgctcgggctggccccggtgcattttttaaatacccgcgagaaatagagttgatcgtcaaaaccaacattgcgaccgacggtggcgataggcatccgggtggtgctcaaaagcagcttcgcctggctgatacgttggtcctcgcgccagcttaagacgctaatccctaactgctggcggaaaagatgtgacagacgcgacggcgacaagcaaacatgctgtgcgacgctggcgatatcaaaattgctgtctgccaggtgatcgctgatgtactgacaagcctcgcgtacccgattatccatcggtggatggagcgactcgttaatcgcttccatgcgccgcagtaacaattgctcaagcagatttatcgccagcagctccgaatagcgcccttccccttgcccggcgttaatgatttgcccaaacaggtcgctgaaatgcggctggtgcgcttcatccgggcgaaagaaccccgtattggcaaatattgacggccagttaagccattcatgccagtaggcgcgcggacgaaagtaaacccactggtgataccattcgcgagcctccggatgacgaccgtagtgatgaatctctcctggcgggaacagcaaaatatcacccggtcggcaaacaaattctcgtccctgatttttcaccaccccctgaccgcgaatggtgagattgagaatataacctttcattcccagcggtcggtcgataaaaaaatcgagataaccgttggcctcaatcggcgttaaacccgccaccagatgggcattaaacgagtatcccggcagcaggggatcattttgcgcttcagccatacttttcatactcccgccattcagagaagaaaccaattgtccatattgcatcagacattgccgtcactgcgtcttttactggctcttctcgctaaccaaaccggtaaccccgcttattaaaagcattctgtaacaaagcgggaccaaagccatgacaaaaacgcgtaacaaaagtgtctataatcacggcagaaaagtccacattgattatttgcacggcgtcacactttgctatgccatagcatttttatccataagattagcggatcctacctgacgctttttatcgcaactctctactgtttctccatacccgttttttggtaccgggccccccctcgagtttattttaggaggcaaaaatgagccagaataacaccttcgagaaattcaccaatcagtacagcctgagcaaaaccctgcgttttgaactgcgtccggttggtaataccgagcagatgctggaagatgaaaacgtgttcaaaaaagatgagatcatccgcaaaaaatacgagcagaccaaaccgttcattgacaaactgcataaagaggtgattaaagatagcctgcacggcaaaaaaatcgaaggtctggatgattacttcaaaaaattcgaaatctatagcaaaaacaaaaaagacagcaaaatcaagaaagaatttaccgataaagaaagcgagctgcgcaaacagctgaatagccattttaaagcagaaagcctgtttagcgaaaaagtgtttagcctgctgaaagaaaaatatggcaccgaagatgagagcttcgtgaaagacgaaaatggtaattttgttctggataccgtgggcgaaaaaatcagcatttttgatgaatggaaaggcttcaccggctactttaccaaatttcagaaaacccgtgagaacttctataaagatgatggcaccagcaccgcaattgttacccgtaccattgatgaaaatctgtatcgcttttgcgagaacatcaaacactttgagagcattaaaaaccgcgtgaactttagcgagatcgagaaaaactttaactttaaactggaaaacctgtttaaagccgacttctacaatagctgtctgctgcaggatggtatcgataaatacaatgatatccttggcggtaaaaccctggaaagcggtgaaaaactgaaaggcctgaatgaaatcatcaacaaatatcgccaggacaacaaggtggaaaaaatcggtttcttcaaaatgctggataagcagattctgggcgataaagagaaaccgagctttattgaaagcattgccgatgataatgagctgctgctgaaacttaaagagttttataccaacgccgaggaaaaaaccgaggttctgaaaaaactgttcagcgacttcagcaaaaataacgatagctacgatctgagcaagatctatattaacaaagtgggcattaacaccattctgctgaaatggtttgatgtggcaggtcgtagcgattttgaaaaaaacattagcacccagaccaaaaaagaaaaaattgtgaccttcgacaaggatagcaacagctataagtttccggaatttctggccttcagccatattaaagaagcactgagcaacggcacctatgaagttaaagaaatctggaaagagcgctattatcagagcgagaacaaagagaaatcagaaaaagcaccgctgaaaaaagatagcgcaattagccattgggaagagtttctgcagatctttagctatgaattcgatctgctgtttgttggtgccgaaagccaggcaggttataatagcaataagaacctgtttgagagcctgatcaaaaaaaacgagaaagggtttagcatcagtccggaagaaaaactggtgatcaagaactttgttgataacaccctgtggatttatcagatggccaaatatttcgcgatcgaaaaaaagcgtaaatggctggaaagtgaatatccgaccgatagcagcttttatgatagcgaagaattcggcttcaaaaacaagttctatgatgacgcctatgataaaatcgtgaaactgcgtatgctgctgcagagccatctgacaaaaaaaccgtttagcaccgataaatggaagctgaactttgaaaatccgacactggcaaaaggttgggacaagaataaagaatcagataattcagcagtgctgctgcgtaaagaaggtcgttattatctggccgttatgaaaaaaggcaacaacaaaatcttcgatgacaagaacaaaagcaactttctggaaaacatcgaaggcggtaaatacgagaaaatggtttacaagcagatgagcgatccgagcaaagatattcagaatctgatggtgatcgacgataaaaccgttcgtaaagtgggtaaaaaagatccgctggatggtgtgaatcgtcgtctggaagaactgaagaaagagtatctgcctcgcgatatcaataccattcgtgaacagaaagcatacctgaaaagcagcgataatttcaatctgggtgatgccaacctgttcatcaactattacaaagatcgtctggtggaataccacaaagacatttttgtgtttagcttccgtgatcgctacagcgattttcatgattttagcaaacatgttgcggagcagacctatagcctgagctttgaagatattagcgagttctacatccaagagaaaaacaataacggcgaactgtttctgttcgagatccataataaagactggaacctggaaaaaaaaggtggcgatcgtaaaagcggtgccaaaaatctgcataccgtttattttgaatccctgttcagcaaagagaacgagaacaacaacttcagcattaaactgaatggtgaagccgagctgttctatcgtccgaaaaccgatgagcagaaactgggtaataagaatgatctgaaaggcaagatcgtgctgaacaaaaaacgttatgccgaaaacaaaacctttattcacattccgattacgctgaatcgtgttgcaagcgaaagcaaatactttaaccagaaactgaacgattttctggtgggcaatccggatattaacattattggcattgatcgcggtgagaaacacctgatctattatgcaggtattaatcaggcaggcgagtttctgaaggatgaaaaaggtaatctggtgctgggtagcctgaataccattaatgatgttaactacgcccaaaagttagaggaacgtgcaaaaggtcgtgttaaagcaaaacaggattggcaagaaatcgaaaacatcaaagatctgaaacgcggttatattagcctggttgttcgtgaactggcagatctgattatcaaacataacgccatcatcgtgtttgaggatctgaatatgcgttttaaacaaattcgcggtggcattgagaaaagcgtttatcagcagctggaaaaagccctgattgataaactgaacttcctggtgaacaaaggtgagaaagatccgaccaaagcaggtcatctgctgcgtgcatttcagctgaccgcaccgattagcgcatataaagacatgggtaaacagaccggtgtgattttctatacccaggcaagctataccagcaaaacctgtccggaatgtggttttcgtccgaatgttcgttgggaaccgaaaagtatcaaagataaaatcaaagaaggcaagctggaaatcacctacaaagaagatggtttcgagatcagctataaactgtccgatttttccaaaagccagaatcagagcaaacgtcgcaatattctgtatacgaatgtgagcaaacaggataaattcaacctgaacaccaaagatgccgttcgttgtaaatggtttcgtaaaacactgagcgaaaacgaactgaataagggcgaacagaagctgaatatccagacagaaaccggtgttaacatcgagtataaaatcagcgattgtctgatcggcctgtttgaaaaatacggtctggattatcagaacaacctgcaagaagagatcaaaaattcaggtgatagtctgccggtgaaattctatgataagctgagcttttatctgcatctgctgaccaatacacgtagcagcgttagcggcaccgatattgatcatatcaattgtccgaattgcggcttctgtagcaaaaatggctttaaaggcggtgaatttaatggtgatgcaaacggtgcatacaacattgcacgtaaaggtattatcatcctggacaagctgaagaactataaaaccgaaaatagcaaccttgaaaaaatgacctggggtgacctgtttattgatattgatgagtgggacaaatttacccagaacaagacctaatggtctagaggtcgaaattcaaattgtgagcggataacaatttgaattttctgtatgaggttttgctaaacaactttcaacagtttcagtggagtgagaatagaaaggaacaactaaaggaattgcgaataataattttttcacgttgaaaatctccaaaaaaaaaggctccaaaaggagcctttaattgtatcggtttatcagcttgctttcgaggtgaattttgaccctctagcgaaaatgcaagagcaaagacgaaaacatgccacacatgaggaataccgattctctcattaacatattcaggccagttatctgggcttaaaagcagaagtccaacccagataacgatcatatacatggttctctccagaggttcattactgaacactcgtccgagaataacgagtggatcccctccaattcgccctatagtgagtcgtattacgcgcgctcactggccgtcgttttacaacgtcgtgactgggaaaaccctggcgttacccaacttaatcgccttgcagcacatccccctttcgccagctggcgtaatagcgaagaggcccgcaccgatcgcccttcccaacagttgcgcagcctgaatggcgaatggaaattgtaagcgttaatattttgttaaaattcgcgttaaatttttgttaaatcagctcattttttaaccaataggccgactgcgatgagtggcagggcggggcgtaatttttttaaggcagttattggtgcccttaaacgcctggtgctacgcctgaataagtgataataagcggatgaatggcagaaattcgaaagcaaattcgacccggtcgtcggttcagggcagggtcgttaaatagccgcttatgtctattgctggtttaccggtttattgactaccggaagcagtgtgaccgtgtgcttctcaaatgcctgaggccagtttgctcaggctctccccgtggaggtaataattgacgatatgatcatttattctgcctcccagagcctgataaaaacggtgaatccgttagcgaggtgccgccggcttccattcaggtcgaggtggcccggctccatgcaccgcgacgcaacgcggggaggcagacaaggtatagggcggcgaggcggctacagccgatagtctggaacagcgcacttacgggttgctgcgcaacccaagtgctaccggcgcggcagcgtgacccgtgtcggcggctccaacggctcgccatcgtccagaaaacacggctcatcgggcatcggcaggcgctgctgcccgcgccgttcccattcctccgtttcggtcaaggctggcaggtctggttccatgcccggaatgccgggctggctgggcggctcctcgccggggccggtcggtagttgctgctcgcccggatacagggtcgggatgcggcgcaggtcgccatgccccaacagcgattcgtcctggtcgtcgtgatcaaccaccacggcggcactgaacaccgacaggcgcaactggtcgcggggctggccccacgccacgcggtcattgaccacgtaggccgacacggtgccggggccgttgagcttcacgacggagatccagcgctcggccaccaagtccttgactgcgtattggaccgtccgcaaagaacgtccgatgagcttggaaagtgtcttttggctgaccaccacggcgttctggtggcccatctgcgccacgaggtgatgcagcagcattgccgccgtgggtttcctcgcaataagcccggcccacgcctcatgcgctttgcgttccgtttgcacccagtgaccgggcttgttcttggcttgaatgccgatttctctggactgcgtgg

SEQ ID NO: 63 - DNA, 10486 bp, Artificial Sequence
  CRISPR/BMC12-Ec vector system
caatcggcgttaaacccgccaccagatgggcattaaacgagtatcccggcagcaggggatcattttgcgcttcagccatacttttcatactcccgccattcagagaagaaaccaattgtccatattgcatcagacattgccgtcactgcgtcttttactggctcttctcgctaaccaaaccggtaaccccgcttattaaaagcattctgtaacaaagcgggaccaaagccatgacaaaaacgcgtaacaaaagtgtctataatcacggcagaaaagtccacattgattatttgcacggcgtcacactttgctatgccatagcatttttatccataagattagcggatcctacctgacgctttttatcgcaactctctactgtttctccatacccgttttttggtaccgggccccccctcgagtttattttaggaggcaaaaatggaaaccaagaacaaaagcatctggggtgatttcaccaacaaatatagcctgagcaaaaccctgcgttttgaactggttccggttggtaaaacccgtgaaaatattcagaaacacaacccggaatttgtgcaggatcagaaaattgaagaagcctaccagattctgaaaagcgtgtttgataaaatccacgaggacttcattaccaagagcctggaaagtgatgaagccaaaagcattaacttcagcgagtatttcgacctgtacaaaaagtggaacgagctgaaaaagaaaaagaccaacgagaagaacatcgagatcaagaaagaaatccagaacgagatcgagaagatctacaaagataatggtggtagcaaaggcgagatccagaaaatcgaggatgaactgcgtaaacgctttgaagaaatctttaaaatccagggcaaaatcttcaaagagaaagcctgcgaactgaacattaaagaaggtcaagagaaagacgacgacgaggaaaaagacgataataagaaaggttttcgcaaactgctgaaagccaaattcctgtatgattatctgtgcaacctgatcgagagcaaaaacatcatctacaaggatttcttcgagaacatcaaaaacaaagaaggcgagagcatcagcaaagaaaagacaaaagatgccctgattcgctttaaaggctttaccacctattttggtggctttgaactgaatcgcctgaactattataccaccaaagaagagaaaagcaccgcagttgcaacccgtattgttaatcagaacctgccgaaattttgcgataacgtgattctgtttgaaatcaaaaagagcgaatatctgaaaatcgatgaattcctgaaaaacaagaacatcagcctgatcagcaaaaatcagaatggtggtgaagtggaactgcacaaaatcaacaaaaactttttcgagatgatgttctttagcaagtgcctgagccagaaagagattcagaaatataacctggaaattggcaatgccaacaacctgattaatcgctataatcagcagcagagcgataaaagccagaaactgaaactgtttaaaacgctgcataagcagattggttgtggtgatcgtggtggttttattccgagcattaaaggtgaagaagatctgcgcgaacgtctgcaagaaattaagaataacagcatcgaatactttgaaaacatcaacgacttcatcgagtacctgaaaaatcacgagaactacgaaaatgtgtattggagcgacaaagccattaataccattagcagcaaatatttcagcgactggctgaacctgaagaaagaaatttggggtaaacgtgatcgcaaaggcaatctgaaagatgaagaaaccaaaattccgcgtgcagtgcagctgaaagatctgctggaaaatctggataaaatcaccgattggaaactggaaggtcgtctgtttaaactgagcctgtttgagaatggtcgtaaagccaaaaagctgcagcaagaggatctgaacaaattcaataaaaacaaaatcgaaaacgagctggaaatcgagaaactgcagattattgaacagaatccgagtccgtttcaggcactgctgaatatgatctttgcagacattaaatccaaagagagcgcatttctggaaagccgcatttttgaaattagcgatttcgtgcacaacgaggacaagcagatcattaaacagtggctggatagcattctggccattaaccagattatcaaatactggcgtgtgaaagatacctttggcaccgaaggcaccctggatgaaaaactgaaaaatatcatttatagcgagaaaaacccgacgcgcttttatgatattattcgcaattacctgaccaagaaaccgcaggatgagctgaataaactgaagctgaattttgagaatagcaccctggcacaaggtctggatgttaataaagaaaaggataacttttgcattatcctgcgcgacgataaacagaaccagtatctgggtattctgaacagcaagaataagaacatcttcgagatcgatcagaacgaggatatctatcaggatgatggtttaggttggagcaagatgatgtataaactgattccgggtgcaagcaaaacactgccgaaaatctttttctcaaaacgctggaccgaaaataatccgacaccggatgaaatcagcaagattaaaaagggcgaaaccttcaagaaaggcgacaatttcattaaacgcgatctgcatgaactgatcaacttctataaagccaaccttgagaaatatccgagcgttaatgaaagctgggcaaaactgttcatcttcaactttagcgataccaaaacctatgagagcatcgatcagttttataacgaggtggataaacagggctataaggtgagctttatcagcatcaataagaataccctggacaactttatcgacaaagagaagctgtacctgtttcagattaagaacaaggacaacaatctggacaaaggcgaaaagaaacagagcaacaaaaatctgcatagcatctattgggaagccatttttggtaaagcactgaacaaaccgaaactgaatggtggcgcagaaattttctatcgtccggcactgagtgaaaagaaaattagtgaactgaaaatcaaagataaaaacggcaagaacattatcatcattaaaaactatcgctatagcaaagacaaattcatttttcactgcccgatcacgctgaactttagtgcaaaaagtagcaaactgaacgacgagatcaacgatcatatcaagaacaagaaagaattttgctttatgggcatcgatcgcggtgaaaaacatctggcatattatagcctggtgaatcagaacggcaaaatccttgataaaggtcagggcaccctgaatctgccgtttgttgataaagatggtaacaagcgttgcatcaaaaccgagaaatacttcgaagaggataagaaagaaaacgaaaagtggaaaccgcgtattattgattgtccggattataactgtctgctggatgcacgtgccagcaatcgtgatctggcacgcaaaaattggcagaccattggtacaatcaaagaactgaaagaaggctatatcagccaggtggttcgtaaaattgttgatctggcgattgaaaacaacgcctttattgttctggaaaacctgaacattggttttaaacgtggtcgccagaagatcgaaaaacaggtttatcagaagctggaactggcactggcacgtaaactgaattttctggttgataaaaaggccatcattggtgaagttggtagcgttaccaaagcactgcagctgacccctccggttaataactttggtgatattggtggcaaaagccagtttggcattatgttttataccaaagcggattacaccagccagaccgatccggttaccggttggcgtaaaagcatttatctgaaacgcggtccggaagattacatcaaagatcagatcctgggtaacaaaaacaaaaacattgaaccggcatttgaggacatttgctttgatggtcaggattattgcttcacctacattaacaaaaataccggcaagaaatggaccctgtacagcagtaaaaatggtaaaagcctggatcgctatcatcgtgaactggtgtatgaaaacagcgataagaaatggctgccgaagaaacaggatgtgctggaaatgctgaataacctgtttgaaggcttcgacaagaaaaagtctctgctgaaacagcttgaaacgaagaatccgaataaaacaggtgaacatccggcatgggaaagtctgcgctttaccattgatctgattcagcagattcgtaacaccgggattaaagaacgtgatgaggatttcattctgagtccggttcgtgacaaaaagggtgatcattttgatagccgtgaagcaagtccggatctgccgaatagcggtgatgcaaatggtgcatacaatattgcacgcaagggcattattatggccaaacatatcgaaaaaggctactttctgtatatcagcgacgaagaatgggatgcatggctggcaggcgaagaatgttggaatcgttgggctgagaaaaataccaaaagcctgctgaagaacaactattaatggtctagaggtcgaaattcaaattgtgagcggataacaatttgaattttctgtatgaggttttgctaaacaactttcaacagtttcagtggagtgagaatagaaaggaacaactaaaggaattgcgaataataattttttcacgttgaaaatctccaaaaaaaaaggctccaaaaggagcctttaattgtatcggtttatcagcttgctttcgaggtgaattttgaccctctagcgaaaatgcaagagcaaagacgaaaacatgccacacatgaggaataccgattctctcattaacatattcaggccagttatctgggcttaaaagcagaagtccaacccagataacgatcatatacatggttctctccagaggttcattactgaacactcgtccgagaataacgagtggatcccctccaattcgccctatagtgagtcgtattacgcgcgctcactggccgtcgttttacaacgtcgtgactgggaaaaccctggcgttacccaacttaatcgccttgcagcacatccccctttcgccagctggcgtaatagcgaagaggcccgcaccgatcgcccttcccaacagttgcgcagcctgaatggcgaatggaaattgtaagcgttaatattttgttaaaattcgcgttaaatttttgttaaatcagctcattttttaaccaataggccgactgcgatgagtggcagggcggggcgtaatttttttaaggcagttattggtgcccttaaacgcctggtgctacgcctgaataagtgataataagcggatgaatggcagaaattcgaaagcaaattcgacccggtcgtcggttcagggcagggtcgttaaatagccgcttatgtctattgctggtttaccggtttattgactaccggaagcagtgtgaccgtgtgcttctcaaatgcctgaggccagtttgctcaggctctccccgtggaggtaataattgacgatatgatcatttattctgcctcccagagcctgataaaaacggtgaatccgttagcgaggtgccgccggcttccattcaggtcgaggtggcccggctccatgcaccgcgacgcaacgcggggaggcagacaaggtatagggcggcgaggcggctacagccgatagtctggaacagcgcacttacgggttgctgcgcaacccaagtgctaccggcgcggcagcgtgacccgtgtcggcggctccaacggctcgccatcgtccagaaaacacggctcatcgggcatcggcaggcgctgctgcccgcgccgttcccattcctccgtttcggtcaaggctggcaggtctggttccatgcccggaatgccgggctggctgggcggctcctcgccggggccggtcggtagttgctgctcgcccggatacagggtcgggatgcggcgcaggtcgccatgccccaacagcgattcgtcctggtcgtcgtgatcaaccaccacggcggcactgaacaccgacaggcgcaactggtcgcggggctggccccacgccacgcggtcattgaccacgtaggccgacacggtgccggggccgttgagcttcacgacggagatccagcgctcggccaccaagtccttgactgcgtattggaccgtccgcaaagaacgtccgatgagcttggaaagtgtcttttggctgaccaccacggcgttctggtggcccatctgcgccacgaggtgatgcagcagcattgccgccgtgggtttcctcgcaataagcccggcccacgcctcatgcgctttgcgttccgtttgcacccagtgaccgggcttgttcttggcttgaatgccgatttctctggactgcgtggccatgcttatctccatgcggtagggtgccgcacggttgcggcaccatgcgcaatcagctgcaacttttcggcagcgcgacaacaattatgcgttgcgtaaaagtggcagtcaattacagattttctttaacctacgcaatgagctattgcggggggtgccgcaatgagctgttgcgtaccccccttttttaagttgttgatttttaagtctttcgcatttcgccctatatctagttctttggtgcccaaagaagggcacccctgcggggttcccccacgccttcggcgcggctccccctccggcaaaaagtggcccctccggggcttgttgatcgactgcgcggccttcggccttgcccaaggtggcgctgcccccttggaacccccgcactcgccgccgtgaggctcggggggcaggcgggcgggcttcgccttcgactgcccccactcgcataggcttgggtcgttccaggcgcgtcaaggccaagccgctgcgcggtcgctgcgcgagccttgacccgccttccacttggtgtccaaccggcaagcgaagcgcgcaggccgcaggccggaggcttttccccagagaaaattaaaaaaattgatggggcaaggccgcaggccgcgcagttggagccggtgggtatgtggtcgaaggctgggtagccggtgggcaatccctgtggtcaagctcgtgggcaggcgcagcctgtccatcagcttgtccagcagggttgtccacgggccgagcgaagcgagccagccggtggccgctcgcggccatcgtccacatatccacgggctggcaagggagcgcagcgaccgcgcagggcgaagcccggagagcaagcccgtagggcgccgcagccgccgtaggcggtcacgactttgcgaagcaaagtctagtgagtatactcaagcattgagtggcccgccggaggcaccgccttgcgctgcccccgtcgagccggttggacaccaaaagggaggggcaggcatggcggcatacgcgatcatgcgatgcaagaagctggcgaaaatgggcaacgtggcggccagtctcaagcacgcctaccgcgagcgcgagacgcccaacgctgacgccagcaggacgccagagaacgagcactgggcggccagcagcaccgatgaagcgatgggccgactgcgcgagttgctgccagagaagcggcgcaaggacgctgtgttggcggtcgagtacgtcatgacggccagcccggaatggtggaagtcggccagccaagaacagcaggcggcgttcttcgagaaggcgcacaagtggctggcggacaagtacggggcggatcgcatcgtgacggccagcatccaccgtgacgaaaccagcccgcacatgaccgcgttcgtggtgccgctgacgcaggacggcaggctgtcggccaaggagttcatcggcaacaaagcgcagatgacccgcgaccagaccacgtttgcggccgctgtggccgatctagggctgcaacggggcatcgagggcagcaaggcacgtcacacgcgcattcaggcgttctacgaggccctggagcggccaccagtgggccacgtcaccatcagcccgcaagcggtcgagccacgcgcctatgcaccgcagggattggccgaaaagctgggaatctcaaagcgcgttgagacgccggaagccgtggccgaccggctgacaaaagcggttcggcaggggtatgagcctgccctacaggccgccgcaggagcgcgtgagatgcgcaagaaggccgatcaagcccaagagacggcccgagaccttcgggagcgcctgaagcccgttctggacgccctggggccgttgaatcgggatatgcaggccaaggccgccgcgatcatcaaggccgtgggcgaaaagctgctgacggaacagcgggaagtccagcgccagaaacaggcccagcgccagcaggaacgcgggcgcgcacatttccccgaaaagtgccacctgaaccccagagtcccgctcagaagaactcgtcaagaaggcgatagaaggcgatgcgctgcgaatcgggagcggcgataccgtaaagcacgaggaagcggtcagcccattcgccgccaagctcttcagcaatatcacgggtagccaacgctatgtcctgatagcggtccgccacacccagccggccacagtcgatgaatccagaaaagcggccattttccaccatgatattcggcaagcaggcatcgccatgggtcacgacgagatcctcgccgtcgggcatccgcgccttgagcctggcgaacagttcggctggcgcgagcccctgatgctcttcgtccagatcatcctgatcgacaagaccggcttccatccgagtacgtgctcgctcgatgcgatgtttcgcttggtggtcgaatgggcaggtagccggatcaagcgtatgcagccgccgcattgcatcagccatgatggatactttctcggcaggagcaaggtgagatgacaggagatcctgccccggcacttcgcccaatagcagccagtcccttcccgcttcagtgacaacgtcgagcacagctgcgcaaggaacgcccgtcgtggccagccacgatagccgcgctgcctcgtcttggagttcattcagggcaccggacaggtcggtcttgacaaaaagaaccgggcgcccctgcgctgacagccggaacacggcggcatcagagcagccgattgtctgttgtgcccagtcatagccgaatagcctctccacccaagcggccggagaacctgcgtgcaatccatcttgttcaatcatgcgaaacgatcctcatcctgtctcttgatcagatcttgatcccctgcgccatcagatccttggcggcaagaaagccatccagtttactttgcagggcttcccaaccttaccagagggcgccccagctggcaattccggttcgcttgctgtccataaaaccgcccagtctagctatcgccatgtaagcccactgcaagctacctgctttctctttgcgcttgcgttttcccttgtccagatagcccagtagctgacattcatccggggtcagcaccgtttctgcggactggctttctacgtgttccgcttcctttagcagcccttgcgccctgagtgcttgcggcagcgtgaagctagctgcataatgtgcctgtcaaatggacgaagcagggattctgcaaaccctatgctactccgtcaagccgtcaattgtctgattcgttaccaattatgacaacttgacggctacatcattcactttttcttcacaaccggcacggaactcgctcgggctggccccggtgcattttttaaatacccgcgagaaatagagttgatcgtcaaaaccaacattgcgaccgacggtggcgataggcatccgggtggtgctcaaaagcagcttcgcctggctgatacgttggtcctcgcgccagcttaagacgctaatccctaactgctggcggaaaagatgtgacagacgcgacggcgacaagcaaacatgctgtgcgacgctggcgatatcaaaattgctgtctgccaggtgatcgctgatgtactgacaagcctcgcgtacccgattatccatcggtggatggagcgactcgttaatcgcttccatgcgccgcagtaacaattgctcaagcagatttatcgccagcagctccgaatagcgcccttccccttgcccggcgttaatgatttgcccaaacaggtcgctgaaatgcggctggtgcgcttcatccgggcgaaagaaccccgtattggcaaatattgacggccagttaagccattcatgccagtaggcgcgcggacgaaagtaaacccactggtgataccattcgcgagcctccggatgacgaccgtagtgatgaatctctcctggcgggaacagcaaaatatcacccggtcggcaaacaaattctcgtccctgatttttcaccaccccctgaccgcgaatggtgagattgagaatataacctttcattcccagcggtcggtcgataaaaaaatcgagataaccgttggcct

SEQ ID NO: 64 - DNA, 10261 bp, Artificial Sequence
  CRISPR/BMC14-Ec vector system
caatcggcgttaaacccgccaccagatgggcattaaacgagtatcccggcagcaggggatcattttgcgcttcagccatacttttcatactcccgccattcagagaagaaaccaattgtccatattgcatcagacattgccgtcactgcgtcttttactggctcttctcgctaaccaaaccggtaaccccgcttattaaaagcattctgtaacaaagcgggaccaaagccatgacaaaaacgcgtaacaaaagtgtctataatcacggcagaaaagtccacattgattatttgcacggcgtcacactttgctatgccatagcatttttatccataagattagcggatcctacctgacgctttttatcgcaactctctactgtttctccatacccgttttttggtaccgggccccccctcgagtttattttaggaggcaaaaatgagccagaacaacatcaaagaaaagagcatctttgacgaatttaccaacaaatatagcctgcagaaaaccctgcgttttgaactgcgtccggttctgaataccgagcagatgctgaccgatagcggtattatcaaactggatgaaaaacgcaaactgaactatgagaaaaccaaaccgtttctgaatcgcctgcatcaagaatttgttaccgaaagcctgaatggtgttcgtctgaaaagtctggatggttatgcagttctgtatgccaattggaagaaaagcatcgataagaaagaaaaggacgcagcctataaagtgctggaaaagaaagaactggaaatccgccaagaaattgtggtgctgtttgatgaaaaagccgttgaatggattggtaaactgcctgcagatgttaaaaagccgaagaaaccgaattatgaattcctgtttgaaccggcaattttcagcatcctgaagaaaaagtatagtgatgaagttggcaccaccattgatgaggaaagcatttttgatagctgggataaatggaccgcctattttggcaaatttttcgaaacccgcaagaacttctataaaagtgatggtaaagcaaccgcagttgcaacccgtattgttaatgaaaatctgcgtcgcttttgtgatgatgtgagcacctttgaaaacatccagagcaaaattgatctgagtccgctggaaaaagaattcgatgttagcctgaaaaaggtgttcgatatccagcattataatcagtgtctgaatcagagcggtatcgatgcatttaataccctgttaggtggtgaagtgcatgaaaatggtgagaaaatcaaaggcatcaacgagtatatcaacgaacatcgtcagaaaaccggtgaaaaactgacccgtctgaagaaactggataaacaaattggcagcgacaaagagaacttcatcgatctgattgaaaccgatgaacagctgaaaaccacactggttacctttattgcaaacgccaaagagaaagttgatctgctggataaaagcgttagctatctgaccaaagataccgatgttaaactgagcggtattttctttcgcaaagaagccattaataccattacgcgtcgttggtttgttagccacgagaaaattagtgatgcactggttagcgcattcagcgataaaaacgttaaattcgatcagaagcgcgaagagtataaattcccggattttatcagctggcatgtgattcagaatgcagtggaaaaactggcatcagatggtgaagaaatttggaagaagtattatctggaagaagagaaactgagcctgctggacaaaaccccgtggcagcagtttctgaccgtttttgaatgtgaatacaacaacctgaaaagcaaaggccatgaaagcgaaggtcgtagctttaccgaactggttcaggatattgaaagtctgctgaaaacggataccctggatcgtaatgatcatgtgaccgaaatcatcaaaagctttagcgatcgtgtgctgaacatttatcgtttcgcaaaatacttcgccctggataaatcatgccagtggaatccggatggtctggatacagatgatttttatgttgcctatgaacagttctatagcgacggctatgaaaagatcgtgaaagtgtatgataaagtgcgcaactacatgaccaagaaaccgtttaatcaggacaaatggaagctgaattttgaaaatccgacactggcaaatggttgggacaaaaacaaagaaacagacaacaccgcaattattctgcgtcgtgcaggtcgttattacctggcagttatggaacgtggtcataatacgctgtttaaaaagattccgatgagcagcagcggttatcagaaaatgacctataaactgtttccggatccgagtaaaatgatgccgaaagtttgttttagcaagaagggccttgaattctttaaaccgagcgcagaaatcatgcgcatttacaaaaatggcgaattcaaaaagggcgatacctttagcctgagcagcatgcatgttctgattgacttttataagaacgccctgaaaacctatgatggctggaccatgtatgatttcagcaatctgaaaaagaccagcgagtataccgaaaacatcggcgaattttatcgtgatgttgcagaaagcggctaccagattaactttgattatatcgccgaacagtatatcgaggatgccaataaagaaggtaaactgtacctgtttgagatccacaacaaagactggaatctgaaagatggtgcaattaaaaccggtagcaaaaatgcacacaccctgtattttgaacaggtgttttcagatgaaaacgcgcagaacaattttgtggtgaaactgaatggcgaagccgaactgtttttccgtccggcaaccagcaccgagaaactgggtaatcattatgatagcaaaggtaacgtggtgaccaaaaataagcgttatgcccatgacaaaatgttctttcatgttccggttacactgaatcgtaccgcaccggatgcacgcaaatttaaccagagcgttaatgtttttctggcgaataatccggataccaacattattggtattgaccgtggcgaaaaacatctggcatatctgagcgttattaaccagaaaggtgacatcctgaaaatcaagagcctgaacaaaatcgaggtgaaagataaagatggcaacgtgatcaaagaagatgattacgcaaaactgctggaagatcgtgccaaaaatcgtgaatcagcacgtcgtgattggaaaagcgttgagcagattaaagatcttaaaaagggctacattagcaacgtggttcgtgaaattgcagatctggtgattaaatacaatgccatcgtggtgtttgaggatctgaatatgcgctttaaacaggttcgtggtggcattgaaaaatcggtttatcagcagttagaaaaggccctgattgataagctgaacttcctggtggataaaaatgaactggatccgcagaaagcaggtcatattctgcatgcatatcagctgaccgcaccgtttgaaacctttaaagatatgggtaaacagaccggtgtgctgttttatacccaggcagaatacaccagccagacagatccggttaccggctttcgtaaaaatgtttatctgagcaatagcgccaccgtggaaaagattaaagcctttgttgaaatgttcgatgtgatcggctgggacgataaactgaaaagctattatttcaagtataacccggtgaacttcgtggaaaccaagtttaaagagaacaccttcagcaaagattgggtgatttatgcaaatgtgcctcgcattaaacgcgaacgcaaaaatggttattgggaagcaaccgttgttaacccgaatgaagaatttctgaagctgttcaaagagtgggatttcgataacatctacgtcgaggacattaaagaacaaattttccagatgttcgaagagggtcgcctggatggcaccaaagaatttgatggcaaaaaccgcaacttttggcacagcttcatttttctgtttaacctgatgctgcaggttcgtaatagcaccgcaacacagtataaaaaggatgaggatggcaacattatcgaaaccgttgaaggtgtggattttattgccagtccggtgtttccgttctttaccaccgatggtggtgattttaccgaaggttgtgtgaatctggcaaaactggaagataaatttgtgggtagcaacgccgataaagaacgcttcaagaaagagtttaatggtgatgcaaatggtgcgtataatatcgcacgtaaaggcattattatgctgaacaatatcaaaaacaaccccgaaaaaccggacctgtttgtgagcaaaaaggattgggataagtttgcacaggccaaccagtaatggtctagaggtcgaaattcaaattgtgagcggataacaatttgaattttctgtatgaggttttgctaaacaactttcaacagtttcagtggagtgagaatagaaaggaacaactaaaggaattgcgaataataattttttcacgttgaaaatctccaaaaaaaaaggctccaaaaggagcctttaattgtatcggtttatcagcttgctttcgaggtgaattttgaccctctagcgaaaatgcaagagcaaagacgaaaacatgccacacatgaggaataccgattctctcattaacatattcaggccagttatctgggcttaaaagcagaagtccaacccagataacgatcatatacatggttctctccagaggttcattactgaacactcgtccgagaataacgagtggatcccctccaattcgccctatagtgagtcgtattacgcgcgctcactggccgtcgttttacaacgtcgtgactgggaaaaccctggcgttacccaacttaatcgccttgcagcacatccccctttcgccagctggcgtaatagcgaagaggcccgcaccgatcgcccttcccaacagttgcgcagcctgaatggcgaatggaaattgtaagcgttaatattttgttaaaattcgcgttaaatttttgttaaatcagctcattttttaaccaataggccgactgcgatgagtggcagggcggggcgtaatttttttaaggcagttattggtgcccttaaacgcctggtgctacgcctgaataagtgataataagcggatgaatggcagaaattcgaaagcaaattcgacccggtcgtcggttcagggcagggtcgttaaatagccgcttatgtctattgctggtttaccggtttattgactaccggaagcagtgtgaccgtgtgcttctcaaatgcctgaggccagtttgctcaggctctccccgtggaggtaataattgacgatatgatcatttattctgcctcccagagcctgataaaaacggtgaatccgttagcgaggtgccgccggcttccattcaggtcgaggtggcccggctccatgcaccgcgacgcaacgcggggaggcagacaaggtatagggcggcgaggcggctacagccgatagtctggaacagcgcacttacgggttgctgcgcaacccaagtgctaccggcgcggcagcgtgacccgtgtcggcggctccaacggctcgccatcgtccagaaaacacggctcatcgggcatcggcaggcgctgctgcccgcgccgttcccattcctccgtttcggtcaaggctggcaggtctggttccatgcccggaatgccgggctggctgggcggctcctcgccggggccggtcggtagttgctgctcgcccggatacagggtcgggatgcggcgcaggtcgccatgccccaacagcgattcgtcctggtcgtcgtgatcaaccaccacggcggcactgaacaccgacaggcgcaactggtcgcggggctggccccacgccacgcggtcattgaccacgtaggccgacacggtgccggggccgttgagcttcacgacggagatccagcgctcggccaccaagtccttgactgcgtattggaccgtccgcaaagaacgtccgatgagcttggaaagtgtcttttggctgaccaccacggcgttctggtggcccatctgcgccacgaggtgatgcagcagcattgccgccgtgggtttcctcgcaataagcccggcccacgcctcatgcgctttgcgttccgtttgcacccagtgaccgggcttgttcttggcttgaatgccgatttctctggactgcgtggccatgcttatctccatgcggtagggtgccgcacggttgcggcaccatgcgcaatcagctgcaacttttcggcagcgcgacaacaattatgcgttgcgtaaaagtggcagtcaattacagattttctttaacctacgcaatgagctattgcggggggtgccgcaatgagctgttgcgtaccccccttttttaagttgttgatttttaagtctttcgcatttcgccctatatctagttctttggtgcccaaagaagggcacccctgcggggttcccccacgccttcggcgcggctccccctccggcaaaaagtggcccctccggggcttgttgatcgactgcgcggccttcggccttgcccaaggtggcgctgcccccttggaacccccgcactcgccgccgtgaggctcggggggcaggcgggcgggcttcgccttcgactgcccccactcgcataggcttgggtcgttccaggcgcgtcaaggccaagccgctgcgcggtcgctgcgcgagccttgacccgccttccacttggtgtccaaccggcaagcgaagcgcgcaggccgcaggccggaggcttttccccagagaaaattaaaaaaattgatggggcaaggccgcaggccgcgcagttggagccggtgggtatgtggtcgaaggctgggtagccggtgggcaatccctgtggtcaagctcgtgggcaggcgcagcctgtccatcagcttgtccagcagggttgtccacgggccgagcgaagcgagccagccggtggccgctcgcggccatcgtccacatatccacgggctggcaagggagcgcagcgaccgcgcagggcgaagcccggagagcaagcccgtagggcgccgcagccgccgtaggcggtcacgactttgcgaagcaaagtctagtgagtatactcaagcattgagtggcccgccggaggcaccgccttgcgctgcccccgtcgagccggttggacaccaaaagggaggggcaggcatggcggcatacgcgatcatgcgatgcaagaagctggcgaaaatgggcaacgtggcggccagtctcaagcacgcctaccgcgagcgcgagacgcccaacgctgacgccagcaggacgccagagaacgagcactgggcggccagcagcaccgatgaagcgatgggccgactgcgcgagttgctgccagagaagcggcgcaaggacgctgtgttggcggtcgagtacgtcatgacggccagcccggaatggtggaagtcggccagccaagaacagcaggcggcgttcttcgagaaggcgcacaagtggctggcggacaagtacggggcggatcgcatcgtgacggccagcatccaccgtgacgaaaccagcccgcacatgaccgcgttcgtggtgccgctgacgcaggacggcaggctgtcggccaaggagttcatcggcaacaaagcgcagatgacccgcgaccagaccacgtttgcggccgctgtggccgatctagggctgcaacggggcatcgagggcagcaaggcacgtcacacgcgcattcaggcgttctacgaggccctggagcggccaccagtgggccacgtcaccatcagcccgcaagcggtcgagccacgcgcctatgcaccgcagggattggccgaaaagctgggaatctcaaagcgcgttgagacgccggaagccgtggccgaccggctgacaaaagcggttcggcaggggtatgagcctgccctacaggccgccgcaggagcgcgtgagatgcgcaagaaggccgatcaagcccaagagacggcccgagaccttcgggagcgcctgaagcccgttctggacgccctggggccgttgaatcgggatatgcaggccaaggccgccgcgatcatcaaggccgtgggcgaaaagctgctgacggaacagcgggaagtccagcgccagaaacaggcccagcgccagcaggaacgcgggcgcgcacatttccccgaaaagtgccacctgaaccccagagtcccgctcagaagaactcgtcaagaaggcgatagaaggcgatgcgctgcgaatcgggagcggcgataccgtaaagcacgaggaagcggtcagcccattcgccgccaagctcttcagcaatatcacgggtagccaacgctatgtcctgatagcggtccgccacacccagccggccacagtcgatgaatccagaaaagcggccattttccaccatgatattcggcaagcaggcatcgccatgggtcacgacgagatcctcgccgtcgggcatccgcgccttgagcctggcgaacagttcggctggcgcgagcccctgatgctcttcgtccagatcatcctgatcgacaagaccggcttccatccgagtacgtgctcgctcgatgcgatgtttcgcttggtggtcgaatgggcaggtagccggatcaagcgtatgcagccgccgcattgcatcagccatgatggatactttctcggcaggagcaaggtgagatgacaggagatcctgccccggcacttcgcccaatagcagccagtcccttcccgcttcagtgacaacgtcgagcacagctgcgcaaggaacgcccgtcgtggccagccacgatagccgcgctgcctcgtcttggagttcattcagggcaccggacaggtcggtcttgacaaaaagaaccgggcgcccctgcgctgacagccggaacacggcggcatcagagcagccgattgtctgttgtgcccagtcatagccgaatagcctctccacccaagcggccggagaacctgcgtgcaatccatcttgttcaatcatgcgaaacgatcctcatcctgtctcttgatcagatcttgatcccctgcgccatcagatccttggcggcaagaaagccatccagtttactttgcagggcttcccaaccttaccagagggcgccccagctggcaattccggttcgcttgctgtccataaaaccgcccagtctagctatcgccatgtaagcccactgcaagctacctgctttctctttgcgcttgcgttttcccttgtccagatagcccagtagctgacattcatccggggtcagcaccgtttctgcggactggctttctacgtgttccgcttcctttagcagcccttgcgccctgagtgcttgcggcagcgtgaagctagctgcataatgtgcctgtcaaatggacgaagcagggattctgcaaaccctatgctactccgtcaagccgtcaattgtctgattcgttaccaattatgacaacttgacggctacatcattcactttttcttcacaaccggcacggaactcgctcgggctggccccggtgcattttttaaatacccgcgagaaatagagttgatcgtcaaaaccaacattgcgaccgacggtggcgataggcatccgggtggtgctcaaaagcagcttcgcctggctgatacgttggtcctcgcgccagcttaagacgctaatccctaactgctggcggaaaagatgtgacagacgcgacggcgacaagcaaacatgctgtgcgacgctggcgatatcaaaattgctgtctgccaggtgatcgctgatgtactgacaagcctcgcgtacccgattatccatcggtggatggagcgactcgttaatcgcttccatgcgccgcagtaacaattgctcaagcagatttatcgccagcagctccgaatagcgcccttccccttgcccggcgttaatgatttgcccaaacaggtcgctgaaatgcggctggtgcgcttcatccgggcgaaagaaccccgtattggcaaatattgacggccagttaagccattcatgccagtaggcgcgcggacgaaagtaaacccactggtgataccattcgcgagcctccggatgacgaccgtagtgatgaatctctcctggcgggaacagcaaaatatcacccggtcggcaaacaaattctcgtccctgatttttcaccaccccctgaccgcgaatggtgagattgagaatataacctttcattcccagcggtcggtcgataaaaaaatcgagataaccgttggcct

SEQ ID NO: 65 - DNA, 10156 bp, Artificial Sequence
  CRISPR/BMC15-Ec vector system
caatcggcgttaaacccgccaccagatgggcattaaacgagtatcccggcagcaggggatcattttgcgcttcagccatacttttcatactcccgccattcagagaagaaaccaattgtccatattgcatcagacattgccgtcactgcgtcttttactggctcttctcgctaaccaaaccggtaaccccgcttattaaaagcattctgtaacaaagcgggaccaaagccatgacaaaaacgcgtaacaaaagtgtctataatcacggcagaaaagtccacattgattatttgcacggcgtcacactttgctatgccatagcatttttatccataagattagcggatcctacctgacgctttttatcgcaactctctactgtttctccatacccgttttttggtaccgggccccccctcgagtttattttaggaggcaaaaatgaatccgacacagaccgataaaaccccgagcaaaccgtttgaaaaattcaccaatctgtactgcctgagcaaaaccctgcgttttgaactgaaaccgattggtaaaacccagaagattctggaagataacaaagtgttcgagaacgataaaaagcgtgccaaaagctatgaagaggccaaaaagtatttcaacaaactgcaccgcgaatttatcgatgaaagcctgaaaaacattaccctgagcaacaatctgatcgagaaattcgagaaaaagtacctgacctggaaaaacagcaaaaacaaagataatagcaccgagctgaaaaagagcgcaaaacgtctgcgtattgttatcctggaaagctttaataagaaagccaacgaatggaacagcgagtatagcaatcaggtgaaaaacgagaagaagaaaaagaaaatccaagaaatcaccggcatcgacctgtttttcaaagttgaagtgtttgacttcctgatccacaaatatccggaagtgcagattaatggcgaaagcatttttagcccgttcaacaaatttagcggctacttcaaaaagtttcacgaaacccgcaaaaacttctataaagatgatggcaccagcaccgcaattccgacacgtattattgatgtgaatctggaaaagtttctggaaaacaaggacatctactataccaaatactttcagaaatacaacagcatcttcaacaaagaagaaaccgacatcttcaaactggaatccttcaaaaattgtctgacccagagccagatcgacaaatacaatgaaagcattgcaaccctgaaaagcaagattaataacctgcgtcagaataacccggaagtgaataaacatgatctgccgttcttcaaagaactgtttcgtcagattctgggccagccgattaagaaagaaacagaacaggataacttcatcgagatcctgaccaatgatgaagtttttccggtgctgcagaaaaacatcgatgagaacgaactgtatattccgaaagcagataccctgtttaaagagtttctgaaatcccagatccaagagacaaacgagtataacatcaacgaaatttatgtggccagccgctttattaacagcattagcaataattggtttgccgagtgggataccattattaacctgctgcgtaccgaactgaaaatcaaacagaatcagaaaaagctgccggattttatcagcattgccagtctgaaacgtgtactgcagaaatcacaggatgaaattgatgccaaagacctgttccgcaacaattatgaaaacctgtttgaatccaccaccgacttctacaaaatcttcctgaaaatctgggagcttgagttcaacgacaacatcaaaaagtacaacctggaaaccgaaaacatccgcaaaatcatcatcgaggataaaaagtatctgccgaacaagaaaagcatcctgaaaaatggtgaaaccggcattatccacaacgagaaaattctggattatgcacagagcgcactgaacatttatcagatgatgaaatacttcagcctggaaaagggtaaagaacgtgaatggaatccggatggtctgaatgaagataccacaggtggtttttatgacgatttcaataaatactaccagaatgtgaacacctggaagtattttaacgaattccgcaactacctgaccaaaaagccgtataaaaccgacaaaatcaagctgtattttggccacaaaagcctgttaggtggctttaccgaaagcaaaacggaaaaatcaaataacggcacccagtatggtgcatatctgctgcgcaaaaagcatggtttaggcggttttgattattatctgggtattagcaccgatccgcatctgatgagctattttgatccgattgatgatagcggtgatagcgaatatgaacgcctgaactattatcaggttctgacccgtaccatttatggtccgagttatgaaggtgattatgagctggataagaaaaacctgagcgaaatcgaaatcatcaagaagattaaacgcagcctgtcctattataccagccgtgttaaaaagatccaggacatcatcaacaacaactatgaatcagtgcgcgatatccacaaagatattaccgatgtgctgaaagaattcggcaccatctttgattataaggtgatcacgaatagccagatccagaaagcctttaattgcgacaaaggcttttacctgttcgagatctatagcaaggattttagcaaagagaaaggcgacaagagcaagaacagtaaagataatctgcataccacctacttcaagagcctgatggatcgtaaacagagcacctttgatttaggtagcggtgaaattttctttcgcgagaaaagcgttcagagcgaaattgatagcatgcgcaaaaccaaaaacaagatcacccgttttaaacgctacaccaaaaatctgatccagttcaatctgagcatcacgctgaataataactgtaccgaagttccgcagaataaaaacgcacgtaaagcgtttatcaacaacttcaatatcgagctgagcaagaaactgctgaccaataatagcgatattaacattattggcatcgatcgcggtgagaaacatctggcatattatagcgtgattgatcagcagagcaatattctggaaacaggcagctttaacaaaattcaagaacgcaaagatcgtgagccgaccgattatcaacagaaactggataaaattcagaaagatcgcgattggcagcgtaaaagttggcaagaaattagcaacatcaaggacctgaaaaagggctatattagccaggtggtgtatgaaattagtaaactggtgaagaagtataacgccatcatcgtttttgaggatctgaacattggctttaaacgtggtcgttttgcaattgagaaacaggtgtatcaaaatctggaactgagcctggcaaagaaactgaattatctggttttcaaagatgccaacgaaggtgaaagtggccattatctgaaagcatatcagctgaccagtccggttaataactttcaggatattggtaaacagtgcggcatcattttctatattccggcaagctataccagcgcaatttgtccgagctgtggttttcacaaaaacattccgaccagcattaaaaagctggccaagaacaaagagttcgtcgaaaaatttgtgatcacgtacgagctgaagaaggatcgtttctatttcggctacaagatcaacgatttctataacagcaatctgcaggacaacgtgatcttttatagcaatgtggaacgcctgcgttacaaacgcaataaagataaccgtagtggtgaagtgcaagagcgtctgccgaatgaagaactgaagaaactgtttgaacagaaccacatcaactacaaagacaatccgcagattagcggtcagatcaaaaatcagaaacttgacaacgaaaagttttacaaaccgctgatctatgaaatcagcctgattctgcagctgcgtaatagcaaaaccgttaaaagcgaagatggcacgattaacaccaatattaaccgcgatttcattagctgtccggcatgttattttcacagcgagaataatctgatgaacctgccgaataaatacaaaggcggtaaaaagttcgaatttaatggtgatgcaaacggtgcctataacattgcccgtaaaggtattctgctgctgaataaactgaacaacattaaagacatcgagaagatcgagtacaacgacctgaatatcagccaagaggattgggataattttgtcaaaaacccgtaatggtctagaggtcgaaattcaaattgtgagcggataacaatttgaattttctgtatgaggttttgctaaacaactttcaacagtttcagtggagtgagaatagaaaggaacaactaaaggaattgcgaataataattttttcacgttgaaaatctccaaaaaaaaaggctccaaaaggagcctttaattgtatcggtttatcagcttgctttcgaggtgaattttgaccctctagcgaaaatgcaagagcaaagacgaaaacatgccacacatgaggaataccgattctctcattaacatattcaggccagttatctgggcttaaaagcagaagtccaacccagataacgatcatatacatggttctctccagaggttcattactgaacactcgtccgagaataacgagtggatcccctccaattcgccctatagtgagtcgtattacgcgcgctcactggccgtcgttttacaacgtcgtgactgggaaaaccctggcgttacccaacttaatcgccttgcagcacatccccctttcgccagctggcgtaatagcgaagaggcccgcaccgatcgcccttcccaacagttgcgcagcctgaatggcgaatggaaattgtaagcgttaatattttgttaaaattcgcgttaaatttttgttaaatcagctcattttttaaccaataggccgactgcgatgagtggcagggcggggcgtaatttttttaaggcagttattggtgcccttaaacgcctggtgctacgcctgaataagtgataataagcggatgaatggcagaaattcgaaagcaaattcgacccggtcgtcggttcagggcagggtcgttaaatagccgcttatgtctattgctggtttaccggtttattgactaccggaagcagtgtgaccgtgtgcttctcaaatgcctgaggccagtttgctcaggctctccccgtggaggtaataattgacgatatgatcatttattctgcctcccagagcctgataaaaacggtgaatccgttagcgaggtgccgccggcttccattcaggtcgaggtggcccggctccatgcaccgcgacgcaacgcggggaggcagacaaggtatagggcggcgaggcggctacagccgatagtctggaacagcgcacttacgggttgctgcgcaacccaagtgctaccggcgcggcagcgtgacccgtgtcggcggctccaacggctcgccatcgtccagaaaacacggctcatcgggcatcggcaggcgctgctgcccgcgccgttcccattcctccgtttcggtcaaggctggcaggtctggttccatgcccggaatgccgggctggctgggcggctcctcgccggggccggtcggtagttgctgctcgcccggatacagggtcgggatgcggcgcaggtcgccatgccccaacagcgattcgtcctggtcgtcgtgatcaaccaccacggcggcactgaacaccgacaggcgcaactggtcgcggggctggccccacgccacgcggtcattgaccacgtaggccgacacggtgccggggccgttgagcttcacgacggagatccagcgctcggccaccaagtccttgactgcgtattggaccgtccgcaaagaacgtccgatgagcttggaaagtgtcttttggctgaccaccacggcgttctggtggcccatctgcgccacgaggtgatgcagcagcattgccgccgtgggtttcctcgcaataagcccggcccacgcctcatgcgctttgcgttccgtttgcacccagtgaccgggcttgttcttggcttgaatgccgatttctctggactgcgtggccatgcttatctccatgcggtagggtgccgcacggttgcggcaccatgcgcaatcagctgcaacttttcggcagcgcgacaacaattatgcgttgcgtaaaagtggcagtcaattacagattttctttaacctacgcaatgagctattgcggggggtgccgcaatgagctgttgcgtaccccccttttttaagttgttgatttttaagtctttcgcatttcgccctatatctagttctttggtgcccaaagaagggcacccctgcggggttcccccacgccttcggcgcggctccccctccggcaaaaagtggcccctccggggcttgttgatcgactgcgcggccttcggccttgcccaaggtggcgctgcccccttggaacccccgcactcgccgccgtgaggctcggggggcaggcgggcgggcttcgccttcgactgcccccactcgcataggcttgggtcgttccaggcgcgtcaaggccaagccgctgcgcggtcgctgcgcgagccttgacccgccttccacttggtgtccaaccggcaagcgaagcgcgcaggccgcaggccggaggcttttccccagagaaaattaaaaaaattgatggggcaaggccgcaggccgcgcagttggagccggtgggtatgtggtcgaaggctgggtagccggtgggcaatccctgtggtcaagctcgtgggcaggcgcagcctgtccatcagcttgtccagcagggttgtccacgggccgagcgaagcgagccagccggtggccgctcgcggccatcgtccacatatccacgggctggcaagggagcgcagcgaccgcgcagggcgaagcccggagagcaagcccgtagggcgccgcagccgccgtaggcggtcacgactttgcgaagcaaagtctagtgagtatactcaagcattgagtggcccgccggaggcaccgccttgcgctgcccccgtcgagccggttggacaccaaaagggaggggcaggcatggcggcatacgcgatcatgcgatgcaagaagctggcgaaaatgggcaacgtggcggccagtctcaagcacgcctaccgcgagcgcgagacgcccaacgctgacgccagcaggacgccagagaacgagcactgggcggccagcagcaccgatgaagcgatgggccgactgcgcgagttgctgccagagaagcggcgcaaggacgctgtgttggcggtcgagtacgtcatgacggccagcccggaatggtggaagtcggccagccaagaacagcaggcggcgttcttcgagaaggcgcacaagtggctggcggacaagtacggggcggatcgcatcgtgacggccagcatccaccgtgacgaaaccagcccgcacatgaccgcgttcgtggtgccgctgacgcaggacggcaggctgtcggccaaggagttcatcggcaacaaagcgcagatgacccgcgaccagaccacgtttgcggccgctgtggccgatctagggctgcaacggggcatcgagggcagcaaggcacgtcacacgcgcattcaggcgttctacgaggccctggagcggccaccagtgggccacgtcaccatcagcccgcaagcggtcgagccacgcgcctatgcaccgcagggattggccgaaaagctgggaatctcaaagcgcgttgagacgccggaagccgtggccgaccggctgacaaaagcggttcggcaggggtatgagcctgccctacaggccgccgcaggagcgcgtgagatgcgcaagaaggccgatcaagcccaagagacggcccgagaccttcgggagcgcctgaagcccgttctggacgccctggggccgttgaatcgggatatgcaggccaaggccgccgcgatcatcaaggccgtgggcgaaaagctgctgacggaacagcgggaagtccagcgccagaaacaggcccagcgccagcaggaacgcgggcgcgcacatttccccgaaaagtgccacctgaaccccagagtcccgctcagaagaactcgtcaagaaggcgatagaaggcgatgcgctgcgaatcgggagcggcgataccgtaaagcacgaggaagcggtcagcccattcgccgccaagctcttcagcaatatcacgggtagccaacgctatgtcctgatagcggtccgccacacccagccggccacagtcgatgaatccagaaaagcggccattttccaccatgatattcggcaagcaggcatcgccatgggtcacgacgagatcctcgccgtcgggcatccgcgccttgagcctggcgaacagttcggctggcgcgagcccctgatgctcttcgtccagatcatcctgatcgacaagaccggcttccatccgagtacgtgctcgctcgatgcgatgtttcgcttggtggtcgaatgggcaggtagccggatcaagcgtatgcagccgccgcattgcatcagccatgatggatactttctcggcaggagcaaggtgagatgacaggagatcctgccccggcacttcgcccaatagcagccagtcccttcccgcttcagtgacaacgtcgagcacagctgcgcaaggaacgcccgtcgtggccagccacgatagccgcgctgcctcgtcttggagttcattcagggcaccggacaggtcggtcttgacaaaaagaaccgggcgcccctgcgctgacagccggaacacggcggcatcagagcagccgattgtctgttgtgcccagtcatagccgaatagcctctccacccaagcggccggagaacctgcgtgcaatccatcttgttcaatcatgcgaaacgatcctcatcctgtctcttgatcagatcttgatcccctgcgccatcagatccttggcggcaagaaagccatccagtttactttgcagggcttcccaaccttaccagagggcgccccagctggcaattccggttcgcttgctgtccataaaaccgcccagtctagctatcgccatgtaagcccactgcaagctacctgctttctctttgcgcttgcgttttcccttgtccagatagcccagtagctgacattcatccggggtcagcaccgtttctgcggactggctttctacgtgttccgcttcctttagcagcccttgcgccctgagtgcttgcggcagcgtgaagctagctgcataatgtgcctgtcaaatggacgaagcagggattctgcaaaccctatgctactccgtcaagccgtcaattgtctgattcgttaccaattatgacaacttgacggctacatcattcactttttcttcacaaccggcacggaactcgctcgggctggccccggtgcattttttaaatacccgcgagaaatagagttgatcgtcaaaaccaacattgcgaccgacggtggcgataggcatccgggtggtgctcaaaagcagcttcgcctggctgatacgttggtcctcgcgccagcttaagacgctaatccctaactgctggcggaaaagatgtgacagacgcgacggcgacaagcaaacatgctgtgcgacgctggcgatatcaaaattgctgtctgccaggtgatcgctgatgtactgacaagcctcgcgtacccgattatccatcggtggatggagcgactcgttaatcgcttccatgcgccgcagtaacaattgctcaagcagatttatcgccagcagctccgaatagcgcccttccccttgcccggcgttaatgatttgcccaaacaggtcgctgaaatgcggctggtgcgcttcatccgggcgaaagaaccccgtattggcaaatattgacggccagttaagccattcatgccagtaggcgcgcggacgaaagtaaacccactggtgataccattcgcgagcctccggatgacgaccgtagtgatgaatctctcctggcgggaacagcaaaatatcacccggtcggcaaacaaattctcgtccctgatttttcaccaccccctgaccgcgaatggtgagattgagaatataacctttcattcccagcggtcggtcgataaaaaaatcgagataaccgttggcct